European Patent Specification EP 3 478 705 B1, published November 29, 2023. Title: Attenuated African Swine Fever Virus Strain Induces Protection Against Challenge With Homologous Virulent Parental Virus Georgia 2007 Isolate. Applicant: Borca, Manuel V. Holinka-Patterson, Lauren G. Gladue, Douglas Risatti, Guillermo R. O'Donnell, Vivian K. The sequence listing filed with the application follows.

SEQUENCE LISTING (42 sequences)

SEQ ID NO: 1 - DNA, 189346 bp, African swine fever virus
gaatataccatattattgctattgccatcaatgagaatgccacgtaggcataggtcatcctatggccggaccaatccatggctgcacttaaaaatatcaaaaaagtttaagttttgggccggcgttaaaatttaaaccttttctggttgatctttagccatgtatagctgcgatgtttggtgccttatctacatgctattggcattcctgatattcgcactaaagtgctatgttacaaccgtcttatgcgtgatttttatccaccttattggccgaagggccgccttgtatttcctgttaggtggtttggccgtattctactggtggcaagcagctatcaataaaatttaatggctctcacttaagatccttgctgtaagcgggcgtttacatactttgatcaagaaaaaaattatttttggacccccccccatgttttatacaaaaatcatataataaagtggcgacaatcaacatattaatcaaccacagcattttatgatgtgttaatcaacatataccatattaatcaaccacagcattttatgatgcgtcaatcaacatattattacggagagcgtcaatcaatataatattgagaacagcgacttgataccgtgtatggtggtggcggcggcatgttgtttgtaacagcatttttcatcattcgaagcttacaaaagatatgtataagatagcatattaatgttattaacagtaatatcaataaggcgtagctatagatcttcactttggtagaccaataatccatggttgcgcttaaaaataccaaaaaaaacattaagttttggagggtaagattggtttttcaccattggtaaagattattattctaaatgtttaccccatagatgtgaaacaatgattcttcatatattaacatattttttgacttatacttttcttcatctagtaaggcgttaattttttccggatctgtcgtttttattgataaaagagaagagtctggactgtaatttttaaataataagatatttattaatatccaattattcgtttggctcgctatttccatgctctcttcgaaagcatcagctcctaaatctatacaaaggaataagttaccttcacaaaaattcattaccgaggtaatcattgcccgattaatgtcagcccccaacataaaacaataatatatagttgtataattacaatcatacatacaggccaactgcatcatttcatcaatgtctatatttgtcttctctttgttataaatttcatgaaggtcaaagacgttgttataagcaaccccacatattaaccgccaatctttaaaatgactatatcgttgataaaaatattggatggcttcagtaagcttatatagtatcgccatactataccaatacctagttagcatttcgttgaatgaaatattatccaatgtaaagttaattgataatgtatctagttcaccaaaaattcttaatttcagttgagcattatttaggaaaaggggattatcagataataattcatggcatagaataatattactgctagttttaacatactgtacattataaaatatttctaaaattttattttcactcaaagctttcctcgcacctaacttttggcataggtcctggtgcactccatattgacagtaaccaacccaaagctgatgtctgcaccccattcggtaaacagctctattaaaccatgattgttttcctgtacagccttcattaatgcaacatttaatgttaaaccatgtttaaaacttgctgtttttattaatatttgttcatctatacaagtatgataaatcgtaattggggcttcatgccaccacaaaccacaacgctctaaaatacaataatcatcttttaacacaggctgtgtagctagtacttttttagtaagtgcttgtaaagtagatggcatcttctatctgcaaaataattatttccgaaaaaaaaatcaaattaaaatactaaattctatttttttttttaataaagcctgtaaattatataataaatctcgcccaccgtattatttccggacacaactttttatacctcattatatttttagatctatagttttttaacaaggcattaattttttctggatctgtcgtttttaaagataaaagagagacgtttgaactataataatctttaaatgataatatttctactaatatatcatgattcttttgttttgctaattctaagctctcttcgaaagcattagctcctaaatctatacaaaagaacaagttattcatataaaagttttttaccgaggtaaccattgcccgattgatgtcagcccccaatacaaaacaatagtaaatggttaaaaaattgctatctctcatacaggccagatatatcatttcatcaatattcatatcaaccttttttatatgatacatttcatgaagatcagacacgttattaaaagaaagcccacatattagccgccaatctttaaaatgactatatcgttgataaaaatattggatggcttcagtaagcttacatagtatcgctatactataccaatatctagttagcatttcgttgaatgttatttcattcaatataaagttgatcgatatcttctctagaaaacaacaaattattacttttaattcctctatattctggaaaaggggattattagataacaatttatggcataaaataatattactactagttttaatacgatgtattttataaaatatttgtacaatatccatttcattcaaaatttttgcgcctaactcccggcagaaattccaagtatgctccgtattgacagtgactaagctagagttgatgtctgcaccccattcagtaaacaactctattagatcatagttgttttcctgcacagttttcattaatgcgagatttaactctaaaccatctttaaaaattgctgattttatcatcaattgattatcctcattagtagaaagcataattggagctccatgccaccacaaaccacaatatttcaaaataaagtagtgttctttagatatgtgctgtgtggccagtatttttttagcaagagcctgcagagaaattggagtagacatatttttttttgcaaaatggtttaagtttttcaagaatacagattggataaattaggttgttgacttagttacaggaggtattaaatattatgtagacataaaaatgagatcctccaaaaaaataaacaacaaaaaaaatatgtttaatattaaaatgacaatttctacattgcttattgctcttattatactacttattattattttagtagtgtttttatactataagaaacaacaaccaccgaaaaaggtctgtaaagtagataaagattgtggtagtggagagcattgtgttcgtggatcatgtagctcattgagctgcttagatgccgtaaaaatggacaaacgaaatattaagatagattctaagatttcctcatgcgaattcactcccaatttttaccgttttacggatactgctgctgatgagcagcaagaatttggaaaaacacggcatcctataaaaataactccatctccaagtgaatcccatagcccccaagaggtgtgtgaaaaatattgttcatggggaaccgatgactgtacaggttgggaatatgttggtgatgaaaaggagggaacatgttatgtatataataatccacatcacccggttcttaaatatggtaaggatcacatcatagccttacctagaaatcataaacatgcataaataaatacattaggctcatcgtatctttttaaaatccataaatattcgtttgatatatgctgaaatttttataaaaaaaataactatttcctataaatcatctagaaatagtcctcgttttgatcggtttatatcttataatattgtgcatcgatgcacaactgctttttttggtccttctggaacatcattatattttctttcattaatataccattcagatgtaaacgttgaataatttttatggcaacaatctaccattgaattatatttagtaacatctaatacatcgtttgttttatcaggctcagctctataatcttgataatttttgttatcagcttctaaagctccatcattatttttcaaagaagtatccataattatgtttggtaaaaatactttaagttttaatgtgatatttaaaatggttgttatataaatttaccgcttacaggtaatctttattcagtgtcataaactatacttttgatgattcagtattttgtgaatcagtacatttattatcattaatatttttaggctgtttttccaatgttttattgttgcaatgagcctgctcctcctttgacgaggaagtgtctgttggagtcatctgtttaggaagagtatcatccatatctattatgaagaaaatatataaatattgatatacaatcaaaaatatttttgatcacgtctttgttatctatcgatattgttgataacgtcttgaataacctacatcatttttttacataaaaaaatagatataatttttattatatctcaattattttaaagataattatcaatacagcaaatatcataagctaacatatttttcgaataatagttttttagtaaagtattaatcttttcaggattggtttcttttgataataagataggattcgctttataaatttttaaagataatatattcacaatgatagaataaccgtatatatctgctaatgtcttactgtgttcaataacattagcccctaaatccatacaaaagaacatattttcaatacaaaagttttttaccgagattaacattgctcgattagcgttggctcccaatgcaaaacagtagtaaatggtcaaaaaattattatcgcgcatacaggccagctccatcattttattaatactcatatgaattttcgttgtgttacatatttcatgaaggtcaaacacattgttgaaagaaagtgcacaaattaatcgccattcatcaaaatgcctgtattcttgacaaaaatattgaatagcttctttaagattatattttaccgctatgccataccaatatttggttagcatctcactaaatgagatctcatttaacatagaatttgttgttaaatccttcaactcccaataaatgatcatccttaaatccaccatgtttacattttgtaaaaaagggttattagaaaataattcatgacacaaaatgacattactacttgttattttacactttgtttcaaagaaaaatcgtaaaatttcacttgtctcaagctcttctttagctcccaattttcggcataggtttcgagtatgctcgttattaataaaaagtaacccataattaatatttgcaccccattcagtaaacaacatgattagatcatcattgttttccttaactgccaataccaatgcagtattaagccttataccctctttaaagcataatgtccttatcattatttgattatcatcatctatatacattgagataggagcttcatgccaccataaaccataacgctctaaaatataataatcatctttagatacgtgttgcgtggccaatgcccttttagcaagtgcttgtaaagtcgatggctgcatgtttattctgttaaaaaaaatcaaattatcgggtaaacataaggatcaacccgtagttaatatttgcagtagtattttttaacaatgaattataataaaaaaataattcattactatctattataaaacccatctttaactttaaagaagaactagatcatcttttttttgttgtgtcagaacttcttcaatttattacccacattttatctaaaaaaataaaaactacatcatatcttgtttcttcatcaaattatcataccatttatagggtgtaggttgggaacattccatcatgtggtaatcagggtatttatatattttttgatagtaacatctatttggcagatgtattgtccaacaatcatgtctaataaaatcattttcacctatgggggaatcatcttaaaaaccttattcctacagattccattttgacagtcccagcaaaagtcacaatattttccatgagtacaccaatgttcaagctctctttcgggaggaatgctgccaattttatgttttttagcttctaactctctgtacaacatcagttgggaaagcagaaagaagattaccaggagaaccattaaatatataatagtctgcaaactacgtttgcgaatgtaatttgcaactaaaacacaacccacaaggtaaaatccataagttaataacttttgccattttcgtatgacagcctcgtgccattcatggttgtgttgtgggcattctgttcggtaaacttcatgaggctttatagaagttacatagtaggtacagaattcattgtgacgaaaaacactgcagttagctatgtagtcattttcaagaatgggagaatggttttcaaagaccttattcttacagatgccatcttgacagtcccaacagaacctacaatgatttgcataggtgcaccagtattcaagctccttttcaggaggggttcttgttagatccaggagctctagctcatatgtataaagaagagttggaatggatagtaaagtaaatatttgcagaccaagcatggctacttgtgaacaagtggctgctcgtcaacaaatagctgtttatcagcaaatagctgtttatcagcaacaactaattatcagcaaatgctgcttgtgggtaagccaataaataggccatacccttgaaaggagaattcagtttgataaaaaaaataacgagttttctaataacccggtcaagcatttaataaatgaatagcatcacacgtctgcatcgtgcattctgcctggaaaatgggcccatctctaatatatttacactgacggtgaatcatacagtgttccatgggatagctatgctcctgtacaggaggcatatcttttagaactttattcttacaaagaccatcttgacaagcccagcaaaaccgacaatttttcacatattgacaccagtatctaagctcctcttccaggggattgtcggtcgaaaacccctgtagactagctaggccagctagcagcaagccgaggtaactaaagaacctcattgtagtgttatattacgaaaaaacatgttaaaatttggaaaaaaaagccctttttatagatctggaaaaaaattttcacaaatctaattaaaagccttacagatcatccttttcataaattttcattaacaattggtgggggcggttgtgaggtactggatcagaacaatccataacatggtaatgtccatttccttcaccatatgtacactggttataccagcgagaaacctcacaagatgtcaaataactgttctcaacaatcaatggcatgctcttattcaccttgttcttgcaaattccatgtgcacattcccagcaaaacttgcagttttccatgtaagtacaccagtatccaagttcttcttgtggaggattatccgttgaacgaagatgccctcctgcctgagtaggtagtcctaagacctgattggccagcaggccaagaatttccaagaagatcaccaacattgctacggctggctgaacagctggcagatagctagctaattagcaaaccaagtgactcgccctctctactcttaatatgagaatttaagattcggtccggcttttttcccatgttttacagggaaaaggtatttttagcctatgaatgtacatggttccgcacattaaaaaaaataaaagaaattatttaatattggctgttattttctttcaactagcaacaagccaggtaactaaagaacttcattgtagttttatattacggaaaaggttaaattttggacaaaaaaatcatatctaattaaaaatcctcacagatctttcttttcataaattttcattaacaattggtaggggcggttgtgaggtactggatcagaacaatccataacatggtaatgcccatttccttcaccatatgtacactggttataccagcgagaaacctcacatgttgtcaagtagctgttttcaataatcaatggcatgctattattcaccttgttcttgcaaattccatgtgcacattcccagcaaaacttgcacctttccatgtaagtgcaccagtatccaagttcttcttgtggaggattatccgttgaacgaagatgccctcctgcctgagtaggtagtcctacgacctgattggccagcaggccaagaattcccaagaagactaccaacattgctacggctggctgaacagctggcagatagctagctaattagcaaaccaagtgactcaccctctctactcttaatatgagaatttaagatccggtccgacatttttccgatattttacaagaaaaagatatttttagctacaaatacacttcatatatccctaaaaaaacaaaaatttatttaattttaactattattttctttccactctctctttaagattttgtaaggattccagggctttggttcagaacaggccattacatggtgaatcccctgtcctagatcatacatacatttatttagccagcgggaaactatacatgattgcacatactcattttcaagaattgttgtattctccaatttgccctcacaaaggccattttgacaattccagcaaaacttgcagttttctgtataagtgcaccagtattcaagttcttcttgtggaggattatccgttggatgaagttgtccagctggttgattaggtagccctaagacctggttgcaattcatggtatggtagatacccttatctaaatcatacatacatttatccagccaacgggaaaccagacatgatttcacatactcattcttgtaaattactgacccatctattttgtttatacaagtgccgtcttggcagtcccagcaaaattggcaactttccatgtaggcacaccagtattcgagttcttcctctggaggctcctctgttggacgaagttgtccaacgagctgacttgaaacctggctggccagaaggccaagaattcccaagaagatcaccaacattgctacggctggctgaacagctgactgaatagctagccaattagcaatccactgtacttttcataagatcatttaagattcggtcggcattttttcaatagtttgctaggaaaaaatttttaattttatagattcacactacttcattctcatgcttaggaaaaaaacaaactaaatcttacaatgtatctggatctaatgagaagctagaattcatcttttttcaaatcctttctgggatgttcattctttttccactccttccttgcaattttataaggattccagggctttgggtcagaacagttcatgctatggtaaatgtgctcctccacatcatatctacataggtcaccccagcgggaaacctcacaatattttacatagtcattctcaataatacttgtggagttgtttccccaaaccctgctggtacaaatcccatcttcacaatcccagcagaaccgacagctttccacataagtgcaccagtatccaagttcattctctgggggttcaaatgttagaggaagatgtccacctacccgagtagaagtggaggatgaaaccaggttgctactggccagcaggccaataattcccaggataatcaccagcattgtgctcaaccagcaacggctagcaacgactagcaactgactagcaatagctagaaatggctagcaatcagtagtagctaacgctctactctttataagaaaatttaaaattcgatcagatttttttagaattgagaatgagtaaaacgcttatattctttttctagctagaaaaaataagctagtttaagataggatttcccttactaacggtttaatttttagcaaaggtataggtaaaatacacttgtacttagctgcaaaaaaataagcttatggcgtataagccgccataagtttatttaattaaaatgttaaactctgtgataagactggaatcttaggcaggtttgatgtggagaacagcatgaaatacaagagtgcctgttacacgaataagttctctcaaaccggggatggtcatactcacatctatgaaatcctggtctaggagattcatttgatgcatgatggccgcacccacacttatgagacactgaagaactaaagggtttaattttgatctgaatggtactatataggatgatggcaatccatatcaagattagagcaatcaaaatcacctcctcaagaagcatgatgtagccttaaatcttagactgctttaaaccttaggccctcactatctttaatgaaggagtttaaattttgatccctttttcaagacccatttagaagaaaaaataaagtttatatcaatctaattcataagtcatctctttcataaatcttcatgtattctctatgtggataagtatgggatgttggatttgcgcagtccatttgatgatctgtatggtttttgggtccttcataataactacatataccattccagcgggaaaccgtgcaatttataatccagtcattttgatgaataactggccaatctgtttgaatcctgtttcggcagataccgtggacgcattcccagcaaaagtcacattggtttgcgtaagtgcaccaataaactagctcatgttcaggaggataacgggttggtagtaaatcttctaatttacgtataggagcggcttgaaggacaaccacccccagtagtactagaatcagtacctttatagtggccaccctacactagacctctaagttgaagacaaagaactaaaatttagagccgtttaattactactaataattatattttttattgtctacaataggattctattaaaaaataatgatttttaccaagaaatatttttataaaaaattaatatattttgtaataaactttatttccaatgactgttaaaataaggaaactatccttagttagtcgaggaagatggttaggttatttcgcaatccgataaaatgtttattttatcgtaggtctcgtaaaatccaggaaaaaaaattacggaagagtttaaaaaagctaaatttttaccaccctccagaagattgttgtcaaatatatcgtttgctagaaaatgttcctggaggaacttactttattacagaaaatatgacgaatgatttaattatggtcgtaaaggattcggtggataaaaaaattaaaagcattaaattatatcttcatggaagttatattaagattcatcagcactattatattaatatttatatgtatcttatgagatatacccaaatttataaatatcccttaatttgttttaacaaatattataacatctaagtaaatattcttggaatggattttcttatagaatggttacaggatatgtcagcgacaggcttaataacaaatttgttaatatttttttgttaaataaatgaacaggccaccatttaatattacccgttgcaaaataagaaaaaaaaacaaacttatagttacaaatcatcttgattaatcacatgtcgttttaactcaatgaaccattctaaatctttgggttgtgaacaattcatgttatgttgatagtgtatcctaaagtgagcttcatacatacaccggtcatgccaccgggaaactgtacaattaacaatataatcattttgcgtaataatagggtggtcactaaacactttatttttacacattccatctttacaggtccagcagaagtcacagtgttttgcataggtgcaccagaacttgagatccctttcaggaggcctacgcatttgcatcggattatctgtggaaagaggtaggttcattattatgttcgtcatcaaaattcctaaaagaacatagaagccaagaaagataagcagtcttgtagcggcttgcattcgcattcgtgagtattgtttgcgaacatagcttatgagagcaatggtagctatcatacaaagacaagtatgtttgatattctcagtgtcaatgaccctatcctcctttatttgcattaactcatcaaaccaatcataatatgtgggatttgtacagctcatgatgtgaaagcggcgtatcctagagtctgtaaagtagctacatctttcattatagcgagaaaccctacatatttgtatgtaatcattttttttgatgagagggtgtttttcaaaaaccttatttttacaaaccccgtgtcgacaattccagcagaagtcacacgattttgcataggtgcaccaatactcaagctctctctttggaggtctccgggtcattggtaactctcctgttcctggaaaagattggctttgaatgaccggctgcatgaccgccagtaccaaaaggaacacaatcaccttcatggctgcaacttataagttgcaacttatgggttgcaatactgcaacgtataggttgcaccttatagatcgcgactcaaaaggtatgaaaaccttaccctcaatacagaatttaagttttaatcctgataatgtatctgtttatgaaaaaaaattttttttactcatgtatgaattcttatacgaatcataatatgtaggctgagaataataattcatatacggtgttgcgggctcaataaaaattttgttaccacaaaaaataaatgctggatttttaagatatatatctattaatgactaaaccctttatacgctgtaggctgaaaacaatccatataatgaatatacggtgatttgggtttaataaaatacatacaacggtcaaaatagcgggcaatactacattgactaatataatcattttgtttaataagaggcatatcatcccacactttatttttacaaataccgttcctacattcccagcagaaatcacagtgttttccatacgtgcaccagtattcaagctctcttataggaggcgtataagtccttggtaaattttgtttcatataaaagatggaaaggggtcgatttaaacccggctgagatagccaaatcaaaatacataaaagagcaagtagtttcatagtggtatttagatgtaaatttttatagtatgcaaatacaatgtaacctacaaatacaatactaaatacaaggtaaaaacaacaatgtcttataatgattggccaataatcaccccccccccccccatttttccatgaatatttcatttcctgtatagggtctaggatgtgaacactccatgttatgatgattaggcattttaactgatatttcataaaaacacccccaggaattgcgattaactatacagtttacaatcgaattcatcgaattagactcatttgttatcttatttttacaaatgccattttgacaatcccagcagaagtcacaattctttacatacgtacaccaatatggaagctcctccttaggaggatgctgggttcttggtaattctggtaattcatgtgcaagaatgaggactgagtagcccaacaaaagtcctagaaccttcatgttgtgtccaaatggcacctgtcattttaaaaaagatttaaattttgctaccgcaaaaaaaatccagtatgtatttttttaatacatataattattgaagtcttataagataaagccgagaacactatattttgtatagatgatgtatccggtattcaaactctcttataagtacatgtaggaaatggtcaattattcaagattggctgagataacaacaaaaccaaaatactcaaaagcataagtaatttcatggttgtactcagtcgtagatttttgcagatcgcaaatgcaacgcaaccagcaaatacaaagctaaatacaaggtaaaaacaataataccttataatgattggccaattcttatccctccatttttccatgaacatttcatgttcataaagtctaggatacgaacaacatttcatgctatgatgattaggtattttaagtgatatttcataaaaacaccacggggttgttggtgattgataggtaagaataaggatggttgaataacctagtaaaagtcctagaaaaaccttcatattgcgttcataccacagatgttatttaaaaaaaatataaattttacagtatgtgatatacacataccacaaaaatgttcttatattaactaaaatatgtgggcagagagcaattcatataatgaatatatggtattttaggctcaataaagtacatacaacgatcaataaaacgggtaatactacatttactgatgtaatcattttgaacaataagaggcatatcatccaaaaccttatttttacaaataccattcttacaatcccagcagaaatcacagtgttttccatacgtacaccaatattcaagttctctcataggaggcgtataggtccttggtaaaatttgtttcgtataaaagatggaaaggggtcgatttaaaactggctgtgctaaccaaaccaaaatactcaaaagaacgaaaagtttcatggttgtactcagacgcagattcttacaaagcgcacatacaaagcagcctgtatatgcaataccaatgatgaaatagagacagtattgctttatagataattgttgatggtcaccccccccccccccccatgtttgcatgaatatttcatttcctgtatagggtctaggatgtaaacattccatgctaaagtgattaggcattttagatgaaatttcatataaacaggattgagtcttggaatcacggaaaactctacagtttacaatagaatgattggagtcaatgaaacgagattccgttatcttatttttgcaaatgccatcttgacagtcccaacagaaatcgcattgtggtacatacgtacaccaatatgaaagctcactcttgggaggatgctgggttcttggtaagtctggtaattcatgtgcgagaatgaggactgagtagcccaacaaaagtcccagaagaaccttcatgttgcgtctaaatgacacctgcacttacaaaaaaaaatttaaattttgaatataacacaaaaaaaccaccttaaaatttcttatattatttcttggatctgccccgacgtcatacaatgtattaaaattatagaccaatcatctttttgtatataggctaatcatctttatatatagattttagatgtttgcttgttgtatcaacttaactgctagcgaagaaaatggataaaaactttctgtatttttataggttgaaatcattttatgcacatcgctaggatctaatattttattttgaagaaccgaatgtgggcttaaaatttttttcttagaaaaaagtagaatcataatattgctatgtttttgtttaatgatttcttgtatcttttttgtatacgggttggcacccaaacctatacaaaaatatacattactcaaataactaccttctatacataatcttttttccccacgtattttcctatttatttccctatttatggaattaaaggatatcaatctctctaaggcacggtcaaggtctgcgcctaaggcaaaacaataatatatacctaatttattcccagggcgtgcacaggcaagaaacatcatgacgtttagccctaaacgtatattttcctgaaaatacgcatgatgaacttcatcaatattacctaagtatatggccgtttgtaaacgccaaagatctaaatgaggaaattttttactaagataatgaataggttttgtgagattaaaatctatggcgaacttataccaaaattttaatacaagtgtatttctcgtcatttcttcttctttttcatctaaatataagataaaacgattgtaaacaaagtctatcaataggtgaaaatcattgctattaaagctgtcgagaatcaaaatattgtcataataaatttcgatcgccagtaaaaccttttttcgtttgacgagataaacaaacatattatacaaccctacatctaaaaattctggattggctcctagttggatacacaggtctttagtctgcttcgttttggcacacatgatgccaaaattaatatcagcaccccataaaacaaataacttgattagatcagtctggttttccttcacagcttttactaaggctctgtcaagctcatagctgtcgacatcagagcatgacatagagccaccggttaccattttacattgcttacaaaaacctatgggtccgttttcccaccatagtccaagctgttgtagaataaaaatatcatcctcatgataatttgaaaaagccttggtttctatcaagactttttttgtaagaacctgtaaagagttcatcgtattattatgaataacaggagtaaacgtaatcaattataaaagtgattttttcgaaaaaaactttagatggttgaaaatgataatgtacatgttcatacaaaaaatagatgcagtgatgtctaaaatcaaaatttaattttctatgtaaaaagtacagacttacttatttgggttaaattgtttattttaaactttaattaaccgtttgagttagcgatgtttgatttatcttccatactcatccggggggggggggtccttatagctctgacattattgtggattattgaatataatgaatacttcatagatgctaaacattttaatagtagttctgaggcttaattgtactctataaatttataaaaactttttgatcaaaatttaatttcttataaaaagagtacagacgtcgcttgtttaagcttcatcatgtttcattcattactttctacaattacggggggggggagtcccctcatagctttagtattgctatggtttactaattattatgtagaatttatagaagcatatgtacctgaaagtatacctactctataaaattaaataatttcagtatattttttttatgaatagaacggaaatgatataaaaataatttaatattgcaaaaaaaattcataatgttggtatgtattataaacataatagcatgtgtaatttataaactgactcctctatataattattagatgaggtaccaacctacttatgatatgccgatgatagatattgtatactataaaacaaaattattttaaatgtattcatggatacattataacatttttaccgcaaattgtctctcagcgaagaaaatgaatgaaacgtttctgtatattcataggttgaaattattttacgcacttcactaggttctaatattttcttatgaagtattgaatgggggcttaaaagtcctttcttaaaaagaagtttcatcataacattcttttcttgtctaagaagagtttcttgtattttttttgtataaggattggcacccaaacttatacaaaaatgtacattactccaaataccataatttgaaaagaaagttatttccctatttacttcatgattaatgaaacctatcaacgtctctaaggccgtattgatatttgcgcctaaggcaaaacaatagtatatacccaatttattttgagggtacatacaagcaagcgacatcatgtcatttggatctaaacgtatattttcctgaaaatatgcatgatggatttcatcaacattacctaagtatacagccgtttttaaacgccaataatctaggtgaggaaatttcttactaagaaaacgaataggttttataagattaaactctatggcgatcttaaaccaaaattttaatacatatgtattttttatcattttttctttttcatctaaatttaagataaaacgattgtaaataaagtctatcaacacgtaaaaatcatggctatcaaaactgtcgagaatcgaaatattgtcataataaatatctatagctaataagaccttttgttgtttaattagatcaacaaacatattatacaaccctacatctaaaaattttggatcagctcctagttgaatacacagaactttcgtcctttccgtcttggcacatatgatgccataattaatgttggcaccccataaaacaaataacttgattagatcagtctggtttttcttcacagccctcaccaaggctctgtcaagctcatagctgtcaacatcagaacatgacatagagccactggttaccattttacattgtttacaaaaacctatgggtccgttttcccaccataatccaagctgctgtaaaataaaaatatcatcctcatgataatttgaaaaagccttgttttctatcaagactttttttgtaagaacctgtaaagaattcatcgtattatcatgaatgaaagcagtaaatgtaatcaattataaaattgacttattgaagagaaatgttaaatgagtgaaatcggtgtttatgatgatgtacatgatcatacgaagaaacacgttcactggtgtccatgatcaaaatttaatgttttacgtaaaaagtacagatgttaactgtttagtttaaacataaatttaacctttagtttaaaccctagttaatgatgtttaatatttcttctatactcattcagggaagtgtaatgattctaatactgttgttatggattattaatgaaaactttacagatgctggagggaataattttaatcatactgttttaatgtagctatataagctttcatcaaaatttaattttttttataaaaatacacgaattaaactaaagtctaaactttagtttgactatttgagttaatgatgcttaacttatcttccatgcttatcaagggggggtcctaatagttttgatactattgttgtggattgttgaatataataaatactttatagatgctgaaatgtttgaaaataatagtacatcaatgttgtaagtttgatcaaaatttaatttctcataaaaaaggtacacatcaacattgctcatttaagtttcatgatgtttgattcattacttcctacaattactgggggggggggggggtctttaatagctttagcattgttatggtttgctgactattatgtagaattcatagaagcacgtttagatagtaatatcactgcagtgtagattatgaaatacatactaaactaatttcagtatattttttttgttcatataagttaaggtacaaaaatgattaaacattgcaaaaaaagaaaatcacaatgctattatacatagtgatcatagtggcttgtatcatttctaaactagttccaaatgaatattgggcaatacatctattttttatcattatgatttttatggtatatatgtatgaaaagttagatatacatcaaaaatctcagttctggaattataccatgtcaggcttatctggacataacgtacaggtaacatgtaagtgttactaaatactatgaagtatctattttttttgttgtaaaaaaaagaacttgatagtattttttaaaaaataaaataattaattgtacgtcaacttccttattttattctttaaaaataactcgtaagtattatttatctattttttgaaaaaatagatgtaatcggtttcatcatttaggtgtgtatttctttttagcatctatcaagaattcattgtttagtgatatgaaaacaatgaatgatcattatcttctatttaacaaccacctaaataaatgaacgtctttttcatcttaactgattaccaaaagttattttgcgaaaaggcatacatatgatcaatatcagacctacaatgaatatttccataatatccctttattgtaataattctatttttgcattccgatatctcatcatctgtgctattatatgtttccataactgtttcatcatcaaacataaatcctgttaaataggcaaaagactttaatcccggatagatttttaccattttcctgagagccgtgtatagcttgtaataaatggccaaaaatatgcaataaagcgtagaaagagagtaatttttggcataaaagattttgaaggtttgatgaatggctaaatcgcatataatataagatacgattttaaagcgcacctgttcacgcagatttgttgaaaaattcgtggaaagatttaacaaataaaaggttattaatagttgctcatcattccccttatacgacatcgtcagacgctctaatattttactactaggcacatctgccacatgttgaacatttaaagcctgttcttcttctgtgttacggcaaaagagccgtgcgtattcaggtgaagctccccaggataacaacgtccttgctacggctaaattttttttgacgatgacttttatcagaaataagtctttatttttgcattgatcactatgcgaatttgtatagttgacgccgttgcattgagtacattgatataatgttttacaattccagcgtagccctaaatggtataaaagaactgtattttcgacataagcatgctgattaacgatgtttttgagacaacacgtcgttaaggacaccatattgtctccaatttgttagataaaagtctttactaaaaaaatagatttttagttttaacaatcgagattttattatttggatgcatcatcaaaaagatttataagtataagaggttgtataagaaaaaaatgatgttatactatttatgttaaaatttaatttatcatataaaaagtacagatttaatcagttggttaaactatttagttaattaaactaaatagtttaaccatttagtcagactacttggttagcaatgtttgagctttcttccattcttatccgggggggggggtcctaatcgttctaatactattgtggatagttgaatataatgaagactttatagatgctataatgatgaattctagtatgcctgtataaaataattaacctttttgatcaaaatttaatttttttataaaaagctacagagtagtgttttattaaacgtggcttatttaaaagttacacaatgttaaaatctctacttactttaattctttgtggggttttattaactttatccatattatggcttactacttaccatgtagaacttatagaggcaatagatgatttctacgactgaaatatagaatagtccattttctatttgtaaaataatgatttatattctttcctaaaaatgatactttatatggtttgaaaacaaatattaacaacttgatttttttttctataaataaactataaatgaaaatagtaaaactcatagagtcttataagtgaacatcttcataatgttactcaaacgttggactattaaaaaatattccgtgtgcattattgcttttaatcagtatgattactttatacgaagccgctattaaaacgcttatcacacaccgaaaacaaattttaaaacaccccgatagccgtgaaattttactagctttggggttgtactgggataaaactcatattcttgttaaatgtcgtgaatgtgggaatatgagtcttaccggaaaacacagtacaaaatgtattaacattaattgtctacttattcttgccataaaaaaaagaataagcgtattgttgataccttgataggaatgggcgcggatgtaacatatatacatcttttaaagaataagataaaactgtcatacaaccagctgtctatgcttaaaagcaactcgcagatttcattgaaggagcttcatgctatatgctatcttttatatggtcggcttcccaaaaaaattaaacaagggatgcgactgtgtaaaacaatggcgggactatgtggtgaacttttatgtgcatttttagctccgtaaatgataatatgtatttaaaacaaacagatattaccaaaatatattctatgtacataatatctgggaaattatttttttttctcatacccttaaatataaaaatattgggtttcttcactaaactttagaggtaaaaatttttctttgttttgcaccatcatgtatgggtttaggctgtcccagggattgtttatttgaatatttcctaaataggaacacaacgccatgatcatatatctttcattctggtaagctttttgatacatcttcaaagatgccgtacctccgagtgtgtaacagcaaacaaacgtccgtacttttccatgggtcgcagcccattccattccgtagctcagcatcttttgctgtatttttttattcgctttataaaaaaagtttttcatccattccacgttctcataaaaacaggcacttaaaaagagcactaggggtagtgtagtcttattatagaatgtaggaatgtatgttttagttatttttttcaacgcgtgttccatactatgttttaccgccataaaaatacaaaaccaataccaactttttctataaaaggttttgctgtacacatataaacgagcaaaatatatttcaaactctatattctttttataaaaaaactcgagacagtcgtttatgttacgactttttctaaatacctcaaaaacagtaattaattcactgtcgctgtggaaatgttcgtaagctaactgtttaatgtctttaggggtcaattctttttttgggagcagtggtttgagattcggcaaaggtcgtctaaagtagtgagcgaacttttcattcgctccccaacacaaaagccgataagccagcatgtagttatcacgttttaccgcgtaaataagcaaatagtttatattgatacatgtaccatgttgctgcccgtttggacatatgttgccgcattctgaacacttatgaatgagatcatagttcttacaacataaccccaaacgggttagtacttctttgtcacgttttaaaaactcgacatgattctttaatgttaatgctttgagcgcaatgttaaataaactctgcattttattaaaatgaggttagtatcatgttttagtataaaatttagcggctgtttacataatgctaaataaacttaacgttcctactaaaccaaaaaaaatcaaattgactaagtcatagagaatttgacgatgttggtaggtaattttttaacatggtatatatttttttagggtcggttatattaggtaataaaagaggacgtgccgttaaagtattttgcttaagatcctttagatccttacaaaaatatagattgttcgtctgatgatgccactgtgttgcagtgatggcttgatcaatatcacctcccaagacaaaacagtagtatatcgttaaaaagttgtaatctttcatacaagccaactgcatcattttatcgatgtccatatgaacgatcttttgctcgtatatttcatgaaggtcaaatacattgttgaagtaaatggcgcacatgagtcgccacatactaaggtgcccatatgtttgatagaaaaaggagatagctcttttaagcttatattttactgctatggcatagcagtatttaacgaatacgttcatgggtacattatctaagatataaaatatgaaaaactttaactctcgatgaatctcttcccccatttcctgtacatttagagcttccaacataggatttttatcaaatatttcatgacataaaataatgttattgctcgttttatgacgcattaaaccggtgaaaatttccttattatttaaactatctttagctcctaactttcgacacagctcctgagtttgttccgtcctagcacaggtcagcccataataaatgtttgctccccactcggtgaacagccttattacgtcatagttattttcttttatggccatgattaatgccacatcaagatgaagaagttcccccttaaagggggttgagcttaaaataacgtaattacagtagtgacataagctaatgggcttgttttgccaccataagccacaatattttaaaatataatgatactcctcaggcacgctctgtttggccacagcctttttggccagggtttgcaaggagagcatgataacttcttgaaaaaaaaactcaaattaagttcctacttttttaaaatattagtatggacagatctaccatcatatgaaggaattctttcatcgttaaacactgaagagataatactttcatcgtatagagaatatcatgtcaatccatatattgaatgttatatatcattaaacccatcattaatatagtgtttatgtgctatggacaggttttttgaatgataatcttttaacatacgttttataacttcgggatcagtttcttttaaagataaagaatcattcatgttataacaatttaatgataacatgctggcaatgaacgagttgtctttttgatgcgctagagtctttccctcctcaaaggcattggcgcctaagtctatacaaaagaatatgtttccgatattatagaactgaatagaatgaaacatggcctgattgatatcagcccctaagacgacgcaacagtaataaatcgttaaatagttatagttcttgcgacaggcccactttagcatttcattcatgtctatgcgaatcctctccttttcgtacacttcgtgaagttcaaacacattattgtaaaaaagggcgcacataagccgccaccgatgtagatgagcatatctctgataaaaatagcaaatcgcctccttaaggttacattctattgccatcgcgtaccaatatttagtaaacatctcgcttaatatatcggtttctaccattaatccctccagttgttcataaatcattccctttacttcaaaacgatttatggtatctaaaatgggattattagaaaatacctcatggcagaaaatgatgttactgctagttagatcacgtttcaatgtgtaaaaaaatcgtaaaatttcctggtcatttaactgttctttggcacctagctgcctgcacaggtctcgggtgtgctccgtgttgacagaaagcaaaccgtagttgatgtttgcaccccactcggtgaacaattctattagatcgtgattgttttcctccacagctttcaccaaggccgcgttaagatttgtgccgttcttaaaatacggcgtccatattttcttttgatgatacatgatagggccattatgccaccatagaccgcagcacttcaaaaaatgaggatggcatttggccggatactggctggccagcacctttttggtgagagtctgcagagagaggaccatatttcttttttttgaaaaaatcaaattaaaaaaatcatgcttgtttagcatacatgtaatattgttataattacgttataattacgttataattacgttataactatattataacaatggtataacaatggtataacaatgttataacaatgttataacgatgtatcattgatgtcatcattcaactaggccaacatactttttaatttatagttttttaatagatgatatattttgttaggatctgcttcttttaacgttaatagcgaggagtctgcactataaatgtctaatgataaatgatgagatatcaaatagtaattccgttgctctgctagggcctttgcctcttcaaaggcgtcggctcccagatctatacaaaagaacaagttatccatattataaaatcgtacgcaggcaagcatagctgaattaatattagctcctaagagaaaacaataatatatggttaaaaaattgttatcttttgtgcaggccatccgcatcatttcatccacgtccatgcggatcttttccttttcatacaaattatgtaggtcaaacagcttattaaaacaaagagcacagattaaccaccacgtatttagatacttaaaatgttggtaaacataagaaatggcctccctaagattatcctgcaatgccactataaaacagtatatcgttaacatatcaccatccgacatattacttaatatgtcggtgtcttctactaaccttttcaacttccaatatatggatgaccttatttcccttataatgacataggctggaaagggattatcattaaaaagtttaagacataagataatattactgctagtagtgccagggtgtattaatttaaagaacatgtgcataatcttctttttatccacgcggtacttggctcctaattcccagcaaaattctcgaacaggcggcgtattggcgcaaattaacccatagttgatgtctgcgccccattctgtaaacagttttattaactgatagttgttttcctttgtagccaacattagtgccgtattaaggtccaagccgtctgcaaagcttggcagctttatcagcatatgtttgcaatcaagggaaattggggccttataccaccatagtccgcagcgttctaagataacatggtactcaatagatacttgctgtctggctagtacctttttggcgaaggattgtaaggaaggaaacatcctgtttctttttttttaaaaatcaattatctttgttcataatcaagaaaaatccccatatttattgagtgataattttttaacatgcaatttattttttcagggtccgtaacgatcgacaacagagaaataaccggattgtaatgctttaatgataaggcatgggctatcagataattttccttttgttctgccaaagctttgccctcctcaaaggcatcggcacccaggtctatacaaaagaacaggtttccaagattatagttttgtatggaaacaagcatggcttgattgatgttggctcccatgataaaacagtagtaaatggccgaatagctataatcttggatgcaggctatgtgcatcatttcatcaatatccatgcggaccctttctatttcgtacagctcgtgaaggtcgaacacgttgttgtaaaaaagggcgcacatgagccgccacctatgtagacgcgggtatttctggtaaaagtagcggatagcatctttgaggtcatagtccaccgctatcgcgtaccagtatttggttaaaacagtgctaaagctatcatcatggtccagcatgaaggttatctccatgagccctcttaactcccacatgatttcccccctcagatccagattatctataatccttaaattggggttattggaaaacacctcgtggcaaaagataatattgctactggttttatcgcgcgttgtatcaaagaaaatttttaaaatatactctctttctaaatattctttggctcccagctctttgcacagatcacgggtattttccgtgagagcacaaatcattccatagttaatatctgcaccccattcagtaaacagctttatcaagtcatgattattctccttcacggctttcatcagtcctatgtttaactcgataccttgactaaaacaggttgaccttataaataatttattgcgtcgaatatgaagcataatggggccattatgccaccacaggccacaacacttcaggacatgatattgatctaccggtatacactgcccggccagtactttcttcgtgagggattgcagggaaggcaacatgcctttccatcctttgacggaaatcaaattatctactaataactatcagtgtttatattaagtatttagatattatcccgggctggatacgtagtatcgctattcacatgtacttccaactctagccggagcctgcagggtcatttatttttaatattgattcttttttgtatttaatcatttagagaaggtcatcataggagccagatgttctctctccagaacttatgtcgaaaaacattacctaaccgtaaacttcctgaattttttgacgaatatatattacaactgctgggattatactgggaaaaccatggaactattcaacgagcaggaaacaactgtgtgcttatacagcaacataccctcattcccgtaaatgaagccctgagaacagcagcatctgaagaaaattatgagatcgtgagccttttattagcgtgggaggggaacctttactatgctattataggggctctagagggcaaccgccacgacttaattcgtaaatatgatgaccaaatcaaggaccatcatgaaattctgccattcattgacgatccagtcatatttcacaaatgccatatcatgcggcaatgcttttttgattgtattttatatcaagctgtaaaatatagtaagtttcgcgttcttctttactttaaacatagattagaggatgatttgcccttcactcatttacttattgaaaaggcatgtaaagatcataattatgaagttattaaatggatatatgaaaacctacatatctacaatatgatagatacctttgaatgtgctattgcccataaggatctacatctatattgtttggggtatagatttatatataacagaatcgtacccgataagtatcatcatttagatattcgcatgctttcaagcctacaactcctacataaggtggcagccaaaggatacttagattttatcctagaaaccttaaagtatgatcataataaagataatataaatattattctaacacaagctgcaacctataaccatagaaaaattttaatctatttcattcctcaatcaacccacgcacagatagaacaatgtttactagtggcgataaaagcaaaatcttccaggaaaaccttgaacttactactgtctcacctaaacctttccatcaacctcatcaaaaaaataagccattatgttgccacttacaattcaacaaatataataggcattctgagtatgcggcggaaaaagaagatatatttagatatcatattgacaaaatttgtaaaaaaagctatttttaataagtttgtcgttcgatgtatggatacattttctataaacccggaaagaatccttaaaatagccgcgcgaataaataggatgatgttagtgaaaaaaatatctgaacatgtttggaaaaatcatgcggttagacttaaataccttaaacatgcggtacacacgatgaagcataaagatgggaaaaatagactcatgaactttatctatgatcgctgttattaccatatgcaaggggaagaaatctttagcctcgcaagattttatgcaatccatcatgcaccaaagttgtttgacgttttttatgattgttgtatcctagatacgatacgattcaaaagccttcttttagattgttcacatatcataggtaaaaacgctcatgatgctaccaatatcaacatcgtgaacaagtatatcggcaacctgtttgttatgggagttcttagcaaaaaagaaatcttacaggactatccatccatttattctaaacaatacatgccttagtttattttttttgcggccgaaacattattcttaccctagaaaacgcttatagtcatcttaaatcataggtaaggaagatcatcatattttttgaaacgtaattttttaacgcatgatctatgatttcagggtccgtgcttttaggcaacggggtggtggccggactataaatctttagggataaaatgttctttataagctcatacccttcccctaaagctgtagtaccctcttcgaaaacatcagcccccagatctatacaaaagaacatgttttctatattatagtactgtattgagctaagcatggcttgattgatgttggcgcccaggacatagcagtagtacatggttgaaaggttgtggtctttgatgcaggcgatccgcatcatctcttctatgtccatatggatcttgtccttttcatacgcctcatgaaggtcaaacacattattaaaacaaagagcacatgttaaccgccacgtattcaggtgtgtatatttttggtaaaaatactgtatggcctctttcaggttatagcgtatggctatagcgtaccagtatttgagtagtaatgtactgagcgaaaactcattatttagcagatcggtttttactattaactcccttaactcccagaaaatttctatcctcatttttatattatttactttttgtaatatcggattgttggaaaacacctcatggcataaaataatgttactactagttttatgaaactttagatctataaaaatttgtaaaatttcttcttcattcaaggtttccttggcacctagctctcgacagaggtcccaggtgtgctccgtgttgacagataccagcccgtagttgatgtccgccccccactctgcaaacagttttataaggttgtagttgttttcccttacagccttcactaacgccgtatttaggtttaagccctctttaatacctgctgattttatgagccttaggttatgatcaaacgtgatcggagcatcatgccaccataggtcataacactttaaaagataatgttggttcgtgggcacgcattgtccagccaacacctttttggtcagagattgcagggaaggcaacatgtctcttcatcttttaaaaaaaaatcaaattaattagccgaataaatttttctttcgagggctttttaaaagagctctttaagagctctttaagagctttttaagagattaaaaaattattcttgctggcattctgccaagtatgcggcattcctatcatctatagtatattatgagaatattcccaaatgatggataagttttttgatttataatcttttaataaactgcttatttcttcggggtcctttaagtttagtggcaaggaagcatctgagctgtaaatatccaaagccaaactatggctcagaaaattataacctttttgttccgctatggcacgaccctcttcaaaggcattaccacccaaatctatacagaaaaatatattaccgatgttataatattgtactgaagtaagcatagcttggttgatgttgccccccagcgcgtaacagtaatatattgttaatggattgttatccttggtagaagccagacatatcatgtcatggacgtctatttggatgttttccttgtggtacatctcatgaagctcatatattttgttataatacaggagacattttaatcgccattcattaagatccgtatatttctcatctagaaaacaaatggcgtccttacaatcgtattgtactgctttggcgtaccaatacttcactagtaaaccatttaactcgtccgtttcttttatttctatgagcccccatagtcttttataaattaagccccttaattgtataacaaatttgttttctaaaataggattattcataaaaatttcatggcacaaaataatactgccgctggttttattgtgcattatcctggtaaaaatacggaaaatatcgttgtcctctagagtttctttggcgcctagctgtctacacaactctcggatgtgcttcgtattgatagaaagcaaaccatagttgatatttgcgccccactctgtaaagagctttatcagactatagttgttttccttaacagctattattaatgccacacgaaggtctatatcttctcctaaaaatcctgattttatttgtattcggccacgatccatacaaagcttgagaggagcatcatgccaccataggccacaatatttcaaaatgcagtgttcatctattgacaaacactggctggctatcgtctttttgacgagggtctgcagagagagcggcaacgacatgtttctttttcaccaaaaaaaatcaaatgttctcgtctttaaaggttaattcatgttcttaaaatgttcatttcatgatagtgattaataatatggtttaataacgctagaaggcttgtttataagacagtcataagcagtctataagacagtctataagcagtctataagacagtctatgacttagtctataactataatttctggatgggctgtaagatactcttcggctcgtttcagattttttgaagtatatgtctttagcatatcatatatttcctggggttcggttacatctaataccaaggtcacatcacggctgaaaagctgctttactaagaaaatgttgctcaagttatacatataagctttgtgcgcaatgagttgtgccctatcaaaatcggcagcccccaaatcaatacagaaaaacatgtttaaagtattattgttatagatagaaagattcatgccataatcgagactagcccccaacctatgacagtaataaatggccgcgtaatttttttcccgcaagcaagcaaatttcatcatcagattagggctgatgcaaatctctttttcacgacacaactcgtgtatgtcaaaaatgttattaaaataaaggctacaagctacccgccaatagaggtgatttttatgccttttatagaaatagtgaatagcctttgtaaaattatgtcgtaatgccagggcaaaccaaaactttgttaataggtggtgcgccgtatcccccgtcaacggaatgtttgaacaggtgtacgtaactgtgtctaaagtggttctagttacggtttccaagagtggattatgacaaaacatgtcataacccagcagaactcctgcacaggattttagcctggccacttcttttaaaatttccagaagacggggttcggatacaggcgttaagcctcccagttccgcacacagccgctttagatacacggcaggaacacgtataagcccatattcaggatttgcgccccaatccacaaataaacgtataagttcaagattatcgctcttcacggcctttactagcgccgcttcgagacaaagatcatcctcagaaaaacactgtaaatgtttatacgaaaaaacttgcttacaattgttacataggtgaataggacctaaatcccaccacaaaccaaaacgctgcaacgtataatcatagtcacttgaaagataattgcatgccacaacttttttggccaacgtttgtaaagacaacatactaagtttaaaacatcttaaatctaagctagctaactttcaagaaaaccctctatccctaagaatatatcttataactagacttatagcagtaaaaatcaactttggttattctttttaatataaaacgtctaattacttgcaaaggactataaagcccattttcctcagctagaatttttattttttaatgaagtagggggatatgttttcccttcaagacctttgccgaaagcatctttttattcttcccgatgtttttggcgagcatgtactacaacgattaggactgtattggagatgtcacggctcccttcaacgcataggagacgaccacatactcatacgacgggatctcatcctttccaccaacgaggccttaagaatggcgggagaggaaggaaacaatgaagtagtaaagctcttgttactgtggaagggaaatcttcattacgccgtcataggagccttgcagggtgatcaatatgacctgatccataagtatgaaaaccaaatcggcgactttcattttatcttaccattgattcaagacgcgaatacgtttgaaaaatgccacgctttagaacgtttttgtggtgtttcatgtctgctaaaacatgctacaaaatacaacatgctccctattctccaaaaataccaagaagagctgtctatgagagcgtatcttcacgaaaccctatttgaactagcatgcctatggcagaggtatgatgtccttaaatggatagagcaaaccatacatgtttacgacctaaagattatgtttaatattgccatctccaagagggatctgactatgtactccttaggatatattttcctttttgatagagggaacaccgaagctacgttgctaacgcaacatctcaagaagacagcggccaaagggctcctccactttgtgctagaaacgttaaaatacggcggcaacatagataccgtcctgacccaagccgtaaagtacaatcatagaaaacttttagattattttctgcgtcaactacctcgtaaacatattgaaaaacttttgttgctggccgtgcaggaaaaggcttctaaaaaaacattgaacttactgttgtcacatttaaactactccgtgaaacgcatcaaaaaactaccgcgctatgtgatagagtacgagtccaccttggtgataaagattttattaaaaaaaagagtgaacctgatagatgccatgttggaaaagatggtaagatatttttctgcgacgaaagtgaggacgatcatggatgagctttcgattagtccggaaagagtcattaagatggctatacagaaaatgagaacggatatcgtaatccatacttcttatgtttgggaggatgatctagaacgtcttactcgtcttaaaaatatggtatacaccataaagtacgaacatgggaaaaaaatgttaattaaagtcatgcacggcatatacaaaaacttattatacggcgaaagggaaaaagtcatgttttatttagccaagctctatgttgctcaaaacgcggccacccaattcagagacatttgtaaggactgttacaaactggatgtggcacggtttaaaccgcggtttaagcaactaatattagactgtttagaaattattactaaaaaatcttgctatagtatcctggaaatcttagaaaaacatattatttccctgtttactatgaaagttatgactgaagaagaaaaaaacctatgtttagaaatattatataaagtaattcattataaaacaatacaatgttaaaattcaatagatatccatcattaatattgattatattttcgaatattatcttctatggtgcaagataatcatctagcgcgtgaaacatgtcctcttctcttcaggaactttgtcgaaaaaagctgcctgactgcatacttccagagttttttgacgactatgtattgcaactgttaggactgcactggcaagatcatggttcccttcagcgtatcgagaagaaccagatacttgttcaacaggaacccatccatatcaatgaagcactcaaagtagcagcatcggaagggaactatgaaatcgtagagctgttgttgtcatgggaggcagatccccgctacgccgtcgtaggagccctagaaagcaaatactatgacctggtttacaaatactatgaccaagttaaagactgccatgatatcttgccgctgattcaaaatccggaaacattcgaaagatgtcatgagttaaacagcacctgttcactgaaatgcttattcaagcatgctgtgataaatgacatgctgccgattcttcaaaaatatacagactatctggataggtgggagtattgcagccagatgctgttcgaactggcatgtagtaaaaaaaaatatgagatggttgtgtggatagagggagttctaggcgtcggcaaagttacatctcttttcaccattgcgattagcaacagagacctacagctgtattctctgggctactcaattatccttgagaatttgtactcctgtggacaggaccccaagtttttactaaatcatttcctgcgagacgtttcaataaaagggcttctaccctttgtaatcaaaaccatagaatatggtggaagcaaggagatagccataactctggctaaaaaatatcagcataaacatattttgaaatacttcgaaacctgggaaagctaggttcagtatggtgtactcactattgtagtgaatcgtatcctgtaaattttgtaaaaaagcttaaacttttgaccacatcatattgttttagaaatctcaaaccagtgaacaacagtcttatcatacattaaaattccagtaaaatttatattttttttggtaaacaaatgttttctcttcaagacatctgtcggaaacatctttttcaacttcctgacgcttttgatgaatatatattacaagcgctaggactatactgggaaaaacacggatctcttcaacgaataagaaaggacgctgtgtttgtacagcgaaacatcgtcctttctaccaatgaggccctgagaatcgcagcctcagagggaaacgaaagggtaataaaacttctgttatcatgggagggaaattttcattatgtgatcataggagctctagagggtgaccaatatgacctaattcataagtatgatagtcaaattaaagactaccacatgattttatcattgatccaaaatgcaaatacctttgaaaagtgtcatcagttatccaatagtaatatgtggtgtcttatacagaatgctataaaatataatatgctccctattctccaaaaacacagaaatattctgacacatgagggagagaatcaggaattgtttgagatggcatgtgaggaacagaaatatgacatagttttatggataggacaaaccctaatgttaaatgagccggagtttatttttgatatcgccttcgaacggatagatttttctttattaacaatgggttatagccttctttttgataacaagatgagtagtatagacattcatgatgaagaagatcttacttcattaccaacagaacacctcgaaaaagcagccactaagggatgtttcttctttatgctagaaactttaaaacatggtggaaatgtaaatatggcagtcttatctaaagctgttgagtataatcatagaaaaattttagaccattttattcggcggcaaaaatgtttatcacgtgaagagattgaaaacctattattaaccgccataaccaattgtgcatccataaaaacgttaaacttactcttgtcttacctaaactattccgtaaaaaatatcattggaaaaatagtacaacatgtcataaaagatggtgattataccatcatattacttttaaaaaaaaagaaaataaacctagtggaacctgttttaacaggttttatagattattactatagctattgttttataaaacattttatccaagagtttgctattcgtccggaaaaactgattaaaatggccgcgcgaaaaggtaaactaaatatgattatcgaattccttaacgaaaaatatgttcataaagatgatcttggaactatatttaaatatctcaaaaccctagtatgtaccatgaaacataaaaaaggaaaagagacattaattgttcttattcataaaatatatcaagatattcatctggagactaaagaaaaatttaaattattaagattttatgtcatgcatgatgcaactatccaatttctatctatgtgcaaagactgttttaatttagccggttttaaaccatttgttttagaatgtttggatattgctattaaaaaaaattaccctgatatgatacaatatatagaaattctatcgaaatctgagtaaaatttatttttttgatcagagtaagaaaatgttctccctccaggagatctgtcgaaagaacatctactttctacctgactggctcggtgagcatgtgattcagcgactaggtctgtactgggaaaaacatggttctcttcagcgaatcggagacaactatgtacttatacaacaggacctcatcatccccatcaatgaagccctaagaatggcaggggaggaggggaatgatgaggtggtacaactcctattactatgggagggaaacattcattatgccatcataggagctttggagagtgaccattatagcctaatacgtaagctctatgaccaaatcgaagactgtcacgacatccttcccttgattcaagacccaaaactctttgaaaaatgccatgaattagataaatcttgtaacattttatgtctcgtattacacgccgtaaaaaacgatatgctttgcattcttcaagagtataaaatgcatctaagtggagaggatattcaagtggtgtttgaaacagcatgccgttcacaaaaaaacgatattgtgtcatggatgggacaaaatattgcaatatacaaccccgaagttatttttgatattgcctttgataagatgaatgtgtccttattatctatagggtatacgcttcttttcaatcatcatataaataatacgaacgaaaatattaattctttattgacacaacatcttgaatgggctgccggcatgggccttcttcattttatgctggaaactttaaagtatggcggggatgtaacgataatagtcttgtctgaggccgtaaaatatgaccacagaaagattttagattattttctccgtcgaaaaaacttgtaccaagaagatcttgaagaactattattgttggcgatacgtgcagattgttctaaaaagaccttaaacttgttattatcttacttaaactattccataaacaatatccgtaaaaaaatattacaatgtgtaaaagaatatgaaacgaccgttattataaaaattttacggaaaagaaagataaatctgatagagcccattttggcagactttataggatatcatagctatacctatatggtagattttatgcgtgagttttccatccatccggaaaaaatgatcaaaatggctgcacgagaatcgagggaggacttgatcataaaattttccaaaaaagtttgcaaagagcctaaagatagacttcactatctcaaaagcttagtgtatactatgcgacataaagaaggcaaacaactgttaatttatacaatccataacttatacaaagcttgtcatctagagagtaaagaaatgtttaatttggcacgattttatgcacggcataatgcagtgatccagttcaaatcgatttgccacgatctctccaagctcaatattaatatcaaaaacttgttgttagaatgtttaggtattgctattaaaaaaaattactttcaacttatcaaaacaatagaaacggatatgcgttatgagtaacatttttagatgagggaagattctaccaaactaactaagacctttcgctagaatgtatcttattgttaatatagatgagatatgtcattgtgaaaaaatagattaggtaggttgtgaaaaacagattaaacttaaaattatgtgtattatgtaaaattttagaaataaaaatttattttttttattgagggtacggaaaatgttctccctacaggacctctgtcggaagaacattttcttccttccaaatgattttagcaagcataccctacaatggctgggattatattggaaagagcatggatccgtccatcgagcagaaaaagacagcataatgatacagaatgaattggttctttctatcaatgatgctttacagcttgcaggagaggagggggacacagatgtagtacagctcttgttattatgggagggaaatctgcattatgccatcataggagccttgaagactgaaaaatataacctaatatgtgagtatcatagccaaattcaggactggcatattctcctacccatgattcaagatccagaaacattcgaaaaatgtcatgatttaagccttggatgtgactttatttgccttctccaacatgctgtaaaatacaacatgctttctattcttgtcaaatataaggaggatctactaaatgcaaggattaggcatcgtatccaatccctgtttgttttggcatgcgaaaatcggagaattgaaattattgattggataggccaaaatctgccaattcctgaacctgatgccatttttagcattgctgttgctacaagagatttagaactgttttccttagggtacaagattatttttgattacatgcaaagacagggaatcattcaattaaccaatggagttcgcatggttgtgctaaatcgtcacattagcatggcaatagataatggtcttttaccttttgttctggaaactttaaaacatggtgggaatatacatagagccttatcttatgcagtaacacacaatagaagaaaaattctggattatcttattcgccagaaaaatatagcccctaatacaattgaaagacttttatatctggccgtgaaaaatcaatcttccaggaaaactttgaacttgttgctatcttacataaattacaaggtgaaaaatgttaaaaagctggtagagcatgtagtaaatgagaaatccactcttgtgttaaaaattttattagaaaaaaaggaaaatctagtggatgctgttttaacaagacttgtaaaacattctacatatttccaggtgagagaatttatccaggagttttccatcagcccagaaaaattcattaaaatagctgtgcgggaaaagaaaaatgtgttaatcgaggctatttctgaagatatttgggaaaatcccacagaaagaattacttatctcaaacagatagtgcacaccataaaatatgaaagtggaaggcgatttttggtagacatcattcacagcatttaccaaagttactcactaaaacacgaagatattcttaaactggcaacattttatgtcaaacacaatgcaatcacccattttaaagacctctgcaaatatctttggctgaacagaggaacagaaagtaagaaactgtttttagagtgtttagaaattgctgatgagaaggagtttcctgatattaaaagtattgtgagtgaatatattaactacttgtttactgcaggagctattaccaaggaagaaatcatgcaagcctatgatgctttagagtagccatgtattaacattctgaaagtagaataaaatatactatatactaaaaaccaaattagccatttttaactatcttcttcttaaaaactctggataaaaatttattttttttaatttgggtagggaaaatgttctcccttcaggacctctgtcggaagaacaccttcttccttccaagtgattttagcaagcataccctgcatttgctggggttatactggaaggggcatggatctatccaaaggataaagaatgatggtgtgcttatagagcatgatcttactctttccatcaatgaagccttaattcttgcaggagaagagggaaacaatgaagtagtaaagctcttgttactatgggaaggaaatcttcattatgccatcataggagctttgaggactgagaactataacctagtatgtgagtaccatagtcaaattcaggactggcatgttctcctccctttgattcaagatccagaaacattcgaaaaatgtcatgatttaagccttgaatgtgatctttcatgccttctccaacatgctgtaaaatataacatgctttcgattcttgttaaatataaagaggatctactaaatgtactatttaggcaacaaattcaaggactatttattttagcatgtgaaaatcggaagcttgagattcttacgtggatgggtcaaaatctgccaattcctgatcctgagcctatttttagcattgctgttgtcacaaaagatttagaaatgttttccttagggtacaagattgtttttgaatacatggaaaaccaaggacttcatttaacccaggtagttcgtatggttatgctaaatcatcactttggcatggtaataaataaaggacttttaccctttgtgctggaaattttaaattatggtgggaatgtaaatagagccttatcttatgctgtcacacaaaataaaagaaagattttagaccatgttgttcgccaaaagaatataccccataaaaccattgaaagaatgttgcatctggctgtaaaaaagcatgctcccaggaaaactctgaacttgttactatcttacataaattacaaggtgaaaaatgttaaaaagttgttagaacatgtagtgaaatacaactctactcttgtgataagactcttgttagaaaaaaagaaaaacctgctggatgctactttgacaagatatgtcaaagattctacatactttcaggtgaaagaatttatgcaagacttctccatcagcccagaaaaattcattaaaatagctgtgcgggaaaagagaaatgtgttgatcaagggtatttctgaagatatttgggaaaatcccgcggaaagaatcaggaatcttaagcagatagtgtgtaccataaaatatgaaagtggaagacaattcctgataaatatcattcacaccatttaccagagttattctttgaaacctgaagaaattcttaaattggcaacattttatgtcaaacacaatgcaaccacccattttaaagatctctgcaaatatctttggctgaacagaagaacagaaagtaagaaactgtttttagagtgcttggaaattgctgataagaaggagtttcctgatattaaaagtattgtgagtgaatacattaactatttgtttactgcaggagctattaccaaggaagaaatcatgcaagcctatgctttggagtatgccatgtattaaatttctgaatcagtaagcaatagatagattttagaatatgctgtattaagttagtttctgaataagtaattaatagatagattttagtttatgtaaaaatgttaacatttgttcataagttttagataccattttagagttacttttttagatattactattttagccattattatcttaaataatcactattttagataggtccccgtattaaaaaccaaattaaccattatctatgtttttaataatactttttaaaaaccctccataaaaatttattttttttcataaaagtagagaaaatgttctccctacaggatctctgtcggaagaacctttttcttccacttgagcccttaggcaagcatgtggttcaacggctgggattatactgggaaggccatggttcagttaaacgagtgggtgattgctttatatgtgtagaccagatttggatgctatcaatccataaggctatacaaattgcagcctcggaaggaaatgagaacattgtcaagcttttcttactatggaaggggagtctacaatatgccatcataggagccttagagggcaggcaatatgatctgattcaaaaatattacaaccaaattggggactgccatcagattctaccactgattcaagatccagaaatttacgaaagatgtcatgaattaaatgttacatgtacctttcaatgcttatttcaacatgctataagagataacatgctgcccattttccaaaaatatggagaagatctgaatggaaacaggagaatggttcaacttctgtatgagatggcatgccgattacaaaattatgatatcatcaaatggataggatctaacctgcatgtttataacttggaagccatttttagcattgcttttgttagaaaggatttaactttgtattctttaggctacatgcttcttctgggtagaatgagtactgaagatagaaactttatctcaatcataacacgccatcttgaatacgcatcaaaaaagggactttttgactttgtactagaatctttgaaatatggaggtcaagtggatacagtgttgtttcaggctgtaaaatacaaccataggaaaattttggcccattttattcatgaaattccccgtgaaacggttgaaaagctgatactccatgctgtggagtcacgggcctccagaaaaacattcaacctgcttttatcttccataaactactgtgtgaacccttttgtcaaaaaactactgcacgctgtggtgaaacacaagtacatgcttatcataaagcttttgctcgagcggcccaaaaagaagataaacctggtagatgctgctctattcaaacttgtaaaatactctacttatacagaaatagtaaaatacatgggtgagttttctgtggacccaaaaagggtggtcaaaatggcagcacgactcatgagagtggacctgattaaaaagatttctaatgatgcatgggaagataaactagagagaatcaagcaccttaaacagatggtaaataccatgaaccacagaaatggaaaaaatctattgatgtacaatattcacaatattactggatatacctatctgaacaccaaagaagcatttaacttaacaagattttatgctgtccacaatgcaacatgtttgtttaaagaaatgtgtaaaagctgttttgtacatgataaaatacagctcagagaattgcttgaagattgtttacatattgctaataggcatgattatatccagattgcagaaaccgcagatgaatgtatcaaatatatagatcttattacatttaagtaaaccatgtatatatcaagtaaatccagattaaatcaggctaattgtaaatagttgtagataccatataatgaatgttttattaggatagtagttcagttaagatagtagtttagttaagatagtagtttagttaagatagtagttatgttaagatagtagttctgttaagataatagtttagttaaaactagttcatgttaagttaatagttttgttaagacaatagttcatttaagtcaatagttcagttaagtcaatagttttgttaagtcaatagtttagttaagtcaatagtttagttaagtcaatagtttagttaagtcaatagttatattaagacattagttctgctaatacattagttttgttaagataataaaaatttattttttttcatcagggtagagaaaatgttctccctacaggagctctgccggaagaacatttacattcttccttaccccttggctaagcatgtacttcaacaactagggctgtactggaagggacatggatctcttcaacgaatcggagatgaccatgtactcttacagcaggacctgatcttttccatcaacgaggccttaagaatggcaggagaggaaggaaacaatgaagtagtaaagctcttgttactatgggagggaaaccttcattatgccatcataggagctttagagggcgaccgatatgaccttatccataaatattatgatcaaattggggactgccacaagattcttcctttaatccaagacccgcaaatctttgaaaaatgccatgaattgagtaactcctgtaatattcgatgccttttagaacatgcagtaaaacacgacatgctttctattcttcaaaaacacaaggagcaaataagattacacatggcattaacccaaatactatttgaattggcgtgtcatgaacgtaaaaatgacatcattagatggatcggttattccctgcacatacaccatctagagactatttttgatgttgcattcgcccataaaaatttatccttatacgttttagggtatgaacttctcatgcacaaagtaaatacagaggctgcatatatagaattacccaatttgctatcatatcaccttcgaactgcggcggcaggaggtcttcttaactttatgttagaaacaataaagcatggtggatatctggataaaacggttttatccgcggctatcaggtacaagcataggaaaattgtggctcattttattcatcaggttccccgtaaaaccgttaaaaaactgttactctatgctgtgcaggctcgggcccccaaaaaaacactgaacctacttttatcttccttaaactactccgtgcacaccatcaccaaacaactcgtacacaatgtcgtcatctacagttccacgcttatcgtaaagcttttactcatgcggcgaaaaaacaagttaaacctagtagatgccgttttagccagacttgtaaaatattccacctatacagacattgtacaattcatgggtgagttttctgtgagcccagaaagggtgatcaaaatggctgcacgggaatccaggacctttctgattgaaatgatctccaaagctgcttggggaaatcacccacagacgttgattcatcatctcaaacaactaaccaataccatgaagcctcaatctggaaaagaccacatcatatataccatccactatatttatctaaactctaatatgctggtagcggaggaggaaaaaaatatttttaaattagcaaaattttatgcgaatcataatgcggtaaacaggtttaaacaaatttgtgaagactattatatattagatgcacgatttaaaacacttattttagaatgttttgaaattgccgtccagaaaaactatcctagaattgcaaatattgtggatgactatattcgattccttttttacaggggaaatataaccgaggaagaaattcgtgaagcctattctttaaaagatgctgaggtttatgtagatttaaaatggttacaacaaggagaaatggtttaaaccaaatccggtttaaactaaatccaatttaaactacatttggtttatcattagtcattgaaaccatcgaaaaaaaagctatttgtttatccccataaactcatcttttttttgtctcaaagtttgacactaaaattcagtgttttatagtgtttataattaagtgttttgcatgcattgcagaaattttcatcttttttaattggttcaataccacatgtcatacaatatgttgtttgattatcaagattaactttatgaaaggaaagtaagtgagccgcaaatttaaaagtaaaatatctttcatttaaaatgatcttatgaatgtattttcgataaggaggaatgaaagcatttgccaaaataaatcgcataaaaggcttggaaaaacccatatcttctaatcttttgtgggtataaaccctattttggtgttttacaaaaacttcattgttataatagtcgttatagctatcaatcatttttttaagtcctataatgcccaaggttgcacgcataaagccacagtttctgctccaaaaagcatgcacctgtaaagggtgcttttcatataaccaattacaaaatttcattccgcaacagtagcatgttatttcagtgggggatgtatagaataatccggcattcgaaaatttttcataattttttatgtcatggattgcgaagctttgatttcgtgcatctatggagctatagcctacatatttaggttttacttcaaataatcgcaaagagatgtatggatctatcgtatttattttaggaaacatttcataattttaaattcttatatataatataaaaaaaattacaaacatttgtaatgatcatcctcaattgaaggctgagttgtaggctttatttttctaattatacgaagaaggtaggttctcataaagccttcaagatgactattgatgtttccaatacattttctcaatgagttcataaacccagacattttgctaatggcttggcaaagtgccaacaagttgtccacaaagtactggtagattgccactagctatagctagctatagtgagccaacctctctgtatgtattttatatatttcattttttaatagatttaatatttttataaaaaatatttagttttttatacaagaatgtcgacaaaaaaaaagcccacaattaccaagcaagagctttactccttagtagcggcagatacccagttaaataaagcattgattgaaagaatctttacaagtcagcaaaaaataatacaaaatgctttaaagcacaatcaagaagttattataccacccggaatcaagttcaccgtcgttacggtgaaagctaaacctgctcgccagggccataatcccgccacaggagagcctattcaaattaaagctaaacctgaacataaagccgtaaagatacgagcattgaaacctgtccatgatatgttaaactaaactataaagtcatattcttctttatcgttattatcttcaatatatttttgccaatcgaaatcgaataaattcagatcctggacatttaaatacttatcatcgtacattttaatataatttaaacatgagttgttgtcaaaaacttttagcgtttttgttaaaattatcatatgaataatttccttattaagagttgccggaataatacaaaacctatttttaggtacatcatccatgataatagtaaaattagtaaaaattgtttcttgtttttcttttgtttcaaataaacgttgtaaggttaaaggtttctcgttcaatggtttctttgaagataaaaagaatgtataatctggtttaaaggtatttttggtttcaatcgtgattccatctgcttgagcatatactaaaccagaccaaatataacggtccactattacaatataatttagcttaagtagcactgcaatttctgcgataaattcactacgatgttttgtaaataatttatgtaattgttccgatgacatttctatggttttatttaacacctgcaatataagatcaccggtggtcgtgtctggattaggaaaatgtatacatatagcattataatccatgcattccaatgtttcttttaatttcattgcctgtgtgctttttcccacaccattgattccctcgatggcaatgagtattccacgcatgattaataaaaggaaaaaaagaattcagtttttaacatttcttacaaatctttttttatacaacattgtacaacactgcattagcggtatatgatgttatagcttcattaaatatttgcttttatataatctttaccaacctatatttggtagatcactgcagatggtcataaataggccataactaagataaaaattatttcagacgctactacggtagtattattaaaatcatgtgtggcaatgtatgacgtcttaatagataaaacatttaaggaaaacaaatttgaataaaaaaataattgttatgatggcgttgttacacaaagaaaagcttatagagtgcatctatcatgagctagaaaatggcgggacaatattgcttctaacaaaaaatattgttgtgtcagaaatttcatacattggcaatacttataaatattttacctttaatgacaatcatgatctgataagcaaagaagatcttaaaggagcaacatccaaaaacattgctaaaatgatttataattggattataaaaaatcctcaaaataataagatttggagtggtgagccgcgtactcaaatttattttgaaaatgatttatatcatacaaattacaatcataaatgtataaaagatttttggaatgtttcaacttcagtcggtcctcatatctttaatgatcgtagcatttggtgtactaaatgcacatccttttacccatttaccaacattatgtcgcccaatatattccaataaattagatatctttgctattaaaatagttaaaaaccttataggataattaggtactttattacgataaattatgatattttataattagttactttattataattaatctctttattaatgaattatcataagataactaattatttttttccatatatcagataataaatctgatatgggctaaaagtatgtttcaaactatttacaatagaatttctgttaagaaaacatacataatttgaataaaatttttttaaatatcaccgaaacaatcaacatggtgttaatagagtttttaacaggtttcttctatttatatggaaagagactgttttccattagtaaagtcatggacatgatatgtctagactattataccattattcctgctcctctggcgatgatgttagcggcaagactaaaaaactatgacctcatgaaacgactgcacgaatgggaaatctctattgactacgctctacttgtagtagatgatgtgccgtctattgactattgcttaagtcttggcgctagatccccgactagagcacaaaaaagagaactgctgagggacaacacgtttaatcccgtgtataagtatcttatgaactgttccggcttcccaacaaagagagaaaaaaacattccttgtgatgttcaatgcgaaagactgcaaaaaaacattataaaagaactggtatttaactgctctgtactgcttgaaatggtactgcacacagaaagagaatatgcatacgccctacactgtgctgcaaaacataaccaattgcccatcctcatgtattgttggcaacaatccacagacgcggaatctattttgttgaaaacctgctgttctgataagaacatcaattgttttaactattgtattctatatggcggcgcccaaaatttggatgctgcaatggtggaagcggcaaagcacgatgcccggatgctgataaactactgtgtcatgcttggtggaagatccttaaacgaagcaaaagaaacggctgccatgtttggacacattgaatgcgcacaacactgttttaaactgcagtcttacgtcgtggacacatcgaatacagacgacactgattaaagcgacaatcttacgtcatgaacgactgtcttttgagtatctatacttacattatatttttttatgaaaaaaatataaaggttgtatacaaacctttgtatacaagaaatttggatcattaaacaataattaatttggacacaggaaacgatctagatcgatcaaaaagctattttttttgcacacagaacatttagataattgagagattactttccatacttgttaagcttttttacacacaggaactttggattctgttcaggaagtttttcatagacattatgtttacagccagtaataataattttgggctttttcttaaaccaccggtggaaaacatccagcttgtaaagagggaaatgcatgtagagaggttttggtagtcatggttaagagatttgactaactccatgtttcctgtaaagactgcccagtcccaagcagtaaaacctctatgatagtctttttgagtcggatctgctccaaattttatgagagaaagcatatttaaagaacggccccgtattgcggccttcatcacaggagtcatcccattaaaattcggtaaacaaattctggtcccattttttccgaaatagcccaacaccccttccaggattaaatgattttttttctcagctaaataatgtaaagcagagtttccatctttatccctcctatgagggttaattatttctccaggataagattcttgttcaaaaagaaattttaaaaagtctatacgtccgtagatgcatatccacatgaataccgaggatccatttttatcgcatctattgacaatccacggatctgttttaaaaaattcctcaaatagtgtaagattcccatttctaatatgttttttaatccatttaacaaacaagttttctatctccctttctggaaacatgtgttccattttgaatgtcgcccctactccactatatgattttactcctttaatttttaatgtccttttttttcggacttctttggataagctgtttattaccatctttaaatgccttatagcggggaggagccaggcccttttcccatatgtgcggtaattcttggtgtttatgcttgcctttggcataaccaggccagtatttttcgatatattcagggtttgtttttacgtattctttaaaggtccgataggcttcttgaatacaggtaggctcaccggtataatttccatgttcatcttcctttaaaaagccattaaccctgtcctttctccacttaagattgtgctttccaaaaatgcgatcaagatcttgcgcctgctggggtggaatcataaatccctttttaggtcgaagctttttattttttccatagcttcggccatcgcgttgcgaaacagtggttaggacgcctgatagtctttccatgggcgtcgcatctaatcctatccatccaccctgatgaatatcaatggcaacaagctctcctttattttgggcaagccaagtttccaagaatgccatgctttcttcccagggataaggcccgccaacaccacgggttgtccaatcttgcaaggactccaggtccgacacctggtaaggctctaaagaagacggttccttgtttttgtactgcaaataagatttaatgacccatttataccatgtgtcgaaccgcagcgtggcgcctccaaagtgaaagccgtcgttgattttaggatatctgcaacatatttcaaccgtacgtttgagttctgcaaaagcggccttccaaggaagtctttcgctgcgggtaagacggtctattttgccctgcgtgccatagcgtatggcatgtcgtgccaattgcaacaattctgacaccgatccgtgggccccgatccagtttatcggataggcaacctccgaagggtttaaaagatgctcgtaaaagcgtggatcttcagatgccaaggcgtctgcaaaggggataatgctagaaaacctgtctagacatacgttttctgtgtttacttctaaaggtagaaaaatggttgcgtgaggcttttgaacctgcttgttcagcggtctgcatatgctttgaataatgtctctaggactatgtcgcggcgctgcaaaaaataccgcgtttagttctggaacctctacgccctcttgaaagagtcgacagtttaataaaataacgggttcctttgaggaacaaaattctgtaaatgttttgaggataacctgtcgcggcagggttgagtgagctatcagggcatagaccccttggtctaccaacgccgcgtatagctccttggcctgtttaatatcacgggtaaataccagcattttaggagccggtatattggtttttaaataggctaaggccattataatttgctttactatgatctgtttcgtggtctcctctttggtactcggttggtgggccaatttaggcgcggctaccatctgcaattcaaaatcatttacatagccggcctctatgccttctcgcagatagtagcgaaaggcaacgccgccaaaaagttcacgatttttcatggaaagcggggtgtcgtacctgggcgttgccgttaaaaaaagtcggtgcccttttttaaagttgagcaacacgtgggtaaagggccgtgtctcccattcgccgcaaatccggtgacattcatcgctaataataagatcgaaatcatccaccagtagcgtggaggattggtaggtggcaatcacaagaagagaaggggcctcccgtatccgttttgcaataaagacaggattggtggtcatttctatattgtcgtgatttagcacaatgcgggtctggtcagaccccacaagcaaaacgttcttcaaagaaattccatactgatagagtttttccagagtctgccgtagtagggacaggcccggcaccaggtacaaaacttttccttgaagataattggagaggataagataggcgacgcgagttttgccgcatcggcaggccatctgcagaatggccctcccacttcgccgcagctcctgatagcccatattggccgcctccttctgataaagtcgatcctcgattgcagtccgtgtctcatctgtagaaaaaaataatacgtcatctgcgaaatgttcatcttccacaggagttatcaccaggtgtctcagtttctccttgcttatcagcggatcagagggcaaagatggctcaaccactatcgtggaatcattcatctcataggcgggagaatcacacaaagtatagcttatgtccagacagtttgcaacatcctcagccaattgttttattttttcgggtaaaagacatacgagttctttgtttttgacgcgaaaaaactgtgcacaatataacacccctgcttcaattttttgcgcatccttctttgtagatgtttccaatgtgaaacaatacttccattcatccgtaaaacaggttgtataagatccatcatgaagcctagcggccaagtttcctgtgtgcccaactttatgtaaggattgggcctccagccagggatgaaccgccacgtaaaatcctgcgcacatgctatatcaaattgcagtttcttaataactgtacacaggatctgaaaaacatgtgattacaaaatttagataagaaatatttaatattaaaaatcacagaatacatgtcactgtgtagagagaaagccaaaaactcctcttgaccgccgtgggaaatcatccagggtagtaggttgtgtttcataaagttgtatgccgtagtgatcaccgtggactccagatggttattggcatctttgcaatactttgccatcttggcagaaaagacgataaatccacaaattctaccccagttgataagatccttaaacagctcagtcacaaccccagtaaactgggttttaatttcttgaacactcgtaagagaaaaggtaattgtaacctgtttgttcaaacactcatcataataggttaaaattttttttatttgttgttgatatgggctaagctcatgctctgaaatatcattaatgtaatatttaatatatcccactagtatttcattaatgatattatgatatattaactcttctccctccatagcggcaccctatatttttttatttaggtttcaatgttatcacaattgcgatacaattgtgatacaattgtgacacaactgtgttgtatacaacaaatgttaggccacgtatagcaacctatatgttaagaaatatttttatcccaacattagttggaaacgagcagccgcaaagaagtcatttaaaataagccatttaaagatttagaatttatatgtatacaactgtacaatggaagcagttcttaccaaactcgaccaggaggaaaaaaaggctctccaaaattttcatcgttgtgcttgggaagaaactaaaaatattataaacgattttcttgaaatccctgaggaacgatgcacctataaattcaactcatacacaaaaaaaatggagcttttatttacccctgaattccacaccgcctggcatgaagttcctgagtgcagagagttcatattaaactttttgagactcatttcgggacatcgagtggtattaaaaggccctacatttgtttttacaaaagagatcaagaatctgggcattcctagtaccatcaatgttgactttcaggccaacattgaaaatatggatgatctacagaagggaaatctcatcggcaagatgaatatcaaagaaggctaaataaaacaactaacatcaaaaaacattaaaggctatgttgtggacgatgcctttgtctcaatagtttcgaggtcatccaataactcatgtaacgtaaaaaagttggtccatttttttgaaaacattaaaagacgttcgtcttcataaataaaaaagtcattcgaaggaaaaatgatatactcaataccatagtcttgtaatattttttttaggtctctcagggtccagggatttaccaggcttctacgcgaagtgagcatcataaaaatatctaatattttttgcgccataagccagcgcggattctcattggcccacaaatcaacaataattctcttatcaaccgtgagcattcctacttgattcgaagaaatgattagatgcccagcagtccaccccatgagtagataacgcagcgttgtagaaatgtcacatatggaaggcattcctccacaacatgaacccaaattaggatgcgtgtgaaacacaaacatagcaggcttgttggccaccctgctataaatatcagcaggcatcatagcctcgctgccaaaataaatgttctctcctgccctataggggcttggaatgatttccactatctcgggtacaccgtttatcatattaatgcggccgcaccattcacggtcatcgtccaaaaattttttgatggcaccccgaacattgtcccagttaagcaacagagtattcacaatctcattacgctccgcccagtattccttaaaacttcttttagacttgctgagctgttcccaggattcgaactcagtccaatgttttttttcttttggggaagacttcccttttgaaacattttttgcggctccaccatctacactatgattttccaaaataatctccttcatcgtttgagttatatgggcattgctaagcaccttagtggtaacctgtttacctatgtgatttagcagaaaaccaagtttgtccatttgtgtctcaaccatttattcttaacaaaacaaaaaaaattaaaaatcatcgtcgtttaaaaagagtttgaaggcaaacgcatcatccttaacacagttctgatactgcgtaggtcttaactcgaaaaagttggttttttctacttcattaagaaagaatttagtcatctgaggaaaagggtttcccaccttataaatgcttttgcactgcatcatgaagcacaaattatctgtaaagtagcgtatatattgaaatagcatttcttttgaaaaaccgggaactcttcctcttgccttgtcaaaggcatagttaataaactcatccaccaactccacagcctccttcaaaattttgtgaatgatcttttcctcgggaatgttatacacgtaatttgagataagaaaacacgcaaaactacagtgcatcccttcatcacgtgagataaactcattatagcttacaagccccggcataatattctgttccttaagaaactggatcgccacaaagtggttttgaaataaaatgccttctacggcggcgaagcccaccagccgctcacctagagtgttcctgtcggggtccatccactgccgcacccactgcgccattttttttatgatagggtgtttttcaatgccgctaaagatgcgctgttgttccttctcatccgggatcagcgtttttacctgtattgagtaggcttcgctatgaacgcactcttgggcagcctgcattgtataaaagtataacacttcctttactttaatttcgcgcataaaattggttaaaaggttttcgataacaatttcgtcggcaacaacaaagaaggctaaaatttgtttataaaattcgcgctgtggctttggcatggcttcccaatcatcaatgtccttacacatgtccacctcctgcgccgtccacgtcaaactttctaattttttataccagttccaacattcggggtgctgaataggaaaaatagtgaaacgttgggaattttcaattagtaattcctccatatttgaaataaatattaacatcttcaaatttattggctgccatggagacgttttttattgagacgttggcatctgatgtgtatggaaaggcgttaaatgttgatttagatagactatcgcaggcgcaggttaaatatacccttcaagagcttatttcctactgcagcgctctaaccattttacattatgactattcaacccttgcggcgcgtctttcggtgtaccagctgcaccagtcaacggcctcctccttctcaaaggcggtgaggctgcaggccgcacaatcctgctcacgcctgtccccccagtttgtggacgtcgtttacaagtacaaagccatttttgacagctacattgactatagcagagattacaagctgtccctcctggggatagaaaccatgaaaaattcttatttgttaaaaaataaagatggggtcatcatggaacgcccgcaggatgcttatatgcgggttgccatcatgatctatgggatgggaagagtggtcaatatgaaaatgattctgctaacctatgacctgctttcccagcacgtcatcacacacgcgtcgcccaccatgttcaatgcaggcaccaaaaagccacaactctccagctgtttcctgctaaatgtaaatgataatttagaaaatttatatgatatggtcaaaacggccggcatcatttcaggcggcggcggtggaatagggctgtgcttgtcaggaatacgggcaaagaatagttttatttctggtagtggtcttaaaagtaacggcatacagaattatattgtgctgcaaaatgcttcacaatgctacgcgaaccagggaggcctacgtcccggagcctacgccgtctacttagagctgtggcaccaagacatctttacatttttacaaatgcctcgcctaaaaggacaaatggctgaacaacggcttaatgcccctaatctcaagtacggcctatgggtccccgacctattcatggaaatacttgaagaccaaatacacaacagaggcgacggcaaatggtacctcttttcgccggatcaggcccccaatctacataaggtctttgatttggaacggtcgcagcacgaaaacgcacaccgcgaatttaaaaagctttactatcagtatgttgctgaaaaaaggtacaccggcgtcacaacggccaaagagattatcaaagagtggttcaaaacagttgttcaagtagggaatccctatatcgggtttaaagatgccataaatcgtaaaagtaatctttcacatgtaggcactatcacgaactccaatctttgtattgaagtcacaatcccctgctgggagggtgataaggctgaacaaggtgtttgtaatctggccgcagtaaatctagccgcctttatacgtgaaaatggctacgactaccgtgggctcatagaagcatcaggcaatgtcacagaaaatttagataatattatagataatggctactaccccacagaagccacgcggagaagcaatatgcgtcaccgacctattggcatcggggtctttggcctagccgacgtgtttgcgtctttaaaaatgaaatttggttcacccgaggccattgccatggatgaggccatccatgcggccctatactacggggccatgcgacgatccatagaacttgcaaaagaaaaaggaagtcatcccagctttccggggtctgcggcctcaaagggtctactgcagcccgacctatgggttcgctgtggtgatttagtttcctcctgggaagaacgcgtggcacagacgacgcagggtgtgttgacgccgaaaaggtggtcgcagctacgcctggcggctatgcagggacttcgaaatggatatgtcacagctcttatgcccaccgcaacctcctcaaattctacaggaaaaaacgaatgttttgagccctttacatccaatctatatacacgtagaacgttaagcggggagtttattgttttaaataagtatttaatagacgatttaaaagaaattaatctttggacagaagccattcaacagcagctactaaatgcgggaggtagcattcagcacattttggatataccggccgagatccgcgatcggtataaaacctccagggaaatgaatcaaaaaattttaacaaaacacgcggccgcacgaaacccctttgtatcccaaagtatgtccttgaactattacttttatgaacctgaactaagccaggtacttacagtgctcgtcctaggctggaaaaaaggtttaactaccggttcctattactgtcattttagccctggagcgggtacccaaaaaaagattataagaaactctgagaaagcgtgtaatgcggactgcgaggcgtgtcttctgtaggtgtctcgcggtaaaagagcagcggggaccatatggtaaaccccaacaagaggataatgaataaaaaaagtaaacaggcatccattagttccatattaaatttttttttcttctatataatggaatattttgttgcggtagacaatgaaacctccttgggggtttttacttctatagagcaatgtgaagaaacgatgaaacaataccccggcctccattatgtcgtttttaagtatatgtgtccggcggatgcagaaaatacagatgttgtatatttaataccctcgttaaccttgcatacccccatgtttgtagaccactgtccaaatcgtaccaaacaagcacgacacgtattgaaaaaaataaacttagtgttcgaggaagagtctattgaaaattggaaggtttcagtaaatactgtgttcccccatgttcacaacagattatctgcgccgaaactttccatcgacgaggctaatgaagccgtagaaaagtttttgatacaagcaggacgactcatgtctctgtaaatgtctcttcctttatgggtgacgtctcttcctttgccgaggaagtctctgttatgggcaagaggtttgaaacaacgcaaggactctgcttaatctgctgtctcacaaagggaatcaaactacctgctttcgtatttttaatgtagtaattacccttgttgtgatgaattttaagaccatagcgtagtcccagtactttattaatgaattttaaaattgtttgagggtccgttttattgggctttttaagcttaaactcaaagctgatcgcgcttaaatcatactgaacaaattcatcaacgagtttcgtcattaattgttcattggtcaatatattagggtcctgaacgcatttaaagccgcacttagttaatagcataatagcgtacatatgagattgaaaactataattaaattgtagatcatgatgctctgcgtgttgcatggcccattgatgaaagtttaattcctgagtttgtaacatagtgagcgactcgtatactgtctttccgcggcttatttggacacggccagtatagttctgttttgtcataaaactattgtattgttcaacaaatttgggagtaattttatgaccgtgccatgcataaaattcgagtagtttatacttttcatacgcaaataggtcttgctggtctactgtgatgccttcctttaagttttgtttaatttgtaaagctttattggcatcaatggtttcagccgaggcaatgtttacatagtcctggtgtttaatttccattttaatgcttgtatattgtttgactgtctccagcttttcacccgtcagtataaacaccttagcgccggtgtcggcgatctggttaataaatcgggttataaagtgattttttgatagatgttgtatccgcattgtttcgagccatagatggtagtatggagttttataatatatcggcctacctgtttccttactatacgtgaaggaaagctggtgattgcttatggtctgaaaaagggtgtcacgtttttgtaacgtaaacatttcaatgtcttcgatggtttctggatagtaattttgtttcccctgtaagcagattttataacacttactttttaattcacgcacgcggcccaacatttggcaacatgtttctacgtcacacgacatattgttaaaaaagccgtataaaacatcaaatctcttatcttcgtatgaaacacccgctgaaatcgtgggcgtatagataaggatatcaacgagcccccaataatacgatacattattaaaatgggattcccgttcatgagcagtgcttttagaactataaaacccaatttttttttccggaaactttttttggataaatgattgcaacagccgggcctccattaatgaatttgtagggataacaatttttttgtcttctagcaaatcctttaaaaggttatttaaccaagtttctcgtgaagaggtaaaataatacgtgtcatgctgggcccttttatattgattccagtgaaagaagatagggacatccccgcgaaaacgctgtagaatattatacgttcgatttcctaggtttgcgtccaagcatataacataatttgccgtttcgagcatccacatgaaaatggcaaaagagggagcaaagtatttgtgcaggccgctattgaattgattaaaaatcgattctacctcatccaaaataagtaggtctacaggctcggctgtggaggttagccggaaaagtgattctacctgaatgatgactctttcgtagctgtccaaatctccagttacttcgctgtacaatgtgaaattcggtagccgggattgtatattttttgagaagatctgtcgaaacgtcacaaaccgtatggtttgttgttttgaaatagaattattgccgtagtatttttgcaaatagttgcgcagttggacggttttacctattttcatttgagcctttacaacaagcgtagggactcgttcatattctcgcatactactttcatcatagatgtgtttttgagtatcaggcagttcttcaaagagaatggactcatgaacctctatgctctttgtcatcacttggtccacatatgtttccacaaaattatttgtgccggaaaggctgcccatgagaaggctatgtttattgtcatggcgacagtgttgatacactttgtttcccgtgactcttaaaattagggtattgtccttatcatgcatacgcttacatatttcgcagtaacttggacttgtacgtttaaacaatactaaatttttatgaacacggaggaagcaatgatttttacatagtgttcctgcaaattttaatacctcttcaagttcactttgttggatagtatcgcaggaactcggtgttgtttcttttacatttgtgaagatacaaggtaaacacgtcgtttcaaagggggttgctataagggtatcactctttttcgtggttgtactggtctcaaacacctctgcaagctcctcattaaacattttaacacgcatgctaccttttttatgagaccctatgatgcgaaaattttgaatacttttgttgacctgggggtcaacaaaaggataaacgtgtttgggaagattttctaacactttggatgtaaagactttggcctcattattgtttaatactgagtatgtataaagtatgatatgaaaggagtatttaagttctcgctttttatttaatccgatagaatctgttagcaaaatttgttcacgcgttagattgatgttataaggtaaagaatatgtctcgtaaaatacatccatgatgacgttaattatcatgtcaaggatgtcatagacattgtcttcgacattatcattgtcatcaacattgtcatcagagtatgacttatttaccggaaagtcgatgtcaaattttaagcgctgaggcaaaaacccaaataccacttcgtggaaacacttctgctcaaagggctgagccgcctcccactcccaaaagtcatcacgacttgaaaaaactctaaaaagattattatattcatctcgcaccacgaagtgattctttaaggtttcgagagaatatttatcctctacggcttctccttgggagttacagcgaagaaacttgaatgtttcttgcattttgatatttaaaattaaatcaattatgatgcggccgctaatgcggcggttgacgcggccgcgccgctgacgcagccatcatacataaagcggcatggccgttttataacgactagtcggccgttatatgacgaactatataaaaatgaattcttttaattagagttaagtattgttgattgtataatccatcatggttgagccacgcgaacagttttttcaagatctgctttcagcagtggatcaacaaatggacactgtaaaaaatgacataaaagacattatgaaagaaaaaacgtcttttatggtatcattcgaaaactttatagaacgttacgataccatggaaaaaaatattcaagaccttcagaataagtacgaagaaatggcggccaaccttatgaccgtcatgacggatacaaaaattcagcttggagccattatcgcccaacttgagattctaatgataaatggcactccacttccggcaaaaaagacaacaattaaggaggctatgcccttaccttcatcaaacacgaataatgaacaaacgagtcctcccgcctcaggcaaaacaagtgaaacacctaaaaaaaatcccacgaatgcgatgttcttcacgcgtagcgaatgggcatcctcgaatacttttcgagaaaagtttttaacaccagaaattcaagccatattggatgagcagtttgcaaacaagaccgggatcgaaagattgcatgccgagggtctttacatgtggagaacccaattctctgacgaacagaagaaaatggtcaaagagatgatgaagaagtaatatttttggtaaaaatatttttatcaaaattttttaccaaataataaaaatatttttactttttttcttcataatatacatagaatgcctacaaaagctggcacaaaaagtaccgcaaataaaaaaacaacgaagggctcctccaaatctggttcttccagaggccacaccggcaaaacccatgcttcttcgtccatgcattccgggatgctctataaagatatggtaaatattgctagatctagaggcattccgatttaccagaatggatcgcgtcttactaaaagtgaattggagaaaaaaattaaacggtcaaaatgaatataatcaggaaacttaagcctggaacaattagccttgtgctgggacccatgtttgccggcaaaactacgtttcttattcattgcatttacatgctcgaacgtttggaaaaaaaagtagtcttcataaaatctaccaaaaacacccgagacaaaactattaaaacacactccggtatacagctacgacccaaacaatgtaaaatcatagaaagcacacagttatctgacgtgggttctctcaccgatatccatgcagttgtcgtagatgaagcgcatttttttgacgatttaatcacatgccgcacttgggcagaggaagaaaaaattattattcttgcgggactcaatgcttccttcgagcagaaaatgtttccgcccatcgttcgtatttttccttactgcagctgggttaagtatattggccgcacctgtatgaaatgtaaccaacataatgcatgctttaatgtgcgtaagaacgcagacaagacgcttatccttgcgggaggaagtgaactgtacgtaacatgttgtaacaactgtctaaaaaatacatttattaagcagttgcaacctattaaatattaaaaatcttatacaataatggatcattatcttaaaaaattacaagatatttatacgaagctcgagggtcatccctttctttttagcccgtcgaaaaccaatgaaaaagagtttattactctgctaaaccaggccttggcctcaacgcagctttaccgcagcatacaacagctgtttttaacgatgtataagctagatcccattgggtttattaactatattaaaacgagtaaacaagagtatttatgcctgttaattaatcctaaactcgttactaagtttttaaaaataacgagctttaaaatttacattaatttcaggctgaaaactttttatataagtcctaataagtataataatttttacaccgctccctctgaagaaaagactaaccatcttctaaaagaagaaaaaacttgggcaaagattgttgaagaaggaggagaagaatcctaagtcgcttacatttttttttgctatttttatagaatgtacacgcatgttgatgttgtcggaatagctgaagcctcagcggccctctacgtgcaaaaagatagggatcgctacttagacgtgctaacaaccattgaaaactttatttaccaacacaaatgcatcataacaggggaaagcgcccacctactctttttaaaaaaaaatatttatctttacgaattttactccaacaatgtggcggagcacagcaaggctttggcgaccctgctttataaacttgatccggaatacctcactcgttacacagtactcattaccaaaattcccaaccattggtatgtgattaacgtagatcagcgagaatttgtgcgcctatatgccatcccggcagttaaacaacacttaccgattcccattttacccttctattgcaccagcgcactcacccagcaagaattgttttgtttaggacctgaactgcagttaatacaaatatattccaagctctgtaaccccaactttgtcgaggaatggcctacgttgctcgactacgaaaaaagcatgcggatgttatttttagaacagtttccgcaaagattggaaatgacgggcgggaagaaggaggagaaggaaaagcatgaaagtatcattaaaaaaataatactagaaatggtctctacccgtcagcgaatcgttgttgggggttacatacaaaaaaacctgtacaaccatgtactcaagaatagaaatcgtttacagcttattacgagcttaaatatttatgaagaaaaagatatcatccagcaattttgtgattcaaatggactgaagatcaaaatacgtatcaacaatccgctcttgcctacaaatccggaattacggcgtttgactatttattttaatcataataatgatgatgatcagtcatatctaatagtagatatgtacaacacgggaagctatgagctagtgcctacaaatcagataaacacgcttgatggcagctttttaataggaacacccttcgtgcaagcgcgatttttgttggtagagatctgggtgcttatgcttattgcgcagcaaactaaaaaggacaccaaaaaaataatacaattttttataaatcaatatgaaatgcttatgaatagtccttggcccagtatggaggccctttttccctcaagcagtaaaagatatttaggcaactatgtagaccctaacgcgctcataaagtgggcacaactcaaattaaaaagaataccgcctttttatcctggaaagccggatgaagaatcatgttaagccgattaaaaaatcatgttaagctggttgaaaaatcatgttaagctggttgaaaaactcttggtgaaagcacggatgtaatattaacattggccgctcgcatttcgtgttgaaatacgatggaagagcgacggctatctaccatgccgatatcggcctggacatcacagttcatgcacttgtagatgggatgactcgcgttatagatggcaggctcgccacagtttctacagatgtaggagatgcagccatccgagtcgtcgtgcgatttttctatgatggtttgcatggcgccctgcgccgtaagcacccaatgctccatttctcccagacgaagacctccgtgcgatcgtttgccgtccaacggctggcctgtgagggcatccgtgggcccatagcttgcaacggcgtatcggtcatccagcacaaatttttgcaggcgctggtgataggtcggtcctatgaagatggccgcatcaaagtactcgccggtctggccgttgaacattttttggcatccattgaagcgtagaccttcttgcgccagtctttctgaaagaagctgcacattaataggcaggaatgcggtgccgtctgttaccaccccctgtagggcatttgctagaccaaccgtggtttctatcatttgaccgttggtcattcgggagggatgtgagtgggggtttacaatgaggtcgggctgcaatccgtcctctgtgaagggcatgtctgaagtgggcagggccagcgccgcaatgcccttgttcccgctgcgagaactcattttgtcgcctatattgagatttctttcatagcgcaggcgcatgaggccaaagatctcgtcattaggcccatggggacgcatcacagcatccacgacggccggctcatcgaagccgtacatgacagaccggtcgatgtatttgttgagttcgtctttttcgccccgtattttggccacttttcctataatgatgtcgccctttttgaccaccgttcctacgggcacgaatccatctacaagcttttcgtaattagcaccaggcttaagatttttggtgattaaagggtcgggcttcccaaacgactctatatcgctttctaattctactttttcttctcggtagaaggtgccggcaaagccgcccctgtcaataaaggactgcgacacgatcacagagtcctcctgattgtagccgccgtagatcatataagccacaatggtattaagcccgttgggtatgacatagttatgtgctatggtctttacaagcggcatttcattgtaaaactggaagaagcggttcatgtcgacacgatatggccagctaaagcaataccagccccccgtttgccggccttggtttgtttcataggtaacacgcgcaggttgggtacagtttgcgtagggggacactagggcggcaaggcccaaaatagcttggggcacgtccacgtgtgtgaaacgacgcgttacatcatgtttatgtttgcgtagctcgatgatggagaaggcaacaagacagttttccgcctcctcgggggtaatgaactcacagatgccctgtgctacgagatcttcaagtgtaagcgttccggctaaaatgtcttttgccatttgaggcgtaaatcgcgtattttgaatgaaagggattttatgtttttcccagtctttatcgcctttttttctggcctctgcggccttgtagcaggcttgattgtatttttcaatattattatctacaatgagtagggggcgggtcagcctaccgacgtccaaccaaaattctacttcgtctaccatgctatcccagtagatggtggtatggggatgcacaaccttgccctcacggcgaagcattctataccgctgagcaagctcaaaggcattggtgcagcagccgatccattctccgttgataaatacgcgcgctaggccctttcgtacaatgtccttgttggaaacatcggctaactgttgaatggccggatctgatagaaggcgttgttttaacgaaagtacttctccggcggtgcagacattggcagtgatggctaactgtttagacatgcctactttttcaccagtatcggctgactgggctacgcagatgtatccaggataggatgcgtgcacgcgacgcatcatgtcagccctttctgtttgtttggatgcgttggtggtgttatgagtatttaccgtacgcaatgctgaaatggtatttaataaattttttctttccaaactttgagtagatactctgtttacaatggggcgctgtcgcaccatgatggttttatttcctgaaatgatagactgttccatactgcgattaagatcggaggcggtattttttgataaagcggcagaaaatgcctcgataatgtttcgctgagtaagctcctcaaaggctgtttgtttaagaagttctttgaacccattgatgatgggtgctatcacggaagtattaaaaatagccttaaaggccttggcgagtgagacccctgagccgtgcacccgcttggtgcggtagctatcacggtccgtgggtggaaacacattcataatgacaagaagtattttatgaataagcaggcctaaaaagcgcagctttcgtacacgtgtatctgcggtttggcccatgtgtggcagcaatattttgtctaaaatagtaagttgtctttcatttaagtattgtaccgcattttcatcgcttttgtaagcagatgggtttgagacaaatttggaaaccttctcggataaaaactggataattttttctcggttcagctcgtgttggaccggttgaaatatggggtctaaaacatgaatggatttttccagaatttctatcatgaaggtattcacaagggagttggattctagatcaaataccacttgctcaatgatgctgtcatcgcctgtcattccaaacatgcgaaagatgagataccaaggtatgcgaagttttgagaacttggtgctattgatttcaatggtaatggcgccggtggtcatgtagcgtataataatttgagagctattttcgaaggcacctcccggttgggagataaactcgccgcgaatgatttcattattcccttgttgcatggtatggtaatggatgtgaagcgtgttaaagcggatgttttctaagaggtctacgacccattccccgcctcgggctataaagtagccgccgggttcattagggtcttctcctatttctttttttgcggtttttgataggtgatgagtgtggcagcggttgctgccccgcatgatgggaaatgtagatacctgaaaaggaggaatacttgctcgttttacctcctgccgaccattgctgtagtgcgccgttaaaataacctcggcggctagattaaccgggcccgaataggaaaggccacacaggcgtgccttattgggtagtaaatttatcttgtttccctgtgaatagtttcgatgttgcgggcgttcaatgttcacatctgtaaagttaaattggatctgaactgattcccgaagcttatctatttcagtatggtcgcgttggtctttataagtaatatccacgttaaacatttgttttacaatttgcggaattccattgtccataagatcgtcgaagcttttgatgttataccctatcaatcctgtagagtttactgcagcggagataaagctcagcatatcagcctctgtaagctcctcattatccacggtttcaatggggccgtaggttatttgcggccgcaagggttccatgattatgaagtactacattaatattcagttattctttaaaataaatctttatttataaatcttatttataatataagaatgccttatgcaagagacatcacaaagtttattacggcaacggaaccagaggtgggtcttcccctgttggcgctgcagcgctccaaatccatcataggggttattcttcttgtaataagtttgttatttattttcattggcattattatattatcagtgagtagtggtcataccacagcagcctctatatttatcgtattgagtcttatcctaggtggcggtggtttttttcttatttataaagataattcttaacccacataaaatttgaaaaaatatagagtaagaaaatgtccaattactattattactatggcggggggagatatgattggttaaaaacagtagaacccactaattttttaaaaatcgggttgccttaccaggcacacccattacatcttcaacatcaggcaactactcccccatctatcttagaaaaatttaaacgagcagacattcttcttaatgaggtgaaggccgaaatggacccactcatgttacaaccagaaaccgaaaaaaaactattccagatattgagtagtattgatatgttcaaaggtctgcgaaaaaaagtagaattcacgtacaatgctcaaattgttacgaatgcttggcttaaaatgtatgagctgctaaataccatgaattttaataatacatctcaggcattttgcaattgtgagcttccaggagggtttataagtgcaattaaccattttaattatacaatgatgcattaccctacttttaactgggtagcttcctccctttaccccagttcggaaacagatgccctggaagatcactatggtctttatcagtgcaatccggataactggttgatgcaatctcctttactgaaaaaaaatatagattataataacggggacgtaaccatcgctagcaatgtaaaaaacctagcgcttagagccacacaaaggctgacgcccatccatctatatacggctgatgggggtattaatgtaggacatgactacaataaacaggaagaattaaatcttaagcttcactttggtcaagcccttacgggtttgttgagtcttagcaaaggcggaaacatgatactcaaacactataccttaaatcatgcatttactctttctttaatatgtgtattttctcacttttttgaggaactatacattaccaaacctacctcctctcggcccacaaactctgaaacctatattgtgggtaaaaacagattacgcttatttacccccaaggaagaacaagtccttctaaaacggctagaattttttaatgatacgcccctcgtagacctaagtctttaccaaaatttacttgaaagcgtttactttgccgtagaaacaatacatctaaaacaacaaatagaatttctaaacttcggaatgaaatgttatcgacatttttataacaagattaaactacttaacgattatttagctccgaaaaaaaagatttttcaggataggtggcgtgtgcttaataagctttatgttcttgaaaaaaagcataaacttaagctttgtgcctcctagggatctgttgcttaatttaacagatgcaatcttaacagatgtaaactaaaaagtgtgttcatacaaggattgtatttatgaatatttattaacatataaggttgtgatgtaacactgtataacctatataactacactatgaagcacggcgtataataatttatattgaacacgatgttgactcatttatttgcaaacaaatatttgtttgcaagacgtttgcatgcatttactaatatgttgttgactagtttatttgcaaactagatgtttgattgcaaactagatgtttgcacgtatttatttgaactaatatacactccttgttttatttgttatatacacagcatacataagtgtatattgtttacacttatgtttataactcgacgtaataacattttacacgctttttttttgcaaatcttaataatattgtatgataaatcaaacaatgtcttatatatgtggtttattattttaggcgccgcaagatgtactccattctcattgcatgcttggtgttattactctgtctagttatatatgtcggtcatcgtgccgatcatgcacgaaaatatttagaaggaatgtggcatggagatccggtttttctaaaacagtcggggctacaatccttttatctctacatacaacctgaccatacatgtttttttagcattgtgaataaaaatggtgaaaagctgatggaaaccaaaataccttgtacgataacaaataaaatatatatgttttttaaacctatttttgaatttcatgttgtgatggaagacatacatagctacttccctaagcagtttaactttctgttagatagtacagaaggtaaacttattttagaaaacaatcacgttatttatgctgtattgtataaggataatttcgccaccgcactaggaaaaacggttgaaaaatatataacacaaaattaatcatgttttctaacaaaaagtacatcggtcttatcaataagaaggagggtttgaaaaaaaaaatagatgattatagtatattaataattggaatattaattggaactaacatcttaagccttattataaatataataggagagattaataaaccaatatgttaccaaaatgatgataagatattttattgccctaaagattgggttggatataataatgtttgttattattttggcaatgaagaaaaaaattataataatgcaagtaattattgtaagcaattaaatagtacgcttactaataataatactattttagtaaatcttactaaaacattaaatcttactaaaacatataatcacgaatctaattattgggttaattattctttaattaaaaatgagtcagtactattacgtgatagtggatattacaaaaaacaaaaacatgtaagtttattatatatttgtagtaaataatatttttaattacttaaaatttttatatataagtttttgatactatattataaaacatatgttcataaaatgataatacttatttttttaatattttctaacatagttttaagtattgattattgggttagttttaataaaacaataattttagatagtaatattactaatgataataatgatataaatggagtatcatggaatttttttaataattcttttaatacactagctacatgtggaaaagcaggtaacttttgtgaatgttctaattatagtacatcaatatataatataacaaataattgtagcttaactatttttcctcataatgatgtatttgatacaacatatcaagtagtatggaatcaaataattaattatacaataaaattattaacacctgctactcccccaaatatcacatataattgtactaattttttaataacatgtaaaaaaaataatggaacaaacactaatatatatttaaatataaatgatacttttgttaaatatactaatgaaagtatacttgaatataactggaataatagtaacattaacaattttacagctacatgtataattaataatacaattagtacatctaatgaaacaacacttataaattgtacttatttaacattgtcatctaactatttttatactttttttaaattatattatattccattaagcatcataattgggataacaataagtattcttcttatatccatcataacttttttatctttacgaaaaagaaaaaaacatgttgaagaaatagaaagtccaccacctgaatctaatgaagaagaacaatgtcagcatgatgacaccacttccatacatgaaccatctcccagagaaccattacttcctaagccttacagtcgttatcagtataatacacctatttactacatgcgtccctcaacacaaccactcaacccatttcccttacctaaaccgtgtcctccacccaaaccatgtccgccacccaaaccatgtcctccacctaaaccatgtccttcagctgaatcctattctccacccaaaccactacctagtatcccgctactacccaatatcccgccattatctacccaaaatatttcgcttattcacgtagatagaattatttaatatgtactatatattaattatttaacctttcaagctggtcttcatttaaatttaaaatccactaataaaatgtattttctagtagcagatcatcgagaacatcatgtgattccttttcttaaaaccgatttccatcacatgcatcaaaatcctatacaaaaaaatcaagctctcctagaaatcaaacagctttttactggagattatctcatctgcaaaagcccttctaccattctggcctgtattgaacgaaaaacctacaaagactttgcggcttctttgaaagatggacgttataaaaatcgccaaaaaatgctgtcgctgcgagaacaaaccaactgtcaactttatttttttgtagaaggcccggcatttcctaaccctcaaaaaaaaattaatcacgttgcctatgcaagcattattactgctatgacgcatcttatggttagagatcatatttttgtcattcaaacgaaaaatgaggcccacagttcccaaaagcttgtgcagcttttttatgccttttctaaggaaatggtgtgcgtcgttcccacctccctcacccccacggatgaagagctatgcatcaagctatggtcttctctttctggtatttcaggcgtgataggtaaaatcttggcaaacacttgttccgtagctcatttggttcatggaaagctttcatcgcagaatattgatcagttaaaaactccctccaaccgaccattccccaaaaaagtaaaacgtatgcttataagcattagcaaaggaaataaggagttagaaataaaattgctctcgggggttcccaatatcgggaaaaaattagctgccgaaattttaaaagatcatgcgcttcttttttttctaaatcagcccgtagaatgcttggcaaatatacaaatcgttcaaaaaacccgtacgattaagttgggaatgaagcgagccgaagcgattcattattttttaaactggtgtggctctgcccatgtaaccgatgatagccaaaatatcacagaggcgtcgcggtccacaatgcaggtcgcgacgcagtccgccgcaatacagcccgctgcaacgcagccattgcacgaagtatcagatgatgcatcatcagatgcttcatcacccgtagggtatcaaacattatctaaagaaatgttattgaacacagcctgatgttaataattcactacatctaaagaaatgttaacctcgatactaaaaagtcattgaacacaactactggggcgctaagttgtccaacacatctaaagaaatgtcaacatcctcgatgctaaaagggtcatcgagccggtcaataatgtcttccccaaaaagtccgggagaactgtaggccgagatgtcgtccatggagctatcttccccagagcacacaaagtcctctccaaaaatcataaagttaaatgcaccgggcttacttaacagcttttcgctttgaataatagtgttgagttctgtcagcgcaaactctctcacaatattcacaacccaggagggctctttaatttcatacagcgttaagaaacttatacataaaaattctatagagtaaagcaaggcgctggcaggatctgttacccgtaggtgtttaaatgtagtgtgatattcattcacaacgttaggcagcaccttttccaaatcctccttttcctcgtacgacaggtgctttacaagcctttcaacatgtataggaggcttgttaaatgtactaacgtgccgcaaacagttataattatataagaaaatacgtacggcagagtcgaccgccatgagccttggatcatccattgaggtaggtggtggcggggcaccctggccttccctgatgtctgcgtaggagcgcccctccatggcccctatggcctctatcacagcaggactgatatccaaaatcttggccgtcttgattatttttccgtaatcgaaagtccatggctcctgtggaggcttgggttgtgtttcggtggagggcgtggtcatatctttctttatttgaatagaacggatcgacatcttttccttatcgtactggtctttataattattataatagtcatgaactaattcgggttgagaaagatgatcgtatataatataggtaaaaagtccgcacttgacacattttttatcctggaagtcgtgtaatcctcccttggggcagcgtgactcgtagaaggcataaaaggtgttaaattctaagctcgcctttagggctgtttggaccttttttatgtttaattgccccacctcatgttgtagcacgtggcatacagaacagcgtagatcggcaagtgcataatggttgtcaattttttttatgacgtctttgcgtgttacttcaatctcggcgggtttctgcgaactgtctacggccttgtaaacgtaaatggtccacttatgaggaagccccctttcatcgtatagggttgaaatgggaagccttttatactcaaacagccgagtccgttggtcggctcttcctgtgttaggatcaaatatgttataaaatccttgctgagcaagcagggccttttgctcgccataagcattttcgtacgttttgaattctgcaagttcggagttaaaattaggtgcattttgtaaatacttaagaaataattcataggctctaaggtaaatgagagttgaggttttttcctcatcccgtcctccccaccacacccgcaggctttcttcttgaaaatagatgtcattcagacgcgtcaactgcgtaaaatcaggccgatatttagaggtataaattttatcataaaattctttttgcgataatagctcggccggggtacgtcctatcacggttttaaactcatattcagcctccttgggagtccgtggtttgtgcatagggatgctgccgtcaatacgggccactgtggcagcataatcatacatggggtccagcagaatctctgtcaaaagtaccttggtgtcgtcctgcacgctaagcccttgtagcccattttggtggataatttttttgaaagcctcccgaaaattattagcaatccactgatccgtaatctcagatagctgatttattataccgctatattgctgcatcattttctccaaaagaaaggtcacgtatgcattcaaagagctatccgccttcattccatgaatggtaatcgtaagaaattctttatttttttgcgagctataaatgagattcaaaatataggcatagatgtagatcacagcatacagctgcgttaaaggatcgtaatcctcttcctttttaatattttcgatgctatacacgagcggcaggcagacatttacggctatattggcaaactgtttcacgtctacaagctttccaaagtggataaacgtgcaggccttcatggtttcctgccaaataaaaacacggagcttactattaagatcgccgatgatgcccacatctgccgtacgatcctcttgaataaaatgggccagctcttcgccacaaattttgcaaaagtaggagtaaataagcccctggttgttttctttctccttgtttattcctgaaaatttcattagcttggttcgcatggtgtcgtaggacgcttctgccgcttgaagctgtataagcatgtccacatggggacaaagcagcttaaacccgcaggctttgcatagattccaattggtggtattgtttttttccttgtagagtacacgaatactttctaatacttttaataactccgcgtattgaagacccgaacgcaactgttttaccagcttgagatgagcacatgcatttttttcttggagttcccactgttttttaatgtttaggtattctgttgtaataagttctgcctcctgtttcccacaggctttaatgacttcttgaaggatgctgttagggtcatccactttaccctccattgtaagaatttcacgtatagcatccgactgcaccctacctattttttcttccataattttaaaatactgtctcgcctgggtaatgacctctgtgagcttcatgtccacctgctgcagaatcatttgctccttttcacgctgttcagcatgttgtaaaaacttttgttctacagggttccaaagcacctccaaatagcctgctctatataggtcataaagcaagggcatgtatcccgatgtaaaaaccggggacaccgagtacatcgtagacaactcttttaaaaaaaatatcacgcgcttaatgttctcctccggttcaatctcctcggtttcaacgatattagatatatgactgccctgatcctcacggtctagctttcggtgtaccatctcctctgctagccgattaatgagccagctatgcccgccgctccgcaaaaacttataaagttcgatatactggtgcgtaaactggatgatgttttccttggtggttacgacaaccccttctccgttttttttccaggtttcttgatccacgcatttcataaatactcgaataaaattggtcaaattggctcctgaggcgacgtagcccaaggtttcaggcgagaaggagcctatctcagccatacgcataaaacactgcggggaaaaagtttttagccgcaacttaagtccatagatttcaatgggggcttctgcgggaacggccaggtgcgtcccattaattaaaaaaatttctttgcgtgtgctagggcgaacacgtaattccttttttttttcactcacgatggggaccacatcggggtctaccagcagttgacgtatgtaggcctctatgggcatggatagatcgggcagctttgactgctcggcgcgaacatggttcacaaaatcttttagagtgaaaagaaagtctattaaacgtatgttttttatatcattagaccctttaagggtagagtagatttcatccactagtgcctcgatttcctcattattgagcgataagatatctgtgccacggtggactatttgcgcgatcgtaattacttcctccattagatagaaactgaatattatatttaaaataaatacaaaatgtcaaatgaaagttttcccgaaacgttggaaaacttactttcaatgttacagaccaaacagcaaaacgcaattcagtcagaggtgattgaatggctgcacagcttttgtgaaacctttcacttaaaaatacactgccataaacagtttattcctagcggggaaaaaaaacgagctaaaatacccgctcaagaaacacagggaaacacgcagccctcccaccatgtgtaccgggttgttctctccagagcacagccagtcaaagcacaggaatctctgctaacaaccatgtgcaacggactggtgctagatgcaaacacatggacatgcctagccattcctccgcctgcgccctttcaacaggcgacccgccaggtccaacacttttaccgtaacaatttctacgaagtggttcccatccaggatggcacccttctcacaatctaccactgggatgaccctgaatatggcccctcctggtgcctagcaagtacccacggatatgatgtgagtaactactgttggataggcgacaaaaccttcgccgagcttgtatacgaattgctgcagcagcactctacctgcgacgtcaccctggaaaaaaataaaacgcggggaacgcgtcttttctttgataacttaaatcccgattactgctatacgattggaatccggcaccataatttacagccgctcatctatgaccctcaaaatatttgggcgattcaatctacaaacctaaaaacgcttaaaacggtatatccagaatactacggctatataggcattccaggaattcagagtcaagttcctgagcttccccagtatgatttaccttatctaatacgatcttataaaactgctatgaatcaagccaaaaatgctataaaaaatggcaaaaaagacaagggatactttaattatggctatttactcatttcgcgagcgcctgccattactaaaagtacttctaatgttttgttaaaatcgcctctgctggtatttttacaaaaaagtgtgtaccagaaaaaacacaatatctctaacagccagcgactagaatttattatactgcaaaactacttgatgcagcattttcgagatcatttcattgctctatttccgcagtacatatcctattatacgaaataccaaaacatgttgaatatgattatccatagtattgcaactaaagataaagatcatccctttgcaggagccgtggtaaaaaaagtgttggaagatattgaaaacgccgaaaacattattgatcatacaaccattcaaaactatgcccatcaaagcaagtacgccatgctttacttgtcaattatttcccatttttaatctaatacggccaaagccgcgggttttttaataaactaacatttaaaaaaactgttttattaaaaattataatacttttattatatatggaacatccatctacaaactatactcccgaacagcaacacgaaaaattaaaacattatgttttaatccctaaacacctttggtcttatattaaatacggaacgcatgtccggtactacaccacacaaaatgttttccgagtcggtggctttgtgcttcaaaatccctacgaagccgttataaaaaatgaggtaaaaacagcaataagactgcaaaatagttttaacacaaaagcgaaagggcatgtaacgtgggccgtcccatatgataatattagcaagctatatgccaaaccagatgcaattatgcttaccatacaagaaaatgttgaaaaagctcttcatgctttaaaccaaaacgtactgacgctcgcatcaaaaatacgttaaatataatttttgtagaggataaaaagctattttagctaaaaaataattcatatacgtttatgcagaggaagaacggtggctttcaaattcagattgcatccacgtagaccgtagcgttttttttgcttctggtttatatcgtaaaccgtaataaacatcatcatttgtatccgttggatctttttcccactccggataaaaaatcggttttcttttttttggtcgttttttgcagtaagctgtaaattaagggaatatagcttatcgaaaagttgttcctgatccatataaatagcagcatatattaaaaaaaataaaaaaagacgcttcaacgagtcagtaccactgcttgccaacgatttacgttggttggtgcattatggtgatatagtaatgagtgcctgcacaagtgcttgcacaagtgcctgcacaagtgcttgcacaagtgcttgcacaagtgcttacacaagtgcttgcacaagtgcctgtacacattactgcatcgccaaagcacctgcaatgcctacttcctcaacagagtacgataactaaatgcttttaagcaccgcttgcgtcgatgtgtccttcggggcaatcgggttcaattggatccaatattattagtcataattacctaatacttattcaattttatcttttttaccttgtaagatttaaacagcgttttagcttgtttaaagcaacgtttaaaacaagctaaaatgctgtttaaaacaacgttttaaacaagttaaaacaaataagcttataaatataccatgacaaaattagcccaatggatgtttgagcagtatgtcaaagatttaaacctaaaaaatcgagggtccccctcgttccgcaaatggctcacattgcaaccctcactgctgcgctattcgggtgtgatgcgtgctaacgcctttgacatcctaaaatatggctatcctatgcagcagtcaggttatacggttgctacgcttgaaatccactttaaaaatattaggtcttcctttgccaacatttactggaaccgtgatagcgaggagcctgagtacgtctgctgttgtgccacctatcaatcgcacgatggcgaataccggtatcgatttgtttggtaccaacccttcatagaggcttataatgccatagaggcggccctggatcccctggaaaccattatcctgaacctcattgcggcacgagatctagacttcgttgttcacatatttccttataataagggccatgaagactatttggcctccacgcaacttattctcaaaatctttattgcgacgcttttaatggacattttaagaattaaagacaacacgttggacgttcacttaaattccgactatattattgtgatggagcggctttggcctcacataaaggatgccatagaacacttttttgaagcccataaggacttactagggtacttaattgcctttcgcaatggggggaactttgcaggaagtcttagaccctcctgtgggcaaaagattgttcccctaacgattcgagaggtcctacaaatgaatgatattaatttagccgtatggcgggaggtgtttattatgcaggaatgttccgacttagtcatcaatgggatagcgccctgtttccccatttttaacacgtggacgtatttgcaaggtattaaccagattttttttgaaaacacgtctttgcaggagaaatttaaaaaagattttattgcccgagagctttccaaagaaattatcaagggccaaaaaacgttgaatgacaaggagtttaaaaagttaagcctacatcaaatccagtacatggaatcctttctacttatgtcggatgttgccattatgattaccacagagtatgttggctatacccttcaatccctgccgggtattatttcgcgatccagctatttatcccccatcgtgaaaaacattttgatggacgaagactcttttatgtccctactatttgacctatgctatggcgcctacgtgttgcataaaaaagaaaatgtgattcacgcggatttgcacctgaataacatgacctactaccatttcaacccaaccagttttacagatcgcaacaaaccaggaaaatacaccttaaaggtcaagaatcctgtgattgcctttataaccgggcccaaagtcgaaaccgaaacgtacgtgttcaagcacatagatgggttcggctgcatcattgactttagcagagccattatggggccaaaccatgcaatcaagcttgagcggcagtacggcctcgcttttgtaaacaccttttaccgcaatcaaagtgagcatattttaaaggtattacggtactattttcctgaaatgctaaccaatcgcgaaaacgaaatacagggggtgattttatcaaactttaatttctttttcaatagcattactgccattgatttttacgccattgctagaaacctacgtagtatgctttctttggactatttacacacctctgaggtgaaacgaaacgtagaaatttcgcaaacatttttggatacatgtcaatttttggaggaaaaggccgtggaatttttgtttaaaaatcttcatactgtcttatctggcaagccggtcgaaaaaacggccggggatgtgcttttacccatcgtatttaaaaaatttttatacccaaatattcctaaaaatatattacggtcttttaccgtaatagatgtatacaattataataatataaagcgttattctgggaaagctatacaaacgtttccaccctgggctcaaaccaaagaaatcttgacgcacgccgagggtcgtacatttgaagatatttttcctagaggagaattagtttttaaaaaggcttacgcagaaaacaaccatttggacaaaattttacagcgtattcgtgagcagcttgctaatgaaaatttgtaaggcttgcagttcttgtatggtcagaacctatgtcgatggaaacattatttttcgctgcagctgcggcgaaagcgttcaaggggatagtcagaacttgctcgtctctagcaaggtgtaccacaccggggaaatggaagataagtacaagatttttattaaaaatgcaccctttgaccccacgaattgccaaataaaaaaggattgcccaaattgtcatttagactatttgacacaaatctgtattggaagccaaaaaatcattatattggtgtgccgctgtggctatatgagcaacagaggataaaccatatcatcccaccgaattatgacattcctttaaaaccgtccgcctaaatagttttcacacctttggtggcagactattttataaaaagtaatgttggttcatgaagataaagtgtgccaaagaaacttttataaacaaatgattaatgtaggtgctagtcgtgtgtacttaaacagggtattctatagccaagtattttctatagccaagtattttctatagccagtattagtcaagtatttagatgtcagggtatttttatagccagtatttttctatatgtacaaactattccagtaaacatatgtgtgttctttattgagcagcatcatggcattaacaagtttattaaactgctctaatgggcattaaatgacaactcggtgcttagcaaaagtgcctataccttttaacaattagggccgggaggcattcccagcttttttctataatcagccatacagtacccctgagcctcatacacgggaataaggtccttccattccttgttgggatcggcgggccagctctcaaatgaggtgtgaatgtaagggtcctgttctttttccttaatgaagcgtttaatctccatttgatgttgtttacttttttgtttgcggcggagcgtgttccgcaccaatacgtaaaaaataccaagaatcacacataaaagaattattaaaaaaaatatcatcatcgcggggtttaaaaaacgatcccatgcaacaggaatcgttcttaaaaccttgtctggcagggctgtaaacatgaagtctcctcctataatcggggtgggactgtagcctaacagttcaaggtcctgtcgttctagatacttattggcgaactgcccaccctttgcccccgtttttttattaatcaagcagcgctgcattttccaccattctaaatcttcaggagaaagctcaatgccatatatcaactttaacgttattgcatctttttcaatatccttatcaatttggctgagcttttgagctttaagcgggtctagtgtgtacttccatttaaacttagtgtcctgtagtttggctacatgaaatacggaacatttcggcggggcctttgtgacgcccttacactgcggaagtttatcattaggacaggcgcatagatgagactgcgccacagcatcgcgaactacatcgcagacggagtacattttcctcctatgttaaacaataaatttttttcatagctgaaatttgtgggcctatcttttcccttgcccggataataattataagggagtgttgaaacatctgggagagaattgcttaaaaaatgggtttttgggaggggtaactgcgactgttgtacgtcgttggccagggagattctatatgccgggctaaaggtgcaacgttcctgtgaacaacttagtacgcgcgttgttaatacaaatggactggtattagcaaacctcgtaaactcttccggacttgtttgtttttgtatgatgtttagcagggagtctgccttttcgagaatccaaagcgtcgcattgtagtaaaataaaaatagcgacttatcggcaggcgttgcaaaagcgccgtatagaaaataaagcagtaagtactggggagacaccacaataaggttatcttgaatgatagatatcgctagctctttaaacatagtgctaaaaaaatgtatgtcgttcgtcttgaatatagggggactatagtccatgtagggctcacatatctcagtcaggtgaaggcccatttcttttatgacttcttccgggttgtacgtcgctaacaccagcgcgggataggctttgggcatatccacggtaagtgttatgtttttatcattcttatggtaggagtaagatggttgtggaaattctgttttccactccgggactttgcaggtaattctcagctcatttagagtctggtacaggagggcgtatgccgcaaagccgtgtatggccacttgtttaaagggaattgaaaacgttttactttcgtatgtcgacttcacaggaacaacgggaatggggtaatatttttctatgaggttataccgctgcaaatcctttttaaacctgctaaaaacatcttcccttggtgggttatcaaaaggaaagcaaaatgctaggtgtagcccggcccgctggtaatcggggtgaatgattttaaggtttttatacgttaatgtgggtatggtgttaaagatattggggggcatatatgaaagatcagcaacccacacaaagtccgtgcgcacccgcatggtctgcacatggatggcgcgcaccgtgcccacctgcttgaagcccttttcatacaaaatgtcagcaagttcgtaggcgtcctcaacgtggttgggggaaaacatatcaaagtcgggtctttctccctcgggataaattgagctgcctttaagatgcagggcataatcaatggcaatccccccgtacaaaataagctttttctttatgataaattcgcggaccacctccaaagccgcctcaatctccacggcatttgcctcacgtttttgagcaatgagccggtacttagaaacattaaaatcagtctttagtaaagacgtcataaatagtgtttaatatatattaaaggtttgaataaaatactaaatagtaaaaatggatgccctattaaaggaaatagaaaagttatcgcagccatccttgcagaaagaaaacaatgatgtatgcgatctctgttttatgcaaatgaaaaaaatttctaactatcagcttttatgcgaagagtgcggtcagctgaaggactggtttgaacctgaatataatgaaaaattcacggtatattctcgtctaaagatcgtgggtgccaatagttcctatcaccagcgcgatttggacaaggccaactcaagtgactatagctccttgcaatttcatcacattttagaggagctcaaatccctaaatgttaagtatatggatgcggggcaaaagccctttcctattcaggtgttaaaagaaactgctcacagttataaccaagtacaacaacatcgggtcatacgcagcattacaaagcttcagatcttagccagtattctacgtagcatttgtttaaaattaaacattgcttgtacggtggcagacgccgcgaggtttactcaacttaataccaaagggatctcaaggggcatggatcttctgcgctccctatttgtagacaataaaattactttaaacgttgatttaaaccctatagacagctttattaatagtacctacagtgccttacaaattaaacaaatccaccaagaactgcaggaggaaaatgtttataatttaaaagaaattgttaagagctttatattatacgcggatgagaagaacatcggcgtcgatcttaacaggagaaccgttgtgattgctacgatgtataatgttttacgccgtgcctactaccccatagaaattgatacggtggtgtatcaatgtaaaatacgaaaaaatacaattacacgtgctcttaaaatgtatgaggattactactcccactttaagtctctttatgagcagtatcatttaaacgcggcaaaaaaattaatttaaactaaacgtttaaactaaatgtttaaactaaacgttaaaactaaacatttcgactaaagtttaaaacctagtctaacagcgggatgcccatttccctggggttccatatttcaacaattttttgaccttcgggtgttaccttgatgcagcgcatgacgagcagtggaattttcctattaaagagttcttgcttagctatatcaataggactgctatatttttttttaagcattgtagatccattaattgccaattgttgcgctctaacggcgaccaaccttgtggcctcaaaggtggttaaaacgttggaggtaatgcgctcgttatcgggtataatgaccaatgtttgcgacgaggcctgcacaaagccctcgcagatggacggagactccacgatctcgtccttgtcctcggactcctcctcactgtcgacgaggttctcctcttccgtttccacatattcctccacgaggtcatccatgataagatcctcgttgtcattatcagccatattacactgttatcaaatgtactgtttaatacgcaaatggatttactacgttttaattgtatgtcttcatgtgcaggctctagtggaaagtaattttctcacaatttttggcaccgttacacttgtgcccacaaaaacccgcgatttttttattttatattacttttggaagtacgagtttaaccagtcgctttcaaaccttatgcgtctatctcgccaaaaaacgctcacagcggtgttggatattacctttaaaaaaataacattaatttttaccacagagggcgtattgcgtatggattctacgaataagccaggcgtgccactcgatatagacccccagttcattgaccttgatagtattttaatggaactggatcattaggacctctcccgcccatttaaatttttagtttctacaataataaaatgcgcgaggaatcatgggaagaccacgataccattcagctcaccgctcagcgcaaatacctcgccgaggtgcaagctctagagacccttttgactcgagagctttcagtctttctcacagagccaggcagcaaaaaaacaaatattattaatagaatcacaggaaaaacctacgcacttcccagcacagagctactaagactctacgagcatctcgagcaatgtcgcaagcaaggcgccctcatgtattttttggaaagacaggggacctactcgggtctcatgttggactatgaccttaaactcaatacaaatgctgttcccccgctggaaccccccgcgctatcacggctttgccatcgaatatttgtgcatataaaaaacagcagtgtgctgcctgagggcagccataaaatccacttcttttttacattaaaacctgaagtggttcagggcaaatatgggttccatgtgctcattcctggtctcaagctggcggcttctaccaaaaaaagcattataggatccctacagcacgatgccaccgtacaaaaaattctacacgagcagggcgttacaaatcctgagtcctgtctggacccccactccgcctccgttccctcgctcctctacggctcctccaaactaaaccacaagccctaccaactgaaaaccggctttgagttagtctttgatagctctgatcccgactacattcccattcatcaaataaaaaatttagaatcttataatttagtttctgagttgagccttacgaatgaacagggaagccttgtaagacctgtctattgcgcggcagacattgccgctgagaaggaggaagagatcccgaccgaggatcactcgctctccatattaatgctacatgatcccgaagcccggtatttacataaaattttaaatctgcttcctccggagtattatgtagagtaccccctatggagcaacgtcgtattcgctttggccaatacatccgctaactatcggcccctcgccgaatggttttcgcaaaaatgccctgaaaaatggaatacgggaggaaaagagaaactagaaaaactttggaatgatgcctcgcaccacactgaaaagaaaatcaccaagcggtccattatgtactgggcccacaaacatgccccccagcaatacaaagaaattgtagaacaaggctacttttccattctcgctgaatatgtgtatagctataacggcatgcttgagcactacatgatcgccaaagtcatctatgctatgatgggcaacaagtttgtagtggacgtggattcaaacgggaagtacgtttggttcgaatttgtgctaccgggccagccaatgaatcagggagaaatatggaagtggcgcaaggaggtaaacccggatgagctgcacatctatatttccgaaaacttttcaagggtgatggaccgaatcacggagcacatcaaataccacctcagtcaaccccatgaaagcaatattttaaattattataaaaaactattaaaagcctttgaacgctctaaaagtaaaatctttaatgacagctttaaaaagggagttatcaggcaagctgagtttttatttcgccaaagaagctttattcaaactctggataccaatccccacctactgggggttggcaacggggttctctccattgagaccatcccggctaagctcattaatcattttcacgagcatcccattcatcagtacacacacatatgttatgtgccctttaatcccgaaaacccctggacaaaactattattgaatgcactccaagacatcatcccagaacttgatgctaggctgtggatcatgttctacctaagcacggccatatttcgcggcctgaaggaggctctgatgcttttgtggcttggaggcggctgcaatggaaaaacttttctaatgcgacttgtggccatggtattgggcgatcactatgcctccaagctcaacatcagccttcttacaagctgcagagaaaccgcggaaaaacccaacagtgcctttatgcggcttaaggggcggggatatgggtactttgaggaaaccaacaaaagcgaggttctaaatacgtcgcggctgaaggaaatggtaaatccgggcgatgtcaccgctcgagagcttaatcaaaaacaggaaagctttcagatgacggccaccatggtcgccgcgtccaactataacttcatcattgacacgacggaccacggcacatggagaagactgcggcattatcggtcaaaggtgaaattctgccataaccccgaccccagtaacccctacgagaaaaaggaagatcctcgctttattcacgagtacatcatggatccagactgccaaaacgcattcttcagcatactcgtctatttttgggagaagctacagaaggaatacaacgggcagattaaaaaagtgttttgtcccaccattgagagcgaaacggaggcgtacagaaagtcacaagatacgctacataggtttatcacagaaagagtcgtggagtcgccctccgcagaaactgtgtacaacctatccgaggtcgtgacggcctacgcggaatggtacaacaccaacattaacgtaaagcgccatattgccctcgagctatcccaggagttagaaaactctgtgctagaaaaataccttcagtggtctcccaacaaaacgcgaattctaaagggttgccgtattttgcataaatttgaaacgctgcagcccggcgaatcctacattggggtgtccacggccggcacactcctaaacacacccatatgcgagccaaaaaataaatggtgggaatggtcccctaatccctctgcccctcctgagaaagaagcgtctgcaccaactccttagggaatatccttagaagcatgtctttcggcagagccattaccggtagcaaaaaagcaacattgagtatattatatgccttagcctgctcataagcgtccttttttttcatggtattttatgtttttaaatatttttaattattttttaaatacgatgaacagttcgtgctccgaaggctgtttactaaaaatcggtgtgaatccgcattctttaaatatggtttcccattcggggatggtatggaaatccatgtctctacgaatagtatggtgcccaagtgcgtcctgcaggctgtgaagccagaaggcctcctgaccttgatgaaggtcgtacatgataagaaaaccatcaggtttcaacagatggtaaagcttgttaaaatcgtttatcgtaagatgatgcgccgccataggtaaccctatgagctccacagagttttcatgctggacatcgtccatatcggtataaaacgtttcacagtaaatgagacgcttaaacgagtatcgatgacaaacatttatttccaagtaggtttgcactacgtttttaggtatatcgggaatcatgttgattaaggttgtttcgggaaacttaatcatctgactaggcttcattttcaactctttaaaggatttcccggagaagtgaaaatgggtctttacgtatttatgtaaaaatacctgaatgggcagagggggctcctcctcttcgttctcgacgcctcccaaaatatttggaatttcctgacgtggcaaaagaaagtttatgtccacgtttacgaatccatcgaggacggacacaaagcttggctctaatctccattccatatactgtttagaaacgggagatagcataatcctaggcgtcacaatgcacgaagggtttttaatcaccgcatcgtggtaagaaaagtgtattccatttcttccagtataaagaagcctatgttcgtcgtagcagaaacaattaaggcggtatgcctcatacatacactgtttcaaagtacaaacacgttttaaaaaggtttctgcattggcggaggccaagcggttttgccattggtggaaggggttcaatcctacaatggccagctcgtttaaaatatcttcgcggcgcgctaaaatctgcaccatagaagaatactttagcatttttttttcgcaccattcgcgaagatgtttagctacattattaaccttattattgataaagtatacgatggcatgttggaagccttcaaaaataaagagcccctccaaaagatcatctgccaatagaagatggatgttggtgtaagcattgtcaatattttgtagaaacggcggaatgcctgccaaaaccgcttcagcaagcatagctccgttccgttgtttactgtccaatagattcgtaagttttttgtccgcaacagacacgacggctaggatggttgcaatgtcagaaatggcggcttgccagaaataacccgaaaagcacatgcgcgcttcttctatagataaaaacgaaaagcgagaggcaatgtctccgagctgcgtgagttgaagacctttttctcctctggttaaaaggcctgccacaatggcccgctcaatggctgatgccagcgcatccgtggggggaggatccagcatatcaatctcctctgccttaaacacgccttccttattttttttaatcgtttctacgacaatgctaagaaaaatggccccagggccttccgtaatgatttcaggatactgctgcactggtatttgctcaaagacgtgttttgtgtaaagcgggtaaaagtgcccaggaaatactctccctacacgcccctttctttgctcgatacggctttgagccgcggggcgcgtaataagccctcccgcccattcgggatagtaggtttcaatgcttctgttccacccgggatctatgacgtacttcagcgtttcaatggtaaggcccgtttccgcaacaaccgtggaaacaatgacccttcttaaaggtttttccactttagcggttaagggatttttcacccacagattcttaatttccgctttcaggccaaggtaggcctcattttcctgcgcaatcgcctcactatcgatcggcaaaatcaacattaacggcagcttttctttggcaaggtccatatttgcattattcagcaacatcgaaaggaagcgtatttcagccataccgggcatgaaaattaaaatatctgcttccgtgggacgatcatgaatgttttctttatgaatagtgagagccgtttcgcaggcggtcttaatgtagttgttggtgttatacagcggccagtgggtttccacaccgtactgtcgtccttccaccaaaataatgttttcttttccgataccaaaataggttgagtatttatgggtatcaatggtggcggaggttaaaattacaaagggaatacgcagcgcccctatgcttcctctttgcaacatgcgctgaagcatacttttaatatacatgagcataaggtcgatgcctagggctcgctcatgggcctcatctataatcataaaggcatagcgggaagctatctcatcatccgtcattgtatgtagctgcgccaacagaacccccgcggttgcataaataaggccccgattgggtttttccgtcagaggcttcgtttggtagcccactgtttggcctaatatcatgtcggggtagtgggttgaggcgccgatgtctttggcgagggtcaccgcggttaggactcttggctgggtacaaataaccgagcgtcccaagtatttttggaaagaatgcgtgttttcatttctcagaattctgaacacgtgtacgggtaaggccgtggattttccggaaccagtgcgtgactttataatgagcacccggtctgcgagggaggttggaatggcccctccaaactccgggagacgttgttttatccaagtgatgatgtaatgaataggaacatcattcttgtgctcagcgggcacgttatagagatgaccaggctccaataaagtcggttttcccatattctattgttttaaggattgattgttcataaatatttttatactctgaccaagaaattatttttttattaagccggttatttacgttgttatggaacgcgaaggtccagtactgaaagtcctccgagttgtttaatgtcaagggattttttgtaagatacgaaaaggcgtggtgctggcacctggtgcatggcagagactcgataaagttcagtatccattggatggcttcatatttttctttccagctaggagcgtctgaaaaaaagatagcatatagatgcaaggatcgccagtatttaggtccccaatgcaacatttataaccttttgaaaaatctcattccatatagaggtaaatattttttttccatggagaatttttttgcactcttgaagggattgcgccacatcgtcaaatgttttttgttttccatgtattttggcgtaattccagccagtatctgtgtcatggtccttaatgtcatccgctaactgaaaggcatgtccaaaacaatgggcagccctttcaatcatcccaatgtcttcaacggatccagttcctaaaacccagcccataataaacgcgatcttaaaaaagggaatggttttttctggagtgtctactaactgaccggaacccgcgctgtttagagagtggcttacaaaggtacacagcagcgctcccagttggttgggatccggaaaccttggacagtgttccttaatccagtcgatttgccggcaaatattttgaaatccttgcatggttagcgccagagcgctcatctgcgccttggctacgccaaagcgggcccacactgtatctttatttcgccgcttcacatcgttgtcaaaggagggcatatcatcgataatcaaagaagctacgtgaaagtactccgctgctagggcggcctctgccggataaataggcgccccaaaggaatgttgcaactgacaggcccgaacaatttccatcaggataatgggacggatatacttcccacctcttagagcgtaagagcaaggctctgttagttgtcccttaaagtccccatcttcaatagcattatttaagatggtctcaaactcttcactaaaggttttataatttttaggattcagtggatgtattccatgaaaaagcgcgacactacgcggtgctgtgattctaaaatacttaggtttgcgcgtataggatattaaaataataataagaactacaatgatggagatatagatgagatgcaacatgctgagttgtctccccgcagggaatggtccttttccgcgcttgttaacggtaccgaggaggcgttgaaatctttaggaaaggtgctgtctagtttggaatctccaattcctcccgtatatttaggtatataattattgtgtctagaaattgtttgctttgaggtatcaaaatattcagcctgaccgctatttcttttagaataattcggtatagggcttgagtagttggcaatactcttaaaccggggcaccaaggtaacaatattttccatataatgggtttgatacgctttgtttaaaaatgggcttaccggctttatgcttgttagttgtgcattgagtaccggtatgtcttctaggatttgtggctttatagaatgattagcaaacacagaatgtagtatattagatacttgtagcatatgtctatttgcggaaaattcctggtattctctgccgtgttgcgaatctttgggcggaaggggaccaagcatcggcacgtccgtgtaggtactggtggattttatgagttcctgctctatgttcggtttgacatgtggatttcctaaaggaatacctctacctgcaatccctttttctaccgacgcaggtagattgtgcgctaaacacaaaatattgtacacgtctttgtgcggaatatatccgttatagtgctggcccggcatctgatcgccaaggtgctgctcatgcttaatggtaccctttgttctgagtttaggaagatcctcgtacgaaaaaaattttgtgtgctcgctgaacctcgtagaaggaaccgaactattttttgggttttttaaggaaggcaatgaggaaggctgggtcagacaatttttctgtgtgccctttaagctagccacctgcggaaatgtttttttttccgtacgaacaacattgcgcctaattaggttttccgtatgggttgaaaaagcaggacgatgatttttaaaatgattaaaaagtttattttttggaatggagctgtacggctccagatcttgcgcatcgccgtaaccaatgtttttgtgctgagggttcagcataaaagaaaagttacgtagatcactgagttgcaatcccttttcagccttttcaggactattagtgtattcattgtatacaggcgcggctccatttttgttgccgcagtaccgggaatttagtatattatcagaataccggttatgacgcggcaaatcgctttcccaaagaggtggatctgacctataatcggctaacagctttgaagcataatcatgatacattgtatataaaagttaattattatattgagaaggcataattacttcttgtaggggtacaagaggctttgaatcaggcaaactgacgggttttgaatcggccggctttggaccggcaggtatctttttaggttgatcttcttctagctcattagacacggatgggggagaaataggaggaataatttcatctccgcccttatatttgtcatggatagaagaaacaattacatccatgtttgatttattataaatgtcgtttaactggtgatttaaaacataataatgcaaaaataatagggctacaatgcatatatatacgtaaatagccgtcttcgtttttcgttttttatccaccggcggattacaaattgcaaaaaatacaactaataccaccgctgtaatgattaaggccacaatgaaaggattttgaaaggatgttttgaacggttcgcacgtataaattttttctcctaaattattgatacccgcaataaaatctacattcattttatatatttataaattatgaaaaatttagagttacatctccgccggaccaatcattgctaaaatttgaagattcttcaaaaaggcccgactggttgaatgtcttctgctcaggtttccaaaaattttccaagaatggattttgaacaataggctcatcttgattttcttcttcaaggatattttctttgatatcaagaacagcttctttaaactcaggtgtatcttgattaaactcaggtttatcctgatcaatcgcaaaaatattatcttcttcagatatatcctgtttaatcgcaagaatagtttcttcctcaggtttatcctgatcaatcgcaagaatattttcttcttcaggtttatcctgaccaaactcaacaatatctttctcgctaaatccgtttttagtgtgaagctcttggttttgaagagaattatcaaaatctattttagttgttgtcctagaccgtggcacgggatagttatctaatggtttacttactatagtcctcgaatgtggcacgggataattgtttggtgacttgctggttagctcttggcttgttaatagttcttgttttctcaataattccatctctactacttctttttgatccgctggtgtctctttttggtattcttcattagaaaaatgttcagagggtaatgtttcaataaactttgtgagtggatagctgctctttgatgtagaagagcgttgaatttgctgataaaggagttgaacaagtcgccggtattcactctgtcttttttcatattttttacgtagcgtggagagatctgctaagagcgacttgttttcagatgttaattcttcaatttgatgaagaaggctgcgattgtatgaactaagtcttgcatacgtttcttctaattctgtctccggctccacataggcctgttttcgcagaaatttattgtatagttccattctttttttgagcagaaaggtaagactataatcttgcatttctttcgtaactttatggtagttttctttccggtttttgataataaagggcagcattttttctgttgtgataaaggtgcccagattgctaatgtagtcgcacagtagcaattccaagatagattctttcttttcaaggcttatagattggctgtattctttaggtatgaaagaatcaacaatcgttgttacgaagtttgaaaagtttaatgttttgctgttaatttgggtaatgttacaaaaatatttgtaaaaactatctagcattttttcataaagttttttattttgtttaacccctaaaatatagccctttacttgatactgatattccgtaacaatggaatgttttttgtatagtgcatttttgtataaaaagttataaaaaatgttgataaaatacgcaccaagggtttcaaaaatacttataacgtgggattcttcctgatccattatatcatatgtaatattattttaataaaaaattactgacgaataacatgcaaaaaaaatatgtttaaacttattttaagctagcacttatttaaaagtgttttaaacacgttttaaattgtatgttaatacacttaaaaattaagccgaaatttgctccaataaggattacttttatcaatgaccacctctttactataaacggctttacataattttaataatgctttagagccaaagctgaaggcagtgggaagcggcactgtactatggtaaaaatgttgccgatgttcatcctcgcggatgtacacaagtttcctatatcctttaaacacaatatggctaatttcttccacatactccttatcctgtttggaatagcggttgctttgacgggaaaaattcgacatacaaatagaggcatttgtaaaaatggaaacaaatgcgtttttacgaagattggcgggtaaatcggtatcatcttggcagcaaataatcatcgaaataaaacagtgacgattttggtaaaaaaactttttaaaaatttcttttgtaaataatgggtgcagttcggccgcgcagtcgtctaatattaaaagtaaacgaggattaagattgatatagtttaacgtaaacttttcatcctctgtaaggcataagtttttatacatatgaatgttctgtataataattttttttaaaagttgctgataaagcgatgtaatcttttcttcttttttttggtccgtttgttcagcctttaagcactccacttttgcaatatttttgttttccttttgctgtatatcgatcggaagtttatgatacaatgtttttagcatatcgatgttgtttactcgactgtagatggaggacatcatagtttgccgctgccagatggcctccaaaaagcgttcagcgcccttgttgtcattttttttttgcttatcggcgagccacaagcggtagtgtattagagttggatgtacaaaaccctcatatgaacgatttgagggttccgagggggcaaccactaaaatttgttcaatatggggttgcaggattttcataatatgtttaacgtacacggttttgcctgtttttgaggggccatatagcacagttgttttatctataaaatgatgtgctttgaactgtagttcaggaattagcttccctgaatgggtcgttagggccatctctatattattacaattctgcttttgtatataaaatttctttttcgagtttattattattgttgacccacatatctacccgtatcgtatcatcaggcacattgagcatttcaagcgcattatctaactgtttttttgtttttatcagctcgctttcttcatcgggggttaaattttctttactaagcagttgcttaattttttcttcgcagtcgtctataaaatcatactctcgagcttttttgatatttccagatgctttttctaggttttttagctccttaaaggaaagcagtcccttaatcccgctatccgtgtgaaaggttgaattatagatggagagccccggagcatccgggccagtttcttgtatattttttgcttttttgtggtaaatagtatttcgtaaaatctcttttcctatctttaggtcttcctcatgacggtccaaaatccgttttattatttcattattttgattaaaataattgtagcgctctctgttggccttaaagcttcccaggagtgtccagttgcctaattgaatggatgaaacctctgagaaaatctggtctttatatttataataaaattcatcaaccttttgttggttgctgctatccaccacatcataaataatgaaggcaaactctaggtcgggtttttctgggtagatgctttccgtagcggcccgcaactcttcgtaattatcctcaatgtaataattccacttataaaaagtatcctgaggtggaatatgctgcgaaagatatctagtaatttttgtgttaaagagaatgggtttaaacgccctcggattttcaagcatatgtttaatgctttggtgaagttctatattttgtaatatgtgggctgctgccctatagccctgtggggtttgggtgattgcatcaatatcggcctgaagctcattaggcacatttaatgttttttgcatgatgtgtaaagggatgcgctcaggatctgctaaatcggtgtattctgtgcttgtacaagtgcttgcacaggtatctacattggtatctgcacacatgcttgcacaggtgtctacattggtatctgcacacatgcttgcacaagtgtctacattggtatctgcacaagtatacgcactttgagcatgaagattaggatcaaacacaaaatgttctcgtaaaaagctatcgatcgttgttttagcttccttgcttttctgcgtctgggttttgcagctatctgctatagataaaattgtatttactaccgattcagagggaacatcattagtttcctgtttcaaagtatcaactaacgttattagctcactgagaagagttttggtcgtgtgggtaggttttgaataggaaggcatccattcctgcagagctttgaagacatatccaataaagctagtcattataagacgtcgaatatactgctcccgcaaatttgtaaaagagcaaaaggccaccctgctatcatttttgaactgtttgtaagggttcgtcctttggtaaagctgtttaagcgtttcttcggatatttcagtagagggatcctccaatacgtttttgagaagctcatcaatattaaattctgccatatcttagagtttattatatacatattaaagctttaatataaggggggtataacaatggacgaaatcatcaataaataccaagctgttgaaaaactttttaaggaaattcagcaaggattggccgcgtatgatcaatacaagaccttaattagtgaaatgatgcactataataatcatatcaagcaggagtattttaactttttaatgattatttcaccttatcttattagggcgcatagcggagaaacgctgcgaaacaaagtaaataatgaaattaaacgtcttattttggttgaaaatatcaataccaaaatatctaaaacgctggtaagtgttaattttttactacagaaaaaactttcaacggacggggtgaaaacgaaaaacatgtggtgcaccaataatcccatgctgcaggtaaaaacagcccacaacctttttaagcaactatgcgacacacagtccaaaactcaatgggtacaaactttaaaatataaggaatgcaagtattgtcataccgacatggtgtttaacaccacgcagtttgggctgcaatgtcctaactgcggttgtattcaagaattgatgggaaccatttttgatgaaacacatttttacaaccatgatgggcagaaagcaaagtcaggtatctttaaccctaaccgtcactatcggttttggatagaacatattcttggtagaaatccagaacaagagttggggaccaaacaagatccctgcggaaccaaggtgttgcaacaactaaaaaaaattattaagcgcgataataaatgcatcgcgcttttgacggtcgaaaatattcgaaaaatgttaaaagagataaaccgcacagacttaaataattgtgtttctcttatattgcgtaaacttaccggagtagggccgcctcaaatatcagagtcgattttactacgaggcgaatacatatttacagaggcaattaagatacgggaaaaagtgtgtaaaaaagggcgtattaataggaattattatccgtattatatatataaaatttttgacgccattttgcctccaaatgataccacgaatcgacgcattttacaatatattcatttgcaaggaaatgatacgctagctaataatgatagtgagtgggaatctatctgtatggagctccctgaaataaaatggaagcccacagatcgaacccattgtgttcattttttttaaagatgaagattttttagatgattttttttagttttttaaaagacgaaaaaattttttaaaagatgaatattcttaaaccccgcaaattacttttttttaggtactgtaacgcagcacagctgaaccgttctgaagaagaagaaagttaatagcagatgccgataccacaagatcagccgtagtgatagaccccacgtaatccgtgtcccaactaatataaaattctcttgctctggatacgttaatatgaccactgggttggtattcctcccgtggcttcaaagcaaaggtaatcatcatcgcacccggatcatcgggggttttaatcgcattgcctccgtagtggaagggtatgtaagagctgcagaactttgatggaaatttatcgataagattgataccatgagcagttacggaaatgtttttaataataggtaatgtgatcggatacgtaacggggctaatatcagatatagatgaacatgcgtctggaagagctgtatctctatcctgaaagcttatctctgcgtggtgagtgggctgcataatggcgttaacaacatgtccgaacttgtgccaatctcggtgttgatgaggattttgatcggagatgttccaggtaggttttaatcctataaacatatattcaatgggccatttaagagcagacattagtttttcatcgtggtggttattgttggtgtgggtcacctgcgttttatggacacgtatcagcgaaaagcgaacgcgttttacaaaaaggttgtgtatttcaggggttacaaacaggttattgatgtaaagttcattattcgtgagcgagatttcattaatgactcctgggataaaccatggtttaaagcgtatattgcgtctactggggcgtccagctataaaacgtgactggcgtacaaaaagtccaggaaattcattcaccaaatccttttgcgatgcaagctttatggtgataaagcgctcgccgaagggaatggatactgagggaatagcaaggttcacgttctcattaaaccaaaagcgcaacttaatccagagcgcaagagggggctgatagtatttaggggtttgaggtccattacagctgtaatgaacattacgtcttatgtccagatacgttgcgtccgtgataggagtaatatcttgtttacctgctgtttggatattgtgagagttctcgggaaaatgctgtgaaagaaatttcgggttggtatggctacacgttcgctgcgtatcattttcatcggtaagaataggtttgctttggtgcggcttgtgcaaatcatgaatgttgcataggagagggccactggttccctccaccgatacctcctggccaaccaagtgcttatatccagtcattttatcccctgggatgcaaaatttgcgcacaagcgttgtgacatccgaactatattcgtctagggaatttccatttacatcgaatcttacgttttcataaagtcgttctccggggtattcgcagtagtaaaccaagtttcggtacgcattctttgtgccgggtacaatgggtcttccaaaaggatctacaagcgtgtaaacggcgccctctaagggtgtttggttgtcccagtcatatccgttgcgaggaaacgtttgaagctgcccatgggcccccatctgggacgtgccctgaatcggagcatcctgccaggatgaatgacatgcacccaatatatgatggcccaccatatcatggaaaaagtctccgtactggggaataccaaaggtaagcttgtttcccaaggtgggggtacccgtatgcgggcgtactttattgtattcaaaccctactggaacataaggcttaaaatgcgcattaaaatgcaccaaatgtgtttcttcgatttgactcaaagtgggttcgggatcgggtttcccataacttttgttcacatttttaatgttagagatcctgctattcagcaagtcttgggccaatataatcttgtcggccttcccatcgttagcaataagacaaaaagctcctcctgatgccatatataatgttataaaaataatttattgtttttattaaatatggcggtttatgcgaaggatcttgataataacaaagagttaaaccaaaaattaattaacgatcagcttaaaattattgacacgctcttgctggcagaaaaaaaaaactttttggtgtatgaactacctgccccttttgacttttcctccggcgaccctttggccagtcagcgcgacatatactatgccatcataaaaagcctcgaggagcgcgggtttactgtcaaaatatgtatgaaaggggatcgtgccctccttttcatcacctggaaaaaaatacaatccattgagataaacaaaaaagaagaatatctgcgcatgcacttcatacaagacgaagagaaagcattttattgtaaatttttagagtctagatgagcttttacgcaatgttgtacagtgttgtatatatgtcttgtaagcatttgttgtagagtaataagtaaaagataaataaaaatgactattaaaataaagcccaaaccattaaaaatatttttatctgttagatttaatttaataaatggctcatggaatgtgtggtgcgccgctgcatgaggtgtggccgcatgggatgtggtcgcataagatgtagctacatgggatgtggcatttgcttgcatgtaaggatcatgatgtgttgggtcttcatcccagcaataatcgccatctttatctagctgaattgtataccccattatatatcacttattatttttttttaatgtttcatgaatttcattataggcggtgaaagggtcctcaggccccttctgtaaaagattatagagatcttcggacgctttatgtttcgtgcgaattaaggcgggatataacaaaagagagggccccagttccaaacaaattttacttagcgggctcatattttgcaccaagtttcccactacttgcgatgtttcataacgcattttaaagagctttatcataaaagtgttatgcaggccggtgtagtctggcctatagttaaggaaggggatttctctggtaccgtcaaacacgatctcaagtcctctagcaagcccgatcaaaatttcttcagcaatggatgagtatctaattcctacattacgaagcgtaagcatttctataacatcatctatttcctgcatagaggaatctattgtaggaattttaatatcatctgtgctgatttgttcattcccaagataggtaagcagcatattaattttttctagctttactagcttagtcttacgctcataatcatgatcttttttataaaaagagttgggatcaccgttggaccgtagatgattaataaggcggtctacttgctttgtactaggtttaatacttttttcactatactcgctttcagcatagtggtttttacgatctcttttagaaatagctgttttttgagatgcctcagactctgcatatttttttctatgcgtagaaagagaataaccgcggtcattacgtgaactactgttgcatgcaaggcctcggcgcgtcttaccgctgcgcacactgccattgcgtatactgccatcgcgcacactgccgctgcgtatactgccattgcgtatactgccgctgcgtatgctgccgctgcgtatgctgccgctacatacactatcactacatatgctgtcagtacatacgctatcgcggcgtatgccgccgtgtaccttatcgccgcccctacccgagggttttttagatataatactgtgtggggagtcaagcgaaaattcagggtcattaaagttaatgcccaatgactttgccaatccattaagctcttcatcaaaatgatcggtaggaaaactttgttgcttgcccatgacctgtttttcaagttcctccaaattggcttgctcatttatatggagattattcataagcgtcgtaattccagcaagatttgctccttctaaaaatgtggtgtcctccatcggatatactatactatttaaaagcttttaaataaaaatgtgtttggaagaaatgctctcttcaagcgtgtgtagctcagatataaatgcctcctcagaaagctttccaccatactcctttctcatcgtataggagggcgccggtttaatgtaggaaatccactgggaggtaaaaaaccggtacaacatatttagcagctcgcgggcctcccaccttttgggctccgtatagtgcacatcaacataagaggcggcgcatgaaaagctgcaaaagttgccgagaacgcccatctcaatctctcctcgctcattttcacgcatataggtgggcacgaattttgggacagtcttgaaatagagatgacatgtccagcatttaaagctagaatgggtaacccatttggaaacagtggtgaatacggagggtagctttttttcgacctcggcttcatcgtcattcgtatttaacgtatcggtggcagtttttttggattgcaagcattcttcaatggtaatcccggataagtataaaatattaggacaattagtttccataattttgatagttatttttatacaacatggatttaattaaagataaatggaggacgaaacggaactgtgttttcggtcaaacaaggtgacgaggcttgaaatgtttgtctgcacatacgggggaaaaattaccagccttgcatgttcgcatatggagttaattaaaatgttgcaaattgctgagccggtgaaggcattgaactgcaactttggccaccagtgcctaccgggctacgaatctttaataaagactccgaaaaaaactaaaaacatgttgcgccgtccgcgcaaaacagaaggcgatgggacttgcttcaatagtgccattgaagcctccattttgtttaaggacaagatgtataaattaaaatgttttcctagtaccggggaaattcaggtcccgggcgtcatttttccggattttgaagacggaaaaaacattatacagcagtgggtagacttcttgcaacatcaacccattgaaaaaaaaatccagattattgaatttaaaacgattatgattaattttaagtttcaaataaacccagtgtctccccgcgtcatcattcatttaaaaaaatttgcagctttgttggaacacatccctactccatatcccatacgtgaaataaagcctccattagaagactcaaaagtatccgcaaaatttatggtcagtccgggaaaaaaagtacgcattaatgtttttcttaaaggtaagataaatattttaggctgcaacacaaaggaatccgcggagaccatttatacgtttttgaaagatcttatcagcgtacattggcaagaaattttgtgcgtgttaccggtacccgattaaagaatgttttcattaataaggtaatcgactatgctaaaaagaataacaagaaaaataccttgaagaactataccaaagtaggtaggttttctgcatgtcacggcatggttaaaattgctaataatgtagtccacaaaagcattgctcaatacgactaaaaatagtaaaaaaaggataagtgctctttttatatccatatactttaaaacttattttttacactaataatttcctgcggccgcaatataaactgtaggtcatctataacgcccagacctgttaaaagtagagtactatgttttaagggatttaaaatatccgccgcaagaatgtgaatataattttcaaagtggtttacaggaatgcgtaagcgtttttttttgcactgcggttggtttagggtcgaatactggcaggaggtatatatattaataagaccgcggtcgatggtttcaatatcttcatagaattcaatgcgcggcgtcaaaagttttttaagatgttgacataactcatcatacgtgtaggactggaggggggaaagaagggtgtagtcaaagttaaaaatgtttttttgaagaacctttaaagcatgttccgcgtccgtggtttccaaaatatgttttatggtatgaatgtcatttaaatctacaaagtctgacagctttgtgtagaactcggtgacggaggttattttctggaaatcggttttttgaaaaagattttcaatgtgtttgcgggttgagttgctttgcagtccatacaagacatcaaaaaattcaatcagcaaaaacttatacaaatggttaatataaaaagctttgttggccttattctgctgaggatatggttcctctaggggatatagaatggcttggtctatatccctaggatcaatagtcaatgttgcgatgggaagcttttccagcgtagcgggaagagtttgggttggagcgtagtaaaagtatagcccggtttttccctctgaaagaaagcccacaaattctttttttatattttgcagcaccgctgagggtacgatttcgtactgtttatactgtttgttgaaaagggtaataaatttccaggtttcttcaaagcttgcaatctgggtgggccgcagatcaaagtcgatgggaatgtcgtcatgaatgtaggatgatagtcttataggaaaataaatagggcgatcggtgtctgaatcgataagtaaagcataacaaaagttatgcctgttgataagttttttaccaaccgtgtagccgggaatgtttttcacgtcatggatatcccaccagttatccttgcacataaactcgctcatagactggatgacctccatcacagggtcatcttcggtaaaaatatactgggcctcactgtttttcagaaatcttttttgctgggtgatggccattgggtagatcccttcgtccgtgtcaaagataatggctatcttcttcgatgggctaagaattttttgtattgtgctgggggacacctcaaacccgatgtcgccctgtttatctttaaaaaagacacagtgaaggtcgtagcatatggcaacaaggtccagaaagatgtcctgccatgtggtgtcccattgaagcagttggtttttttgttcaacaaaggtttgtaagataaggtttgccagctccgcgccgctggaaaacatgttgccggccccattccccaaaatatagtactgcggtgtgttggccgcctttgcaatttcaatggcaagggccttgggggcaagatccaaaattcgagcaagggaataaaaaagcccggcattgctaattccaagcatggtttgctccacccccacaatgcaaaaaatgtcgggctcttttatcgtatttaaaaacagttcatctgctatctggtggggtagaaaggcaatccggttcaccggtattttttttccataggacaaggtatgacgcgatgtttgtgtattaagatcctccaggtcttgttctacaaacgtgtgcttggtgaggcaggtattgttaatatagaaccgctttgtgcccagcagggccttcgtcttttggcagcacggcagacagtaatttagggggtggcggccttctagtaggcttagatgagggtagtcaggatgcgggcagctatagtaggcaggtaccccctccgtgaaattccaatactttactagctccttgcgcttggctggcggcatggacttcacctcggcctctgagtaaatgacgggtggccgtgggtgctggcataggacggagtaaaccgttgcctgcgtgtcgtacttgcgcaggtcatacaggtcggggtcctgttcttgaagcgcacgtagctgagaggctccctttccttgttgtttatcgtgcagttgagagagtttattaaccaaaattttgtcaggcccggtgatcaagttatctaaaaacacaaataggtaaacccaaagatagttaaactcttcctgggtaatgttaaacatttctattttgatatctgtaaccctatggtagatgcgaatgttgcggccgccgtagattgtttcccaccgggccgcaacatttgtgtcaaagaggtacgcatacgtgttttggagcaacgcaacattgatgtccattttgcgccccggaccggaggaaataatgatcatccgttcgatttcgtggggatcatacgaataaatcccctttttaaataaaaaattgtagaccccggtttgctggaggccccgcacggaaataatccctgcttgctcgtattcccgccaacgacttttgagctcggtaaatcccttgctagaaagcgtatagggccaaaaggtggacaccgacatggagctgatagaaatttggatgtcctcgttggagggaaggggcagactccctccacgaggaaacgcggcaggccccatatcattaattgtatgaataataggatttatgaaattatttagggtggacaccacggagttaaagtcgtggcgctcgttttctgaccaattgctttcgataaagtagtgcccattattttgtatggtaagaataaaggcctttttattgataaagcgtattaaaataatagtgggtacacggaatgttttattgctgaatttttcaggctccgtggaagttatgtggtgtttggaaaccacggtgggacctgttttactataaaagaacaccaccagctgaggaatatcgggagtagctggaaataggtcgaaaacattgcgcacattaatttgaatatttacgaggggtgaaattttaatcattgccgaggtgacggccaacgtgccgcgtgttagtctattcccctcgtacttggcaatgacttgttgtgctctggcatacgtaaagtttattagtttttgctctaggagaagcctctttttaagactggtcaaggatggagaaagagcaggatactgtttttccatttgtaagggagattgtaccaatagtttaaaggcatcgggggaaagaagaggccaatacttcataataaggccgtaatagagtaagtcaaattggtaattatcctctatggcaatggagatttggcgccgcatgggggccactagcgtgttgaggtctgctacaaagatgtgatgaatgttttttatgagctggaagctgtcgagcgcttccacatagagctcatctttttgactttccatagatgcgtcgatgttcaccccacccacctgttgaaactcctttttgtagtcgcgaatgtctaacgccaccccgctaccgcttaacaataggcgatacgttacctgaagcgcattgttttgaaaaaagaaaatgtgttgtctataaggggggatccctgtggcaacgtaaattttttctcgaatgtctttaaaagtgtcttcagggaaaatactatactcgctatacatcgtctcaatttctggcatcatcacgtttgtctcctcgccacgatcctccacaaaaagtttttcaaactcatctaaatcatcgctatctccacccaccacgtattgggaaagctttttctcccaatcctcgccgtaaaaattttgtaaaatttctttgtccttaggggttcgctgcaggtctttgcggcaggcctgtaacacgtttgcaggaacggatcccaaaaaaataaacgtcttcgtgtactcattttccacaggattataaagagtaactcgtagaggatttgttaaaaagtcattttggaaatccattatacccggtatagaaaataaaatttaaaataaaaacggatgatatctatcatggaccgttctgagattgttgcacgggagaacccggtgattacccaacgagttacaaatctcctacaaaccaatgctcctctactattcatgcccattgatatccatgaagtacgatatggagcctacacacttttcatgtatggttccctcgaaaacggttacaaagcagaagtaaggattgaaaacatcccagttttctttgacgtacagattgagttcaatgatacaaaccagctttttttaaagtcgctactgacggctgaaaatattgtgtatgaacggctggagacgctcacccagcgtcctgtaatggggtaccgcgagaaggaaaaagagtttgcaccatacattcgaatattttttaaaagcctgtatgagcgacgaaaagccattacttacttaaataatatgggctacaacacggccgcggacgacacaacctgttattaccgaatggtttcccgagaattaaaactacctcttacaagttggatacagcttcagcactattcctacgagcctcgcggcttggtacacaggttttccgtaacccccgaggatcttgtttcctatcagaatgatggccccacagaccacagcatcgttatggcctacgatatagagacctatagccctgttaagggaaccgttccggacccaaatcaggcaaacgacgtggtgttcatgatatgcatgcgcattttttggattcactccacagagcctctagcgagcacgtgcatcaccatggcaccctgcaaaaagtcctcagagtggaccaccattctatgctcctctgaaaaaaatttgttgttaagctttgctgaacagtttagccgctgggctcctgatatatgcacagggttcaatgattctcggtacgactggccctttatcgttgaaaaatctatgcagcacggtattctagaagaaatctttaacaaaatgagccttttctggcaccaaaagctggataccattctaaaatgctattacgtaaaggaaaagagagtcaaaatctcggccgaaaaatcgatcatttcctcctttttgcatacccctggatgcctacccattgatgtccgcaacatgtgtatgcagctttaccctaaagccgaaaaaacaagcttgaaagcgtttttagaaaattgtgggttagattcgaaggtagacctgccgtaccatctcatgtggaagtattatgaaacacgagacagcgaaaaaatagccgacgtggcctattactgcattatagatgcccagcgctgtcaggaccttctggtgcgccacaatgttatccccgatcgcagagaggtaggaattctgtcatacacctcgctgtatgactgtatctactacgcgggaggacacaaggtatgcaatatgctcattgcctatgccatccatgatgaatacggccgtattgcttgcagtaccattgcccgaggtaagcgggaacacggaaaatatcccggcgcctttgtgatagaccccgttaaagggcttgaacaggataaacccaccacaggtctcgactttgcgtcgctgtacccctcactcatcatggcctacaacttttcgccagaaaaatttgtagcctctcgggatgaggcaaatagcctcatggccaagggtgaatctcttcactacgtctcctttcactttaacaatcgtctcgtggaaggatggtttgtgcggcataataacgttcctgataaaatgggattgtacccaaaagtactcatcgatctacttaacaaacggaccgcccttaaacaagagcttaaaaaactaggtgagaaaaaagaatgtatccatgaatcccatcctgggtttaaggaactacagtttcgccatgccatggtagacgcgaagcaaaaggcgttgaaaattttcatgaacacgttttacggcgaggcaggtaacaatttgtcgcccttctttctgcttcctctagccggaggagtcaccagttcgggtcaatataatcttaaacttgtctataactttgttatcaataaaggttacggcatcaagtacggtgacaccgactcattatacattacatgcccagatagtctttatacagaggtaacagacgcatatttaaacagccaaaaaacgataaaacattatgagcaactctgccacgaaaaagtgcttctgtctatgaaagccatgtctacactatgcgccgaggtgaatgaatacctgcgacaagataatggcaccagttacctacgtatggcctacgaggaagtactctttcctgtgtgctttacaggcaagaaaaagtattatggtattgctcatgtaaacacacccaattttaatacaaaagaattattcatccgcggaatagatatcattaagcagggtcaaacaaaactcaccaaaacgataggaacgcgaattatggaagaatccatgaaactacgccgccctgaggaccatcgcccccctcttattgaaatcgttaaaacggttttgaaggatgctgtggttaacatgaagcagtggaattttgaagacttcatccaaacagatgcgtggagaccggacaaagacaacaaagcagtccaaatctttatgtctcgcatgcacgctcggcgtgagcaactaaaaaaacacggcgctgcagcatcgcaatttgctgagcccgagccgggagaacgcttctcctacgttatcgtggaaaaacaggtacagtttgatatccagggccaccgcacagattcctccagaaagggggacaagatggaatacgtctctgaagcaaaggctaaaaatcttcctattgatatattgttttatatcaacaactatgttctaggcttgtgcgcgagattcattaatgaaaatgaagaatttcaaccccctgacaacgtcagcaataaggatgaatacgctcagcgccgagctaaatcctacctacaaaaattcgtgcaatccattcaccctaaagacaagtctgtcattaagcaaggcaatgttcatcgacagtgctacaaatacattcaccaagaaattaaaaaaaaaataggcatctttgccgacctttataaggaattttttaacaacaccacaaaccccatcgaaagctttattcaaagcactcagtttatgatacaatactttgatggagaacaaaaagtaaaccattctatgaaaaaaatggttgaacagcatgctacggctagtaatcgagctggtaagcccgctggtaatccagccggcaatgcgctgatgcgggctatatttacgcagctgattacggaagaaaaaaaaattgtacaagccttatacaataagggggatgcaatacacgatcttctcacctatatcattaacaatataaattacaaaattgccacgtttcagacgaaacagatgttgacgttcgagttttccagtactcatgtagaactgctattaaagctgaataaaacgtggcttattttggctggaattcatgtggcaaaaaaacatctgcaagcttttttggattcatataacaatgaatcgccgtctagaacattcattcagcaggctatagaggaagaatgtggcagtattaaaccatcttgctacgactttatttcctaatacttcttaagaaactctttaaacaaggacttcgcatggtcaaaggttctaaacccatggcccttatgattcgccaaaaaagcggtttcatcaagattttctaaccctttcacggatgaagaaataaggtgttcggcctcgtttgcccattttctatgattttttttcacctcgggttctagatctgttttctccatatactcattgtggtcatatttttttttgggaggaggcgtgggtggaggaatgggtggaggaagtacacccgactttcccgcttcaaccgttttataaaaaaatagaagcataatacaaagaataaggactatcgcaaatatgataaccagtgtcccagtcgagggcattttgttatataagtaacgttttttttattttttataattcgaatgaagaaccatgttgaatagtcttctactcaaagacattttgttatacggtaaatgagaatttataaaatccgaatatcactatcatactgtttatctgagaaggtctcactgggtcctgtgatggagaacccatactctgtaatgctggggtttataatgtggtcaggactgacaagcacatttctgaactgcgagagttctaggtttagacgcagtcgtaatagtcgctgtatatttgtaataaatattagattgcgtatgaggcgagtgtcaaagcgatcctttccaatttgtactaaggtgggcttttgtattccaactcccacttgtttaacgatggaccagggtccttcttcccgattttgttccgtgatataggtcagcacactattttctgtatatgaggtatgatgtcgcatattaatacctggtgccattccaactggcggttgtgcaattcgggctgtaccgggacccaaccatcgtggagttttataaacatatcgttctagcgtatttaaaaattccttaaggttatttacgagtagcatgaagggtgctattaaaacaggtggatggtttataaccattgtcataaaccattgcattgcttcaatatcattttgtaatgcttgacggggaggcggggcaggtaatccacgtatgttgaataaagcggttaattgtgcaccggctgtttggggcgtaatattttgtattaaatttatcatcgaattggcttgcccggcatttcctataagatcgattaaattggttatttgacctcgatattgttgtacccagttttgaatggcagcgatgatctcaggggttggattgttttgaatttcaggtgtttgtattagattattcacttctcttcgtgtatcttcaagctgagtcctaaatgcatttaactcgcctataatttggtttctatcaataacatttcttaaacctcgaactgtttcagccaatcgtatagtacgcacaatttcatgtaaggcctggtttatgtatattgacatgggatggccccaccgctcacgtccacgttgaatacctgcggccaaactaggacctgcctcgtcataatcaaattgtgtaggataaaggcttccaaatagcactttattgaaaatttggtcagaaagaaatttagggcggcccatatttagcgcgttgtcccctctaaagatgcgtgacatgtatccggcgttgcctttggatagtaactcattcccatattgagtaatagagaccgagacataggggtttataagaagttttagcataaattctcgagtatttatggggggacgattcggaatgtttaatacctctgcaacatctggttgaggagccgtggtgtccagagatcgtactttttcagccgaaatgccgtacataagacaagcaatttcttcaaaactatagtcatagttgtaaatattggcaagtggtatagatcgcatcagcgcatttacattgataggtataatattcatatcaaacaagttaaatatgcgctcgcgctctctattagagccaagagtgcgtgtttgacctttcggcgacactattttgtgaatatgattgatttgctcctcttggtaagagctttccacgaaggaaattacgtcttgcaatgttttacgaagcgaatacactgcattcatccctattcccgctgttataatgggtttatcgtctctgttctcgctaataagattaactccaccaaaagtattttcattgtacatcatcactgttttaaaactacggatatttatgataaatcggagagcctgaatggcgtgggtataaaagtgttcaaatcgcgtgggagtaatttgttcgcgagcaactaccgtttcattatagtttttcatgataagctgtactccgggcatatctgagagctgtaccggatcatttcccagtaattttcttgtgccgtatagtagtttaaactcgggggagccgctttcaaggttcgggtaaagaagaggatcatatacctcattattttctattcttaggtcatgtaaataatagagcgaaagtgaaaatggcataagaggctccttattgtaccgggacatatagttttgaatgaagtgttcttctgtttcaagatagatgggatgatcggtaagctcgtgcaggacctccatggcagaatctgccagagtgtgagagcctctaatgatcccgtcgatcactgcgaccagtcgctttcgcacaacatcgctcgtattattttgtgcgtctcctaggggcataagcgtaacattgggacgaaatacgccgccaattccccgcagggccgcctgaccgacggatagtcctgtcgcaggaacattgttattattataataaataacggaatcattattggctcccaagagtgccgtcagattagggcgagctagttggacatttgtgtattgtataaattgttttagaagctctccctggctaataagaatattaaacattttgttaaatagtggaagattggctctataattttctttaaggtaaatgggaatttctgttaaagtagaaataagatgctgactcaggccctggcgattggtatccttaataagccgctgaagtataagtcccaaagacagaagaagcaccgactgctctgtggggtcgcctctatgaccaaagacgttgttattgcgtgctaagtcagggtgagcatatcccatctccatcactgcttggctaaagttcccattagcgaatgcattaataagatttagatatatttttccgctgggagcatcataaaatcgggtaatatatgaagctatgagctggttaaacaccatcatcatactacgattattttgaataccatagtctgatccgtataggcgataacgtcgaaggttgtttgcggcatcattgacattggcataggttctgagcgctatgttgtcccagtagctaagagtattttcctcctgggcgttgttggtacgaataagattggagagtctaaagtctcctagtgccacctgctctacacgaagtccagagttattctccaaagcatcgtaaaatacgagtctactgaatactcttccgtattgttcaaagcgttcagaggattggggattgttatttatttgaatattagccgcgtcccttctttgcgccccacctcgaagttgcagtacattataaggctttgtaagcaaggtgtaggttttattaatgatttggttaaccccctccaggcccaattcaccgccaggaagcggccttcctccggcatcggtaggtggtttaataagtttgtcaattaaatgttcttccaaccagtaaaatgagccaggattagatctattttcatagtattgaataatgtttttatcaatatgcgggcgtagaagatcaagaaaatacttcgtgtcggccatcaaagaatcaattaaggaaataagacctgtaaaatctaaatgcacttgagcggtgctggtttcagggaagcgaacttgaaccattttgttaaaactggaggtcatttcgaagatattggtcaacaggagctgcatgattcgctgattatctactaaataccttgcggccaactcttgctccggacgaactcctccaccagcaggaatacccacatatggtacaatccaagcaaaaagagtttctgtggttaaatttcggtcttgggctgctgcagccgcttcggtagtgggatcagggtacaccatagaaagccgcatattgatttctttaatgactaatcctggatttctaatctcagagatggccccgtgttttcttccgagccagtcaataagattggcgcggttcacgttggcagcttgtgtctctcgtaaccattcgataatgcttttttgaatcgtatctaggtctaaacctttaatgttattacgaaagttattaagaagtacgtaaatagcactcaataagttaagacctgtaataacggtttcatgaaacagaaatattttgttaacatctgtatctgccagtgactcagagccttgaataagttttgaaacgatttgaattttatcggtatgctcctttttgagttcattgatagcctggcgaatgagttcttggtaggaaattttgcccaattcttgttgcagactgggatcttcaaacatctcactaagctgtttcctaaatttttgtaccaaatcccactgggagttgggctgcagcattcctgtttggacatccacagagtctatattgtatagtgccgggcgccacttgggggtaggctgggttgaaggactaataaacctatcggagggaagtaattgtgaggattgtgtatagccatcctcatcaggaagaatggagtagttggtttgattcatcattccaaaatcattcatagttcgcgcttcctgaacaatgcgttgaaatttttcccattcggtgcgtgtaatgacaccgaatctgcggtttatttcatttacaaaatggataagcgcttttttggttgcttcttgttcaccatactctaagttaaagtgttggtaaatgacgtttatttctttgataagctgacgaatttcggtttctgagtagtcaccaatgttaataagctcaataggacgcataaagataatgcgaataagtcctgagaagattccttccagctcaggaagcatcgagatctgtacattttcatctctaaaggaaaacaacttttgataaaattcggcgaggcggggaaggcggaagtaaagctctgctgcctcgggaattacctcgggctctagctcatcggcaccccccaatatcatacgcgtgggtataagtttgtacacgggctcaggccgttcaaacatgtcgtaaatccctaatacaataaaaatcttggcggccatacttttcagcatgaaggtgaagaagacgtcctcggtttcccagcgggttgatagggcgtcgttaactctcacagtagagaggtagacccgctgagccgcttcctcggcagtctgtgcaagcgccatcctttgtcctccaatttctgattgatttagatttttaagtcccacggaaagcgcagaatgttgaagatattcaagcaaggttttatagatttgcaggggcgacatgggcaccatttgccgcagctcctctcccccaagcatgtccccaatccgggcaaaggcattgatgatatttttaagcgcctgaaagttagaaagagagcgcccgataaggtcgcgaatgtttttagcctggcttgctctgacgggacggagggtaccaacgcttcggccttgttggatttcagccgcaactttttcgtagtagtggcccgcaggagcattatccgtaaagacgttggagtcgttgcctgtggaggtgggaaaactttcaaagacttgtgcaagcgtgtcccctgttgtctcggtgaaccatcgtcctataatgcgcacgccatccagcatctgttggactgtttgaatagaatctatgttgtttacaaacgttttggtaatgtttttaagataaagatctagcccttccagagctcgatagaatcggcgttttacatcatactccagctcgatggcgcttacggttgccttccagtctacttcctgggcacctccaggatttgggcccacgtgtcctctggcaagatctacagccggagaattaatgcgcgcatttttttccgtatccaactgcatgaggcgtcccgcaatagcatctccgagaatagtggcatagttttcctcgtaggattgaaactcctgtttgttatgcgttaaattggagtaaatctgggccacataatagtaatacataaaggtgttaattgcctggttgaggtcaacctgcgatcgcgcggccttgctgagcccaagctcttcaactgttagggcagcaccgcctacccttgtacactcgcagtcctcctcgcctccatactttttttgcacaatatcggtataaaaatcaataatctgtagcaagcgagagcaggagtcataaagatttttaaaattagggtcggttttagatatctcctccaaaacatttttaacaagcgtaagctgtgttaagaaggtttcgcgttcttctcgtgcggccgcattggtgtaaaagccgataagacttagatcaagtgcgatggtgcccatatcattaatgcgcgaaagagcatctcgaagcctcgttatgttcggcgtcaaggcaatttctttaacaagtttgatgcctatttttttcacattttccaaaaagtcgttataggcttgtgtgcttttattcaaaaattccatgaggatgtgctttctatccagtctttgcgcttcaatcctcctatctagtggcgttttctcctcatcgcccccctttttggcacaactgttctcaaggattttgtggcgttcattaaaggtctgtcgcaacaggttcacggctttttcaaactcagcaatgttttctgcggagacaagaccactaaaccttttgaggtcaagctccttgtcaaactccgcccagtttttgctttgaaggtactgttcaaccttgagtcctactttctggagagccttattaattttattcgcaacagacgcagcaatacctagattacaaagtgtgtacgaaagtacttttccaaaatttttggttcccaagacactatttgtatcatttaaaagtttaataatatccacctcatccgtctgcagtttatcaagttccttttgggtgggagttaaaatattgtcaataaaattcgttaaaatgttgatttgcaggttttgttcatttaaaagtcgacgatatactgcttcaatcatggtgactgcattaatgacttcctcattgggggctgctttggttacctccgtcaccatgcgctcgtgaagttgcttaatggcgtcgtttaacagcttgatattttcaagtgtattttctatactgccgtgtacatcaagatactctgcgcgcagtccatgagttagggagttaatgtacagaactatttgtcgacatatactggcggccccttcggtggtatctataagcttatcctgacctaaatcaataaattcctggttaatggcgtctgcaatcattttacagacggtctcctgtttttccgcattttttacaaaggtggaaccggctcgaggatcgggcagttgttttttgatatctttaagaatatcttcgatgggctgctttgtgtctactttgaaccctattttggcaatcgccctgataattccttctataatccgcagctttgctttactcgatacggagtctatgtgataatctttaatgtgttgtacaggatttttgtcccccccgccattaaaatatcctccccctgaaaaaggacgagtttgtctttgtatatgatcctgtaacttcgcatatatatttgcttctgatgaaggcagtggtctactagaggttgaagatccacggttacccattataataaaaaaaataaagatttaaaactacaaatattttgctgtttataaacccaatcatataagactaactaaaacattaaatgtaggtgagataaaagcttattttttttaaaagtttaataaccatgagtcttaccacctctttttcttcttcctttagaggggttccataaatggtttgaataaaattatgtgctctaataaccttgttaaaatcaggtgcctttccatattgttcaatatgttgcacagtcttttgtgcaagcatatacagcttggagtctttaggtacctccgatgagggctcttgctcaaacaacgtttcaaaggaggatgtgcattcattggtttcattatcatttttttcatgaatgttctccgaagatgctgaggattccgtctcctcttcaaacagcacatgcagaatcatattccattcttcttgagcctgatgttcagtatacccttgccctgcatatatacgagcagatttcacaatatcatacttaacagtactaagcaatgtttttatagcggtcgtaacaattctaccgctattgataatctcaacagaaaaccaattatacaggctacccgcatgaaacacaacttgtgaagatgatcttaaatccgttttgaagatgacctccattttcatggatatatttaaaataaaatccattcaattttaaaattataaaataataagaagatgccctctaatatgaaacagttttgcaagatttctgtatggctacagcagcacgatccagatttattagaaattatcaacaacttatgtatgcttggcaatttatccgcggcaaagtacaaacacggagttaccttcatttaccccaaacaggcaaagatccgcgatgaaataaaaaaacatgcctactccaatgacccttcacaagccataaagaccttagaatcactcatccttccattttacattcccactccagcggagttcaccggggaaatcggctcctacaccggagtgaaattagaggttgaaaaaacggaggcgaataaagttattttaaaaaatggagaagcggtcctagtaccggcggccgattttaagccctttcctgatcgccgactagcggtctggatcatggagtcaggctctatgcccctggagggtcccccctataagcggaaaaaggagggtggggggaatgacccgccggttcctaagcatatctcgccgtatactccgcgcacgcgtattgccattgaggtggaaaaggcctttgatgactgtatgcgtcaaaactggtgtagtgtcaataatccctatcttgccaagtcggtctccttgctgtctttcttgtcgctcaaccatcccaccgagtttattaaggtactgccgcttatagactttgaccccttggtgaccttttatctacttcttgagccctataaaacgcatggggatgactttttaattccggaaaccattttattcggccctaccggatggaatggtacagatctgtatcaaagtgccatgctggagtttaaaaagttttttacccagattactcgccaaacctttatggacatagccgattcggctactaaggaggtagatgttcccatatgttactcggatcccgaaaccgtacattcctatgccaatcacgtgcgtactgaaattttgcatcacaatgccgtcaataaggttacaacacctaacctcgtcgtgcaggcctataatgagctcgagcaaaccaataccatacgacattacggccctattttcccggaaagtaccatcaacgcactgcgtttttggaaaaagctgtggcaggatgaacagcgatttgttatccacggcctgcaccgcacgttgatggatcaacccacctatgaaacctctgagtttgcagagatcgttagaaatttacggttttcgcgtcccggcaataactatataaacgagcttaatattacaagtcccgctatgtacggcgacaagcataccaccggagatattgcgcccaatgatagatttgccatgttggtggcctttatcaacagtactgactttttatacaccgcgattcccgaggaaaaggtaggggggaatgaaacccaaaccagtagccttacagacctagttccaacacggctacactcttttttaaatcataatctaagcaaacttaaaatcttaaaccgcgcgcagcaaacggttagaaatattctttcaaatgattgtcttaatcaactgaaacattatgttaaacacacgggaaaaaatgaaatactaaagttacttcaagaataagtatgttgatacctgtggtgtgttttacctgtgggtttcctattggaacctacgcggcaatttttgacaaggctcgtaccgagtatattaaaaccaaaatgggcggaacattgccgcaaaatatcccattagatgcttctctccagattgagttaaaagacctcattacagctctgggaatcccaatgcgggtgtgttgtcgcactcatttaattactacgttggattatcgtaaatattattaatatctaaaattgaaaaaatatttttaatgttactagtaaaaatgactacacacatctttcacgcagatgatctcctacaagcattgcaacaagcaaaagcagaaaaaaatttttcatctgtattttctttagattgggataaattacgcacagcgaagcgtaatacaacggttaaatatgttacggtcaatgtcatagtaaaaggcaaaaaagctccgctaatgtttaactttcaaaatgaaaaacatgtaggaaccattcctcccagtaccgatgaagaggttatacggatgaatgctgaaaatccaaagtttttggtgaaaaaacgtgacagggatccctgtttgcagttcaacaaatacaaaatctcgccgccattggaagatgatggtctcactgttaaaaagaatgagcagggtgaagaaatataccccggcgacgaagaaaaatctaagttgtttcaaattattgaactgttagaagaagcctttgaagacgctgtgcaaaaaggtcctgaagccatgaaaacgaaacatgttataaaattaattcaaagaaaaatttctaatagcgcggttaaaaacgcagacaaacctttgccgaatcctatcgcacgcattcgtattaaaatcaatcccgctacaagtatactaacaccaatattgcttgataaaaataagcccattactttacagaatggtaaaacaagctttgaagagttaaaagatgaagacggcgttaaggccaatccggataatattcataagcttatagaatcgcattctatacatgatggcatcattaatgctagatctatttgcatcagcaatatgggcatttcatttccgctttgcttggaaatgggagttgtaaaagtttttgaaaaaaataatgggattgatgtgaactccatttatggctcagacgatatttcaactcttgttaatcagattgctattgcttaaacaatttgctcaaaacaagcttataaacgtttcttaggtatgcgatacgtaaatcctaattctttaataagttctttttcagtagtgatttttagaggtactaaagtttgatttttaaataatccatactgatttagcttataattctttttttttaacgcagctcgaattcttattaaataagaaacgggacccgtaaaatgaagtactgcgtatggcttttcctcggctaaggccgtaaaaagatcaagttgatatgtgttttttttccattcaataaaaagtacacactttcgttctccgcagacttttacagaaaaagaaagatcctttatgcgaatgttgggcaggacgtgttttaaaagttttttttctggaacaataataagaagatccacgtcattaagcattttctcttcgcgtcttaagctaccaacagcaacgatgttttttgataaaatttttataagttgtccattatattcaaacgcaagtcgggagcgtaagtcatttacaattttttttccttgaataagcgttaacattttatatttaatattaaaatcttttcattttatatattatatacgcaaaatggcacttgatggttcaagtggtggaggctctaatgtagaaacattacttatagtagcaatcattgtggttattatggcaatcatgctttactatttttggtggatgccccgccagcaaaaaaaatgtagcaaggctgaagaatgcacatgtaataacggaagctgttccctaaaaacaagttaaaacatgcaattatatgcatgcatataaacgcatgcatataaacgcatacatataaaatgcgtaaatactatataaaaaactataacatatcaatcaaggaatcaacacttttataattttccgtaatatatttttcatccataatgatgtcagagtacatggtccctatgcgaggaacagagcccataagggtaggcgcggcaataccgtaaatgggattcacggcggagtcaaccgcagcatctgtcaagacctggactggagacgacaaggccattcgcaacaacacgttggaaggctctcttgcattaagccctgccttttctagagaggtaacctgtcccgttcttgtcatgagatctgcgtacatgagtaaatgacgatggttgggacccttgtcccccataaccgttctaatttcactaataattttttgccgtgccgcttctatgccgtaaagctccatggtgtctcctatagaggacgatacgatggtgtatgggtcgatgttatcatcaagcattgcgccaaaaatattagtcccgtttgttttgatggcgtagatattgtctagtcttaccagtttcccctgggcatccacacggtggcgcataagcttaacaacattcgcatttttgatgcctggtattcctctaatcgtgctatttaatagtttatccaccacatttacggcaattttttcatccgtagccattcgggtattggtactgcgtctaaaggcgctttcccgtaggtatatgcgaataatgatgggaatccctgaggccgtgttttccacagaatgcatgatgtaggtgttggggtgtttagctcttagactattaataatactttctagactaatgctttttaatatcatggttgttttgtttaattccaagcggatacaccagtttgcaatatcctctgggggctgtagtagaggatggttttccagaaaatccgtcatccattccacatcacttgcaaaatcggggtacatcacatttttttttgtgcttgaatacgtttcgtacaataggtgccactgcaatatcaaccgttcgaacgttataagctctatgctgttagcaatttcttgcgcatatgttttatttgtttccacttccgggttctttagacgtaaaagcatttcagaggattgttcagcctctacgggcttcgcgctaaagatctcctggggccgcacaattcccgacttgttggttcccccggccacggaccggtggtgggagtccagcatatattgtgtcaagggctctgatacggactgcgccgccaggattcccactgcctcaccgtagttaataagactttgagtatattgtagccttatgaggtccaggatggcactcatctgctcgcaggtaatgtttaatgttttaacggttgccagttcgatgcgaataagcatgcgcatcagagaggcagcccgtttaagataaacgggtatgggcgtttgtagtcgttcctgaatgttgttaataaacacgtatggaagatttttgcaaaacgttttgaccatcgcgtatttttgtagaatacttttttcgtcgaagggaagcacgccactggtggagctcagtagaatgttttttacgatgctggccacgtttaccggcacctgtctaacatctgtaagcagctgactgaaattaaaattttcgacgtttaggaagatctgtcgatatttatctctatcctttttaaggcgtgaaaattcttcttcaaacaagggcgattgtatcccggtgtacttgaatttgtcttcaagttcctggtccgacagcatgatggtttcaaaccgtacggtttcaagctggcgcgcatcaaggccgtcctctccgtacaactgctgcacaagacgcgtatcgatggaaacccgtcggtaataatccacaatacaggattgaaggccaaagatggctttacggttggcatagcctgtggatgatgtcgataatgctttgttgatcaagtcgaatcttccattcatttccccaaagataaattcaggggaggtaaggcccgcaatatagctgttgcagatgaacccgtaggcctgcgcctccagggcaaacctggggtagtacaccagggtcctaccgaaggaaaactggggttgaatgcgttgtgtattaatttcaatttggccgatgcccgccatgatgtgaatcatattggggtttgagcccttggcgccagtggccaccatctgaaaaagcccattggtttccggattaatggaattcataatcggctttaaaattctatcgggaaatttaagcgcattcagctgcaatttttcgtagaagtcatgcgttgtcaggcctataggcggcatgatgtctccatgaagcagccggttgtttatttcctccgactcaagcagcagttcattgataatttcttggacctcctgatgtgcctccggggttaggagcatgtcggccgtggacactgtgaatccggcgttgcgcacgtagtttagggcgagctgctgggtcgcaaatatcattttcaaggcctgctgcggcccatacctacgcgaaataaggtgatagattccaccggaggaacccgctccgacggcctttttgtcaaggacgccttcaatgagttcgccgttgcgtatttgtgtagagatgtcctgcttgttataatgcatgtagggtgcatacacttctgagtaccatgtgggggctcgttgataattgatgggggtctgcctcagtagcatagatacaaccgatttgccatccagcaggtcagttggggagtagttggcaaaacaaggtgggtcggtttgggttgtttgaaacaaccccatggcgtgcagcttgttcatcacatttttccccatgggggtgttcgtgcgtgtaagcaaaaagcttcccaccgtggagtcctgcacctgcccattaacgggacccgagctctttgtggaaatgaaccagtttcgcacagaacaaagtagttcggcctcaacgcggctcatgacgctccagggaacccagagattcatctgatccccgtcaaagtccgcattataccaggcacatgcgctgacattcatttgaaacgtagaaatttttgggttttcaagaacgacaatccggtgaacccctatgctgcttcgttcgagagaaggctggcgattaaaaaacgcgacgtcgccagtgacgacgtcacggtaaaggatgtctcctacctccagcctaaagtcttgtttgagaccctcaatgtcgtgaacggattgtgttatttgcttatacactcttgaacaaccagggtactggcgctttccatttaaaaaatagggcattaatctattaatattataatgttgcactgtttccgcaacttgcagcgttcgtgcaaaggaaatgggatagccaacctcgtccaggtgaaggtctgagttcccgcagatggtggaccggctgatcgaccatacctggctgcccagtagggatttacgaattcttccctccttgcgaggaagtcttcgcatgatggagggagcagggcgtgcccccatgacgatcccacgctttcccgtgcctccctgggttgcggtggtggaaacggaatccaacaaaaagttatagtaaagttgctgtatggtttgcaaattgcggtcaatatttaaaggtattttttggccgcgcacgatttgtaggtccttcgggatcagcagattctttcgaaccagatactgaatcacgttgttaatgtcgtgaaagctttgggggcctgacccgattcccaatctgatgccaggtcgtatgctgatgggggggatctgaatggccttaagcacaagtttttcgggatgggagtttttacttcgccccagttttacaacggtgtcgtaggttacgcgcgaaaaaatctctctgatgatctgcgggtacagtttgtcaatcttgccctgctgatccgcccaaaaggtaaaataatcttccgagtccttaacaattttggggtgtactgccttacagacgtagcactgctttccttcggtttggcttgaagccgcttcaataagacgcttaggcctaataaggtgctcgtacctctttaggtcaacgatgggagccccgcagttgagacatataacccttaaccatcgtcgtatttcggcgatgaagagcggctgaagcaccggagcatgcatctgcagtatcccagggtgtcccatacattgcttgcgctggtgtgagcaagtgatgcatttataatggtgatcggtggttcccattcgcgcatcatagatacccccttcggcgggaagggtgccctcaaataaattagaaatggtaacctccataacgccttgcctcttatgatcattgtcaccggcaatattgaactgaacggcggctatttcggcatatccagcctccatatttttgctaaatacataataaaacttcaaatgttaaaaaaaataacatcggttggcatatttttttgttaaaaccaagtgttaaatgatttctaaaacatttatcggttcacgaaaacctaccgcacgggcctgaagaggaatgccagttttgggggaaagctcggcatattccacggtaagctcttttccataaagatgttttttaaataaggcgggcgtgagtttttgaaaaagagcataacgatccgcgtacgtcaaatgcttaggagtgactacaaaccgctttttgtttggcaattcgcaaacccataaaatggcgcctaagtcctttcccttttttccctgagtatagtccactaaaataaattcagcgtctagcagcggtttcagcttggcaagatgcgctgagtggtagttgttgtatcccggctcatagggcccattggcattgcgtacgatggctccctcgtagccctccttaataaactgcgccttaagcctaagggcctcatccacattcttcacgctaaaattttcaacttggtggataaaggtaagatcttccttctgtttaaaaatatttgttaatagctgttgtctcttgttggaaggcatttgaagctgatcactccaaaaacagtcaaacacgtaaaagtgcagctcggaggaatctgtcttcgcattcgcctgccccgcgatccattgcagaggtttgcggtgtaaataaagctcaccatccaaatatactctcacgtctataaataaataaagctgtttgagctcttttttaatattgtcaagacctaaaaattcctttttcgtgcgcgaatacaagagaatgctaccatcgccctgctggcaggccacagctcgaacgccattacgcttgcgctgcacgatgggatctgtttcttcttcaaaaaatgtcttaggaattatattaaaatattttaccagcataggggggataattcctctatttgtgtgggctccccgcttttgtctggcatggcgattatatttactaagggcgtccttgaatgcctgatggactaccgttgtggcattttttttacccaagttttttccctcggtaacacgtgtcatttttgatatccgcaccgccccttcttccacaaaaaattttgtgaaaatttcagcaacggcgtcttttacatctgtggaaaacatctcatctgtgatgggaatgatcgtgttgtgctgcaccacttgcacacaaataatccatgaggccttttttccgcttttcgtttcagactcaatcggaggaaaacaaaaaatgttgtttgaatattgcccaggaaattgatttagcatggttttaacaataaaataagcctatcaatttttttataatttgaatagttattccaaattcaatatggcttctttagataatttagtggcacgatatcagaggtgctttaatgaccagtctcttaaaaatagtactattgaacttgaaatacgttttcaacagataaattttttattattcaaaaccgtatatgaggcacttgtggcacaagagatccctagcaccatctcccacagcatccgctgcatcaaaaaagttcaccatgaaaaccactgccgggaaaaaattttgccgtcggaaaatctttacttcaaaaaacagcctctcatgttttttaagttttcagagcctgcatctctgggctgtaaggtctcgctggccatcgagcagcccattcgtaaatttatcttggactcctccattctcgttcggctcaaaaatcgtacgacctttcgggtatctgaactttggaaaatagagcttaccattgtaaagcagctgatgggaagcgaggtctctgcaaaacttgccgctttcaaaacgcttctgtttgacaccccagagcaacaaacgacaaaaaatatgatgacgttaataaacccagatgacgaatatctttacgaaatagaaatagagtatacaggaaagcccgaatccctaacggcggcagatgttataaaaattaaaaacacggtgttgacacttatttctccaaaccatttaatgctaacagcctaccaccaggccattgaattcattgcctcccatatactgtcctcagaaatccttcttgctcgtattaagagcgggaagtgggggcttaaacgcctcctcccccaggtgaaatccatgaccaaagcggattacatgaaattttatccgcccgttggctactatgtaacggacaaagcagatggaattagaggcatcgccgtcattcaggacacgcaaatttatgtggttgcagaccagttatacagcctaggtaccaccggcattgaaccccttaaaccaaccattttggacggtgaatttatgcctgaaaaaaaagaattttatgggtttgacgtcatcatgtatgagggcaatctattgacgcaacaggggtttgaaacaagaattgagtctttaagcaagggcattaaagtcttacaagcgtttaacataaaagcagaaatgaagccctttatttcgctaacaagtgcagatcccaacgtgctcctcaaaaactttgaaagcatttttaagaaaaaaactcgcccatattctattgatggcatcattttagtagaacctggcaattcttatctaaatacaaacacctttaagtggaagcccacctgggataacacattagactttttggtgcgaaaatgtccggagagtttaaacgtaccagagtacgcgcccaaaaaagggttttccctgcatctactatttgtaggcatctccggagagctttttaaaaaattagcgctaaattggtgtccaggatatacgaaactattccccgttacacagcgcaaccaaaactactttccagtacagttccagccatcggattttccattggcatttctttattaccacccagatacctcgtcattttctaatatagatggaaaggtccttgaaatgcgttgtcttaagagagaaatcaatcacgtcagctgggaaattgtaaaaatccgggaggataggcagcaggatcttaaaaccggcgggtattttggcaatgatttcaaaacagccgaactcacatggcttaactatatggatcccttttcctttgaggagctggcaaagggcccttctggaatgtacttcgccggtgccaaaaccggcatataccgcgctcaaacagcacttatttcctttattaaacaagaaatcatccaaaaaataagtcaccaatcctgggttatcgatcttggaataggaaaagggcaggacctaggacgttacctggacgcagggataaggcatcttgttgggatcgataaggatcaaaccgcgcttgcggagcttgtttatcgaaaattttcgcatgctacgacccgacagcacaagcacgctaccaacatttacgtgttgcatcaagacctcgcagagcctgcgaaagaaatcagcgaaaaggtacaccaaatttacgggtttcccaaggagggagcttcttccattgttagcaacctgtttattcactatcttatgaaaaacacgcagcaggtggaaaacctggccgttctgtgccataagcttcttcagccggggggaatggtgtggtttaccaccatgttgggagaacaggtcttagaattacttcatgaaaatagaatagagctcaatgaagtatgggaggctcgtgaaaacgaagtggtcaaatttgctattaaacgtctctttaaagaggatatattacaggaaactgggcaagaaattggagtcctgttacccttcagcaatggcgacttctacaatgaatatcttgtgaacacagcgtttttaattaaaatatttaaacatcacggcttttccctagttcaaaagcagtcctttaaggactggattccagaatttcaaaactttagtaaaagtttgtataaaattcttacagaagccgataaaacttggacaagcctttttgggtttatttgtctgcgcaaaaattaaatattttttcataagaagtactacccaggttttaaagaaatagctaaaaatatcatatggatactgccatgcagcttaaaacgtctattggtttaattacatgtcgtatgaacacccaaaataaccaaatagaaactattctggttcaaaaacgttacagccttgctttttcagaatttattcattgtcattactctataaatgctaatcaaggtcatctgattaaaatgtttaataacatgacaattaatgaacgactgcttgtcaaaacactggattttgaccgcatgtggtatcatatttggattgaaactccagtctacgaactataccacaaaaaataccaaaaatttaggaaaaattggcttctcccggataatgggaaaaagcttatttcattaatcaaccaagcaaagggctcaggaacacttctatgggaaatccctaagggtaagccgaaggaagacgagtcggaccttacctgtgccatacgggagtttgaagaagaaaccgggattacccgcgaatattaccagattctcccagagtttaaaaaatctatgtcatactttgacggtaaaacagaatataagcatatctacttccttgcaatgttatgtaagtcgttggaggaacccaatatgaatctttctttacaatacgaaaaccgaattgccgaaatttctaaaatttcttggcaaaatatggaggctgtacgttttattagcaaacgccagtcattaaacctggagcctatcatcgggcctgcatttaattttattaaaaactatttacgatacaagcactaggatgccgcattaaaatgccacataaggtaatacactaggaatgtcgcacacgcacaagaatacaacgtcgccggagatttattatctagtacacgttttatgtatgtacaatccgccttcatttaatatattgagcggatgtactatgtatttattttaacaaaaaacattattttttttaatcttcatcatctgtttttataaactcagtaatatcaaaagtagcttgtggggtttcagagggttcaccttggttatcctccgtgaggataacatgttcttcaggttcgtcgtcactggagaacccatcatttaattcctcttcactcaacatctgtaaaaaatcttccaagctttcgctatcgttaaaatcctcatcatccataagaataatggtaccttcctcatcgtttcctccttgtttcgtgtctaaataggcctgcatggcatttgcaaaagtatcaaaataggctgagtcagattgctgttccaaaatatggccttgcgtattaaatgtggttgcatcgttgttaaatgcttgcaaatacagtaagggatttatatccattattattaagcaaaaaaaatttaaattatttttcgaccgatgttaggtaaaattaaacaattgctataggtgttaagcaatgtttattgattttaagtactcaacaaccatgatgtaaatactatacagcacttttggatttttaatcaaatccagattaatactaacttcttttgtgatacagttcgtaataatagtatcctgctcatcgttttgtaagatttcttttaatatatttttttttaccgggatactaagcaattgattattttcttttaaaaactccttttgatattcaatcgtcttattcattgaatatttgtatataactataattacaaatgttcaatgaattgttattcatgtcgggagatggctatttaaaaatcatgtcctatttttctttgctcaataagcatccaaatattttcatggcgttttattaattgttcattattgaacgtatcacaaagatcatttataaattgcagatagtttattatttctttcaagagagtaacaaacattacttcagcagaacatataataggtaattcagtggcgttaaaagaattttgatcttgttgatacgccaatggcgaggacttaaggagatttgggggtcttgcccaaaaccctaggctgctgttcttgttttttagggcgtcataaagaaatgaaagcacattgcaaggcttaagccgcgacatctccttccccttgggccctttccatatttttagatctaagatctcatccgagcttatagagtaggtatagtaaagtttttcaaaaaagcatatctgcttgaagtcttttttagaacgactttcaagaagcatttctataatgttaacaagttttgttaggtttaaggcctgttcctgtgtaagctcctcttgcacgtgatagactgaaaaagtgtgcttaggaatgaaaatactccccgtggcactggcctgttgtctgccaggtatatagtacacgctgctgttagcaagctgtaccggcacaatttgccccacttctgcaacattattttgcgattcggacgagggtatgacaatagttacgggttcagtcaataggctttcgccgagaataatattactgtcatttttaataattttaacggccgctattaaatcaaaggcatttaagtaagaaacaacagcagaaaatcttacatgcatatatcctcttccgctattattcgtacgcataataaaacaaggggagcgttgtataacgccagtaatattaagaataaaactgtttttgaaacacttacccacataaatgttttcaagctccttcaaaagatgagcctccacatttgtacaaaaattggtaggatcatcaatattcaacgttgtctcaaaaattttttggtcgatcatatctataatatattctgtctatttcaatttaaataatatacgaataaataacgagattattttattaaataagcaatggtgtatacactttgtatttactttgagatatactttgtgtatcacaacgtgccctaagatgtgtgcacaagtgacggcattttgtcgttaaaaaggtaaaaccagcggattccatcctgcattccatttggttgattacgagcctccatttctttttgcaaaaggttattgcgaatgagtaagcagagcttgatggcactaatctttgtaaggtttaaacttatgcccaattggtcagcaattttttgttgctcctcccgtccgcgtgtttcgcatacggctccccggtttagcatgcgaatatcagtaatctcattcttttttaaaacctggataggtgggcggattttaaatttaagggcctttcccttgctttccatatagcctatgacgatgtcgttttcttttcgtttaacattaatattaagcatataaagcggaatttcatgccaggttttatcttctcgcgaggtaataagtcgcacggagtcctccgtggcatagcccactagagtgttgtcatccccaggcacgtggcttataattttaaaaatgtccggaaatggctgaatatctttttttgaaaaagcgatgaaaaactttttataaacctcgacaagggcccccatacctgcaagattatctataataagtgcttctagcatcgtatagtgaaatgaagcggggtagtggatgagtacctgctccattggctcatcctgaaaatccttctgaaacttttcatacaatacttgaaagggttctttggtctgcgagtgttcgaggtatttggtaatacggatgctgtgcatcgcgggaggctgaaaatcccgaatatatgtttcaatatctaataccggttcctttttatggttaagcaccgcagcgacgtacaaatgctcaggctttgccggcacatgcataatggtgcaaagacgattctgtatccataattccttgcactggttttttgagtagcatagagaaatgagcgccagcgcgaagttgtcctctgagaagagtttattatcgatggtaattccctgtatgagcttgggagtggaaacagccttccatagctcggagtacgtccacacggggcgtgccataaacaaagatataataatattagaaattgtttttacctcttgctccccgtatccataggcctcaaaggtattgaggacggtggctccgacgtttgccggcgtgatggatggactaaggggcagactttccaacataggcttatcaatcttaatctggttggtgaacccatcaatggcgtgctttcgcagcgccttatccccctcctgtattaaaatgtattcttttaatttttgtgcgtacttagcgagctctggccctccatcgggtgttgtcgatacgtacaaataaattgtcacgttgcgctcactgggggggagctccatgtgtgaattttttcgcaccaccctcccaaatacctgaataagccggggaatatcaaggggcaatgacataatcatctcgtaccgcacggcctgaaagttcaaaccctccacaatcaccttggacccgatgagaatacgcagctggtggccttccaggttggacgaggcgttaaaaagagccaggcttcgttcgcgtacagcgggctctatttcgctgtgcagaatggtgaaccgtactggaataaactgatggtcgctatgtgtgtgctcatcgcgaatcgcggcgcagatggagcagcgggtcgttcccacaggggacgaaacttcatttaaaatgccattactttgtaaaatttcttgcaagataagaacccccgacatgcggacccgattgtggtaaattaaaattttcccccggccttgccgaataatggaaagaatgtctttcatcatttgagtgtattttccgctataaaaggccaatcccgagatgtgcgttggtggctgcagcgacaaaaagctgccactcacattaaagggggctctacgcgaaggctcaataatctgtaccccgttttccagaagccagtctgtgcttgccatagaaagggcggtgggggtttccgtcgagttaaacaggccgtaagccttgggttccgtttgttttgaaaattttgggttgggaaacaccatgtcataaatgctgtacgcattactcgagattttagggtcagggcccagctgtttaagcgtttcaagctgatactcagacatggggcattcgatgaaatgtaagtacggcaatgtttcgtctttataggacaacatctttccggcaaatattctttcggggtaaaaattggtgttggtatccaacaaaaaagatacccttccggtgctcagtctttccacaagagctagggcgtcctttttccatttaacggaatgcccactgctgtcaaacagttgctggcgctggaggggctggccgttgggcagctcatgccgcggaaccaaaaggtttaacaggtcgacgtattccatgacactcccggttacgggcgttgccgacatgaagacggccctgggggcctggtgaggtggaaaggcatccaggacatactgtaaagcgatgccataattatttcgttcctggatattgtacacgttgtgtatttcatccgcaatgagcagtcctcccctaagttgctccatgattttttgattcacccggatgaggccgtttgtctcggcctcgctaattttttgcacgaactgagatatatcgttctcattcaatgtatcttctgcttcgtcagaacgatgaaacagagaaagcacatcaaagtttttctcttcacccttactcgtaatattgaaaagcttggatgcaaattccttatagccgtaaaactgaaaaaagcctccgcggtttctatcggttaaacggcgctttaacgtactaacgaacccatttagatgccgtgattcgaccgacgtggtgctgccagactgctttgcaatgtgaagaagccggtgtagctcagcgacctccttgtaagaaacaaatcccagctcaggacgtcttagcatttctgtttgaatgatggcgcgtgtaaagcctaccacaaaaatccagggcgcattttcaataaaattcatgtagtggttcataaattgacgcgcgatggcaatcgcggcaatgctttttcccgtcccggtctgccagtttaataaaagacgcgagtagggcgtgttgggattttgaaagttttggacgaaaagctgggcattatgcaattggagacccttgatggaaggaaagggcgacgcgtaggggtcacacggaaaaaacgctcgcccccccttctcgcagccaggcccaccgatctggacaaaatgagcccgcagatcacgaatgagctctttttggtcgacaggaggggaaatcaacgatttaaactcctttcttcgcgccaactgctgcaaaaagtctgcggcatccaattcgggatacgccatattatcataaaaaaataaacctttttatgaaaacttttatgtgattctgtattgcaattgttttttatgaatactgtaaataagcgtatcaacttgtttttctaacgaagaggcgttattctttttttctggatataaaataataataagtataataattaagactaaacagcaggcaatcactatcaaactcatattatacttacttttttataaaaagtattatatcttatgaatgcgcaagttcagctaattgttcgtcgcttggaatgtgggactgcagggaggtggagtttttcctttttctaaagaataccgggaaatggtggtgaggctcaggttgttgtacatagtagctaggaggaggtttaggtatgctcgacttgcagtcaatagtccggttatagtaaacgatggcaacgatgataagaataataatgagcaaaatcaaaatgcccaggagaatcgcagttgttccgggatatttggcgattgtatgggctaaaaggccttgggtgctttgtttaattccctcgcgggttgacaggttatgagaaagcagtggagacgtttcagtgtccatttattacaattgaacagttatattaatctcaaataaaatataacacaaaattaattatggccatgcaaaagttatttacgtatatttacgagtttattgaatatcgtaagatggtgctgttggaagaaaaggtaccatatgataagtttgttcaaatggtacttaatacaggattttttcgtattaacgcggagacgctgaatcacggaatcgtatccgtgtttatctttggagcaaatggcaagtacgttcaccacggaggcgacatgagaacgcttttaacgaatacgcttaatgaaaaaaaacattatgaagaattaattttaatcgttgataagcccgttttaagcaaaaaaaatattttagatataatcgtcgagcagcgcgctgcaaatcccacgattgtaataaacatatatccctaccacctgttctgcattaacattcccaaggtgagtgccattcctaaacataaactaattactcaggaggaggcgcaggagtttttaggtcgcgaatatctgcaaccgcaggacctcatgcaaattagcgcgtcagaccccccggtggtctggctgggaggaagaccgggagactttgtgcaaattgagcggccctcagagacagctatgcacgctgttgttatccgctttatcaccaagtccaaaatttgagtcccgtgtttaaagatgacagacagctaagtaagcatatctgtaaaattgtcgatgtcctctgtggatagagcgctttcctctgagcagcaaattttttcatacatctccatgggggatggcgaggctttaatagtatgtaggtcacgtaagaactgttgtatgatgggatatttgtcttttaaaaactggggatgtttcataactggaattatttgaaagataaagaccttccatccaaagtagccaaccacatttggcatttcgggacacgcggtttcataaggcatagaatagtgaatagtgtactgatctttttgatacagcgtttcaagtagttggcgaaatgtttccgcgtcgagcgtgccaaaatcttgaggagcctcggtgtgctcctgtgtagagcagatcgtgatgattccccaggcaagcgggagcatggactctggagggtggatatccgtattggtctcattattcgatcccagctgatgaatgccgcacacgcgaaacatggcctcgacgtagatgcccatagagataggcggcgaaagggcaagaccggattgtatttgcggcatatagtaggagggcaccgagttttttatttttcggttgaatggggactttatttctaccagcacggggatgcgtttcgtggcctcatagcgtacgttgttaaaaattgttttgatttcccaggactgttgagtgtatcccagcgttaggtgacaaaacccatcggggctattactatgtccggggtatcccaaataggtcccatcaatatgaatattgtcacctatgacggtggtttggcagaacaactcaagcagatctttactaacacgctcaaaaagggttccccagctacaagcagcgcggttcaaattcttcttaaaaagatttgctttttccgccaaggttatataatagcttttgtaagggtttaaacctaaaacgctggcaaggtcagagccacccacctgagtgcgacgaatagcatgccaggcatcggagcgctgctgaggagagtctttaaacaggcgtacaaaggtttccattatacttgttttaacaggaattcaatataaaaagtcaacacagtttgcaatttttccaatctcaagatatagccatacatttttttttccaattggcgaatatgtttaagctcatgtgtttcaatattagcatccggaaatttaaatgcataaagatgttcaaaggcctgatttatacacgtatcaaaggatctgtggtatgttattagcttcagcatgtgtgccagatcttcaagatggtctaaatttatacggttttccacgtggtggatcatgtctgccacatcttgagcccccatccaggggatcacaaggtactcccccttaaagatgattcgtcgtttttttaaaaaatcatgaaaacgttttaaagcttcaagaaaggggcagttgggctttgaccccaaaatgctgacgacgatatcctcgggcatgatgtattcgcagtgaggatagtagtttacggactctaattcagcggcccgccgttttatttcgtatcttgcccagttattcagagagtactccacgcctccgaccacaacagacatcctatctattaaaaaataacaataaaaaccttatgaaatctatgtatagtggccgctaaaatgtctatattagaaaaaattacgtcaagtccctctgaatgcgcagagcatcttacaaacaaagatagctgtttaagtaaaaaaatacaaaaagagctcacctcttttttggaaaaaaaagagacactcggttgcgattcggagtcctgcgtaattacccaccccgccgtgaaggcctatgcgcaacaaaagggactggacctctccaaagaactggagactcggtttaaagcgccaggacccagaaacaacacgggtcttcttacaaacttcaatattgatgaaacgctgcagaggtgggccataaaatacaccaagtttttcaactgtcctttttccatgatggactttgagagggtccattataaatttaatcaagtggatatggtaaaggtatataagggagaagagctacaatatgtagaaggcaaagtggtcaagcgtccttgtaacaccttcggatgcgttttaaacacggacttttcaacgggcactggaaaacactgggtagccatctttgtggatatgcggggcgactgctggagcatcgaatattttaattcgacgggaaattctcctccaggtcccgttattcgttggatggaacgggtcaaacagcagctattaaaaatacaccacaccgtgaaaacgcttgcagttaccaacattcgtcaccaacggtcgcagaccgagtgcggcccctacagcctgttttacatcagggcacgcctcgacaacgtgtcatacgcccattttatatccgctaggattaccgacgaagacatgtataagtttagaacccatctgtttcgcatcgcataaactaataaagtttgaattctttataggaataaaaatggaagcgtttgaaatcagcgatttcaaagagcatgcgaagaaaaaaagcatgtgggctggcgccctcaacaaagtcactatttcgggtcttatgggggtctttaccgaagatgaggaccttatggcgttacccattcacagagaccactgccccgctttgttaaaaatttttgacgagatcatcgtaaatgccacggatcatgaaagagcttgccataacaaaacaaaaaaggtaacttacattaaaatttcgtttgataaaggtgtgttttcttgcgaaaacgatggcccgggaatccccattgcaaagcatgagcaagccagtcttatcgccaagcgcgatgtgtatgttcccgaggtggcttcatgtcactttttagccggaacgaacatcaataaggccaaggactgtatcaaggggggaaccaacggcgtcgggctgaagctcgccatggtgcattcgcagtgggccattcttaccaccgccgacggcgcgcaaaagtatgttcaacatatcaaccaacgcctagatatcattgagcctcctaccattacaccctccagggaaatgtttacacgtatcgagctcatgcccgtataccaggaactagggtacgcggagcctctgtctgaaacagagcaggcggatctttccgcctggatttaccttcgcgcctgccaatgcgcggcctacgtgggaaaaggcaccaccatttattacaatgataagccttgccgcacgggctctgtgatggcgctagccaaaatgtacaccctgttgagcgcgcctaatagcacgatacatacggcgaccattaaggccgacgcaaagccctatagcctgcaccccctgcaggttgcggcggtcgtgtcccccaagtttaaaaaatttgaacacgtgtccgttatcaacggggtaaattgcgtaaaaggagaacatgtcacctttttgaaaaagactattaatgaaatggtcgttaaaaaatttcaacaaacgattaaagataaaaaccgcaaaacaacattacgagacagctgttcaaacatctttatcgttatagtgggttccattccaggaatagaatggaccggccagcggaaggatgaacttagcatcgcggaaaatgtttttaaaacgcattactccattccttctagttttttaacaagtatgacaaagtctatcgtggatattcttctgcaatccatttctaaaaaagataaccataaacaggtcgacgtagacaaatatacgcgtgcccgcaatgcgggaggaaaaagggcgcaggactgcatgctactcgcggcggaaggggatagcgcactttccctgctgcgcacgggactaaccctgggaaagtccaacccaagcgggccctcctttgacttctgcggcatgatctccctgggaggagtcatcatgaatgcctgcaaaaaggtgacaaacattacaacggactctggagaaaccattatggtgcgcaacgaacagcttaccaataataaagtgttgcagggaatcgtgcaggtattgggtctagacttcaactgccattacaaaacacaggaagagcgagcaaagctgagatacggctgcattgttgcgtgcgttgatcaagatctggatgggtgtggaaaaatccttggactgctgctggcctactttcacctgttttggcctcagcttattatccatggtttcgtaaaacgactgcttaccccgctgatacgtgtgtatgaaaagggtaagaccatgcccgtggaattttactatgaacaagagtttgatgcctgggcaaaaaagcagaccagcttagccaaccataccgtaaaatattacaagggattggcggcgcatgacacccatgaagtaaaaagcatgttcaaacattttgacaacatggtgtacacgtttaccctggatgactcagcaaaggagttgtttcatatttattttggcggggagtcggagttgcgaaaaagagagctttgcaccggcgtggtgccgctcaccgaaacccagacgcagtccattcatagtgtccgacgaattccttgcagcctgcatctgcaagtagataccaaggcttacaagctggatgccatcgagcggcagattcccaacttcttagacgggatgacgcgggcgcggcgcaaaattttagccgggggggtgaaatgcttcgcctccaacaaccgtgaacgaaaggtttttcagttcgggggctacgttgcagatcacatgttttatcaccatggcgacatgtcgttaaacacaagtattataaaagccgcccagtattacccaggctcctcccacctctatccggtattcataggcataggaagttttggctccaggcacctgggaggaaaggatgcaggatccccaagatacatcagtgtgcagcttgcgtctgaatttattaaaacaatgttccccgcggaggactcatggcttctcccctacgtctttgaggacggccagcgggcggaaccagagtactacgtgcctgtgttgccgcttgctattatggagtacggcgccaacccatcggagggctggaagtacaccacttgggcccggcaactggaagacattttggccttggtgagggcctacgtcgacaaagacaacccaaaacacgagctactgcactatgcaataaaacataagattactatactcccgctgcggccctccaattacaatttcaagggccatttgaagcggtttggccaatactactacagctacggcacgtacgtcatctcagagcagcgaaatataattactattacggagcttcctctgcgtgttcctacggttgcatacatcgaaagtataaaaaaatcgagtaaccgcatgacatttattgaagaaatcatcgactacagtagttcagaaactattgaaattctggtgaaattaaagccaaatagtcttaaccgtatcgtggaagaatttaaggagactgaagagcaagattccatagaaaattttctgcgcctgcgcaattgtttacattcacatctaaactttgtaaaacctaaaggtggcattatcgagtttaacacgtattatgaaattttgtatgcgtggctaccttacaggcgtgagctttaccaaaagcgtcttatgcgtgagcacgcggtgcttaagctgcgcattatcatggaaactgctattgtacgctacatcaatgagtctgcagagctaaatctttcccattatgaggatgaaaaggaggcaagccgcattctaagcgagcatggatttcccccgctgaaccacacgctgatcatttcccctgagtttgcctctatagaggaactcaatcaaaaagcactgcagggctgttatacctatatactatctttgcaggctcgagaattgcttatcgcagccaaaactcgtcgggtggaaaaaataaaaaaaatgcaagctcgtcttgataaggttgagcagcttttgcaagagtctccctttcccggcgccagcgtatggctggaggaaattgatgcggtggaaaaggctattataaaaggaagaaatactcagtggaaatttcattaaacgctaccggttttatgatgtccaataggtgttaagcaatcagttcatcaacatttttttcaagaatttgaaaagtttggataatgttctgaatacttttttctaaaagagttatcaaatcttcttgtgaggccttatgaataattgttaataccatttcttgcttatggggaacacactgataccccacaaagctaatatcaggaatcatttcataaatatatgtttttagcagatttccgatggtatgggtttcatcttttatcgtgataatggcctttgttttttcctcatccatggaaaacagcacaagttccggctgcggctcttcaaagttttcataaattttttgaatgctttggattcggccaataatgatccggcaggcgttttttaaatacgtgcgaacggcctggttgatatgtggcagcggcaccgctggaaagcaaagccccaggcggtggtgacgcgggtctgaggtcatagagctttgcttgtaaccgctaagcgccatatattcttttttatccgttgggtactgttcaatgtcaaggtgggaaaaatgtgttttaacggcaagattaaaggcggcatgctttcgtcctatgccctttttaatatagatatcctctataatcaacgattttccgggttgtaggaagccaatctcaaaggtaggattaaaaatcgggtatttaagcttagggcctgccacctggatgagatcgcggctatagatggttttaacctcacagctattgtttaaactccgcagagcaaataccagtgtctcgtttttcgcataaatcggaatgaaattaatgcggtttctaataaattgttccgtcataaacaggtccgtggaatcctcgatcttatacccaccgggcttaatatctagcatataattgggaatttcatcttgcaagacccgcgacaggccgtggaccgcggctctgctaatgcccttaaagtccataacaacattgaccgggacgaggggcaactgctcctcgagctgaaatagttttttggccgcatttttaataaagaggttggaaaagtctatcaaaaacggtttgatttccacgttttggaaaattttttccatttgtattataaatatatctatatatattcaaattatggtagtttatgacttgctcgtttctttaagtaaggaatccatagatgtgctacggtttgtagaggcaaaccttgcggcgtttaaccagcagtatatttttttcaatatccaaagaaaaaactcgatcacgacaccccttctcattacgccgcagcaggaaaaaatttcgcaaattgttgagtttttaatggatgaatataataagaacaatagaaggccctccgggccgccgcgtgagcagcccatgcacccattattgccgtatcaacaatcctcggacgaacagcccatgatgccgtatcaacagcccccggggaatgatgatcagccatatgagcaaatataccataaaaaacacgcgtcgcagcaagtaaatactgaactgaacgattattatcaacatattcttgcattaggcgatgaagacaaaggtatggacagcatgttaaaacttccagaaaaggcaaaaagggatagcgatgatgaggacgacatgttttctataaaaaactaacgacgtaacaattaaacaaaaataaaaatcattataaaatgaatcttgaatacgtccaagttgttcaaaaatttaatcaagtactcctagaacttaccaaaaaagtatgtaccgttgtgggcgggagcaaacccacctattggtatcaccacattagaagggtttgctcagaatgtccatccatgccgatgagtatgataggtccgtatctgaatgtctataaagcccaaattctaacaagggacaagaatttttttatgaatttcgatcccgcgcataatgagtacacctttatcattcaaaaactaaaagaagcagcccgaaatatgccggaagacgaattagaacagtactgggtaaaacttttatttttacttaaaagctacataaaatgtaagccctttattaattaaagaattgatgcataactaataaatggccggtcgtgttaaaataaaacagaaagagctcatagactctactgtaaaaaacaaaaatgtgatgaatctgttccatgaaattataggctcaaaaggcaatattaattttagcgttgtctggcccaagtttaaaaaaatcaaacagagcgtttatgactacatttccactctttctgtgctggaaaaagcaaacgttatgcaaaactttgaagctgataagaaactgttggaactttttgtacaaaagctgtgggctgcctatgaaggctatttcaaatatcccgagattgaaaaatatgaggtggaaggccaggtaaatttcaatctcgtacctcagtgcgtcctcgaaaagtttagccagttgtataggataagaatcaattcagagcttgtcacactcatcctaaacagctgtgcctttatgagtaaatataacgattatattctcaaaaaagatccctacatactaaccataacccccggcctatgcttttcccccattcccaacttcgaggacctaaattttaaacatctttacaacagtgataaaaattctcagcatgacaaagagtttatcatgtttatattatataagctttatacggctgccctaggagtgtacaatgccatctcgattccagacatcgacgtagaagaccttgaaaatatcatcctatcctcggtgagccagattaaaaaacaaattccgcgctgcaaagacgccttcaacaaaattgaatcttcggtacacctgttgcgcaaaaattttaacacatattacagtgactatgtgggctcaggctacaacccaaccatcattatggaacagtacattaaagacatatcacaggattccaagaacatatcaccacgcatttcctaccagtttagaaccatcatcaagtattaccgcgacatgattgccaccaggcatcaaacgatggacccccaggtattaaacctcgtaaagcacgtcgaaaagaaattagatatgcttgatagagaaaaaaattagtatatatagttatggtgaatctttttcctgtttttaccttaattgtgattattacaattttaattacgactcgagaactatccaccacgatgcttattgtttctcttgtaacagattatattattattaatacacagtatacggaacagcagcatgaaaacaatacatttttcatgccgcaaaaaaattcttttaacgaatcttataataaagacaaaaaatctaatatacatattccctaccagtggctggcgcctgaactgaaggaagctgagagcaagtactggtggggcaattatgatcctcatagcgagcccgttctcgctggcgcatcttgaatatcttcatacgtggcacgtcaccatcaaaaacattgcccaacagcacgggcttgatataaaggtggccattgtggtctcaacatcgcatttaaataattttttgccaatttccggggcgcttaacatcgaatgtataaccttccccagttgcggcatcaaggagatagacctcctatgggcgcgcattaaactatttcaacattactgcgccatcggtgcccgtcttttatggctggtaagtgctgacatcaggccccctgtttcagcgtggccagccatcgccgacagtctaaaaaagggagcagatgcggtcgttattccctacccctcccgatggaacaatcttatacctaccgtcatcaaagaaatagttgtccaccaaaaaaaatgccttgtggcggtggatgcacgccaccttgatacagatacccagattgtaggggccgggatgggctgcatcgtcctaaccctaaaggcccttatggtgcgcctaagtattggcaaacagcccgttaagatactgtggcccgaccttcacggcactgccgagggcattcctctggagggggtggaggttggctggtttttaaacgcttatgcgcataaattaaatatacgctgcctaggggctgatcatattgcgcagcacttaacttaattctttatttaaaaagtccacgcatccagtggcggcctacattaagggcctacgcacataaatatacactggctagaagtacgccttcatttaaaccattgaattatttatataatggctgcaaacattattgcaacaagagccgtgccaaagatggccagcaaaaaagagcatcaatactgtctgctagactcccaggaaaagcgtcatgggcattatcccttttcatttgaattaaagccttatgggcaaacaggcgcaaatatcataggagtacagggctcacttacccatgttatcaaaatgacagtatttccatttatgattccttttcctttacaaaaaactcatatagatgattttattggtggacgcatttatttattttttaaggaactggacatgcaagcagtttctgatgtaaatggaatgcaataccacttcgagttcaaggttgttcctgtaagccccaaccaagtagagcttcttcctgtgaataataaatataaatttacatatgctataccggtagtgcaataccttaccccaatcttttatgatctttcgggaccgctagatttcccattagatactctttcggtccatgtggatatcctctccaatcatatacagcttcctatccaaaaccataacctaacaacgggtgatcgtgtttttatttctggatataaacacctgcaaacgattgaattatgtaaaaataacaagatttttatcaaaaatataccgccgctttcatccgaaaaaataaaactatatatactaaaaaatcgaatcagaattccgctatactttaaatctttaaaaacgtctaagtaataacatttttatagtctactcctagttccgaaataggctgaatttcttttttaagtcctttaaaccaaggatgtgatacaagactcttaaaggaaagccgcttattttcattaattgttaaacattccgtgataaactgttttcccgtctctgaaatgttctcgggaatataattttcccgtttcaggatatcatttaaataaaaattttctgcacgaaatctaaaaagattaaccgcgaccatacctatcgtccacacggttaaaggaagctggtagtaataaccataataataaaattctggacacacgtattcccatgttccaaacatattatattggggacgggtttcgtctaatctaacagcgcttccaaagtcaatgaccttaatgatcttttgatttatgtctataataaggttctcatccttaatatccccatggataaagcccttctcataaatgttttgtataataagaataagctggaatattatttttttggcttcggtttcctcaagttttttaaagtaatgataatgaagtagatcaacactatttggaatatattctatgattagtatatgatacatagcattttcggtatattcgataagcttaataacaccgggagtatcttgcagggctttcaacacgatgacttcatttcctggaatttcttttttagaaacgtacttaaatataatgggttgccctacttgatgacccaaaaagacgttatttctgccaccctcaaacatgggtctcgtcgcaatgaaatacatgtgctgcgttgtggagatcctttccacctttgctgtaggataaaacgcatattgtgcctggggattttttaacatttttttaagctgttgttccggcctggacatgttttattagctttatatataaagggttagaaggtttaatttcaatatatgccttaatgatgggattatattcgtaaaaggtatagcctaatcctacgtctttgtttttttggtaaaaaaactgtttgccctcgtaggatatgctataggcttttacttcggcttttacaagcggttggcagggattgggcaaacgtaaatcgcgttcaaagttttcatgaaaaagcaaagcatttgtgggctgacacatcagacagccgctttcgccattgaaggcacattcaatggccgccctttttagtaaatcgcggaaagcagaattaagatggctcttttcaagccccctttcgtgaaaacgctcatcaatcgttttttgttcctgactgccttcgggaatactataaaacattttttgattagccaccgcgatgtacaaaaaaggctgtacggttttctcctcgggcggtagcgcatcgtggctaccaatgcgtataatgcgcgccttcacttgatcctctcgggccttatcccagtacggctctaggatatgaacctgccgcccgtatttgagatccaatccctcagctcctgttttagagacgagtaaaattttaataacctctccgtgtatattcagcggcgaattccaaagctgctggatcatgtcgcgctctttagataaaattttccctgtaataagcgtaaatcgtgttattttggaggacaggactaacgtatgggtcggcccatcttccgcaaagtttttcaccataagatctttcccatccttatgaaggaggatggtgttgtgcccttcttccaatacttttaggggctgaaggcactggtagccctctatttctaaaaagcgggccacgacgtgaaggcccaattccacaaactgtgagtaaatgagcacagggcccggagacgttttaatattttttagcatgcgtactattttgggactagaattttctgtgaaggcctctttgggcagctgctgaacagcctctgataatttttcatcctcctttactgttagcatttcggacgcgaagatgctgatcatacgggaacgcacatagtaggaggagcctgactcttgctccgatcctggcaggcagagggcggcggcatttattttttcatacattcctgagctggcgtgcttttccgcgttttcaacgtctcgggccagcagatattgcctatactgctcgggtgacatttcaaccttttctataataagaggaagctctgtggggaatagcttgttgagctcattctggtttccagcgtagcttatcatacccactaggcggtttagtagtttgtccgcgtttaaagggctattcgttgttttattgacataagcggtgtagaatctttcatagtgaagaggtaataagattcgcccgcttagcatattaaaacagggcaccatttcaaaggggtccttcgaacacggggtgcctgttaaaaacagaatacgaatatttttagcttgcataatattattgtacagctggcgggcatttgttttatcattggcgctattgataattcctctaaagaggttgtgtgcctcgtcaacgatgagcaggcatccatttagggaccctcccgcctttatgatctgctgccccatgttgtaagcgtctagggacacaaacctgaagcgccgcgagattttttgtagctctttggagtgatccgtcgtttccggatataaaagtttaataagctttaacaaagactgttggaagtttgagtgcaacgacttgggtgcgatcagaatcgggttgtaaatatgtgaaagtgagatggcaagcgacaggctcaaaatggttttccccatgcccatctggtgatagatgaggaggccccgtgtgttttccccctggcctatcccaaatttaggatccgaaaaggcggtgtaaattaaaaactggtagtatttcagggctcgtgcaaagcgggcagtgagtgaggtgtctttgctttcctgaagctctttatatttttcatatacctcttttaggtatgcttctatttggacggggaaggaggtgttgttgtgcacgcaagacatgactcgttataaggatcccatattaaaacttcattagaagaatagggctgctgatagctagcgctgcacttaaaaatggggtagccctttttcttgtaaatccggtgcctgtcgtagacctggctagaaagcgggcttagtgtatctttaatgtccacaacgatgcgtacctttttttcatccgatccctgccgggtaatacgtcccaagatttgctccatgttgtttctgcggggcgttgccatgatgatcgatgtcatatgcttgaaggaaatgcctctacgcccgtagccataggtcagcaagataatggaagcgctgtgtgcctgagaaagagcggtatttgaaaccccgccgcataggagcgccacctccggaacgataatttgaacatctttgaattctttggaaagcgcctgataaaaaatttctaaaagtttgcgaaattccacgaaaatgatgatgccatacggctcatcggtcccccatttgtgaggctcagcggtatgcagggagtaaagccgctttgcctcatttacgacaagttgtatacgcgaaggatcttgaagtagtttatcaatggtggcaatggccgataccttttcattaatatacacagggctaacgaagtcaggatgtccctgatattcgatttccctcacgtacccggaaaaggttgtggtgggacttacagtcctctggggctgtcctagatggtgaataataatcttgtccataccatcgggccggtccaggggtgtagcggacagtcctaatatccgactaagttgtattttccaaaaaattttgtaattctccggcgagtgtaattcatgtgcctcatctaacacgactagaccaaagggctcaaagaactgctcaggcttcttgcgcagggtattaatgattcccacgatgacgtcgtactctttgctcgtcatgtcctttttcttgcacgctgcattattgtaagcagctacacgtaggtggggcaggagcaatgttagctcgtcgatccactgtatttgaatcgccttggtgggcacgatgaccagggtagggtacaaaagtttttgaataatgctgatcgcaatacgcgttttccccaaaccggtatttagatgtaggtaaaagcgcccatagggggacaggagctttttatgaatcttatcgaccatttcttgctggtagttaaatagtggaaattctgtttcaacgcatgggagggcccgcagcgacacggggcgcgtcgtgtaaaccatgttaaacatttcaaactgcttttgcagcaatatgggaaaataaatgtattccccctgcagcgtgaaggcagtttcctgtcttatggctatgtgctttggctgcccgggtaatgcccgcgccgtaacggtgagcgccttaagaacgcgcccgaaatcatgttgtaatttactttgtagcttcttataatttattcctattccagcaaaggatataatggcctccattctcacgctggacgggttatatgcagaggttccaaaattcttaccagaggcgttacgagagggctgtgctggcaagaatcctctaagcttttatattcaacaaattttaaatttaatgggatgtgacggtaacgagtaccatgttctttttaccagcagctccgaggaagcaaatactcatatgatcatggccgccgtgcgtcgccatttgctgcggacgcagcaaaggcctcatgtcattatcggagcagccgagccccctagcgtcaccgaatgtgtgaaggcattggcgcaggaaaaacgctgcgtatacaccatcatccccctaaaaaattttgaaatagatcctgttgcggtatacgatgccatacaaagcaatacctgcttagcgtgcatttcaggcactaatgctgttgtcaaaacgttcaacaaactccaggacatcagcaacgtgttaaaaggtattcccctgcactcagaagtgagtgatcttgtttatcaaggatgtattcaacaaaatccgcccgctgatagtttttcaataaatagtctctacggcttcctgggagtcggtgttttgggaatgaagaaaaaggtcatgcaaggattggggccgctcatttttggaggagggctgagaggcggaagccctaatatacccggaattcatgccatgtataaaacgctaacccagcaaaggccttctatgaaaaaaaataaatacaatacatacgctgttcatgaaaactttaaaaaacatcagcatgtatatctacccatagggggcgtgtctgcagaggacacgtctgcagaaaacatatctacaaaagacatgcctgttgaaggcccgaagggactcccgggctatattttatttagcgttggccgtcgcgccgaggagctacaaaaaaaaattttcactaaatttaatataaaggttggccgtgttgttgacttacaagagatactgtttcgtatcaaaataccccaaaaatactgggagacattattgttcatccaattaagagataatttgaccaaagaggacataaaaagagttatggttgttttgatgcatttagataccatcactcctcgtggctctcttcctcctccgagccactcttcttctttttcttaatcgtttttgtttgttctataataagggaaaagaactccgtgggatcttgttccccgtacaggttatctgcgaccataaggatgcttagaatggtaaacaggtgagaatacataagggtttgcgttttaagaaaaccctgacgttgaatcataattgaaaacaccttgcaaagccgactcatcagttgttctgtaatggcgttaagcattttctggaatttttcttggttttcgggtgtgattttatattcatgtagaaagtgtttcacacctgaggagaagaatctttcctccttcgagagcccatctttgatgatgggaagttccttgatcagggcaaaccattcctcctcttgggcttgcggattctgaagatactgatggcagatatggtttagaatggtgcacacgtagctaataagctctgagctgattctttggttggttttcaaatgttggcgaaagtagtttttcaccgaagtgcatgtaataaacgtcttcattttcttataatatacaacagtatgttgagtctttaatttaaaattacaaggagttttctaggtctttatgcgtataggtgtttctttgtcgtaaattttcaatagccgacattgtttgtgaagcagtgttctgagtagtgactgtcgtgtaaggctcagccggatgagcaggagcactcgcggccgcaggtgcggccgccggcccgccagttgccatgactagtctgtccgtaactgggttgtccgtaactggtttgtttgttgctggtctgtttgttgccggtctgcccgtgactggcttgcctacacttgctgtagtcgctccagctggtttagaggtacctggttgtggagtgacttctacccactgctgatcttgataaggatttataaactgtatatcttcctcctcaatagcagcagcttttttctttcttgaagagaatagatagattagaacgatgataatgatgactaagaccacgatagcaatgagaatagtatacatatgtgtggagaagaagcttggtgtagtgactggtgacaaacactcaccataatgccgcggataaaccggttgaaaaaattcagaatccatttaagatactattataaataatatataaaaatgttgtggcgcaatgaaattacagaatttatggaccaactttccaagtattctcaagaaatcttaaaaacgtttaagcaattgcgtcctagtgaatataaacaatacaatgaatttttaacacaagttacaccgttgctgcaaaaaacccctgaaaaaattccagagttggttgaccatatattcaattacctagacaacgttgaaaaaatttgtgagctcctcgtgaatgctagctcaattattattagttcaaaaatacgagaacaagtaaaacacggaatgagcttcagctataaagccgacctcgactccttggcggacattctctctcaaaaacagtacgtgcttatgcatctttcaaaaaatattgcggccgagtattttaatacgtgtttaaaccaagggaaatccaagttagatctcaaagctgcctctgtattttatagtagtcgttcccgaacggcaagctcagcagaactctatagaaaaatgctatacgcctatggttcaccgcaggaaattaattattatactgaaaaagcccgaaataagacgttggatgtggaggagagcgacagcatggccatcatcgaacgaacggcccgacacaacctttcccttatgcacccgctagaagccatggggcttacctttggggcaaccaacacggacgccgacccggaggatctgaaggacaaaacggtgataaatttaacgctcccgcaggcaacagaaagcatcacctaccatcttaaatccctaatgcagctaaaaaaagtaagtacggcttcaggactaaatacaaacattttgaaagcatttgataatattatttccacccctgtgaaaaaaaataaaatggcctccaagttggcgcccgggatggatgtcgtgttcactagcgataacggaaaaacattttttactaaaaacattttaagcaaaaacatgctagcggggcccaaagagcgggtgtttgcatataataatctcattagtaatttaaataactcctgtttcatacaaaatcacaacgattttttaagacagcaggactcttggcccttctatgacgcgcacaattttaccaacaagtttttaatgcagcctattttttcggggcagacccgtcctcggcttcagggagccatggaggcggcgcatgtggaaacgcatctcacggcatttttacaaagtattcagccctctaggccacaagatccctctgttttggcttcccccaagttatctgctctaatcttgaactaaaaacagcctttcttggacttaaatgatggtctaccagtttttgaaataacttagagaactatgaagattttcatgaaatttaaattagagatttgcaaaggttacttgcggtcattttctgttgaattaaataattattcgaatagtataatgtctgaagatattcgtcgtggtcctggcagaccgccaaagaaaagggttgttcccaactttgagcgcaagggcattctggaaaaaccagttcggccacaaagccgtctcgagttttcctatgataacccgctgatatttaaaaatctttttatttactttaaaaaccttaaaagtaaaaatattttggtgcgatgtacccccaccgagattacctttttttcacgtgaccagtcgcaggcaagctttgttattgccaccatcgacggaaaaaacgtgaaccattattacgccagtgatgtcttttggctaggcatcaacagagagctcgttgaaaaaatgtttaacagcattgatcgctcttttttaaaaattaccatcgttcaccgctatgacaagcctgaaaccctgttttttatctttacggattttgacattgacaaggagtgcacgtatcagattacggtctcggagcccgagctcgatatggaccttatcgaaatggaaaaaagcatcagtgaagaaagactcaagaactatcctctgcgctgggagtttacctccaagcagctcaagaaaacatttagcgacttatcaaactacaccgagctcgtgaccattgaaaaactcggcggcgatacgccgctgcacctgtatttccaaaagtttaactccatctcataccacgagatgtataaatcttccaacaagatcaacctgacctcgaccattcctaagtcgcaggtgttccagataaatgttaaaattgctcacatcaagtcgctggcctcggctatggtcaccgacaagatccgcattctgtgcgaagaaaatgggaacctaatctttcaatcggaaatggatgcccttatgttaaatacgattaccttgaacaccacgatatagttcggtaacattagatgttctaatatttagcatctaaataatacgctgtagtccggtcagggttgcgtcacagttttcccatttttttgcctcgtcggcggtggccaccgttgccctatcatttacgcccggtaagacaaagctaaaggcgttcagcggggcttggcaatgcccgcccagcgtgaaggagctcggaggattttgcgcatcccgaaatcccttagccatgttgtttaacacttcggttacgtcaatcgagtgaagggatcccttgggatccgtgaatgtaaagacgcagtttctaaagcgcatgtatgcgatggacgattcatcgggggttttgaaggtaacagtgttccccttgctgtacttaaagggggaccatccggtaaaattataccaaatgaaagcaataataattaaaataaccaacacaatagttatagacaacacaaagtctgtagtgccgcccattattaaataaaaatattttagaccgccggcttaaaatttacttattgctcatagcttaagtctattttattcatagcttaagtttattgctcatggcttaagtctattgcttatagcttaagtctattttattcatagcttaagtctattgttcatggcttaagtttgttgctcatagcttaactccattactgatagcttactgatcatgacttaaataaaaatattttgcccgcttaaaaattgtttaggtttgaaaaaataagagatggagggggcaacttatcgtcattgtgtttacccccactggaagacatcaaacggtaaataattataagaatcaaaatgattaatataagggttaaaaaaggatgattcatcacattaattaaaaacgtatttataacgctgttgcagttgaaattttggtataggtcggaaatattgcccgagcctccgtattctgcaatgttctgacatatggtgagtccggaggggcactgcttgttggtcaaaatatttctttgctccgttgttttataggcatttttatttccattacacggagcaaacgcacattcaggccatagggtgccggagttcacacaggcacaatactggctatacgcatactcatcctttgagcacaatccctgtttatcgcatatgctcccaataatattgtcatcctccgccgtttgttgatttgtatgcgagcgtaaaatagcggcccaggccttgggctcctttttttgcagctcggaaatcgaagggcctgtacagctaaagtcgacccaaatatcattgcatttcgtggaaactggcatgcaagacataattgaaataattaataagtatatatcatggcaacaaatttttttattcaacctatcaccgaagaagctgaagcatactacccaccttccgtgataacgaataaacggaaggacctgggggtagacgtatactgttgctccgacctagtgcttcaacctggactaaatattgttcgcctgcatattaaagtagcatgcgaacacatgggcaaaaaatgcggttttaaaatcatggcgagaagcagtatgtgcacccatgaacggctgctcatccttgcaaacggaattggtttaatagacccgggttatgtgggcgagctcatgctcaagatcattaatcttggcgacaccccggtccaaatatgggccaaagaatgtttggtgcagttggtggcccaaggtgaccatgtgcctgaccatatcaacatcctaaaaagaaaccaaatatttccgctgtttgcgcctaccccaagaggcgagggtagatttgggagcacgggcgaggccgggattatgagaacttaattttattttttttcttaacataatgggaggctctacaagcaaaaattcctttaaaaatacgaccaacattatcagcaattccattttcaatcagatgcaaagttgtatttccatgttggatggcaaaaattacataggcgtattcggtgatggaaatattttaaaccacgttttccaggatttaaacttatcattaaacacaagttgcgtgcaaaagcacgtaaacgaggaaaatttcattacaaatctttcgaaccaaattactcaaaatttaaaagaccaagaagttgcgttaacccaatggatggacgcaggaactcacgatcagaaaacggatatagaagaaaatataaaggtaaacttaacaaccacacttattcaaaactgcgtttcatccctgtcgggtatgaacgtgctggtggtgaaggggaatggcaacattgttgaaaacgcaactcagaagcagtcgcagcaaatcatctctaactgcttgcaggggagcaagcaggccatagacaccacaaccggcatcactaacacggtaaatcagtactcacactacacctcaaaaaacttttttgacttcattgcagacgcaatttcggctgtttttaaaaacatcatggtcgcggctgtagttatcgttctaatcatcgtagggtttatagccgtcttttactttttgcattcacggcaccgccatgaggaggaagaagaagctgaaccactcataagcaacaaggtattaaaaaatgctgccgtttcgtaataatttaattaaaagtaaaaaaaaaggtattgttatagtgatggcagattttaattctccaatccagtatttgaaagaagattcgagggaccggacctctataggttctctagaatacgatgaaaatgccgacacgatgataccgagcttcgcagcaggcttggaagagtttgaacccattcccgactatgaccctaccacatcaacttccctgtattcacaattgacccacaacatggaaaaaatcgcagaggaagaggatagtaattttctacacgatactagggagtttacttcactggtccccgatgaggcagacaataaaccggaagatgacgaagaaagcggtgcaaaacctaaaaagaaaaaacatttgtttccaaaattaagctcgcataaatcgaagtaaaaattgaagcgaaaaaaagtagaaaaaaaatgtttggagcttttgtaagccaccgtttgtggtcagatagtggttgtacgaccacctgcatcacaaacagcattgctaattatgtagccttcggcgaacaaattggatttccctttaaatcagctcaggtatttattgccggccctagaaaggctgtgataaatattcaggaagatgataaagttgagcttttaaagatgattgttaagcacaatctttgggttgttgctcatggaacctacttagatgtgccctggtcccgtaagagtgcgtttgttacacattttatacaacaagaactacttatatgcaaggaagtcggtattaaagggttagttttacacctaggcgctgtggagcctgaacttattatggaaggactaaaaaaaattaagccggttgagggggttgtcatttacctggaaaccccgcataacaaacatcatacatataaatacagtacaattgagcagatcaaagaattgtttttacggatacgaaataccaggttgaaacagattggtttatgcattgatacggctcacatctggtcttccggtgtcaacatctccagctataatgacgcggggcaatggctgcgctcgctggaaaacattcattccgtgatcccaccaagccacattatgttccacctaaatgatgccgccacagaatgcggaagcggtatagaccgacatgcaagtctttttgaaggaatgatttggaaatcatatagccataaaataaagcaaagcggtttatattgttttgttgaatacgttacgcgacaccagtgtccggctatattggagagaaacctcgggtcttccatgcaattacaaaccgctttaaccgcagaatttactacattaaaatcgttattaaaataaggatgagttttagcgaatgtcccttagttattagtgcatgcaaaaaatttctacaaaagcgtattacaatagagaatgaagcacttataaatgccttaataaccgctttagcgcagaccagcacgttgaatgatctttgtttattacctattcaaacctatttgcttagttataaaaatgcttttgagtggatacacttcgtatgtattgcaatcaccactattttggataataagtataactggaaggactgtacggtagatattaattatatttttctccatgtaacctatatttacaatattaaaaccaaggaatacctagactactgttcttaaactttattttttctatatttacgccaaagagaatatttaaagtttttttgaaaaaaataatatatgtagataaaattcagttacatgatatatgtgtaaacatgtgtggtaaacaacatatggttatgctttataagataaatgcgcataatatatgtaaacaaaatatggttatgtgttaaatgcatataaatgtattttaacgtatatcttgtgataatggatatatgcatttattaaaagaggctgtatttattataaatcttgctaaggatgccattgtcaacatatatcccatgttggacaaattgcgttgcgatccagttctttttttttgattttgtttaatgctatcctttttgaagggatggttgtccaccatatttattcgatgttcaatgaataggtctgctttttcgtaaggcagtgaaggtcgttccaagactccttgaacgatggacgtgttttcttggatccacttaaaaagcacgtggcattcaaaaacaggacagtgattggatccttggatatgctttggacagccaatgcttgaagagatgtagtcccttttctttaggacaagcttctccacgctggggcaacagagatcgttcaagttctggacggtcgcatttggaatgttgaaacttcgtatccattcaccctcgggtcctcccttatgaagaaggagtatttgctcatggtccttagtaatcttaaccaaatgttggaagatcatttttttacctgctttaaaggcctgaagggtgtcagttggcaaagctattgaattcgggagtgggctttcatcaagcgtgaaatggtgaatgtgacgcgactggaaagaaaacgaccgttgatttattttttcaaagattgggtcgattccgccatgaaagaacagctgcaagattttagaaggcgtatttttttcccaataaaaaatgaccacttctcgtgggattaaaatcgtctgtgtcccattttcattatataattggcccataaagccatcaacgtcaatcaacaccaaaagcatggtatagagagcttttagaaccggagttcgttaaaaaaatacaaagttcgtttaaaacgtgtaatgttactaaaaaaatgtaatgtttaaatgataatgataccacatgcattaatgaaaaaaacttttaaatttttgttttaatatttgcatgaaaatggaaacatttttagtctgtttatttcacaatgcagatggtttacatcaacagattcaggaaattttgtatttattgcggatgcatatttacgaaacaaatctttacttaaagcaggaactatcacggcttatatatccaaataggcaactttcttttgtgttacttatgcccctttcccttctaagaaactgggatgacattgaatatttaacggacgttgtagatgataagcagactctacattacgcggcaaatttgctgacaaactacgttctacatctatccatgtttcaaaagctgacaaaaccatacttccttttagcggtcaagcgggtcagcgaaaaactcaacaaaaagcagcgacattcattttacgaggtattggtaacctccgaaaccttgaataattatgaaaacctatctaaaaacattttaaatacgttgatgtttgccgtgcgctacgtatttaaacctacgccgaactattcagaaattctcgcagagttggaaaaaaaaaataaaattcaccatattatttttaatatggtaattacggattttgcgcaaatccgtgaacaacaaatggataaacatctgtgtgaaacaaataatgagcttcgtcaggaatgtaaagaaactatttttgatttaaaggtggtaggaaatgtttagccaataaactcatgcccgcattttttacaggtacaaaatatcgtggatggctcatcgagggcgcgtgtttgtacttctctgtaggtacacatacgctgcttgcagttgggacacttataaagttgtgacgtcttttcggcgaccttttgctgcgaacgtagagtaatttctgtcttctcctttaaggcggcagaggggcaaagctcggcgaacgtcatgctaccaattgcctccggttttagctcgccagaaattagcttattaagggcatcgttatcctgttgttggtgactttttttttcgcagttaataatatgattgatcgtcccacaacgggttgaatattcttctaaaaaggttttttcttgttgctggtacgtataatgataacacgaggcctcgattttttgcgcgtattcggtgcataaatcagtatgttccttaaaaaacatatgtttttgaagcgttctaaaaaacatcatttggatgatatcacgcatttccaaaataatatagggttctagtcttttggaatctttcataactagatcggtggtaatattcttagtcatacaatttattaaaaatggtttaatatattgtaaatattttttaggcgtgtcagcctgtaaaaaacattcttgttcaatcttatttgtaaggatagtattttgcaaatacttatttagcaaaaatacgatagaatcgcgggctatatgcattttcatataatttttttttaaaatttaatacaaaaaaaagaagtatagactcttcttctagtccggttagttcgttggttgcctcaacatggagactcagaagttgatttccatggttaaggaagccttagaaaaatatcaataccctcttactgctaaaaatattaaagtagtgatacaaaaagagcacaatgtcgtcttacctacaggatctataaatagcatactgtacagtaactcagaactttttgagaagattgataagacaaataccatttatcccccgctttggatacggaaaaactaattgtaaccagtagtacatttaaggatagtttaagcagtaaatgtagaataacacagttaagcaataaataacaagtatataggaatatataggaatatatagaaatatatagaaatagctaagcttaatactaattcagctttttttttaactaaaacctgaatagatgcgaagtagcggacatatacatactaaaataagccatacatttactttcttcttgaacatgaaacctttttttcttctgttgttggtatataaacaataggactgtttgctgaggttgtatgatcttctacaactgctgtctcaggatgacgatgtttttttaaactaaaagtgtaggatggaatgagtggaatatagttatggctcgacttatcctgtttcgtacaggaatattttttacaaatagaacgcaacaagcatatgaataaaaacagaaatgatatacaggagcataaaatagatatgaacactaaggggtagcagcttttataacgttccgtatttttcttagctatcaattgatttaccgtaatatttatctcgggaaactttgttctacaatattttgtttggtattccagaaactcatgtcctggcttattcccgcagcttaaaaaatgatacaaaaatgtgttattgttactaaaattaattcttcttaagaaaaactgcggaagacgctttaggtacgtctgttcctgttttagtaggaagtagtataagggacaatttctttttccacacattagattattgtaatataggtaggttggggtgttggagcgaataagttttctgagtatgttataatctatgacttgtaaatcgttataccttaggtccaaaaacttgagttctttaccaaagccacctgcaatttcagaaatatttttcatcccgcagcggataatacggatgtcctgaaacgtctttaaaatacttgtattgtagtgaatacttatgttatttttttgtaaataatctatgtcatgacaagtgcatgaaatgccagcagcattgcttggtatagtattatatgcaggaagaactatactactattgagaatagtcacattgtacttataccatgtattattttctgatataaagtatttgcaggtgacctgtggtttaatcctacctgttaagccacttcctaaaaaaacaaaaaatatgaaaacccttagcatcctgtatatactattaaaaatttataaaattttctgtttaaatttcatttagacaaaaaaataatatatatacatcagcaagaaattatatacagattatataattttctgatttttttttgccacaataagcatcattatatgcattaaaatctcaatactaaacactaaaatctaaattctaagcattaaattctaagcattaaattctatgcactaaactgtaagcactaaaatctaagtaactaaaatcaacactaaatgtatgcaacctaaaatgtaaagcattactcatcatcctcctcttcttcatcctcatcatcataggttaagatatatgtgtcatcctccatttcttcacattcatcttcataagcatcactgggtattggtggaacattggatgcagcatttttaaaatattctatgtcttctggtgaacactcatctaatgattttttgacagtccttttaacttccatgggatatgattccaaatcctctttatataagagtttacggtagcttttagctgcatccacatttgctggagaatctggatttggctcattgagcagtgaaattacactaagaagaatggtatcaatcttttgagccggagaccaagtcattccctgttcttcagcattgtctccgtgtaagatagagatacatagttttccatcagagtaaatattaggatgccacatttcagaggtgaatgttaatctgggtggtgcatatgggtattctggaggaaaggcgatttttgccttgaataagcctccctcataaaaagtgtcaggtgggccccttaagatcacatcccattcagtcatatccttctcattcaccgaaattttgaaattctcagagggattctctatcaggtgtctgtactctgctattaaaaacctggaaaccatggttatttaatattaattaaattccctggtttattcctccttaaaagtagatgaacctcttttgttttttattgggttcatttttactaaatttatgaactggaaaaaactttaacggcataattatcaaatgcgaagggggatccgtataaaatcctagcttgccggtaatggctattaagttaaatttggtaccagtaacactaatatttaaaaagccctgatcattaactttccacattaaaagattattatattcgaatgtttgtccaatatggacaactttgtcaccagatgttacatttgatttggttgttagtggctgaagcttggcacaatcaaaaataagcccattaacactaagatatagaggagtgggttgatctattttctcatagtttaatattccatctttccacgtaatagcttgataattatccgcagcaatgagttgaaattttataaatagtacaggggttttagttgtcgttatacatttaaagggtgttttataaaaataaaaataataattgttaaaagtatgataataatcgccaaaataatttcatacattttttataagaattatacatagtatggtatttaaaatattagctaaatttaaaaaaacttcatgatttttaaaacagggaaaaaggggattaggttgaataaaaaaggtaagcacttgtctatatattttttttacaatgttgccttgagtcgcatttttaactggctggggagtatcagagtggaatatcactgtagtaggtctataaggtcttgttaaaatatgatcggtcattgttttcgtactagtgtcatttagggtcgacctgatagctcgatataaagttataggggataacctatcaaatacagtcttatctgtgctgaaatgtatatcgtcttctttatcactaataatattaggaatggctgtcattaaataattactacttgttgttgtgggtgaaatagttgtactggtattattggaaatggctgtcattaaataattactacttgttgttgtgggtgaaatagttgtactagtattattagaaatggctgtcgttaaataattactacctattacaagtaaactaatgctaactacatttttaacctcaataaacctaaaaagccatactaaatacctaaacaacatcctgttataatatgagcagaaaaaaaaataagtataattagggaattattcttattcgcttactattaagaataattcagaatcttatttagttagaaactatcataaagtgaataggactcatcgtcggatgaagattccgtttcagagatagtttctttttcttcctcagaataatctgttcctacaatagaatcggtgtcatcctcagaaagagaagtatttaaatatggactatctatagcaatatcctcttctatctcgcaatcctcctcctccatttccatagtgtgtaggagaatatttttatcatcatgctcacttctttttttgttgaaagatgaaccgtcctcaatacggttcatgttaagttccttcatcttatgtataatttccgtaatccgtgatgtttttgacatgtaagatggttttaaggttatatccacaataacaggagaatctctatcattttcatttgataaactttgatctttgatttcttcgtctaaaattcttgtctttttttgggtactagatgaaatagaggaattcatattctgaaacgatatatcaaggggagctggacgcttttttccaattaaaccgtttttcgagatactatgattagatgaatgatctttagccaagctgtccttggatatactatagttagatattttacctttaaataatattcttctatacaagttattcttaggtaaagaattagtatggattcctatatttttatctgaaggagtgtccatatcggagaacgtcctcttacgaatattttgaccacgagccatttcatccactataggcagtattttggctggctatggttctttgttgtgacaattctatgagatttgattgcaaatcaatttttagttttaaatatattggtacctaggacaaagaaagtatatatagccaataattattccactaaattgatttccagactgatgggtatggagccatgttgtctctgcagacgatcgcaaaaatggccgtagcaacaaacacctactccaagtatcactatccaatactgaaggtctttgggctgtggtggaaaaacaatacgctaaatggccctattaaaatatgtaaccattgcaacaacataatggtaggagaatatcctatgtgttacaatcatggaatgagtctggatatagctttgattcgggcagtaaaggagcgtaatatatccttagtccagcttttcaccgaatgggggggaaatattgactatggggcactttgtgctaacactccatctatgcaaagattatgtaaaagtttgggagccaaaccaccaaagggccgaatgtatatggatgctcttatacatctttcagataccttgaatgataatgatctgattagggggtatgagatttttgatgataatagcgtgttggattgtgtcaatctcatacgactcaaaataatgcttaccttgaaggcccgtatacctctcatggaacaactagaccaaattgccttaaaacaacttctgcagcgatactggtatgccatggctgtacaacacaacttaacaatcgctatccactattttgataatcatattcctaatataaagccatttagtctgcgctgtgctttgtattttaatgatccctttaaaatccatgatgcttgcagaactgtaaatatggatcctaatgagatgatgaacattgcttgtcaacaggatttaaactttcaaagcatttactattgttatcttttaggggctgatattaatcaggctatgctaatgtctttaaagtatggtcatctttctaatatgtggttttgcatagatttgggggcggatgcctttaaagaggcaggggcgcttgctgagaaaaaaataaaagagtgttacaacacatattaggtcttaatatctttaagcgagagttgattcccccctgtaaagatcctgatccttatcaaatccaaattctgttaaaaaactacattctaaaaaatgtctcaactgtttttacatattattgccagtagccattgtttatatcagaaaataacccatttgtttatctttttttgtggggcaaccattaagacccgacgcaaaaaaagattaatcttttatcagatacctaaaacgttctataagggagtctatgagatggatcatattttgatggtcatagtaagaagcaagctttttggcgaaaacaacggagttaaagaatttaacccgctcatgtttggataggacttttaacagcgagccaaaacagtatttaaaaatttggcaatagtttttttgggatgcaataaacaaacacttgatcagtgcccgcttcactttctgatcagacatgtttgccgcataacaggcctttttaaacttagtaatataattatgttccgcaagcaccattaacaagggaacgatgggaagctgcttttcttggtgaaatttacgtaaatattcgatggccaccgcttggacgactgtgtaatttactaagttagaaatgatagctttcatggttgtaaaaatatacataggattttctttttctgtatacagtttgaaaagcttatgattacgtgaaatgatggccatttttaatacaagatggtatagtgtatctttaggtaaaaatgccttgcaagccgcgatgatgtcgatgttgtctccatgaacagcgatagaaactaatgtttccaatctaaatgtttttatctgcattaatagaagaatgcagtcaatgttattatacttaataatactgtaatacaccgaatcaatgaccgtcatctgagaatcaagctgacttattagtaaatttaacgtttttttggaggcatgacctttgatcgcggcactaagtgcacacagtatagcaaaattgttaaatacattttgatttaggagaaggagtaatattttccttcggttatagtacgcagcatctgtgatgattattggccgataaatgttaaaatgtgttaacagctttttaaaaaaacggaagtaatttttttggatcgctgtttgcatcatcgaaataatgagataatcagggtatataatgggtaggtcacatgctacctctaacaaagaatagtcgcccaatctaaaggctgtgttgaaaagcgtactatcatcatacgtatcgagtacccctgctgttacaaaccaagcgataagatgaatgtgccgttccttgcaagctatcgcaaatagggagtttcctatggaatgtcgaataatgtactccctatttttttccaaaatgtttggaaaattgtatagcgttgcggcatacagtagacactccattctggcgttataatttttacttttacatatgaataggtggaagaactcgaataattcttgagaacttgttaaatgcataatatggtgatattttggtgtcgttaaatggtatgagaaaatgcattctaatacatcttttcggttatgctttagcgcctgagctaaggcatattcaggctcgacccataggactagtgtttctataattgagatattcgcctgctttgccagggcatactttaagacgctccggttagaaaaaatgttgttatgaagatggataaccgtatccatttttacgatgggaccattccagtatagtcctaaatgctgtagcagatcttttgttagttgtgaagcgttctcgggtgtcatataaatatgttgcagggcttttttctgtaaggagaacatttcgtcgtaatcgtacaaaaaaaattaaaatttgggcatggatgattcaaacataacaaaatcaagattttataacagtttgcattaacctatacatatatgcaagtaaatgagatattatctatcataacgaatcaagggatatttgtatatatcaggagtttctgaaataaagatatgaagattatcatagtagtatccatcaatcacaatgcaacttcctttaaggcataatttagtaaactcagcactcccatcttctggatgctttacaactaacattaaaaactcctcagtcatattatctgtaataaaataagatcctcctggagccatttgtagcatgtctcttattcctacaaaatcttttttgggatggtaaaaactcagcagtttcaaactcttttttagttttttttcctggtatttaagccatttgttataaaacagttttcttatgaaaatgcatttgaaaatattgggaatgtttaaccatgcttcttccgagcacatctccagatacttactttctttgtttcccatgtctaatttattgctcactaagttagtaatgaatctattttaataatctactttactaatctatcttaataacctatcttataatctatcttaataacctaattataacctatttataattggctaatgctgccggcatttcatgcctatctaaacaactcctactaagcaatctactattacatatatagattcactttttatatttgtaaatcatgagaattataaaatcattactcatttttattgtaaattagtgggtatttgtaaaaatcttcaaacgttttaagatagttttctagagagaagtaatctttgccatcaatatataatgcttttcctttaaactccagttttgctatgtttagtgagccgtttctagatctttttgggcaataaatagattttcattggttgcatcgtccgtaagcagaaaggtaccactaggcacgttaaaaaacatacgttctatttcatggtcggatttttgagaatagaaaaaatctaattttttaatccgcgttaactcttttttatcaatctttccagactgttttatatatactttattgcaaatcttacaatcctctatggcttcattatacttattttgcttatcctctattgacatgtccgtatttgataggtaacttccgttaaggcggttccccatggttttagatagatttttaattcagttgtatacttttattatgaggctaaaatatagaagtttgatcctaaaaaaataaaaagattttgtacatttatttatggtttatagcggtatagaggccgataaaaggtatccgggtagtctcctatgatatcgtcaattttggtataataacagttgttatggtagtattgtccaaaccgagtatgtatgcgccggtgaagcgtccgcccgctaatggtacagttccaggttaagacaatcatatcacacccaaaaagagaggaaacagcataggtgcccaaaggttcattatataacatacgccgcatatattttagttttttttctccatggtaataatcacaggttttcatgtcctgcttaataggatgattccccatgtatgataatatataataaatttagtttttagctttttcaaaaaattgggcgctcgaaactaaattttccttatcacagcgtttggagaaagcgtatttaaagatatatcttcttctaacaagactgcaaaaaaaatcttaccccttatttttataatgttcatcatagcgtttgaagatatcagaaggtgccaggttttataaaaatatcctttaggatttataacgatacaagggtctataaaatatatgcgggtataatcttataaaatcatcgattttttcataatattctccgtttatacaataaagatcataacagatattgatgcgtagatgcattattcgcgtgttcgttgggcagctaaaggatatcacaacgtagttttttttaagaaaagacgaaactacataagtccctaagggttcattgaatagtaaacgccatatttgttttaaattttgttgttcaccatagtagtattcgcactttttcaagtcttttttaataagcctattccccatgtatgcttataaataaaaatttagaaatgtgctatattatttgttgatgaatcatgaacacgtcttatatgttgatatgttactttaaaaacatttgtattttcaacagacgcgttctattcttattaagaatgatgccgtctttattttaaaccttggtttaaaatttaaagaagtatttataaactataatcatgggaactttttcagtaactgcctctgcaaaaagtgacgatgctgtttgtaagtatttagaagaaccaatagatgaaaattacagaaacatattaagaaatgagcatgttaaaaaaaatttaaatgaggctctgaatcgacatattactacctataatccagtagttgattggtgtaataactattcaacattttcatctcaggatttcgatgaatataaaatttatatacatagcgatcttatggatggacgacctcgtccaaaaaaaacatggtgtgtcatcatgtaatgtttgttagttttatataaacgcaaaaatattcttctaggagatgttgatatactacctattgaattcaatatattaaagtacatttctggctattcccattacggtattattattactatttttaagagctagatgtggatttaagtaataataacattctcccgttcctcctagagacacctcatcaaattcccatcctatgcaacctttatgttgtaaacataatgattgacagcattcatcttcttttgaccaagtcgtccaaatcctaccaagatctatacgtgtttttccaaatggagattgaagatcagcagtagtggcattaaacctataaaaaccaggtgcataatcacatgaacggatcgtaggatctaatttaatatcttttatatcttgttttactgcttctagacaacttttatcagtacatgttccacgtacacagtggtgtcctttatccttacaatccgtatctgtcttacatttttttttcggcggtttatgtttcagatggtaaaaacccagtattaaaataatcacaagaataattcctataagtacttgaacaacaggataaaacattttaatattaaatatattttttaattaaatgaatagatttaatccaagtagtattaaaattttttagaaatagtgttctacaaataatgaaatgaatggtccaaaaaaaataaggtgtacaataatgtaatatattgttaggctaagtaaatttaatattttaaagtatttggaaaaatattttttaacatatgatgtctaggaatattttttagacatttaaaaccatatagttactttatttattacactgaacttgaaaagacttattacctaaaatattaatagatgaagtaatattgtgtaattgagtccataacatgggtgggaaacaaaaatctcgtaatatgaaaaataaacatcctaaaaagagtgcaattgttataagtttatgtaactttattttaaagtaagaatataaaaatatgagtacaagaggaataggggccattactaacattggctccaacatcctgttgtctacaaaaaaaaatattttttttagcaaaaaaaaatccatggaaggatattaatacacataattatttgacatcacattagtgtacttaccaaatagtaatatacaaccatcctaatattcacctttatgaaatgatcccaacctatacggtaaaatagtataggttttaataaagaaaaaagatattctgtggtttttatttttgtatagtgtgtgaatacaaaataaaatcccaaattttaaccttttcttttttttctatacaggatgttagaaatagtattggcaacgctgctaggcgacctgcagcggctccgggttcttacccctcagcagcgggcagttgccttctttcgagccaatactaaggagctagaggacttcttatgctcagatgggcagtctgaggaggtactgtctggcccccttcttaaccgtctactagaaccctcaggccctcttgatattttaaccggatatcacctatttcgtcagaatcccaaggcaggtcagttgcgcggccttgaggtcaagatgcttgaacggttatacgatgctaatatttacaatatactgtctcggctgcggcctgaaaaagttcgcaacaaggctattgagctatactgggttttccgagctatccatatttgtcatgctcctttagttttagatattgtacgatatgaggaaccggactttgctgaactggcctttatttgtgctgcttactttggtgaacctcaggtaatgtatttgctctacaaatatatgcctctgacccgcgcagttcttacggatgccatccggataagtcttgagagcaacaaccaggtagggatttgctatgcttacttgatgggaggcagcctcaagggactagtctccgccccactgcgtaaacgtctgcgcgccaaactacgctcgcagcgcaaaaagaaggacgttctttcaccccacgacttcttactgctgctccagtagctttttttgccgcaggagcaccgcggataggagctcctccacgctcgcgatccggcgctggaagcggaaccgatcgaccgccacctgctcccagggacccttgcgctcgatgtcgtcggcttcccacacctcgacggctgtggcaaaatggacatgcttcgcgtcgttcgtccgttttttgcgccgcctccccattattcttcctgtaagattagtgtttaatacctataataacataattttaagatttaatataccaaaacttaaactatttttgtatagtaactattagcatgtctacacatgattgttctctaaaagagaaaccggttgatatgaacgatatatctgagaaatcagttgtcgtggataatgcacccgagaaaccagctggagcgaatcatatacctgagaagtcggcccgcgaaatgacatcatcagaatggattgctgaatattggaaaggtataaaacgtggaaatgacgtgccatgttgttgtccaagaaaaatgaccagtgcagacaaaaagttttcagtatttggtaagggatccctaatgcgctccatccagaagaataattaaaaaaaatattttttttagcaagtttttaaactatttaaataaatgtggtaaaaaaattcacataataattaaagtgaacgtgttagaattaatatttttttataatcggatataatatccattaaatcaataaatgatagtgttgctaccacactaaacaataacaaacagaaacgcacgatacctttcctcatgatttataatagcgtgttatctaaagatttttttgaaaaaaatattaaattttagttgattatttttttcagttacaacattgctttagaaaaaatacctaattactacatagcaaataaagcgagcgcattgttacaaacaacattttttttgcgcctggatactcctatatatgagaactataatacggtatattaatcctattaccaacattgtcaataatagtatgtaggcaatgacatactttaaataccaaatatccatggttatttctaaaaatcttgaaaaaacgttaaattttagatcggtcacctacgacagtaatactaattttaataattgatgactgaaatcataatataatgccgtgcgaaaaataattatttttcggttaaagataccattacataaaaaatatgccatctactctacaagtgcttgctaaaaaggtattggccttaggggagcataaagaaaatgaacatatatctagagaatattattatcatatattaaagtgttgcggtttatggtggcatgaagctccgattatactttgttatgatgggagtgagcaaatgatgataaagactccaatctttgaagaaggcatattacttaatactgcattaatgaaagctgtacaggagaataattatgaattaataaagttgtttactgaatggggagcaaacatcaattatggattaatttccattaataccgagcatgcccgggatctatgtcgaaaattaggagctaaagaaatgcttgaaggaaatgaatttatacaaattatattcaaaacattagatgataccaccagtagtaatataattttatgtcatgaattattcaccaacaatcctcttttagagaatgtaaatatgggggaaatgaggatgataatttattggaggatgaaaaatttaacgaacctattattaaataatgactctattagtgaaatattaactaaattctggtatggtatagcagtaaaatataatcttaaggatgcgatccaatatttttaccagagattcatggacttcaacgagtggcgagtaacatgtgctctttcttttaataatgtgaatgatcttcataagatgtatataacagagaaggttcatatgaataatgacgaaatgatgaatctagcctgcagcattcaagacagaaatttatcaaccatttactattgttttctattggggggctaacatcaatcaagcaatgttaacctcagtattaaattataatatttttaacttattcttttgtatagacttaggggctgatgcctttgaagagggtaagaccctggcgaaacaaaaggggtataatgaaatagtggaaatcttatcattagatatcatttatagtccaaatactgacttctcatcaaaaatagaacctgaacatattagttctttgttaaaaaacttttatccaaaaaatctgttcgcttttgatcgttgcaaccccggtttatattattcttagaggaccgctacaaaaattattttttttcttgatcaaagctccaaaataattattagattaaagtcgcctatagcagcagcccactccaaaaaaagtattttatagtacaaaaaacacgaaaaatagtttgcggccggcggcaaactatttgttgttgtctaaaacttaatgtttttttaatatttttaaatgcaaccatggattgttggactatcagggagaagaactatagctacatcatattgtcaatactggtaatactattaatatggtatcttatacttaactattgtcgatcgaaaaaaaatgcagttacaaacaacatgccgccaccatacacggtgtcaagtagctgttctcaataatagggttgattgacgctcttcgtaataatatgttgattgacgcatcataaaatgctgtggttgattaatatgttgattgtcgcctactttattatataagtaatgatttttgtataaaatacgggtttgtgagggctttattttttcttattagaacaaagcatgcaatttaaggcctacagcaagagtaatttaacacctacaacagtaattttaaggtcagtaataatgtttaattaaggcctgaccactaaaacttaaacgattttgtaaaaaaaaatgtctactccactttctctacagactcttgttaaaaaagtgctggccacacagcacatatctaaagaacactactttattttgaaatattgtggtttatggtggcatgaagcgccgattacgatttgcattgatgaggatagccaaatattgataaaatcggcaagcttcaaagaaggcttatctttagatatcgcattaatgaaagtcgtgcaagaaaataaccatgatttaatagagttgtttaccaagtggggtgcagatatcaactctagcttagttactgttaatacggagtatacccggaacctttgtcagaaattaggcgcaaaggaagctttgaatgaaagggatattttacaaatattttataaaacacgtcatcttaaaactagcagtaatattattttatataatgaattgttttctaataatctccttttccaaaatatagagagattgagtttaatagtttataggggcttgaaaaacttatcaatcaactttatattggatgatatttcatttagcgaaatgttaactagatactggtatagtatggcgatattatataaccttactgaagccatccaatatttttatcaacgatataggcattttaaagattggcggcttatatgtgggctttcttttaacaatttgtctgaccttcatgaagtatataacttagagaagacggatatagacattgatgaaatgatgaagttgacctgtagtacgtatgatggtaattattcgactatttattattgttttatgttgggggctgacatcaatcgggcaatgttaacctcggtaataaactttcatattggtaacttgttcctttgtatagatttaggagctgatgctttcgaagacagcatggaactagcaaaacaaaagaataataatatattagtagaaatattatcatttaaaaattattatagttcaaatacctctcttttatcaataaaaacgacagatccggaaaaaattaatgccttattagatgaagaaaagtatgagtcaaaaaatatgttaatgtatgaagaattatctcattgatacaaaattattttttataacagaactctctgatggtgacaaatctccgataggaatatatgacgtaacataattatttttttcgcccagaaaaaaattataaatgttattattgccagcacttttatcaactatacgtacaaaaaggtgttgaccaaaaaaataattttttttcttgatcaaagtatgtaaacgcccgcttacagcaaggatcttaagtgagagccattaaattttattgatagctgcttgccaccagtagaatacggccaaaccacctaacaggaaatacaaggcggcccttcggccaataaggtggataaaaatcacgcataagacggttgtaacatagcactttagtgcgaatatcaggaatgccaatagcatgtagataaggcaccaaacatcgcagctatacatggctaaagatcaaccagaaaaggtttaaattttaacgccggcccaaaacttaaactttttttgatatttttaagtgcagccatggattggtccggccataggatgacctatgcctacgtggcattctcattgatggcaatagcaataatatggtatattctacttatctattgccgatcgaaaaaaaatgttgttacaagcggtaatacgctcgctttagcgccaatatcgcatatgtgaaaaatgttcgccgaaaaaaacattaaaatttagaaccgccgcggcatctcaggggcggcaacatttttttttatatggatattgtcacacaccacctcatctatgacgcaatatattactgctaatatcaggttccccaatagtatgtagagaaaccacacaagatagatattcatggcgatttttgacgaaaaaacattaagttttagcttctttgacgcctgtgtactaataatgtttaacgcctgtagtataataattgatacctacagcagtaattgatacctacggcgataatgtctctctggccgccccaaaaaaaagtatttacggtagggtttattaccggcggcgtaacaccagttatggtcaattttgtctggcccgccgcccagccgcaaaaaaaaatcaattacaaccgcaaaaaaaaatatttccggccgcggcgtttcaaaaaataatctttgcgaaataattccgcatcttgtgaaatgaacgcctacagtaataattttaatctttgacacctacagcagtagtaataattttaatctttaacgcctgcagcagtactaatattttaatctttaacgcctacagcagtagtaataattttaatgtttaacgcctacagcagtagtaat

SEQ ID NO: 2 - protein, 119 aa, African swine fever virus
MLHWGPKYWRSLHLYAIFFSDAPSWKEKYEAIQWILNFIESLPCTRCQHHAFSYLTKNPLTLNNSEDFQYWTFAFHNNVNNRLNKKIISWSEYKNIYEQSILKTIEYGKTDFIGAWSSL

SEQ ID NO: 3 - DNA, 192535 bp, African swine fever virus
gaatataccatattattgctattgccatcaatgagaatgccacgtaggcataggtcatcctatggccggaccaatccatggctgcacttaaaaatatcaaaaaagtttaagttttgggccggcgttaaaatttaaaccttttctggttgatctttagccatgtatagctgcgatgtttggtgccttatctacatgctattggcattcctgatattcgcactaaagtgctatgttacaaccgtcttatgcgtgatttttatccaccttattggccgaagggccgccttgtatttcctgttaggtggtttggccgtattctactggtggcaagcagctatcaataaaatttaatggctctcacttaagatccttgctgtaagcgggcgtttacatactttgatcaagaaaaaaattatttttggacccccccccatgttttatacaaaaatcatataataaagtggcgacaatcaacatattaatcaaccacagcattttatgatgtgttaatcaacatataccatattaatcaaccacagcattttatgatgcgtcaatcaacatattattacggagagcgtcaatcaatataatattgagaacagcgacttgataccgtgtatggtggtggcggcggcatgttgtttgtaacagcatttttcatcattcgaagcttacaaaagatatgtataagatagcatattaatgttattaacagtaatatcaataaggcgtagctatagatcttcactttggtagaccaataatccatggttgcgcttaaaaataccaaaaaaaacattaagttttggagggtaagattggtttttcaccattggtaaagattattattctaaatgtttaccccatagatgtgaaacaatgattcttcatatattaacatattttttgacttatacttttcttcatctagtaaggcgttaattttttccggatctgtcgtttttattgataaaagagaagagtctggactgtaatttttaaataataagatatttattaatatccaattattcgtttggctcgctatttccatgctctcttcgaaagcatcagctcctaaatctatacaaaggaataagttaccttcacaaaaattcattaccgaggtaatcattgcccgattaatgtcagcccccaacataaaacaataatatatagttgtataattacaatcatacatacaggccaactgcatcatttcatcaatgtctatatttgtcttctctttgttataaatttcatgaaggtcaaagacgttgttataagcaaccccacatattaaccgccaatctttaaaatgactatatcgttgataaaaatattggatggcttcagtaagcttatatagtatcgccatactataccaatacctagttagcatttcgttgaatgaaatattatccaatgtaaagttaattgataatgtatctagttcaccaaaaattcttaatttcagttgagcattatttaggaaaaggggattatcagataataattcatggcatagaataatattactgctagttttaacatactgtacattataaaatatttctaaaattttattttcactcaaagctttcctcgcacctaacttttggcataggtcctggtgcactccatattgacagtaaccaacccaaagctgatgtctgcaccccattcggtaaacagctctattaaaccatgattgttttcctgtacagccttcattaatgcaacatttaatgttaaaccatgtttaaaacttgctgtttttattaatatttgttcatctatacaagtatgataaatcgtaattggggcttcatgccaccacaaaccacaacgctctaaaatacaataatcatcttttaacacaggctgtgtagctagtacttttttagtaagtgcttgtaaagtagatggcatcttctatctgcaaaataattatttccgaaaaaaaaatcaaattaaaatactaaattctatttttttttttaataaagcctgtaaattatataataaatctcgcccaccgtattatttccggacacaactttttatacctcattatatttttagatctatagttttttaacaaggcattaattttttctggatctgtcgtttttaaagataaaagagagacgtttgaactataataatctttaaatgataatatttctactaatatatcatgattcttttgttttgctaattctaagctctcttcgaaagcattagctcctaaatctatacaaaagaacaagttattcatataaaagttttttaccgaggtaaccattgcccgattgatgtcagcccccaatacaaaacaatagtaaatggttaaaaaattgctatctctcatacaggccagatatatcatttcatcaatattcatatcaaccttttttatatgatacatttcatgaagatcagacacgttattaaaagaaagcccacatattagccgccaatctttaaaatgactatatcgttgataaaaatattggatggcttcagtaagcttacatagtatcgctatactataccaatatctagttagcatttcgttgaatgttatttcattcaatataaagttgatcgatatcttctctagaaaacaacaaattattacttttaattcctctatattctggaaaaggggattattagataacaatttatggcataaaataatattactactagttttaatacgatgtattttataaaatatttgtacaatatccatttcattcaaaatttttgcgcctaactcccggcagaaattccaagtatgctccgtattgacagtgactaagctagagttgatgtctgcaccccattcagtaaacaactctattagatcatagttgttttcctgcacagttttcattaatgcgagatttaactctaaaccatctttaaaaattgctgattttatcatcaattgattatcctcattagtagaaagcataattggagctccatgccaccacaaaccacaatatttcaaaataaagtagtgttctttagatatgtgctgtgtggccagtatttttttagcaagagcctgcagagaaattggagtagacatatttttttttgcaaaatggtttaagtttttcaagaatacagattggataaattaggttgttgacttagttacaggaggtattaaatattatgtagacataaaaatgagatcctccaaaaaaataaacaacaaaaaaaatatgtttaatattaaaatgacaatttctacattgcttattgctcttattatactacttattattattttagtagtgtttttatactataagaaacaacaaccaccgaaaaaggtctgtaaagtagataaagattgtggtagtggagagcattgtgttcgtggatcatgtagctcattgagctgcttagatgccgtaaaaatggacaaacgaaatattaagatagattctaagatttcctcatgcgaattcactcccaatttttaccgttttacggatactgctgctgatgagcagcaagaatttggaaaaacacggcatcctataaaaataactccatctccaagtgaatcccatagcccccaagaggtgtgtgaaaaatattgttcatggggaaccgatgactgtacaggttgggaatatgttggtgatgaaaaggagggaacatgttatgtatataataatccacatcacccggttcttaaatatggtaaggatcacatcatagccttacctagaaatcataaacatgcataaataaatacattaggctcatcgtatctttttaaaatccataaatattcgtttgatatatgctgaaatttttataaaaaaaataactatttcctataaatcatctagaaatagtcctcgttttgatcggtttatatcttataatattgtgcatcgatgcacaactgctttttttggtccttctggaacatcattatattttctttcattaatataccattcagatgtaaacgttgaataatttttatggcaacaatctaccattgaattatatttagtaacatctaatacatcgtttgttttatcaggctcagctctataatcttgataatttttgttatcagcttctaaagctccatcattatttttcaaagaagtatccataattatgtttggtaaaaatactttaagttttaatgtgatatttaaaatggttgttatataaatttaccgcttacaggtaatctttattcagtgtcataaactatacttttgatgattcagtattttgtgaatcagtacatttattatcattaatatttttaggctgtttttccaatgttttattgttgcaatgagcctgctcctcctttgacgaggaagtgtctgttggagtcatctgtttaggaagagtatcatccatatctattatgaagaaaatatataaatattgatatacaatcaaaaatatttttgatcacgtctttgttatctatcgatattgttgataacgtcttgaataacctacatcatttttttacataaaaaaatagatataatttttattatatctcaattattttaaagataattatcaatacagcaaatatcataagctaacatatttttcgaataatagttttttagtaaagtattaatcttttcaggattggtttcttttgataataagataggattcgctttataaatttttaaagataatatattcacaatgatagaataaccgtatatatctgctaatgtcttactgtgttcaataacattagcccctaaatccatacaaaagaacatattttcaatacaaaagttttttaccgagattaacattgctcgattagcgttggctcccaatgcaaaacagtagtaaatggtcaaaaaattattatcgcgcatacaggccagctccatcattttattaatactcatatgaattttcgttgtgttacatatttcatgaaggtcaaacacattgttgaaagaaagtgcacaaattaatcgccattcatcaaaatgcctgtattcttgacaaaaatattgaatagcttctttaagattatattttaccgctatgccataccaatatttggttagcatctcactaaatgagatctcatttaacatagaatttgttgttaaatccttcaactcccaataaatgatcatccttaaatccaccatgtttacattttgtaaaaaagggttattagaaaataattcatgacacaaaatgacattactacttgttattttacactttgtttcaaagaaaaatcgtaaaatttcacttgtctcaagctcttctttagctcccaattttcggcataggtttcgagtatgctcgttattaataaaaagtaacccataattaatatttgcaccccattcagtaaacaacatgattagatcatcattgttttccttaactgccaataccaatgcagtattaagccttataccctctttaaagcataatgtccttatcattatttgattatcatcatctatatacattgagataggagcttcatgccaccataaaccataacgctctaaaatataataatcatctttagatacgtgttgcgtggccaatgcccttttagcaagtgcttgtaaagtcgatggctgcatgtttattctgttaaaaaaaatcaaattatcgggtaaacataaggatcaacccgtagttaatatttgcagtagtattttttaacaatgaattataataaaaaaataattcattactatctattataaaacccatctttaactttaaagaagaactagatcatcttttttttgttgtgtcagaacttcttcaatttattacccacattttatctaaaaaaataaaaactacatcatatcttgtttcttcatcaaattatcataccatttatagggtgtaggttgggaacattccatcatgtggtaatcagggtatttatatattttttgatagtaacatctatttggcagatgtattgtccaacaatcatgtctaataaaatcattttcacctatgggggaatcatcttaaaaaccttattcctacagattccattttgacagtcccagcaaaagtcacaatattttccatgagtacaccaatgttcaagctctctttcgggaggaatgctgccaattttatgttttttagcttctaactctctgtacaacatcagttgggaaagcagaaagaagattaccaggagaaccattaaatatataatagtctgcaaactacgtttgcgaatgtaatttgcaactaaaacacaacccacaaggtaaaatccataagttaataacttttgccattttcgtatgacagcctcgtgccattcatggttgtgttgtgggcattctgttcggtaaacttcatgaggctttatagaagttacatagtaggtacagaattcattgtgacgaaaaacactgcagttagctatgtagtcattttcaagaatgggagaatggttttcaaagaccttattcttacagatgccatcttgacagtcccaacagaacctacaatgatttgcataggtgcaccagtattcaagctccttttcaggaggggttcttgttagatccaggagctctagctcatatgtataaagaagagttggaatggatagtaaagtaaatatttgcagaccaagcatggctacttgtgaacaagtggctgctcgtcaacaaatagctgtttatcagcaaatagctgtttatcagcaacaactaattatcagcaaatgctgcttgtgggtaagccaataaataggccatacccttgaaaggagaattcagtttgataaaaaaaataacgagttttctaataacccggtcaagcatttaataaatgaatagcatcacacgtctgcatcgtgcattctgcctggaaaatgggcccatctctaatatatttacactgacggtgaatcatacagtgttccatgggatagctatgctcctgtacaggaggcatatcttttagaactttattcttacaaagaccatcttgacaagcccagcaaaaccgacaatttttcacatattgacaccagtatctaagctcctcttccaggggattgtcggtcgaaaacccctgtagactagctaggccagctagcagcaagccgaggtaactaaagaacctcattgtagtgttatattacgaaaaaacatgttaaaatttggaaaaaaaagccctttttatagatctggaaaaaaattttcacaaatctaattaaaagccttacagatcatccttttcataaattttcattaacaattggtgggggcggttgtgaggtactggatcagaacaatccataacatggtaatgtccatttccttcaccatatgtacactggttataccagcgagaaacctcacaagatgtcaaataactgttctcaacaatcaatggcatgctcttattcaccttgttcttgcaaattccatgtgcacattcccagcaaaacttgcagttttccatgtaagtacaccagtatccaagttcttcttgtggaggattatccgttgaacgaagatgccctcctgcctgagtaggtagtcctaagacctgattggccagcaggccaagaatttccaagaagatcaccaacattgctacggctggctgaacagctggcagatagctagctaattagcaaaccaagtgactcgccctctctactcttaatatgagaatttaagattcggtccggcttttttcccatgttttacagggaaaaggtatttttagcctatgaatgtacatggttccgcacattaaaaaaaataaaagaaattatttaatattggctgttattttctttcaactagcaacaagccaggtaactaaagaacttcattgtagttttatattacggaaaaggttaaattttggacaaaaaaatcatatctaattaaaaatcctcacagatctttcttttcataaattttcattaacaattggtaggggcggttgtgaggtactggatcagaacaatccataacatggtaatgcccatttccttcaccatatgtacactggttataccagcgagaaacctcacatgttgtcaagtagctgttttcaataatcaatggcatgctattattcaccttgttcttgcaaattccatgtgcacattcccagcaaaacttgcacctttccatgtaagtgcaccagtatccaagttcttcttgtggaggattatccgttgaacgaagatgccctcctgcctgagtaggtagtcctacgacctgattggccagcaggccaagaattcccaagaagactaccaacattgctacggctggctgaacagctggcagatagctagctaattagcaaaccaagtgactcaccctctctactcttaatatgagaatttaagatccggtccgacatttttccgatattttacaagaaaaagatatttttagctacaaatacacttcatatatccctaaaaaaacaaaaatttatttaattttaactattattttctttccactctctctttaagattttgtaaggattccagggctttggttcagaacaggccattacatggtgaatcccctgtcctagatcatacatacatttatttagccagcgggaaactatacatgattgcacatactcattttcaagaattgttgtattctccaatttgccctcacaaaggccattttgacaattccagcaaaacttgcagttttctgtataagtgcaccagtattcaagttcttcttgtggaggattatccgttggatgaagttgtccagctggttgattaggtagccctaagacctggttgcaattcatggtatggtagatacccttatctaaatcatacatacatttatccagccaacgggaaaccagacatgatttcacatactcattcttgtaaattactgacccatctattttgtttatacaagtgccgtcttggcagtcccagcaaaattggcaactttccatgtaggcacaccagtattcgagttcttcctctggaggctcctctgttggacgaagttgtccaacgagctgacttgaaacctggctggccagaaggccaagaattcccaagaagatcaccaacattgctacggctggctgaacagctgactgaatagctagccaattagcaatccactgtacttttcataagatcatttaagattcggtcggcattttttcaatagtttgctaggaaaaaatttttaattttatagattcacactacttcattctcatgcttaggaaaaaaacaaactaaatcttacaatgtatctggatctaatgagaagctagaattcatcttttttcaaatcctttctgggatgttcattctttttccactccttccttgcaattttataaggattccagggctttgggtcagaacagttcatgctatggtaaatgtgctcctccacatcatatctacataggtcaccccagcgggaaacctcacaatattttacatagtcattctcaataatacttgtggagttgtttccccaaaccctgctggtacaaatcccatcttcacaatcccagcagaaccgacagctttccacataagtgcaccagtatccaagttcattctctgggggttcaaatgttagaggaagatgtccacctacccgagtagaagtggaggatgaaaccaggttgctactggccagcaggccaataattcccaggataatcaccagcattgtgctcaaccagcaacggctagcaacgactagcaactgactagcaatagctagaaatggctagcaatcagtagtagctaacgctctactctttataagaaaatttaaaattcgatcagatttttttagaattgagaatgagtaaaacgcttatattctttttctagctagaaaaaataagctagtttaagataggatttcccttactaacggtttaatttttagcaaaggtataggtaaaatacacttgtacttagctgcaaaaaaataagcttatggcgtataagccgccataagtttatttaattaaaatgttaaactctgtgataagactggaatcttaggcaggtttgatgtggagaacagcatgaaatacaagagtgcctgttacacgaataagttctctcaaaccggggatggtcatactcacatctatgaaatcctggtctaggagattcatttgatgcatgatggccgcacccacacttatgagacactgaagaactaaagggtttaattttgatctgaatggtactatataggatgatggcaatccatatcaagattagagcaatcaaaatcacctcctcaagaagcatgatgtagccttaaatcttagactgctttaaaccttaggccctcactatctttaatgaaggagtttaaattttgatccctttttcaagacccatttagaagaaaaaataaagtttatatcaatctaattcataagtcatctctttcataaatcttcatgtattctctatgtggataagtatgggatgttggatttgcgcagtccatttgatgatctgtatggtttttgggtccttcataataactacatataccattccagcgggaaaccgtgcaatttataatccagtcattttgatgaataactggccaatctgtttgaatcctgtttcggcagataccgtggacgcattcccagcaaaagtcacattggtttgcgtaagtgcaccaataaactagctcatgttcaggaggataacgggttggtagtaaatcttctaatttacgtataggagcggcttgaaggacaaccacccccagtagtactagaatcagtacctttatagtggccaccctacactagacctctaagttgaagacaaagaactaaaatttagagccgtttaattactactaataattatattttttattgtctacaataggattctattaaaaaataatgatttttaccaagaaatatttttataaaaaattaatatattttgtaataaactttatttccaatgactgttaaaataaggaaactatccttagttagtcgaggaagatggttaggttatttcgcaatccgataaaatgtttattttatcgtaggtctcgtaaaatccaggaaaaaaaattacggaagagtttaaaaaagctaaatttttaccaccctccagaagattgttgtcaaatatatcgtttgctagaaaatgttcctggaggaacttactttattacagaaaatatgacgaatgatttaattatggtcgtaaaggattcggtggataaaaaaattaaaagcattaaattatatcttcatggaagttatattaagattcatcagcactattatattaatatttatatgtatcttatgagatatacccaaatttataaatatcccttaatttgttttaacaaatattataacatctaagtaaatattcttggaatggattttcttatagaatggttacaggatatgtcagcgacaggcttaataacaaatttgttaatatttttttgttaaataaatgaacaggccaccatttaatattacccgttgcaaaataagaaaaaaaaacaaacttatagttacaaatcatcttgattaatcacatgtcgttttaactcaatgaaccattctaaatctttgggttgtgaacaattcatgttatgttgatagtgtatcctaaagtgagcttcatacatacaccggtcatgccaccgggaaactgtacaattaacaatataatcattttgcgtaataatagggtggtcactaaacactttatttttacacattccatctttacaggtccagcagaagtcacagtgttttgcataggtgcaccagaacttgagatccctttcaggaggcctacgcatttgcatcggattatctgtggaaagaggtaggttcattattatgttcgtcatcaaaattcctaaaagaacatagaagccaagaaagataagcagtcttgtagcggcttgcattcgcattcgtgagtattgtttgcgaacatagcttatgagagcaatggtagctatcatacaaagacaagtatgtttgatattctcagtgtcaatgaccctatcctcctttatttgcattaactcatcaaaccaatcataatatgtgggatttgtacagctcatgatgtgaaagcggcgtatcctagagtctgtaaagtagctacatctttcattatagcgagaaaccctacatatttgtatgtaatcattttttttgatgagagggtgtttttcaaaaaccttatttttacaaaccccgtgtcgacaattccagcagaagtcacacgattttgcataggtgcaccaatactcaagctctctctttggaggtctccgggtcattggtaactctcctgttcctggaaaagattggctttgaatgaccggctgcatgaccgccagtaccaaaaggaacacaatcaccttcatggctgcaacttataagttgcaacttatgggttgcaatactgcaacgtataggttgcaccttatagatcgcgactcaaaaggtatgaaaaccttaccctcaatacagaatttaagttttaatcctgataatgtatctgtttatgaaaaaaaattttttttactcatgtatgaattcttatacgaatcataatatgtaggctgagaataataattcatatacggtgttgcgggctcaataaaaattttgttaccacaaaaaataaatgctggatttttaagatatatatctattaatgactaaaccctttatacgctgtaggctgaaaacaatccatataatgaatatacggtgatttgggtttaataaaatacatacaacggtcaaaatagcgggcaatactacattgactaatataatcattttgtttaataagaggcatatcatcccacactttatttttacaaataccgttcctacattcccagcagaaatcacagtgttttccatacgtgcaccagtattcaagctctcttataggaggcgtataagtccttggtaaattttgtttcatataaaagatggaaaggggtcgatttaaacccggctgagatagccaaatcaaaatacataaaagagcaagtagtttcatagtggtatttagatgtaaatttttatagtatgcaaatacaatgtaacctacaaatacaatactaaatacaaggtaaaaacaacaatgtcttataatgattggccaataatcaccccccccccccccatttttccatgaatatttcatttcctgtatagggtctaggatgtgaacactccatgttatgatgattaggcattttaactgatatttcataaaaacacccccaggaattgcgattaactatacagtttacaatcgaattcatcgaattagactcatttgttatcttatttttacaaatgccattttgacaatcccagcagaagtcacaattctttacatacgtacaccaatatggaagctcctccttaggaggatgctgggttcttggtaattctggtaattcatgtgcaagaatgaggactgagtagcccaacaaaagtcctagaaccttcatgttgtgtccaaatggcacctgtcattttaaaaaagatttaaattttgctaccgcaaaaaaaatccagtatgtatttttttaatacatataattattgaagtcttataagataaagccgagaacactatattttgtatagatgatgtatccggtattcaaactctcttataagtacatgtaggaaatggtcaattattcaagattggctgagataacaacaaaaccaaaatactcaaaagcataagtaatttcatggttgtactcagtcgtagatttttgcagatcgcaaatgcaacgcaaccagcaaatacaaagctaaatacaaggtaaaaacaataataccttataatgattggccaattcttatccctccatttttccatgaacatttcatgttcataaagtctaggatacgaacaacatttcatgctatgatgattaggtattttaagtgatatttcataaaaacaccacggggttgttggtgattgataggtaagaataaggatggttgaataacctagtaaaagtcctagaaaaaccttcatattgcgttcataccacagatgttatttaaaaaaaatataaattttacagtatgtgatatacacataccacaaaaatgttcttatattaactaaaatatgtgggcagagagcaattcatataatgaatatatggtattttaggctcaataaagtacatacaacgatcaataaaacgggtaatactacatttactgatgtaatcattttgaacaataagaggcatatcatccaaaaccttatttttacaaataccattcttacaatcccagcagaaatcacagtgttttccatacgtacaccaatattcaagttctctcataggaggcgtataggtccttggtaaaatttgtttcgtataaaagatggaaaggggtcgatttaaaactggctgtgctaaccaaaccaaaatactcaaaagaacgaaaagtttcatggttgtactcagacgcagattcttacaaagcgcacatacaaagcagcctgtatatgcaataccaatgatgaaatagagacagtattgctttatagataattgttgatggtcaccccccccccccccccatgtttgcatgaatatttcatttcctgtatagggtctaggatgtaaacattccatgctaaagtgattaggcattttagatgaaatttcatataaacaggattgagtcttggaatcacggaaaactctacagtttacaatagaatgattggagtcaatgaaacgagattccgttatcttatttttgcaaatgccatcttgacagtcccaacagaaatcgcattgtggtacatacgtacaccaatatgaaagctcactcttgggaggatgctgggttcttggtaagtctggtaattcatgtgcgagaatgaggactgagtagcccaacaaaagtcccagaagaaccttcatgttgcgtctaaatgacacctgcacttacaaaaaaaaatttaaattttgaatataacacaaaaaaaccaccttaaaatttcttatattatttcttggatctgccccgacgtcatacaatgtattaaaattatagaccaatcatctttttgtatataggctaatcatctttatatatagattttagatgtttgcttgttgtatcaacttaactgctagcgaagaaaatggataaaaactttctgtatttttataggttgaaatcattttatgcacatcgctaggatctaatattttattttgaagaaccgaatgtgggcttaaaatttttttcttagaaaaaagtagaatcataatattgctatgtttttgtttaatgatttcttgtatcttttttgtatacgggttggcacccaaacctatacaaaaatatacattactcaaataactaccttctatacataatcttttttccccacgtattttcctatttatttccctatttatggaattaaaggatatcaatctctctaaggcacggtcaaggtctgcgcctaaggcaaaacaataatatatacctaatttattcccagggcgtgcacaggcaagaaacatcatgacgtttagccctaaacgtatattttcctgaaaatacgcatgatgaacttcatcaatattacctaagtatatggccgtttgtaaacgccaaagatctaaatgaggaaattttttactaagataatgaataggttttgtgagattaaaatctatggcgaacttataccaaaattttaatacaagtgtatttctcgtcatttcttcttctttttcatctaaatataagataaaacgattgtaaacaaagtctatcaataggtgaaaatcattgctattaaagctgtcgagaatcaaaatattgtcataataaatttcgatcgccagtaaaaccttttttcgtttgacgagataaacaaacatattatacaaccctacatctaaaaattctggattggctcctagttggatacacaggtctttagtctgcttcgttttggcacacatgatgccaaaattaatatcagcaccccataaaacaaataacttgattagatcagtctggttttccttcacagcttttactaaggctctgtcaagctcatagctgtcgacatcagagcatgacatagagccaccggttaccattttacattgcttacaaaaacctatgggtccgttttcccaccatagtccaagctgttgtagaataaaaatatcatcctcatgataatttgaaaaagccttggtttctatcaagactttttttgtaagaacctgtaaagagttcatcgtattattatgaataacaggagtaaacgtaatcaattataaaagtgattttttcgaaaaaaactttagatggttgaaaatgataatgtacatgttcatacaaaaaatagatgcagtgatgtctaaaatcaaaatttaattttctatgtaaaaagtacagacttacttatttgggttaaattgtttattttaaactttaattaaccgtttgagttagcgatgtttgatttatcttccatactcatccggggggggggggtccttatagctctgacattattgtggattattgaatataatgaatacttcatagatgctaaacattttaatagtagttctgaggcttaattgtactctataaatttataaaaactttttgatcaaaatttaatttcttataaaaagagtacagacgtcgcttgtttaagcttcatcatgtttcattcattactttctacaattacggggggggggagtcccctcatagctttagtattgctatggtttactaattattatgtagaatttatagaagcatatgtacctgaaagtatacctactctataaaattaaataatttcagtatattttttttatgaatagaacggaaatgatataaaaataatttaatattgcaaaaaaaattcataatgttggtatgtattataaacataatagcatgtgtaatttataaactgactcctctatataattattagatgaggtaccaacctacttatgatatgccgatgatagatattgtatactataaaacaaaattattttaaatgtattcatggatacattataacatttttaccgcaaattgtctctcagcgaagaaaatgaatgaaacgtttctgtatattcataggttgaaattattttacgcacttcactaggttctaatattttcttatgaagtattgaatgggggcttaaaagtcctttcttaaaaagaagtttcatcataacattcttttcttgtctaagaagagtttcttgtattttttttgtataaggattggcacccaaacttatacaaaaatgtacattactccaaataccataatttgaaaagaaagttatttccctatttacttcatgattaatgaaacctatcaacgtctctaaggccgtattgatatttgcgcctaaggcaaaacaatagtatatacccaatttattttgagggtacatacaagcaagcgacatcatgtcatttggatctaaacgtatattttcctgaaaatatgcatgatggatttcatcaacattacctaagtatacagccgtttttaaacgccaataatctaggtgaggaaatttcttactaagaaaacgaataggttttataagattaaactctatggcgatcttaaaccaaaattttaatacatatgtattttttatcattttttctttttcatctaaatttaagataaaacgattgtaaataaagtctatcaacacgtaaaaatcatggctatcaaaactgtcgagaatcgaaatattgtcataataaatatctatagctaataagaccttttgttgtttaattagatcaacaaacatattatacaaccctacatctaaaaattttggatcagctcctagttgaatacacagaactttcgtcctttccgtcttggcacatatgatgccataattaatgttggcaccccataaaacaaataacttgattagatcagtctggtttttcttcacagccctcaccaaggctctgtcaagctcatagctgtcaacatcagaacatgacatagagccactggttaccattttacattgtttacaaaaacctatgggtccgttttcccaccataatccaagctgctgtaaaataaaaatatcatcctcatgataatttgaaaaagccttgttttctatcaagactttttttgtaagaacctgtaaagaattcatcgtattatcatgaatgaaagcagtaaatgtaatcaattataaaattgacttattgaagagaaatgttaaatgagtgaaatcggtgtttatgatgatgtacatgatcatacgaagaaacacgttcactggtgtccatgatcaaaatttaatgttttacgtaaaaagtacagatgttaactgtttagtttaaacataaatttaacctttagtttaaaccctagttaatgatgtttaatatttcttctatactcattcagggaagtgtaatgattctaatactgttgttatggattattaatgaaaactttacagatgctggagggaataattttaatcatactgttttaatgtagctatataagctttcatcaaaatttaattttttttataaaaatacacgaattaaactaaagtctaaactttagtttgactatttgagttaatgatgcttaacttatcttccatgcttatcaagggggggtcctaatagttttgatactattgttgtggattgttgaatataataaatactttatagatgctgaaatgtttgaaaataatagtacatcaatgttgtaagtttgatcaaaatttaatttctcataaaaaaggtacacatcaacattgctcatttaagtttcatgatgtttgattcattacttcctacaattactgggggggggggggggtctttaatagctttagcattgttatggtttgctgactattatgtagaattcatagaagcacgtttagatagtaatatcactgcagtgtagattatgaaatacatactaaactaatttcagtatattttttttgttcatataagttaaggtacaaaaatgattaaacattgcaaaaaaagaaaatcacaatgctattatacatagtgatcatagtggcttgtatcatttctaaactagttccaaatgaatattgggcaatacatctattttttatcattatgatttttatggtatatatgtatgaaaagttagatatacatcaaaaatctcagttctggaattataccatgtcaggcttatctggacataacgtacaggtaacatgtaagtgttactaaatactatgaagtatctattttttttgttgtaaaaaaaagaacttgatagtattttttaaaaaataaaataattaattgtacgtcaacttccttattttattctttaaaaataactcgtaagtattatttatctattttttgaaaaaatagatgtaatcggtttcatcatttaggtgtgtatttctttttagcatctatcaagaattcattgtttagtgatatgaaaacaatgaatgatcattatcttctatttaacaaccacctaaataaatgaacgtctttttcatcttaactgattaccaaaagttattttgcgaaaaggcatacatatgatcaatatcagacctacaatgaatatttccataatatccctttattgtaataattctatttttgcattccgatatctcatcatctgtgctattatatgtttccataactgtttcatcatcaaacataaatcctgttaaataggcaaaagactttaatcccggatagatttttaccattttcctgagagccgtgtatagcttgtaataaatggccaaaaatatgcaataaagcgtagaaagagagtaatttttggcataaaagattttgaaggtttgatgaatggctaaatcgcatataatataagatacgattttaaagcgcacctgttcacgcagatttgttgaaaaattcgtggaaagatttaacaaataaaaggttattaatagttgctcatcattccccttatacgacatcgtcagacgctctaatattttactactaggcacatctgccacatgttgaacatttaaagcctgttcttcttctgtgttacggcaaaagagccgtgcgtattcaggtgaagctccccaggataacaacgtccttgctacggctaaattttttttgacgatgacttttatcagaaataagtctttatttttgcattgatcactatgcgaatttgtatagttgacgccgttgcattgagtacattgatataatgttttacaattccagcgtagccctaaatggtataaaagaactgtattttcgacataagcatgctgattaacgatgtttttgagacaacacgtcgttaaggacaccatattgtctccaatttgttagataaaagtctttactaaaaaaatagatttttagttttaacaatcgagattttattatttggatgcatcatcaaaaagatttataagtataagaggttgtataagaaaaaaatgatgttatactatttatgttaaaatttaatttatcatataaaaagtacagatttaatcagttggttaaactatttagttaattaaactaaatagtttaaccatttagtcagactacttggttagcaatgtttgagctttcttccattcttatccgggggggggggtcctaatcgttctaatactattgtggatagttgaatataatgaagactttatagatgctataatgatgaattctagtatgcctgtataaaataattaacctttttgatcaaaatttaatttttttataaaaagctacagagtagtgttttattaaacgtggcttatttaaaagttacacaatgttaaaatctctacttactttaattctttgtggggttttattaactttatccatattatggcttactacttaccatgtagaacttatagaggcaatagatgatttctacgactgaaatatagaatagtccattttctatttgtaaaataatgatttatattctttcctaaaaatgatactttatatggtttgaaaacaaatattaacaacttgatttttttttctataaataaactataaatgaaaatagtaaaactcatagagtcttataagtgaacatcttcataatgttactcaaacgttggactattaaaaaatattccgtgtgcattattgcttttaatcagtatgattactttatacgaagccgctattaaaacgcttatcacacaccgaaaacaaattttaaaacaccccgatagccgtgaaattttactagctttggggttgtactgggataaaactcatattcttgttaaatgtcgtgaatgtgggaatatgagtcttaccggaaaacacagtacaaaatgtattaacattaattgtctacttattcttgccataaaaaaaagaataagcgtattgttgataccttgataggaatgggcgcggatgtaacatatatacatcttttaaagaataagataaaactgtcatacaaccagctgtctatgcttaaaagcaactcgcagatttcattgaaggagcttcatgctatatgctatcttttatatggtcggcttcccaaaaaaattaaacaagggatgcgactgtgtaaaacaatggcgggactatgtggtgaacttttatgtgcatttttagctccgtaaatgataatatgtatttaaaacaaacagatattaccaaaatatattctatgtacataatatctgggaaattatttttttttctcatacccttaaatataaaaatattgggtttcttcactaaactttagaggtaaaaatttttctttgttttgcaccatcatgtatgggtttaggctgtcccagggattgtttatttgaatatttcctaaataggaacacaacgccatgatcatatatctttcattctggtaagctttttgatacatcttcaaagatgccgtacctccgagtgtgtaacagcaaacaaacgtccgtacttttccatgggtcgcagcccattccattccgtagctcagcatcttttgctgtatttttttattcgctttataaaaaaagtttttcatccattccacgttctcataaaaacaggcacttaaaaagagcactaggggtagtgtagtcttattatagaatgtaggaatgtatgttttagttatttttttcaacgcgtgttccatactatgttttaccgccataaaaatacaaaaccaataccaactttttctataaaaggttttgctgtacacatataaacgagcaaaatatatttcaaactctatattctttttataaaaaaactcgagacagtcgtttatgttacgactttttctaaatacctcaaaaacagtaattaattcactgtcgctgtggaaatgttcgtaagctaactgtttaatgtctttaggggtcaattctttttttgggagcagtggtttgagattcggcaaaggtcgtctaaagtagtgagcgaacttttcattcgctccccaacacaaaagccgataagccagcatgtagttatcacgttttaccgcgtaaataagcaaatagtttatattgatacatgtaccatgttgctgcccgtttggacatatgttgccgcattctgaacacttatgaatgagatcatagttcttacaacataaccccaaacgggttagtacttctttgtcacgttttaaaaactcgacatgattctttaatgttaatgctttgagcgcaatgttaaataaactctgcattttattaaaatgaggttagtatcatgttttagtataaaatttagcggctgtttacataatgctaaataaacttaacgttcctactaaaccaaaaaaaatcaaattgactaagtcatagagaatttgacgatgttggtaggtaattttttaacatggtatatatttttttagggtcggttatattaggtaataaaagaggacgtgccgttaaagtattttgcttaagatcctttagatccttacaaaaatatagattgttcgtctgatgatgccactgtgttgcagtgatggcttgatcaatatcacctcccaagacaaaacagtagtatatcgttaaaaagttgtaatctttcatacaagccaactgcatcattttatcgatgtccatatgaacgatcttttgctcgtatatttcatgaaggtcaaatacattgttgaagtaaatggcgcacatgagtcgccacatactaaggtgcccatatgtttgatagaaaaaggagatagctcttttaagcttatattttactgctatggcatagcagtatttaacgaatacgttcatgggtacattatctaagatataaaatatgaaaaactttaactctcgatgaatctcttcccccatttcctgtacatttagagcttccaacataggatttttatcaaatatttcatgacataaaataatgttattgctcgttttatgacgcattaaaccggtgaaaatttccttattatttaaactatctttagctcctaactttcgacacagctcctgagtttgttccgtcctagcacaggtcagcccataataaatgtttgctccccactcggtgaacagccttattacgtcatagttattttcttttatggccatgattaatgccacatcaagatgaagaagttcccccttaaagggggttgagcttaaaataacgtaattacagtagtgacataagctaatgggcttgttttgccaccataagccacaatattttaaaatataatgatactcctcaggcacgctctgtttggccacagcctttttggccagggtttgcaaggagagcatgataacttcttgaaaaaaaaactcaaattaagttcctacttttttaaaatattagtatggacagatctaccatcatatgaaggaattctttcatcgttaaacactgaagagataatactttcatcgtatagagaatatcatgtcaatccatatattgaatgttatatatcattaaacccatcattaatatagtgtttatgtgctatggacaggttttttgaatgataatcttttaacatacgttttataacttcgggatcagtttcttttaaagataaagaatcattcatgttataacaatttaatgataacatgctggcaatgaacgagttgtctttttgatgcgctagagtctttccctcctcaaaggcattggcgcctaagtctatacaaaagaatatgtttccgatattatagaactgaatagaatgaaacatggcctgattgatatcagcccctaagacgacgcaacagtaataaatcgttaaatagttatagttcttgcgacaggcccactttagcatttcattcatgtctatgcgaatcctctccttttcgtacacttcgtgaagttcaaacacattattgtaaaaaagggcgcacataagccgccaccgatgtagatgagcatatctctgataaaaatagcaaatcgcctccttaaggttacattctattgccatcgcgtaccaatatttagtaaacatctcgcttaatatatcggtttctaccattaatccctccagttgttcataaatcattccctttacttcaaaacgatttatggtatctaaaatgggattattagaaaatacctcatggcagaaaatgatgttactgctagttagatcacgtttcaatgtgtaaaaaaatcgtaaaatttcctggtcatttaactgttctttggcacctagctgcctgcacaggtctcgggtgtgctccgtgttgacagaaagcaaaccgtagttgatgtttgcaccccactcggtgaacaattctattagatcgtgattgttttcctccacagctttcaccaaggccgcgttaagatttgtgccgttcttaaaatacggcgtccatattttcttttgatgatacatgatagggccattatgccaccatagaccgcagcacttcaaaaaatgaggatggcatttggccggatactggctggccagcacctttttggtgagagtctgcagagagaggaccatatttcttttttttgaaaaaatcaaattaaaaaaatcatgcttgtttagcatacatgtaatattgttataattacgttataattacgttataattacgttataactatattataacaatggtataacaatggtataacaatgttataacaatgttataacgatgtatcattgatgtcatcattcaactaggccaacatactttttaatttatagttttttaatagatgatatattttgttaggatctgcttcttttaacgttaatagcgaggagtctgcactataaatgtctaatgataaatgatgagatatcaaatagtaattccgttgctctgctagggcctttgcctcttcaaaggcgtcggctcccagatctatacaaaagaacaagttatccatattataaaatcgtacgcaggcaagcatagctgaattaatattagctcctaagagaaaacaataatatatggttaaaaaattgttatcttttgtgcaggccatccgcatcatttcatccacgtccatgcggatcttttccttttcatacaaattatgtaggtcaaacagcttattaaaacaaagagcacagattaaccaccacgtatttagatacttaaaatgttggtaaacataagaaatggcctccctaagattatcctgcaatgccactataaaacagtatatcgttaacatatcaccatccgacatattacttaatatgtcggtgtcttctactaaccttttcaacttccaatatatggatgaccttatttcccttataatgacataggctggaaagggattatcattaaaaagtttaagacataagataatattactgctagtagtgccagggtgtattaatttaaagaacatgtgcataatcttctttttatccacgcggtacttggctcctaattcccagcaaaattctcgaacaggcggcgtattggcgcaaattaacccatagttgatgtctgcgccccattctgtaaacagttttattaactgatagttgttttcctttgtagccaacattagtgccgtattaaggtccaagccgtctgcaaagcttggcagctttatcagcatatgtttgcaatcaagggaaattggggccttataccaccatagtccgcagcgttctaagataacatggtactcaatagatacttgctgtctggctagtacctttttggcgaaggattgtaaggaaggaaacatcctgtttctttttttttaaaaatcaattatctttgttcataatcaagaaaaatccccatatttattgagtgataattttttaacatgcaatttattttttcagggtccgtaacgatcgacaacagagaaataaccggattgtaatgctttaatgataaggcatgggctatcagataattttccttttgttctgccaaagctttgccctcctcaaaggcatcggcacccaggtctatacaaaagaacaggtttccaagattatagttttgtatggaaacaagcatggcttgattgatgttggctcccatgataaaacagtagtaaatggccgaatagctataatcttggatgcaggctatgtgcatcatttcatcaatatccatgcggaccctttctatttcgtacagctcgtgaaggtcgaacacgttgttgtaaaaaagggcgcacatgagccgccacctatgtagacgcgggtatttctggtaaaagtagcggatagcatctttgaggtcatagtccaccgctatcgcgtaccagtatttggttaaaacagtgctaaagctatcatcatggtccagcatgaaggttatctccatgagccctcttaactcccacatgatttcccccctcagatccagattatctataatccttaaattggggttattggaaaacacctcgtggcaaaagataatattgctactggttttatcgcgcgttgtatcaaagaaaatttttaaaatatactctctttctaaatattctttggctcccagctctttgcacagatcacgggtattttccgtgagagcacaaatcattccatagttaatatctgcaccccattcagtaaacagctttatcaagtcatgattattctccttcacggctttcatcagtcctatgtttaactcgataccttgactaaaacaggttgaccttataaataatttattgcgtcgaatatgaagcataatggggccattatgccaccacaggccacaacacttcaggacatgatattgatctaccggtatacactgcccggccagtactttcttcgtgagggattgcagggaaggcaacatgcctttccatcctttgacggaaatcaaattatctactaataactatcagtgtttatattaagtatttagatattatcccgggctggatacgtagtatcgctattcacatgtacttccaactctagccggagcctgcagggtcatttatttttaatattgattcttttttgtatttaatcatttagagaaggtcatcataggagccagatgttctctctccagaacttatgtcgaaaaacattacctaaccgtaaacttcctgaattttttgacgaatatatattacaactgctgggattatactgggaaaaccatggaactattcaacgagcaggaaacaactgtgtgcttatacagcaacataccctcattcccgtaaatgaagccctgagaacagcagcatctgaagaaaattatgagatcgtgagccttttattagcgtgggaggggaacctttactatgctattataggggctctagagggcaaccgccacgacttaattcgtaaatatgatgaccaaatcaaggaccatcatgaaattctgccattcattgacgatccagtcatatttcacaaatgccatatcatgcggcaatgcttttttgattgtattttatatcaagctgtaaaatatagtaagtttcgcgttcttctttactttaaacatagattagaggatgatttgcccttcactcatttacttattgaaaaggcatgtaaagatcataattatgaagttattaaatggatatatgaaaacctacatatctacaatatgatagatacctttgaatgtgctattgcccataaggatctacatctatattgtttggggtatagatttatatataacagaatcgtacccgataagtatcatcatttagatattcgcatgctttcaagcctacaactcctacataaggtggcagccaaaggatacttagattttatcctagaaaccttaaagtatgatcataataaagataatataaatattattctaacacaagctgcaacctataaccatagaaaaattttaatctatttcattcctcaatcaacccacgcacagatagaacaatgtttactagtggcgataaaagcaaaatcttccaggaaaaccttgaacttactactgtctcacctaaacctttccatcaacctcatcaaaaaaataagccattatgttgccacttacaattcaacaaatataataggcattctgagtatgcggcggaaaaagaagatatatttagatatcatattgacaaaatttgtaaaaaaagctatttttaataagtttgtcgttcgatgtatggatacattttctataaacccggaaagaatccttaaaatagccgcgcgaataaataggatgatgttagtgaaaaaaatatctgaacatgtttggaaaaatcatgcggttagacttaaataccttaaacatgcggtacacacgatgaagcataaagatgggaaaaatagactcatgaactttatctatgatcgctgttattaccatatgcaaggggaagaaatctttagcctcgcaagattttatgcaatccatcatgcaccaaagttgtttgacgttttttatgattgttgtatcctagatacgatacgattcaaaagccttcttttagattgttcacatatcataggtaaaaacgctcatgatgctaccaatatcaacatcgtgaacaagtatatcggcaacctgtttgttatgggagttcttagcaaaaaagaaatcttacaggactatccatccatttattctaaacaatacatgccttagtttattttttttgcggccgaaacattattcttaccctagaaaacgcttatagtcatcttaaatcataggtaaggaagatcatcatattttttgaaacgtaattttttaacgcatgatctatgatttcagggtccgtgcttttaggcaacggggtggtggccggactataaatctttagggataaaatgttctttataagctcatacccttcccctaaagctgtagtaccctcttcgaaaacatcagcccccagatctatacaaaagaacatgttttctatattatagtactgtattgagctaagcatggcttgattgatgttggcgcccaggacatagcagtagtacatggttgaaaggttgtggtctttgatgcaggcgatccgcatcatctcttctatgtccatatggatcttgtccttttcatacgcctcatgaaggtcaaacacattattaaaacaaagagcacatgttaaccgccacgtattcaggtgtgtatatttttggtaaaaatactgtatggcctctttcaggttatagcgtatggctatagcgtaccagtatttgagtagtaatgtactgagcgaaaactcattatttagcagatcggtttttactattaactcccttaactcccagaaaatttctatcctcatttttatattatttactttttgtaatatcggattgttggaaaacacctcatggcataaaataatgttactactagttttatgaaactttagatctataaaaatttgtaaaatttcttcttcattcaaggtttccttggcacctagctctcgacagaggtcccaggtgtgctccgtgttgacagataccagcccgtagttgatgtccgccccccactctgcaaacagttttataaggttgtagttgttttcccttacagccttcactaacgccgtatttaggtttaagccctctttaatacctgctgattttatgagccttaggttatgatcaaacgtgatcggagcatcatgccaccataggtcataacactttaaaagataatgttggttcgtgggcacgcattgtccagccaacacctttttggtcagagattgcagggaaggcaacatgtctcttcatcttttaaaaaaaaatcaaattaattagccgaataaatttttctttcgagggctttttaaaagagctctttaagagctctttaagagctttttaagagattaaaaaattattcttgctggcattctgccaagtatgcggcattcctatcatctatagtatattatgagaatattcccaaatgatggataagttttttgatttataatcttttaataaactgcttatttcttcggggtcctttaagtttagtggcaaggaagcatctgagctgtaaatatccaaagccaaactatggctcagaaaattataacctttttgttccgctatggcacgaccctcttcaaaggcattaccacccaaatctatacagaaaaatatattaccgatgttataatattgtactgaagtaagcatagcttggttgatgttgccccccagcgcgtaacagtaatatattgttaatggattgttatccttggtagaagccagacatatcatgtcatggacgtctatttggatgttttccttgtggtacatctcatgaagctcatatattttgttataatacaggagacattttaatcgccattcattaagatccgtatatttctcatctagaaaacaaatggcgtccttacaatcgtattgtactgctttggcgtaccaatacttcactagtaaaccatttaactcgtccgtttcttttatttctatgagcccccatagtcttttataaattaagccccttaattgtataacaaatttgttttctaaaataggattattcataaaaatttcatggcacaaaataatactgccgctggttttattgtgcattatcctggtaaaaatacggaaaatatcgttgtcctctagagtttctttggcgcctagctgtctacacaactctcggatgtgcttcgtattgatagaaagcaaaccatagttgatatttgcgccccactctgtaaagagctttatcagactatagttgttttccttaacagctattattaatgccacacgaaggtctatatcttctcctaaaaatcctgattttatttgtattcggccacgatccatacaaagcttgagaggagcatcatgccaccataggccacaatatttcaaaatgcagtgttcatctattgacaaacactggctggctatcgtctttttgacgagggtctgcagagagagcggcaacgacatgtttctttttcaccaaaaaaaatcaaatgttctcgtctttaaaggttaattcatgttcttaaaatgttcatttcatgatagtgattaataatatggtttaataacgctagaaggcttgtttataagacagtcataagcagtctataagacagtctataagcagtctataagacagtctatgacttagtctataactataatttctggatgggctgtaagatactcttcggctcgtttcagattttttgaagtatatgtctttagcatatcatatatttcctggggttcggttacatctaataccaaggtcacatcacggctgaaaagctgctttactaagaaaatgttgctcaagttatacatataagctttgtgcgcaatgagttgtgccctatcaaaatcggcagcccccaaatcaatacagaaaaacatgtttaaagtattattgttatagatagaaagattcatgccataatcgagactagcccccaacctatgacagtaataaatggccgcgtaatttttttcccgcaagcaagcaaatttcatcatcagattagggctgatgcaaatctctttttcacgacacaactcgtgtatgtcaaaaatgttattaaaataaaggctacaagctacccgccaatagaggtgatttttatgccttttatagaaatagtgaatagcctttgtaaaattatgtcgtaatgccagggcaaaccaaaactttgttaataggtggtgcgccgtatcccccgtcaacggaatgtttgaacaggtgtacgtaactgtgtctaaagtggttctagttacggtttccaagagtggattatgacaaaacatgtcataacccagcagaactcctgcacaggattttagcctggccacttcttttaaaatttccagaagacggggttcggatacaggcgttaagcctcccagttccgcacacagccgctttagatacacggcaggaacacgtataagcccatattcaggatttgcgccccaatccacaaataaacgtataagttcaagattatcgctcttcacggcctttactagcgccgcttcgagacaaagatcatcctcagaaaaacactgtaaatgtttatacgaaaaaacttgcttacaattgttacataggtgaataggacctaaatcccaccacaaaccaaaacgctgcaacgtataatcatagtcacttgaaagataattgcatgccacaacttttttggccaacgtttgtaaagacaacatactaagtttaaaacatcttaaatctaagctagctaactttcaagaaaaccctctatccctaagaatatatcttataactagacttatagcagtaaaaatcaactttggttattctttttaatataaaacgtctaattacttgcaaaggactataaagcccattttcctcagctagaatttttattttttaatgaagtagggggatatgttttcccttcaagacctttgccgaaagcatctttttattcttcccgatgtttttggcgagcatgtactacaacgattaggactgtattggagatgtcacggctcccttcaacgcataggagacgaccacatactcatacgacgggatctcatcctttccaccaacgaggccttaagaatggcgggagaggaaggaaacaatgaagtagtaaagctcttgttactgtggaagggaaatcttcattacgccgtcataggagccttgcagggtgatcaatatgacctgatccataagtatgaaaaccaaatcggcgactttcattttatcttaccattgattcaagacgcgaatacgtttgaaaaatgccacgctttagaacgtttttgtggtgtttcatgtctgctaaaacatgctacaaaatacaacatgctccctattctccaaaaataccaagaagagctgtctatgagagcgtatcttcacgaaaccctatttgaactagcatgcctatggcagaggtatgatgtccttaaatggatagagcaaaccatacatgtttacgacctaaagattatgtttaatattgccatctccaagagggatctgactatgtactccttaggatatattttcctttttgatagagggaacaccgaagctacgttgctaacgcaacatctcaagaagacagcggccaaagggctcctccactttgtgctagaaacgttaaaatacggcggcaacatagataccgtcctgacccaagccgtaaagtacaatcatagaaaacttttagattattttctgcgtcaactacctcgtaaacatattgaaaaacttttgttgctggccgtgcaggaaaaggcttctaaaaaaacattgaacttactgttgtcacatttaaactactccgtgaaacgcatcaaaaaactaccgcgctatgtgatagagtacgagtccaccttggtgataaagattttattaaaaaaaagagtgaacctgatagatgccatgttggaaaagatggtaagatatttttctgcgacgaaagtgaggacgatcatggatgagctttcgattagtccggaaagagtcattaagatggctatacagaaaatgagaacggatatcgtaatccatacttcttatgtttgggaggatgatctagaacgtcttactcgtcttaaaaatatggtatacaccataaagtacgaacatgggaaaaaaatgttaattaaagtcatgcacggcatatacaaaaacttattatacggcgaaagggaaaaagtcatgttttatttagccaagctctatgttgctcaaaacgcggccacccaattcagagacatttgtaaggactgttacaaactggatgtggcacggtttaaaccgcggtttaagcaactaatattagactgtttagaaattattactaaaaaatcttgctatagtatcctggaaatcttagaaaaacatattatttccctgtttactatgaaagttatgactgaagaagaaaaaaacctatgtttagaaatattatataaagtaattcattataaaacaatacaatgttaaaattcaatagatatccatcattaatattgattatattttcgaatattatcttctatggtgcaagataatcatctagcgcgtgaaacatgtcctcttctcttcaggaactttgtcgaaaaaagctgcctgactgcatacttccagagttttttgacgactatgtattgcaactgttaggactgcactggcaagatcatggttcccttcagcgtatcgagaagaaccagatacttgttcaacaggaacccatccatatcaatgaagcactcaaagtagcagcatcggaagggaactatgaaatcgtagagctgttgttgtcatgggaggcagatccccgctacgccgtcgtaggagccctagaaagcaaatactatgacctggtttacaaatactatgaccaagttaaagactgccatgatatcttgccgctgattcaaaatccggaaacattcgaaagatgtcatgagttaaacagcacctgttcactgaaatgcttattcaagcatgctgtgataaatgacatgctgccgattcttcaaaaatatacagactatctggataggtgggagtattgcagccagatgctgttcgaactggcatgtagtaaaaaaaaatatgagatggttgtgtggatagagggagttctaggcgtcggcaaagttacatctcttttcaccattgcgattagcaacagagacctacagctgtattctctgggctactcaattatccttgagaatttgtactcctgtggacaggaccccaagtttttactaaatcatttcctgcgagacgtttcaataaaagggcttctaccctttgtaatcaaaaccatagaatatggtggaagcaaggagatagccataactctggctaaaaaatatcagcataaacatattttgaaatacttcgaaacctgggaaagctaggttcagtatggtgtactcactattgtagtgaatcgtatcctgtaaattttgtaaaaaagcttaaacttttgaccacatcatattgttttagaaatctcaaaccagtgaacaacagtcttatcatacattaaaattccagtaaaatttatattttttttggtaaacaaatgttttctcttcaagacatctgtcggaaacatctttttcaacttcctgacgcttttgatgaatatatattacaagcgctaggactatactgggaaaaacacggatctcttcaacgaataagaaaggacgctgtgtttgtacagcgaaacatcgtcctttctaccaatgaggccctgagaatcgcagcctcagagggaaacgaaagggtaataaaacttctgttatcatgggagggaaattttcattatgtgatcataggagctctagagggtgaccaatatgacctaattcataagtatgatagtcaaattaaagactaccacatgattttatcattgatccaaaatgcaaatacctttgaaaagtgtcatcagttatccaatagtaatatgtggtgtcttatacagaatgctataaaatataatatgctccctattctccaaaaacacagaaatattctgacacatgagggagagaatcaggaattgtttgagatggcatgtgaggaacagaaatatgacatagttttatggataggacaaaccctaatgttaaatgagccggagtttatttttgatatcgccttcgaacggatagatttttctttattaacaatgggttatagccttctttttgataacaagatgagtagtatagacattcatgatcaagaagatcttacttcattaccaacagaacacctcgaaaaagcagccactaagggatgtttcttctttatgctagaaactttaaaacatggtggaaatgtaaatatggcagtcttatctaaagctgttgagtataatcatagaaaaattttagaccattttattcggcggcaaaaatgtttatcacgtgaagagattgaaaacctattattaaccgccataaccaattgtgcatccataaaaacgttaaacttactcttgtcttacctaaactattccgtaaaaaatatcattggaaaaatagtacaacatgtcataaaagatggtgattataccatcatattacttttaaaaaaaaagaaaataaacctagtggaacctgttttaacaggttttatagattattactatagctattgttttataaaacattttatccaagagtttgctattcgtccggaaaaactgattaaaatggccgcgcgaaaaggtaaactaaatatgattatcgaattccttaacgaaaaatatgttcataaagatgatcttggaactatatttaaatatctcaaaaccctagtatgtaccatgaaacataaaaaaggaaaagagacattaattgttcttattcataaaatatatcaagatattcatctggagactaaagaaaaatttaaattattaagattttatgtcatgcatgatgcaactatccaatttctatctatgtgcaaagactgttttaatttagccggttttaaaccatttgttttagaatgtttggatattgctattaaaaaaaattaccctgatatgatacaatatatagaaattctatcgaaatctgagtaaaatttatttttttgatcagagtaagaaaatgttctccctccaggagatctgtcgaaagaacatctactttctacctgactggctcggtgagcatgtgattcagcgactaggtctgtactgggaaaaacatggttctcttcagcgaatcggagacaactatgtacttatacaacaggacctcatcatccccatcaatgaagccctaagaatggcaggggaggaggggaatgatgaggtggtacaactcctattactatgggagggaaacattcattatgccatcataggagctttggagagtgaccattatagcctaatacgtaagctctatgaccaaatcgaagactgtcacgacatccttcccttgattcaagacccaaaactctttgaaaaatgccatgaattagataaatcttgtaacattttatgtctcgtattacacgccgtaaaaaacgatatgctttgcattcttcaagagtataaaatgcatctaagtggagaggatattcaagtggtgtttgaaacagcatgccgttcacaaaaaaacgatattgtgtcatggatgggacaaaatattgcaatatacaaccccgaagttatttttgatattgcctttgataagatgaatgtgtccttattatctatagggtatacgcttcttttcaatcatcatataaataatacgaacgaaaatattaattctttattgacacaacatcttgaatgggctgccggcatgggccttcttcattttatgctggaaactttaaagtatggcggggatgtaacgataatagtcttgtctgaggccgtaaaatatgaccacagaaagattttagattattttctccgtcgaaaaaacttgtaccaagaagatcttgaagaactattattgttggcgatacgtgcagattgttctaaaaagaccttaaacttgttattatcttacttaaactattccataaacaatatccgtaaaaaaatattacaatgtgtaaaagaatatgaaacgaccgttattataaaaattttacggaaaagaaagataaatctgatagagcccattttggcagactttataggatatcatagctatacctatatggtagattttatgcgtgagttttccatccatccggaaaaaatgatcaaaatggctgcacgagaatcgagggaggacttgatcataaaattttccaaaaaagtttgcaaagagcctaaagatagacttcactatctcaaaagcttagtgtatactatgcgacataaagaaggcaaacaactgttaatttatacaatccataacttatacaaagcttgtcatctagagagtaaagaaatgtttaatttggcacgattttatgcacggcataatgcagtgatccagttcaaatcgatttgccacgatctctccaagctcaatattaatatcaaaaacttgttgttagaatgtttaggtattgctattaaaaaaaattactttcaacttatcaaaacaatagaaacggatatgcgttatgagtaacatttttagatgagggaagattctaccaaactaactaagacctttcgctagaatgtatcttattgttaatatagatgagatatgtcattgtgaaaaaatagattaggtaggttgtgaaaaacagattaaacttaaaattatgtgtattatgtaaaattttagaaataaaaatttattttttttattgagggtacggaaaatgttctccctacaggacctctgtcggaagaacattttcttccttccaaatgattttagcaagcataccctacaatggctgggattatattggaaagagcatggatccgtccatcgagcagaaaaagacagcataatgatacagaatgaattggttctttctatcaatgatgctttacagcttgcaggagaggagggggacacagatgtagtacagctcttgttattatgggagggaaatctgcattatgccatcataggagccttgaagactgaaaaatataacctaatatgtgagtatcatagccaaattcaggactggcatattctcctacccatgattcaagatccagaaacattcgaaaaatgtcatgatttaagccttggatgtgactttatttgccttctccaacatgctgtaaaatacaacatgctttctattcttgtcaaatataaggaggatctactaaatgcaaggattaggcatcgtatccaatccctgtttgttttggcatgcgaaaatcggagaattgaaattattgattggataggccaaaatctgccaattcctgaacctgatgccatttttagcattgctgttgctacaagagatttagaactgttttccttagggtacaagattatttttgattacatgcaaagacagggaatcattcaattaaccaatggagttcgcatggttgtgctaaatcgtcacattagcatggcaatagataatggtcttttaccttttgttctggaaactttaaaacatggtgggaatatacatagagccttatcttatgcagtaacacacaatagaagaaaaattctggattatcttattcgccagaaaaatatagcccctaatacaattgaaagacttttatatctggccgtgaaaaatcaatcttccaggaaaactttgaacttgttgctatcttacataaattacaaggtgaaaaatgttaaaaagctggtagagcatgtagtaaatgagaaatccactcttgtgttaaaaattttattagaaaaaaaggaaaatctagtggatgctgttttaacaagacttgtaaaacattctacatatttccaggtgagagaatttatccaggagttttccatcagcccagaaaaattcattaaaatagctgtgcgggaaaagaaaaatgtgttaatcgaggctatttctgaagatatttgggaaaatcccacagaaagaattacttatctcaaacagatagtgcacaccataaaatatgaaagtggaaggcgatttttggtagacatcattcacagcatttaccaaagttactcactaaaacacgaagatattcttaaactggcaacattttatgtcaaacacaatgcaatcacccattttaaagacctctgcaaatatctttggctgaacagaggaacagaaagtaagaaactgtttttagagtgtttagaaattgctgatgagaaggagtttcctgatattaaaagtattgtgagtgaatatattaactacttgtttactgcaggagctattaccaaggaagaaatcatgcaagcctatgatgctttagagtagccatgtattaacattctgaaagtagaataaaatatactatatactaaaaaccaaattagccatttttaactatcttcttcttaaaaactctggataaaaatttattttttttaatttgggtagggaaaatgttctcccttcaggacctctgtcggaagaacaccttcttccttccaagtgattttagcaagcataccctgcatttgctggggttatactggaaggggcatggatctatccaaaggataaagaatgatggtgtgcttatagagcatgatcttactctttccatcaatgaagccttaattcttgcaggagaagagggaaacaatgaagtagtaaagctcttgttactatgggaaggaaatcttcattatgccatcataggagctttgaggactgagaactataacctagtatgtgagtaccatagtcaaattcaggactggcatgttctcctccctttgattcaagatccagaaacattcgaaaaatgtcatgatttaagccttgaatgtgatctttcatgccttctccaacatgctgtaaaatataacatgctttcgattcttgttaaatataaagaggatctactaaatgtactatttaggcaacaaattcaaggactatttattttagcatgtgaaaatcggaagcttgagattcttacgtggatgggtcaaaatctgccaattcctgatcctgagcctatttttagcattgctgttgtcacaaaagatttagaaatgttttccttagggtacaagattgtttttgaatacatggaaaaccaaggacttcatttaacccaggtagttcgtatggttatgctaaatcatcactttggcatggtaataaataaaggacttttaccctttgtgctggaaattttaaattatggtgggaatgtaaatagagccttatcttatgctgtcacacaaaataaaagaaagattttagaccatgttgttcgccaaaagaatataccccataaaaccattgaaagaatgttgcatctggctgtaaaaaagcatgctcccaggaaaactctgaacttgttactatcttacataaattacaaggtgaaaaatgttaaaaagttgttagaacatgtagtgaaatacaactctactcttgtgataagactcttgttagaaaaaaagaaaaacctgctggatgctactttgacaagatatgtcaaagattctacatactttcaggtgaaagaatttatgcaagacttctccatcagcccagaaaaattcattaaaatagctgtgcgggaaaagagaaatgtgttgatcaagggtatttctgaagatatttgggaaaatcccgcggaaagaatcaggaatcttaagcagatagtgtgtaccataaaatatgaaagtggaagacaattcctgataaatatcattcacaccatttaccagagttattctttgaaacctgaagaaattcttaaattggcaacattttatgtcaaacacaatgcaaccacccattttaaagatctctgcaaatatctttggctgaacagaagaacagaaagtaagaaactgtttttagagtgcttggaaattgctgataagaaggagtttcctgatattaaaagtattgtgagtgaatacattaactatttgtttactgcaggagctattaccaaggaagaaatcatgcaagcctatgctttggagtatgccatgtattaaatttctgaatcagtaagcaatagatagattttagaatatgctgtattaagttagtttctgaataagtaattaatagatagattttagtttatgtaaaaatgttaacatttgttcataagttttagataccattttagagttacttttttagatattactattttagccattattatcttaaataatcactattttagataggtccccgtattaaaaaccaaattaaccattatctatgtttttaataatactttttaaaaaccctccataaaaatttattttttttcataaaagtagagaaaatgttctccctacaggatctctgtcggaagaacctttttcttccacttgagcccttaggcaagcatgtggttcaacggctgggattatactgggaaggccatggttcagttaaacgagtgggtgattgctttatatgtgtagaccagatttggatgctatcaatccataaggctatacaaattgcagcctcggaaggaaatgagaacattgtcaagcttttcttactatggaaggggagtctacaatatgccatcataggagccttagagggcaggcaatatgatctgattcaaaaatattacaaccaaattggggactgccatcagattctaccactgattcaagatccagaaatttacgaaagatgtcatgaattaaatgttacatgtacctttcaatgcttatttcaacatgctataagagataacatgctgcccattttccaaaaatatggagaagatctgaatggaaacaggagaatggttcaacttctgtatgagatggcatgccgattacaaaattatgatatcatcaaatggataggatctaacctgcatgtttataacttggaagccatttttagcattgcttttgttagaaaggatttaactttgtattctttaggctacatgcttcttctgggtagaatgagtactgaagatagaaactttatctcaatcataacacgccatcttgaatacgcatcaaaaaagggactttttgactttgtactagaatctttgaaatatggaggtcaagtggatacagtgttgtttcaggctgtaaaatacaaccataggaaaattttggcccattttattcatgaaattccccgtgaaacggttgaaaagctgatactccatgctgtggagtcacgggcctccagaaaaacattcaacctgcttttatcttccataaactactgtgtgaacccttttgtcaaaaaactactgcacgctgtggtgaaacacaagtacatgcttatcataaagcttttgctcgagcggcccaaaaagaagataaacctggtagatgctgctctattcaaacttgtaaaatactctacttatacagaaatagtaaaatacatgggtgagttttctgtggacccaaaaagggtggtcaaaatggcagcacgactcatgagagtggacctgattaaaaagatttctaatgatgcatgggaagataaactagagagaatcaagcaccttaaacagatggtaaataccatgaaccacagaaatggaaaaaatctattgatgtacaatattcacaatattactggatatacctatctgaacaccaaagaagcatttaacttaacaagattttatgctgtccacaatgcaacatgtttgtttaaagaaatgtgtaaaagctgttttgtacatgataaaatacagctcagagaattgcttgaagattgtttacatattgctaataggcatgattatatccagattgcagaaaccgcagatgaatgtatcaaatatatagatcttattacatttaagtaaaccatgtatatatcaagtaaatccagattaaatcaggctaattgtaaatagttgtagataccatataatgaatgttttattaggatagtagttcagttaagatagtagtttagttaagatagtagtttagttaagatagtagttatgttaagatagtagttctgttaagataatagtttagttaaaactagttcatgttaagttaatagttttgttaagacaatagttcatttaagtcaatagttcagttaagtcaatagttttgttaagtcaatagtttagttaagtcaatagtttagttaagtcaatagtttagttaagtcaatagttatattaagacattagttctgctaatacattagttttgttaagataataaaaatttattttttttcatcagggtagagaaaatgttctccctacaggagctctgccggaagaacatttacattcttccttaccccttggctaagcatgtacttcaacaactagggctgtactggaagggacatggatctcttcaacgaatcggagatgaccatgtactcttacagcaggacctgatcttttccatcaacgaggccttaagaatggcaggagaggaaggaaacaatgaagtagtaaagctcttgttactatgggagggaaaccttcattatgccatcataggagctttagagggcgaccgatatgaccttatccataaatattatgatcaaattggggactgccacaagattcttcctttaatccaagacccgcaaatctttgaaaaatgccatgaattgagtaactcctgtaatattcgatgccttttagaacatgcagtaaaacacgacatgctttctattcttcaaaaacacaaggagcaaataagattacacatggcattaacccaaatactatttgaattggcgtgtcatgaacgtaaaaatgacatcattagatggatcggttattccctgcacatacaccatctagagactatttttgatgttgcattcgcccataaaaatttatccttatacgttttagggtatgaacttctcatgcacaaagtaaatacagaggctgcatatatagaattacccaatttgctatcatatcaccttcgaactgcggcggcaggaggtcttcttaactttatgttagaaacaataaagcatggtggatatctggataaaacggttttatccgcggctatcaggtacaagcataggaaaattgtggctcattttattcatcaggttccccgtaaaaccgttaaaaaactgttactctatgctgtgcaggctcgggcccccaaaaaaacactgaacctacttttatcttccttaaactactccgtgcacaccatcaccaaacaactcgtacacaatgtcgtcatctacagttccacgcttatcgtaaagcttttactcatgcggcgaaaaaacaagttaaacctagtagatgccgttttagccagacttgtaaaatattccacctatacagacattgtacaattcatgggtgagttttctgtgagcccagaaagggtgatcaaaatggctgcacgggaatccaggacctttctgattgaaatgatctccaaagctgcttggggaaatcacccacagacgttgattcatcatctcaaacaactaaccaataccatgaagcctcaatctggaaaagaccacatcatatataccatccactatatttatctaaactctaatatgctggtagcggaggaggaaaaaaatatttttaaattagcaaaattttatgcgaatcataatgcggtaaacaggtttaaacaaatttgtgaagactattatatattagatgcacgatttaaaacacttattttagaatgttttgaaattgccgtccagaaaaactatcctagaattgcaaatattgtggatgactatattcgattccttttttacaggggaaatataaccgaggaagaaattcgtgaagcctattctttaaaagatgctgaggtttatgtagatttaaaatggttacaacaaggagaaatggtttaaaccaaatccggtttaaactaaatccaatttaaactacatttggtttatcattagtcattgaaaccatcgaaaaaaaagctatttgtttatccccataaactcatcttttttttgtctcaaagtttgacactaaaattcagtgttttatagtgtttataattaagtgttttgcatgcattgcagaaattttcatcttttttaattggttcaataccacatgtcatacaatatgttgtttgattatcaagattaactttatgaaaggaaagtaagtgagccgcaaatttaaaagtaaaatatctttcatttaaaatgatcttatgaatgtattttcgataaggaggaatgaaagcatttgccaaaataaatcgcataaaaggcttggaaaaacccatatcttctaatcttttgtgggtataaaccctattttggtgttttacaaaaacttcattgttataatagtcgttatagctatcaatcatttttttaagtcctataatgcccaaggttgcacgcataaagccacagtttctgctccaaaaagcatgcacctgtaaagggtgcttttcatataaccaattacaaaatttcattccgcaacagtagcatgttatttcagtgggggatgtatagaataatccggcattcgaaaatttttcataattttttatgtcatggattgcgaagctttgatttcgtgcatctatggagctatagcctacatatttaggttttacttcaaataatcgcaaagagatgtatggatctatcgtatttattttaggaaacatttcataattttaaattcttatatataatataaaaaaaattacaaacatttgtaatgatcatcctcaattgaaggctgagttgtaggctttatttttctaattatacgaagaaggtaggttctcataaagccttcaagatgactattgatgtttccaatacattttctcaatgagttcataaacccagacattttgctaatggcttggcaaagtgccaacaagttgtccacaaagtactggtagattgccactagctatagctagctatagtgagccaacctctctgtatgtattttatatatttcattttttaatagatttaatatttttataaaaaatatttagttttttatacaagaatgtcgacaaaaaaaaagcccacaattaccaagcaagagctttactccttagtagcggcagatacccagttaaataaagcattgattgaaagaatctttacaagtcagcaaaaaataatacaaaatgctttaaagcacaatcaagaagttattataccacccggaatcaagttcaccgtcgttacggtgaaagctaaacctgctcgccagggccataatcccgccacaggagagcctattcaaattaaagctaaacctgaacataaagccgtaaagatacgagcattgaaacctgtccatgatatgttaaactaaactataaagtcatattcttctttatcgttattatcttcaatatatttttgccaatcgaaatcgaataaattcagatcctggacatttaaatacttatcatcgtacattttaatataatttaaacatgagttgttgtcaaaaacttttagcgtttttgttaaaattatcatatgaataatttccttattaagagttgccggaataatacaaaacctatttttaggtacatcatccatgataatagtaaaattagtaaaaattgtttcttgtttttcttttgtttcaaataaacgttgtaaggttaaaggtttctcgttcaatggtttctttgaagataaaaagaatgtataatctggtttaaaggtatttttggtttcaatcgtgattccatctgcttgagcatatactaaaccagaccaaatataacggtccactattacaatataatttagcttaagtagcactgcaatttctgcgataaattcactacgatgttttgtaaataatttatgtaattgttccgatgacatttctatggttttatttaacacctgcaatataagatcaccggtggtcgtgtctggattaggaaaatgtatacatatagcattataatccatgcattccaatgtttcttttaatttcattgcctgtgtgctttttcccacaccattgattccctcgatggcaatgagtattccacgcatgattaataaaaggaaaaaaagaattcagtttttaacatttcttacaaatctttttttatacaacattgtacaacactgcattagcggtatatgatgttatagcttcattaaatatttgcttttatataatctttaccaacctatatttggtagatcactgcagatggtcataaataggccataactaagataaaaattatttcagacgctactacggtagtattattaaaatcatgtgtggcaatgtatgacgtcttaatagataaaacatttaaggaaaacaaatttgaataaaaaaataattgttatgatggcgttgttacacaaagaaaagcttatagagtgcatctatcatgagctagaaaatggcgggacaatattgcttctaacaaaaaatattgttgtgtcagaaatttcatacattggcaatacttataaatattttacctttaatgacaatcatgatctgataagcaaagaagatcttaaaggagcaacatccaaaaacattgctaaaatgatttataattggattataaaaaatcctcaaaataataagatttggagtggtgagccgcgtactcaaatttattttgaaaatgatttatatcatacaaattacaatcataaatgtataaaagatttttggaatgtttcaacttcagtcggtcctcatatctttaatgatcgtagcatttggtgtactaaatgcacatccttttacccatttaccaacattatgtcgcccaatatattccaataaattagatatctttgctattaaaatagttaaaaaccttataggataattaggtactttattacgataaattatgatattttataattagttactttattataattaatctctttattaatgaattatcataagataactaattatttttttccatatatcagataataaatctgatatgggctaaaagtatgtttcaaactatttacaatagaatttctgttaagaaaacatacataatttgaataaaatttttttaaatatcaccgaaacaatcaacatggtgttaatagagtttttaacaggtttcttctatttatatggaaagagactgttttccattagtaaagtcatggacatgatatgtctagactattataccattattcctgctcctctggcgatgatgttagcggcaagactaaaaaactatgacctcatgaaacgactgcacgaatgggaaatctctattgactacgctctacttgtagtagatgatgtgccgtctattgactattgcttaagtcttggcgctagatccccgactagagcacaaaaaagagaactgctgagggacaacacgtttaatcccgtgtataagtatcttatgaactgttccggcttcccaacaaagagagaaaaaaacattccttgtgatgttcaatgcgaaagactgcaaaaaaacattataaaagaactggtatttaactgctctgtactgcttgaaatggtactgcacacagaaagagaatatgcatacgccctacactgtgctgcaaaacataaccaattgcccatcctcatgtattgttggcaacaatccacagacgcggaatctattttgttgaaaacctgctgttctgataagaacatcaattgttttaactattgtattctatatggcggcgcccaaaatttggatgctgcaatggtggaagcggcaaagcacgatgcccggatgctgataaactactgtgtcatgcttggtggaagatccttaaacgaagcaaaagaaacggctgccatgtttggacacattgaatgcgcacaacactgttttaaactgcagtcttacgtcgtggacacatcgaatacagacgacactgattaaagcgacaatcttacgtcatgaacgactgtcttttgagtatctatacttacattatatttttttatgaaaaaaatataaaggttgtatacaaacctttgtatacaagaaatttggatcattaaacaataattaatttggacacaggaaacgatctagatcgatcaaaaagctattttttttgcacacagaacatttagataattgagagattactttccatacttgttaagcttttttacacacaggaactttggattctgttcaggaagtttttcatagacattatgtttacagccagtaataataattttgggctttttcttaaaccaccggtggaaaacatccagcttgtaaagagggaaatgcatgtagagaggttttggtagtcatggttaagagatttgactaactccatgtttcctgtaaagactgcccagtcccaagcagtaaaacctctatgatagtctttttgagtcggatctgctccaaattttatgagagaaagcatatttaaagaacggccccgtattgcggccttcatcacaggagtcatcccattaaaattcggtaaacaaattctggtcccattttttccgaaatagcccaacaccccttccaggattaaatgattttttttctcagctaaataatgtaaagcagagtttccatctttatccctcctatgagggttaattatttctccaggataagattcttgttcaaaaagaaattttaaaaagtctatacgtccgtagatgcatatccacatgaataccgaggatccatttttatcgcatctattgacaatccacggatctgttttaaaaaattcctcaaatagtgtaagattcccatttctaatatgttttttaatccatttaacaaacaagttttctatctccctttctggaaacatgtgttccattttgaatgtcgcccctactccactatatgattttactcctttaatttttaatgtccttttttttcggacttctttggataagctgtttattaccatctttaaatgccttatagcggggaggagccaggcccttttcccatatgtgcggtaattcttggtgtttatgcttgcctttggcataaccaggccagtatttttcgatatattcagggtttgtttttacgtattctttaaaggtccgataggcttcttgaatacaggtaggctcaccggtataatttccatgttcatcttcctttaaaaagccattaaccctgtcctttctccacttaagattgtgctttccaaaaatgcgatcaagatcttgcgcctgctggggtggaatcataaatccctttttaggtcgaagctttttattttttccatagcttcggccatcgcgttgcgaaacagtggttaggacgcctgatagtctttccatgggcgtcgcatctaatcctatccatccaccctgatgaatatcaatggcaacaagctctcctttattttgggcaagccaagtttccaagaatgccatgctttcttcccagggataaggcccgccaacaccacgggttgtccaatcttgcaaggactccaggtccgacacctggtaaggctctaaagaagacggttccttgtttttgtactgcaaataagatttaatgacccatttataccatgtgtcgaaccgcagcgtggcgcctccaaagtgaaagccgtcgttgattttaggatatctgcaacatatttcaaccgtacgtttgagttctgcaaaagcggccttccaaggaagtctttcgctgcgggtaagacggtctattttgccctgcgtgccatagcgtatggcatgtcgtgccaattgcaacaattctgacaccgatccgtgggccccgatccagtttatcggataggcaacctccgaagggtttaaaagatgctcgtaaaagcgtggatcttcagatgccaaggcgtctgcaaaggggataatgctagaaaacctgtctagacatacgttttctgtgtttacttctaaaggtagaaaaatggttgcgtgaggcttttgaacctgcttgttcagcggtctgcatatgctttgaataatgtctctaggactatgtcgcggcgctgcaaaaaataccgcgtttagttctggaacctctacgccctcttgaaagagtcgacagtttaataaaataacgggttcctttgaggaacaaaattctgtaaatgttttgaggataacctgtcgcggcagggttgagtgagctatcagggcatagaccccttggtctaccaacgccgcgtatagctccttggcctgtttaatatcacgggtaaataccagcattttaggagccggtatattggtttttaaataggctaaggccattataatttgctttactatgatctgtttcgtggtctcctctttggtactcggttggtgggccaatttaggcgcggctaccatctgcaattcaaaatcatttacatagccggcctctatgccttctcgcagatagtagcgaaaggcaacgccgccaaaaagttcacgatttttcatggaaagcggggtgtcgtacctgggcgttgccgttaaaaaaagtcggtgcccttttttaaagttgagcaacacgtgggtaaagggccgtgtctcccattcgccgcaaatccggtgacattcatcgctaataataagatcgaaatcatccaccagtagcgtggaggattggtaggtggcaatcacaagaagagaaggggcctcccgtatccgttttgcaataaagacaggattggtggtcatttctatattgtcgtgatttagcacaatgcgggtctggtcagaccccacaagcaaaacgttcttcaaagaaattccatactgatagagtttttccagagtctgccgtagtagggacaggcccggcaccaggtacaaaacttttccttgaagataattggagaggataagataggcgacgcgagttttgccgcatcggcaggccatctgcagaatggccctcccacttcgccgcagctcctgatagcccatattggccgcctccttctgataaagtcgatcctcgattgcagtccgtgtctcatctgtagaaaaaaataatacgtcatctgcgaaatgttcatcttccacaggagttatcaccaggtgtctcagtttctccttgcttatcagcggatcagagggcaaagatggctcaaccactatcgtggaatcattcatctcataggcgggagaatcacacaaagtatagcttatgtccagacagtttgcaacatcctcagccaattgttttattttttcgggtaaaagacatacgagttctttgtttttgacgcgaaaaaactgtgcacaatataacacccctgcttcaattttttgcgcatccttctttgtagatgtttccaatgtgaaacaatacttccattcatccgtaaaacaggttgtataagatccatcatgaagcctagcggccaagtttcctgtgtgcccaactttatgtaaggattgggcctccagccagggatgaaccgccacgtaaaatcctgcgcacatgctatatcaaattgcagtttcttaataactgtacacaggatctgaaaaacatgtgattacaaaatttagataagaaatatttaatattaaaaatcacagaatacatgtcactgtgtagagagaaagccaaaaactcctcttgaccgccgtgggaaatcatccagggtagtaggttgtgtttcataaagttgtatgccgtagtgatcaccgtggactccagatggttattggcatctttgcaatactttgccatcttggcagaaaagacgataaatccacaaattctaccccagttgataagatccttaaacagctcagtcacaaccccagtaaactgggttttaatttcttgaacactcgtaagagaaaaggtaattgtaacctgtttgttcaaacactcatcataataggttaaaattttttttatttgttgttgatatgggctaagctcatgctctgaaatatcattaatgtaatatttaatatatcccactagtatttcattaatgatattatgatatattaactcttctccctccatagcggcaccctatatttttttatttaggtttcaatgttatcacaattgcgatacaattgtgatacaattgtgacacaactgtgttgtatacaacaaatgttaggccacgtatagcaacctatatgttaagaaatatttttatcccaacattagttggaaacgagcagccgcaaagaagtcatttaaaataagccatttaaagatttagaatttatatgtatacaactgtacaatggaagcagttcttaccaaactcgaccaggaggaaaaaaaggctctccaaaattttcatcgttgtgcttgggaagaaactaaaaatattataaacgattttcttgaaatccctgaggaacgatgcacctataaattcaactcatacacaaaaaaaatggagcttttatttacccctgaattccacaccgcctggcatgaagttcctgagtgcagagagttcatattaaactttttgagactcatttcgggacatcgagtggtattaaaaggccctacatttgtttttacaaaagagatcaagaatctgggcattcctagtaccatcaatgttgactttcaggccaacattgaaaatatggatgatctacagaagggaaatctcatcggcaagatgaatatcaaagaaggctaaataaaacaactaacatcaaaaaacattaaaggctatgttgtggacgatgcctttgtctcaatagtttcgaggtcatccaataactcatgtaacgtaaaaaagttggtccatttttttgaaaacattaaaagacgttcgtcttcataaataaaaaagtcattcgaaggaaaaatgatatactcaataccatagtcttgtaatattttttttaggtctctcagggtccagggatttaccaggcttctacgcgaagtgagcatcataaaaatatctaatattttttgcgccataagccagcgcggattctcattggcccacaaatcaacaataattctcttatcaaccgtgagcattcctacttgattcgaagaaatgattagatgcccagcagtccaccccatgagtagataacgcagcgttgtagaaatgtcacatatggaaggcattcctccacaacatgaacccaaattaggatgcgtgtgaaacacaaacatagcaggcttgttggccaccctgctataaatatcagcaggcatcatagcctcgctgccaaaataaatgttctctcctgccctataggggcttggaatgatttccactatctcgggtacaccgtttatcatattaatgcggccgcaccattcacggtcatcgtccaaaaattttttgatggcaccccgaacattgtcccagttaagcaacagagtattcacaatctcattacgctccgcccagtattccttaaaacttcttttagacttgctgagctgttcccaggattcgaactcagtccaatgttttttttcttttggggaagacttcccttttgaaacattttttgcggctccaccatctacactatgattttccaaaataatctccttcatcgtttgagttatatgggcattgctaagcaccttagtggtaacctgtttacctatgtgatttagcagaaaaccaagtttgtccatttgtgtctcaaccatttattcttaacaaaacaaaaaaaattaaaaatcatcgtcgtttaaaaagagtttgaaggcaaacgcatcatccttaacacagttctgatactgcgtaggtcttaactcgaaaaagttggttttttctacttcattaagaaagaatttagtcatctgaggaaaagggtttcccaccttataaatgcttttgcactgcatcatgaagcacaaattatctgtaaagtagcgtatatattgaaatagcatttcttttgaaaaaccgggaactcttcctcttgccttgtcaaaggcatagttaataaactcatccaccaactccacagcctccttcaaaattttgtgaatgatcttttcctcgggaatgttatacacgtaatttgagataagaaaacacgcaaaactacagtgcatcccttcatcacgtgagataaactcattatagcttacaagccccggcataatattctgttccttaagaaactggatcgccacaaagtggttttgaaataaaatgccttctacggcggcgaagcccaccagccgctcacctagagtgttcctgtcggggtccatccactgccgcacccactgcgccattttttttatgatagggtgtttttcaatgccgctaaagatgcgctgttgttccttctcatccgggatcagcgtttttacctgtattgagtaggcttcgctatgaacgcactcttgggcagcctgcattgtataaaagtataacacttcctttactttaatttcgcgcataaaattggttaaaaggttttcgataacaatttcgtcggcaacaacaaagaaggctaaaatttgtttataaaattcgcgctgtggctttggcatggcttcccaatcatcaatgtccttacacatgtccacctcctgcgccgtccacgtcaaactttctaattttttataccagttccaacattcggggtgctgaataggaaaaatagtgaaacgttgggaattttcaattagtaattcctccatatttgaaataaatattaacatcttcaaatttattggctgccatggagacgttttttattgagacgttggcatctgatgtgtatggaaaggcgttaaatgttgatttagatagactatcgcaggcgcaggttaaatatacccttcaagagcttatttcctactgcagcgctctaaccattttacattatgactattcaacccttgcggcgcgtctttcggtgtaccagctgcaccagtcaacggcctcctccttctcaaaggcggtgaggctgcaggccgcacaatcctgctcacgcctgtccccccagtttgtggacgtcgtttacaagtacaaagccatttttgacagctacattgactatagcagagattacaagctgtccctcctggggatagaaaccatgaaaaattcttatttgttaaaaaataaagatggggtcatcatggaacgcccgcaggatgcttatatgcgggttgccatcatgatctatgggatgggaagagtggtcaatatgaaaatgattctgctaacctatgacctgctttcccagcacgtcatcacacacgcgtcgcccaccatgttcaatgcaggcaccaaaaagccacaactctccagctgtttcctgctaaatgtaaatgataatttagaaaatttatatgatatggtcaaaacggccggcatcatttcaggcggcggcggtggaatagggctgtgcttgtcaggaatacgggcaaagaatagttttatttctggtagtggtcttaaaagtaacggcatacagaattatattgtgctgcaaaatgcttcacaatgctacgcgaaccagggaggcctacgtcccggagcctacgccgtctacttagagctgtggcaccaagacatctttacatttttacaaatgcctcgcctaaaaggacaaatggctgaacaacggcttaatgcccctaatctcaagtacggcctatgggtccccgacctattcatggaaatacttgaagaccaaatacacaacagaggcgacggcaaatggtacctcttttcgccggatcaggcccccaatctacataaggtctttgatttggaacggtcgcagcacgaaaacgcacaccgcgaatttaaaaagctttactatcagtatgttgctgaaaaaaggtacaccggcgtcacaacggccaaagagattatcaaagagtggttcaaaacagttgttcaagtagggaatccctatatcgggtttaaagatgccataaatcgtaaaagtaatctttcacatgtaggcactatcacgaactccaatctttgtattgaagtcacaatcccctgctgggagggtgataaggctgaacaaggtgtttgtaatctggccgcagtaaatctagccgcctttatacgtgaaaatggctacgactaccgtgggctcatagaagcatcaggcaatgtcacagaaaatttagataatattatagataatggctactaccccacagaagccacgcggagaagcaatatgcgtcaccgacctattggcatcggggtctttggcctagccgacgtgtttgcgtctttaaaaatgaaatttggttcacccgaggccattgccatggatgaggccatccatgcggccctatactacggggccatgcgacgatccatagaacttgcaaaagaaaaaggaagtcatcccagctttccggggtctgcggcctcaaagggtctactgcagcccgacctatgggttcgctgtggtgatttagtttcctcctgggaagaacgcgtggcacagacgacgcagggtgtgttgacgccgaaaaggtggtcgcagctacgcctggcggctatgcagggacttcgaaatggatatgtcacagctcttatgcccaccgcaacctcctcaaattctacaggaaaaaacgaatgttttgagccctttacatccaatctatatacacgtagaacgttaagcggggagtttattgttttaaataagtatttaatagacgatttaaaagaaattaatctttggacagaagccattcaacagcagctactaaatgcgggaggtagcattcagcacattttggatataccggccgagatccgcgatcggtataaaacctccagggaaatgaatcaaaaaattttaacaaaacacgcggccgcacgaaacccctttgtatcccaaagtatgtccttgaactattacttttatgaacctgaactaagccaggtacttacagtgctcgtcctaggctggaaaaaaggtttaactaccggttcctattactgtcattttagccctggagcgggtacccaaaaaaagattataagaaactctgagaaagcgtgtaatgcggactgcgaggcgtgtcttctgtaggtgtctcgcggtaaaagagcagcggggaccatatggtaaaccccaacaagaggataatgaataaaaaaagtaaacaggcatccattagttccatattaaatttttttttcttctatataatggaatattttgttgcggtagacaatgaaacctccttgggggtttttacttctatagagcaatgtgaagaaacgatgaaacaataccccggcctccattatgtcgtttttaagtatatgtgtccggcggatgcagaaaatacagatgttgtatatttaataccctcgttaaccttgcatacccccatgtttgtagaccactgtccaaatcgtaccaaacaagcacgacacgtattgaaaaaaataaacttagtgttcgaggaagagtctattgaaaattggaaggtttcagtaaatactgtgttcccccatgttcacaacagattatctgcgccgaaactttccatcgacgaggctaatgaagccgtagaaaagtttttgatacaagcaggacgactcatgtctctgtaaatgtctcttcctttatgggtgacgtctcttcctttgccgaggaagtctctgttatgggcaagaggtttgaaacaacgcaaggactctgcttaatctgctgtctcacaaagggaatcaaactacctgctttcgtatttttaatgtagtaattacccttgttgtgatgaattttaagaccatagcgtagtcccagtactttattaatgaattttaaaattgtttgagggtccgttttattgggctttttaagcttaaactcaaagctgatcgcgcttaaatcatactgaacaaattcatcaacgagtttcgtcattaattgttcattggtcaatatattagggtcctgaacgcatttaaagccgcacttagttaatagcataatagcgtacatatgagattgaaaactataattaaattgtagatcatgatgctctgcgtgttgcatggcccattgatgaaagtttaattcctgagtttgtaacatagtgagcgactcgtatactgtctttccgcggcttatttggacacggccagtatagttctgttttgtcataaaactattgtattgttcaacaaatttgggagtaattttatgaccgtgccatgcataaaattcgagtagtttatacttttcatacgcaaataggtcttgctggtctactgtgatgccttcctttaagttttgtttaatttgtaaagctttattggcatcaatggtttcagccgaggcaatgtttacatagtcctggtgtttaatttccattttaatgcttgtatattgtttgactgtctccagcttttcacccgtcagtataaacaccttagcgccggtgtcggcgatctggttaataaatcgggttataaagtgattttttgatagatgttgtatccgcattgtttcgagccatagatggtagtatggagttttataatatatcggcctacctgtttccttactatacgtgaaggaaagctggtgattgcttatggtctgaaaaagggtgtcacgtttttgtaacgtaaacatttcaatgtcttcgatggtttctggatagtaattttgtttcccctgtaagcagattttataacacttactttttaattcacgcacgcggcccaacatttggcaacatgtttctacgtcacacgacatattgttaaaaaagccgtataaaacatcaaatctcttatcttcgtatgaaacacccgctgaaatcgtgggcgtatagataaggatatcaacgagcccccaataatacgatacattattaaaatgggattcccgttcatgagcagtgcttttagaactataaaacccaatttttttttccggaaactttttttggataaatgattgcaacagccgggcctccattaatgaatttgtagggataacaatttttttgtcttctagcaaatcctttaaaaggttatttaaccaagtttctcgtgaagaggtaaaataatacgtgtcatgctgggcccttttatattgattccagtgaaagaagatagggacatccccgcgaaaacgctgtagaatattatacgttcgatttcctaggtttgcgtccaagcatataacataatttgccgtttcgagcatccacatgaaaatggcaaaagagggagcaaagtatttgtgcaggccgctattgaattgattaaaaatcgattctacctcatccaaaataagtaggtctacaggctcggctgtggaggttagccggaaaagtgattctacctgaatgatgactctttcgtagctgtccaaatctccagttacttcgctgtacaatgtgaaattcggtagccgggattgtatattttttgagaagatctgtcgaaacgtcacaaaccgtatggtttgttgttttgaaatagaattattgccgtagtatttttgcaaatagttgcgcagttggacggttttacctattttcatttgagcctttacaacaagcgtagggactcgttcatattctcgcatactactttcatcatagatgtgtttttgagtatcaggcagttcttcaaagagaatggactcatgaacctctatgctctttgtcatcacttggtccacatatgtttccacaaaattatttgtgccggaaaggctgcccatgagaaggctatgtttattgtcatggcgacagtgttgatacactttgtttcccgtgactcttaaaattagggtattgtccttatcatgcatacgcttacatatttcgcagtaacttggacttgtacgtttaaacaatactaaatttttatgaacacggaggaagcaatgatttttacatagtgttcctgcaaattttaatacctcttcaagttcactttgttggatagtatcgcaggaactcggtgttgtttcttttacatttgtgaagatacaaggtaaacacgtcgtttcaaagggggttgctataagggtatcactctttttcgtggttgtactggtctcaaacacctctgcaagctcctcattaaacattttaacacgcatgctaccttttttatgagaccctatgatgcgaaaattttgaatacttttgttgacctgggggtcaacaaaaggataaacgtgtttgggaagattttctaacactttggatgtaaagactttggcctcattattgtttaatactgagtatgtataaagtatgatatgaaaggagtatttaagttctcgctttttatttaatccgatagaatctgttagcaaaatttgttcacgcgttagattgatgttataaggtaaagaatatgtctcgtaaaatacatccatgatgacgttaattatcatgtcaaggatgtcatagacattgtcttcgacattatcattgtcatcaacattgtcatcagagtatgacttatttaccggaaagtcgatgtcaaattttaagcgctgaggcaaaaacccaaataccacttcgtggaaacacttctgctcaaagggctgagccgcctcccactcccaaaagtcatcacgacttgaaaaaactctaaaaagattattatattcatctcgcaccacgaagtgattctttaaggtttcgagagaatatttatcctctacggcttctccttgggagttacagcgaagaaacttgaatgtttcttgcattttgatatttaaaattaaatcaattatgatgcggccgctaatgcggcggttgacgcggccgcgccgctgacgcagccatcatacataaagcggcatggccgttttataacgactagtcggccgttatatgacgaactatataaaaatgaattcttttaattagagttaagtattgttgattgtataatccatcatggttgagccacgcgaacagttttttcaagatctgctttcagcagtggatcaacaaatggacactgtaaaaaatgacataaaagacattatgaaagaaaaaacgtcttttatggtatcattcgaaaactttatagaacgttacgataccatggaaaaaaatattcaagaccttcagaataagtacgaagaaatggcggccaaccttatgaccgtcatgacggatacaaaaattcagcttggagccattatcgcccaacttgagattctaatgataaatggcactccacttccggcaaaaaagacaacaattaaggaggctatgcccttaccttcatcaaacacgaataatgaacaaacgagtcctcccgcctcaggcaaaacaagtgaaacacctaaaaaaaatcccacgaatgcgatgttcttcacgcgtagcgaatgggcatcctcgaatacttttcgagaaaagtttttaacaccagaaattcaagccatattggatgagcagtttgcaaacaagaccgggatcgaaagattgcatgccgagggtctttacatgtggagaacccaattctctgacgaacagaagaaaatggtcaaagagatgatgaagaagtaatatttttggtaaaaatatttttatcaaaattttttaccaaataataaaaatatttttactttttttcttcataatatacatagaatgcctacaaaagctggcacaaaaagtaccgcaaataaaaaaacaacgaagggctcctccaaatctggttcttccagaggccacaccggcaaaacccatgcttcttcgtccatgcattccgggatgctctataaagatatggtaaatattgctagatctagaggcattccgatttaccagaatggatcgcgtcttactaaaagtgaattggagaaaaaaattaaacggtcaaaatgaatataatcaggaaacttaagcctggaacaattagccttgtgctgggacccatgtttgccggcaaaactacgtttcttattcattgcatttacatgctcgaacgtttggaaaaaaaagtagtcttcataaaatctaccaaaaacacccgagacaaaactattaaaacacactccggtatacagctacgacccaaacaatgtaaaatcatagaaagcacacagttatctgacgtgggttctctcaccgatatccatgcagttgtcgtagatgaagcgcatttttttgacgatttaatcacatgccgcacttgggcagaggaagaaaaaattattattcttgcgggactcaatgcttccttcgagcagaaaatgtttccgcccatcgttcgtatttttccttactgcagctgggttaagtatattggccgcacctgtatgaaatgtaaccaacataatgcatgctttaatgtgcgtaagaacgcagacaagacgcttatccttgcgggaggaagtgaactgtacgtaacatgttgtaacaactgtctaaaaaatacatttattaagcagttgcaacctattaaatattaaaaatcttatacaataatggatcattatcttaaaaaattacaagatatttatacgaagctcgagggtcatccctttctttttagcccgtcgaaaaccaatgaaaaagagtttattactctgctaaaccaggccttggcctcaacgcagctttaccgcagcatacaacagctgtttttaacgatgtataagctagatcccattgggtttattaactatattaaaacgagtaaacaagagtatttatgcctgttaattaatcctaaactcgttactaagtttttaaaaataacgagctttaaaatttacattaatttcaggctgaaaactttttatataagtcctaataagtataataatttttacaccgctccctctgaagaaaagactaaccatcttctaaaagaagaaaaaacttgggcaaagattgttgaagaaggaggagaagaatcctaagtcgcttacatttttttttgctatttttatagaatgtacacgcatgttgatgttgtcggaatagctgaagcctcagcggccctctacgtgcaaaaagatagggatcgctacttagacgtgctaacaaccattgaaaactttatttaccaacacaaatgcatcataacaggggaaagcgcccacctactctttttaaaaaaaaatatttatctttacgaattttactccaacaatgtggcggagcacagcaaggctttggcgaccctgctttataaacttgatccggaatacctcactcgttacacagtactcattaccaaaattcccaaccattggtatgtgattaacgtagatcagcgagaatttgtgcgcctatatgccatcccggcagttaaacaacacttaccgattcccattttacccttctattgcaccagcgcactcacccagcaagaattgttttgtttaggacctgaactgcagttaatacaaatatattccaagctctgtaaccccaactttgtcgaggaatggcctacgttgctcgactacgaaaaaagcatgcggatgttatttttagaacagtttccgcaaagattggaaatgacgggcgggaagaaggaggagaaggaaaagcatgaaagtatcattaaaaaaataatactagaaatggtctctacccgtcagcgaatcgttgttgggggttacatacaaaaaaacctgtacaaccatgtactcaagaatagaaatcgtttacagcttattacgagcttaaatatttatgaagaaaaagatatcatccagcaattttgtgattcaaatggactgaagatcaaaatacgtatcaacaatccgctcttgcctacaaatccggaattacggcgtttgactatttattttaatcataataatgatgatgatcagtcatatctaatagtagatatgtacaacacgggaagctatgagctagtgcctacaaatcagataaacacgcttgatggcagctttttaataggaacacccttcgtgcaagcgcgatttttgttggtagagatctgggtgcttatgcttattgcgcagcaaactaaaaaggacaccaaaaaaataatacaattttttataaatcaatatgaaatgcttatgaatagtccttggcccagtatggaggccctttttccctcaagcagtaaaagatatttaggcaactatgtagaccctaacgcgctcataaagtgggcacaactcaaattaaaaagaataccgcctttttatcctggaaagccggatgaagaatcatgttaagccgattaaaaaatcatgttaagctggttgaaaaatcatgttaagctggttgaaaaactcttggtgaaagcacggatgtaatattaacattggccgctcgcatttcgtgttgaaatacgatggaagagcgacggctatctaccatgccgatatcggcctggacatcacagttcatgcacttgtagatgggatgactcgcgttatagatggcaggctcgccacagtttctacagatgtaggagatgcagccatccgagtcgtcgtgcgatttttctatgatggtttgcatggcgccctgcgccgtaagcacccaatgctccatttctcccagacgaagacctccgtgcgatcgtttgccgtccaacggctggcctgtgagggcatccgtgggcccatagcttgcaacggcgtatcggtcatccagcacaaatttttgcaggcgctggtgataggtcggtcctatgaagatggccgcatcaaagtactcgccggtctggccgttgaacattttttggcatccattgaagcgtagaccttcttgcgccagtctttctgaaagaagctgcacattaataggcaggaatgcggtgccgtctgttaccaccccctgtagggcatttgctagaccaaccgtggtttctatcatttgaccgttggtcattcgggagggatgtgagtgggggtttacaatgaggtcgggctgcaatccgtcctctgtgaagggcatgtctgaagtgggcagggccagcgccgcaatgcccttgttcccgctgcgagaactcattttgtcgcctatattgagatttctttcatagcgcaggcgcatgaggccaaagatctcgtcattaggcccatggggacgcatcacagcatccacgacggccggctcatcgaagccgtacatgacagaccggtcgatgtatttgttgagttcgtctttttcgccccgtattttggccacttttcctataatgatgtcgccctttttgaccaccgttcctacgggcacgaatccatctacaagcttttcgtaattagcaccaggcttaagatttttggtgattaaagggtcgggcttcccaaacgactctatatcgctttctaattctactttttcttctcggtagaaggtgccggcaaagccgcccctgtcaataaaggactgcgacacgatcacagagtcctcctgattgtagccgccgtagatcatataagccacaatggtattaagcccgttgggtatgacatagttatgtgctatggtctttacaagcggcatttcattgtaaaactggaagaagcggttcatgtcgacacgatatggccagctaaagcaataccagccccccgtttgccggccttggtttgtttcataggtaacacgcgcaggttgggtacagtttgcgtagggggacactagggcggcaaggcccaaaatagcttggggcacgtccacgtgtgtgaaacgacgcgttacatcatgtttatgtttgcgtagctcgatgatggagaaggcaacaagacagttttccgcctcctcgggggtaatgaactcacagatgccctgtgctacgagatcttcaagtgtaagcgttccggctaaaatgtcttttgccatttgaggcgtaaatcgcgtattttgaatgaaagggattttatgtttttcccagtctttatcgcctttttttctggcctctgcggccttgtagcaggcttgattgtatttttcaatattattatctacaatgagtagggggcgggtcagcctaccgacgtccaaccaaaattctacttcgtctaccatgctatcccagtagatggtggtatggggatgcacaaccttgccctcacggcgaagcattctataccgctgagcaagctcaaaggcattggtgcagcagccgatccattctccgttgataaatacgcgcgctaggccctttcgtacaatgtccttgttggaaacatcggctaactgttgaatggccggatctgatagaaggcgttgttttaacgaaagtacttctccggcggtgcagacattggcagtgatggctaactgtttagacatgcctactttttcaccagtatcggctgactgggctacgcagatgtatccaggataggatgcgtgcacgcgacgcatcatgtcagccctttctgtttgtttggatgcgttggtggtgttatgagtatttaccgtacgcaatgctgaaatggtatttaataaattttttctttccaaactttgagtagatactctgtttacaatggggcgctgtcgcaccatgatggttttatttcctgaaatgatagactgttccatactgcgattaagatcggaggcggtattttttgataaagcggcagaaaatgcctcgataatgtttcgctgagtaagctcctcaaaggctgtttgtttaagaagttctttgaacccattgatgatgggtgctatcacggaagtattaaaaatagccttaaaggccttggcgagtgagacccctgagccgtgcacccgcttggtgcggtagctatcacggtccgtgggtggaaacacattcataatgacaagaagtattttatgaataagcaggcctaaaaagcgcagctttcgtacacgtgtatctgcggtttggcccatgtgtggcagcaatattttgtctaaaatagtaagttgtctttcatttaagtattgtaccgcattttcatcgcttttgtaagcagatgggtttgagacaaatttggaaaccttctcggataaaaactggataattttttctcggttcagctcgtgttggaccggttgaaatatggggtctaaaacatgaatggatttttccagaatttctatcatgaaggtattcacaagggagttggattctagatcaaataccacttgctcaatgatgctgtcatcgcctgtcattccaaacatgcgaaagatgagataccaaggtatgcgaagttttgagaacttggtgctattgatttcaatggtaatggcgccggtggtcatgtagcgtataataatttgagagctattttcgaaggcacctcccggttgggagataaactcgccgcgaatgatttcattattcccttgttgcatggtatggtaatggatgtgaagcgtgttaaagcggatgttttctaagaggtctacgacccattccccgcctcgggctataaagtagccgccgggttcattagggtcttctcctatttctttttttgcggtttttgataggtgatgagtgtggcagcggttgctgccccgcatgatgggaaatgtagatacctgaaaaggaggaatacttgctcgttttacctcctgccgaccattgctgtagtgcgccgttaaaataacctcggcggctagattaaccgggcccgaataggaaaggccacacaggcgtgccttattgggtagtaaatttatcttgtttccctgtgaatagtttcgatgttgcgggcgttcaatgttcacatctgtaaagttaaattggatctgaactgattcccgaagcttatctatttcagtatggtcgcgttggtctttataagtaatatccacgttaaacatttgttttacaatttgcggaattccattgtccataagatcgtcgaagcttttgatgttataccctatcaatcctgtagagtttactgcagcggagataaagctcagcatatcagcctctgtaagctcctcattatccacggtttcaatggggccgtaggttatttgcggccgcaagggttccatgattatgaagtactacattaatattcagttattctttaaaataaatctttatttataaatcttatttataatataagaatgccttatgcaagagacatcacaaagtttattacggcaacggaaccagaggtgggtcttcccctgttggcgctgcagcgctccaaatccatcataggggttattcttcttgtaataagtttgttatttattttcattggcattattatattatcagtgagtagtggtcataccacagcagcctctatatttatcgtattgagtcttatcctaggtggcggtggtttttttcttatttataaagataattcttaacccacataaaatttgaaaaaatatagagtaagaaaatgtccaattactattattactatggcggggggagatatgattggttaaaaacagtagaacccactaattttttaaaaatcgggttgccttaccaggcacacccattacatcttcaacatcaggcaactactcccccatctatcttagaaaaatttaaacgagcagacattcttcttaatgaggtgaaggccgaaatggacccactcatgttacaaccagaaaccgaaaaaaaactattccagatattgagtagtattgatatgttcaaaggtctgcgaaaaaaagtagaattcacgtacaatgctcaaattgttacgaatgcttggcttaaaatgtatgagctgctaaataccatgaattttaataatacatctcaggcattttgcaattgtgagcttccaggagggtttataagtgcaattaaccattttaattatacaatgatgcattaccctacttttaactgggtagcttcctccctttaccccagttcggaaacagatgccctggaagatcactatggtctttatcagtgcaatccggataactggttgatgcaatctcctttactgaaaaaaaatatagattataataacggggacgtaaccatcgctagcaatgtaaaaaacctagcgcttagagccacacaaaggctgacgcccatccatctatatacggctgatgggggtattaatgtaggacatgactacaataaacaggaagaattaaatcttaagcttcactttggtcaagcccttacgggtttgttgagtcttagcaaaggcggaaacatgatactcaaacactataccttaaatcatgcatttactctttctttaatatgtgtattttctcacttttttgaggaactatacattaccaaacctacctcctctcggcccacaaactctgaaacctatattgtgggtaaaaacagattacgcttatttacccccaaggaagaacaagtccttctaaaacggctagaattttttaatgatacgcccctcgtagacctaagtctttaccaaaatttacttgaaagcgtttactttgccgtagaaacaatacatctaaaacaacaaatagaatttctaaacttcggaatgaaatgttatcgacatttttataacaagattaaactacttaacgattatttagctccgaaaaaaaagatttttcaggataggtggcgtgtgcttaataagctttatgttcttgaaaaaaagcataaacttaagctttgtgcctcctagggatctgttgcttaatttaacagatgcaatcttaacagatgtaaactaaaaagtgtgttcatacaaggattgtatttatgaatatttattaacatataaggttgtgatgtaacactgtataacctatataactacactatgaagcacggcgtataataatttatattgaacacgatgttgactcatttatttgcaaacaaatatttgtttgcaagacgtttgcatgcatttactaatatgttgttgactagtttatttgcaaactagatgtttgattgcaaactagatgtttgcacgtatttatttgaactaatatacactccttgttttatttgttatatacacagcatacataagtgtatattgtttacacttatgtttataactcgacgtaataacattttacacgctttttttttgcaaatcttaataatattgtatgataaatcaaacaatgtcttatatatgtggtttattattttaggcgccgcaagatgtactccattctcattgcatgcttggtgttattactctgtctagttatatatgtcggtcatcgtgccgatcatgcacgaaaatatttagaaggaatgtggcatggagatccggtttttctaaaacagtcggggctacaatccttttatctctacatacaacctgaccatacatgtttttttagcattgtgaataaaaatggtgaaaagctgatggaaaccaaaataccttgtacgataacaaataaaatatatatgttttttaaacctatttttgaatttcatgttgtgatggaagacatacatagctacttccctaagcagtttaactttctgttagatagtacagaaggtaaacttattttagaaaacaatcacgttatttatgctgtattgtataaggataatttcgccaccgcactaggaaaaacggttgaaaaatatataacacaaaattaatcatgttttctaacaaaaagtacatcggtcttatcaataagaaggagggtttgaaaaaaaaaatagatgattatagtatattaataattggaatattaattggaactaacatcttaagccttattataaatataataggagagattaataaaccaatatgttaccaaaatgatgataagatattttattgccctaaagattgggttggatataataatgtttgttattattttggcaatgaagaaaaaaattataataatgcaagtaattattgtaagcaattaaatagtacgcttactaataataatactattttagtaaatcttactaaaacattaaatcttactaaaacatataatcacgaatctaattattgggttaattattctttaattaaaaatgagtcagtactattacgtgatagtggatattacaaaaaacaaaaacatgtaagtttattatatatttgtagtaaataatatttttaattacttaaaatttttatatataagtttttgatactatattataaaacatatgttcataaaatgataatacttatttttttaatattttctaacatagttttaagtattgattattgggttagttttaataaaacaataattttagatagtaatattactaatgataataatgatataaatggagtatcatggaatttttttaataattcttttaatacactagctacatgtggaaaagcaggtaacttttgtgaatgttctaattatagtacatcaatatataatataacaaataattgtagcttaactatttttcctcataatgatgtatttgatacaacatatcaagtagtatggaatcaaataattaattatacaataaaattattaacacctgctactcccccaaatatcacatataattgtactaattttttaataacatgtaaaaaaaataatggaacaaacactaatatatatttaaatataaatgatacttttgttaaatatactaatgaaagtatacttgaatataactggaataatagtaacattaacaattttacagctacatgtataattaataatacaattagtacatctaatgaaacaacacttataaattgtacttatttaacattgtcatctaactatttttatactttttttaaattatattatattccattaagcatcataattgggataacaataagtattcttcttatatccatcataacttttttatctttacgaaaaagaaaaaaacatgttgaagaaatagaaagtccaccacctgaatctaatgaagaagaacaatgtcagcatgatgacaccacttccatacatgaaccatctcccagagaaccattacttcctaagccttacagtcgttatcagtataatacacctatttactacatgcgtccctcaacacaaccactcaacccatttcccttacctaaaccgtgtcctccacccaaaccatgtccgccacccaaaccatgtcctccacctaaaccatgtccttcagctgaatcctattctccacccaaaccactacctagtatcccgctactacccaatatcccgccattatctacccaaaatatttcgcttattcacgtagatagaattatttaatatgtactatatattaattatttaacctttcaagctggtcttcatttaaatttaaaatccactaataaaatgtattttctagtagcagatcatcgagaacatcatgtgattccttttcttaaaaccgatttccatcacatgcatcaaaatcctatacaaaaaaatcaagctctcctagaaatcaaacagctttttactggagattatctcatctgcaaaagcccttctaccattctggcctgtattgaacgaaaaacctacaaagactttgcggcttctttgaaagatggacgttataaaaatcgccaaaaaatgctgtcgctgcgagaacaaaccaactgtcaactttatttttttgtagaaggcccggcatttcctaaccctcaaaaaaaaattaatcacgttgcctatgcaagcattattactgctatgacgcatcttatggttagagatcatatttttgtcattcaaacgaaaaatgaggcccacagttcccaaaagcttgtgcagcttttttatgccttttctaaggaaatggtgtgcgtcgttcccacctccctcacccccacggatgaagagctatgcatcaagctatggtcttctctttctggtatttcaggcgtgataggtaaaatcttggcaaacacttgttccgtagctcatttggttcatggaaagctttcatcgcagaatattgatcagttaaaaactccctccaaccgaccattccccaaaaaagtaaaacgtatgcttataagcattagcaaaggaaataaggagttagaaataaaattgctctcgggggttcccaatatcgggaaaaaattagctgccgaaattttaaaagatcatgcgcttcttttttttctaaatcagcccgtagaatgcttggcaaatatacaaatcgttcaaaaaacccgtacgattaagttgggaatgaagcgagccgaagcgattcattattttttaaactggtgtggctctgcccatgtaaccgatgatagccaaaatatcacagaggcgtcgcggtccacaatgcaggtcgcgacgcagtccgccgcaatacagcccgctgcaacgcagccattgcacgaagtatcagatgatgcatcatcagatgcttcatcacccgtagggtatcaaacattatctaaagaaatgttattgaacacagcctgatgttaataattcactacatctaaagaaatgttaacctcgatactaaaaagtcattgaacacaactactggggcgctaagttgtccaacacatctaaagaaatgtcaacatcctcgatgctaaaagggtcatcgagccggtcaataatgtcttccccaaaaagtccgggagaactgtaggccgagatgtcgtccatggagctatcttccccagagcacacaaagtcctctccaaaaatcataaagttaaatgcaccgggcttacttaacagcttttcgctttgaataatagtgttgagttctgtcagcgcaaactctctcacaatattcacaacccaggagggctctttaatttcatacagcgttaagaaacttatacataaaaattctatagagtaaagcaaggcgctggcaggatctgttacccgtaggtgtttaaatgtagtgtgatattcattcacaacgttaggcagcaccttttccaaatcctccttttcctcgtacgacaggtgctttacaagcctttcaacatgtataggaggcttgttaaatgtactaacgtgccgcaaacagttataattatataagaaaatacgtacggcagagtcgaccgccatgagccttggatcatccattgaggtaggtggtggcggggcaccctggccttccctgatgtctgcgtaggagcgcccctccatggcccctatggcctctatcacagcaggactgatatccaaaatcttggccgtcttgattatttttccgtaatcgaaagtccatggctcctgtggaggcttgggttgtgtttcggtggagggcgtggtcatatctttctttatttgaatagaacggatcgacatcttttccttatcgtactggtctttataattattataatagtcatgaactaattcgggttgagaaagatgatcgtatataatataggtaaaaagtccgcacttgacacattttttatcctggaagtcgtgtaatcctcccttggggcagcgtgactcgtagaaggcataaaaggtgttaaattctaagctcgcctttagggctgtttggaccttttttatgtttaattgccccacctcatgttgtagcacgtggcatacagaacagcgtagatcggcaagtgcataatggttgtcaattttttttatgacgtctttgcgtgttacttcaatctcggcgggtttctgcgaactgtctacggccttgtaaacgtaaatggtccacttatgaggaagccccctttcatcgtatagggttgaaatgggaagccttttatactcaaacagccgagtccgttggtcggctcttcctgtgttaggatcaaatatgttataaaatccttgctgagcaagcagggccttttgctcgccataagcattttcgtacgttttgaattctgcaagttcggagttaaaattaggtgcattttgtaaatacttaagaaataattcataggctctaaggtaaatgagagttgaggttttttcctcatcccgtcctccccaccacacccgcaggctttcttcttgaaaatagatgtcattcagacgcgtcaactgcgtaaaatcaggccgatatttagaggtataaattttatcataaaattctttttgcgataatagctcggccggggtacgtcctatcacggttttaaactcatattcagcctccttgggagtccgtggtttgtgcatagggatgctgccgtcaatacgggccactgtggcagcataatcatacatggggtccagcagaatctctgtcaaaagtaccttggtgtcgtcctgcacgctaagcccttgtagcccattttggtggataatttttttgaaagcctcccgaaaattattagcaatccactgatccgtaatctcagatagctgatttattataccgctatattgctgcatcattttctccaaaagaaaggtcacgtatgcattcaaagagctatccgccttcattccatgaatggtaatcgtaagaaattctttatttttttgcgagctataaatgagattcaaaatataggcatagatgtagatcacagcatacagctgcgttaaaggatcgtaatcctcttcctttttaatattttcgatgctatacacgagcggcaggcagacatttacggctatattggcaaactgtttcacgtctacaagctttccaaagtggataaacgtgcaggccttcatggtttcctgccaaataaaaacacggagcttactattaagatcgccgatgatgcccacatctgccgtacgatcctcttgaataaaatgggccagctcttcgccacaaattttgcaaaagtaggagtaaataagcccctggttgttttctttctccttgtttattcctgaaaatttcattagcttggttcgcatggtgtcgtaggacgcttctgccgcttgaagctgtataagcatgtccacatggggacaaagcagcttaaacccgcaggctttgcatagattccaattggtggtattgtttttttccttgtagagtacacgaatactttctaatacttttaataactccgcgtattgaagacccgaacgcaactgttttaccagcttgagatgagcacatgcatttttttcttggagttcccactgttttttaatgtttaggtattctgttgtaataagttctgcctcctgtttcccacaggctttaatgacttcttgaaggatgctgttagggtcatccactttaccctccattgtaagaatttcacgtatagcatccgactgcaccctacctattttttcttccataattttaaaatactgtctcgcctgggtaatgacctctgtgagcttcatgtccacctgctgcagaatcatttgctccttttcacgctgttcagcatgttgtaaaaacttttgttctacagggttccaaagcacctccaaatagcctgctctatataggtcataaagcaagggcatgtatcccgatgtaaaaaccggggacaccgagtacatcgtagacaactcttttaaaaaaaatatcacgcgcttaatgttctcctccggttcaatctcctcggtttcaacgatattagatatatgactgccctgatcctcacggtctagctttcggtgtaccatctcctctgctagccgattaatgagccagctatgcccgccgctccgcaaaaacttataaagttcgatatactggtgcgtaaactggatgatgttttccttggtggttacgacaaccccttctccgttttttttccaggtttcttgatccacgcatttcataaatactcgaataaaattggtcaaattggctcctgaggcgacgtagcccaaggtttcaggcgagaaggagcctatctcagccatacgcataaaacactgcggggaaaaagtttttagccgcaacttaagtccatagatttcaatgggggcttctgcgggaacggccaggtgcgtcccattaattaaaaaaatttctttgcgtgtgctagggcgaacacgtaattccttttttttttcactcacgatggggaccacatcggggtctaccagcagttgacgtatgtaggcctctatgggcatggatagatcgggcagctttgactgctcggcgcgaacatggttcacaaaatcttttagagtgaaaagaaagtctattaaacgtatgttttttatatcattagaccctttaagggtagagtagatttcatccactagtgcctcgatttcctcattattgagcgataagatatctgtgccacggtggactatttgcgcgatcgtaattacttcctccattagatagaaactgaatattatatttaaaataaatacaaaatgtcaaatgaaagttttcccgaaacgttggaaaacttactttcaatgttacagaccaaacagcaaaacgcaattcagtcagaggtgattgaatggctgcacagcttttgtgaaacctttcacttaaaaatacactgccataaacagtttattcctagcggggaaaaaaaacgagctaaaatacccgctcaagaaacacagggaaacacgcagccctcccaccatgtgtaccgggttgttctctccagagcacagccagtcaaagcacaggaatctctgctaacaaccatgtgcaacggactggtgctagatgcaaacacatggacatgcctagccattcctccgcctgcgccctttcaacaggcgacccgccaggtccaacacttttaccgtaacaatttctacgaagtggttcccatccaggatggcacccttctcacaatctaccactgggatgaccctgaatatggcccctcctggtgcctagcaagtacccacggatatgatgtgagtaactactgttggataggcgacaaaaccttcgccgagcttgtatacgaattgctgcagcagcactctacctgcgacgtcaccctggaaaaaaataaaacgcggggaacgcgtcttttctttgataacttaaatcccgattactgctatacgattggaatccggcaccataatttacagccgctcatctatgaccctcaaaatatttgggcgattcaatctacaaacctaaaaacgcttaaaacggtatatccagaatactacggctatataggcattccaggaattcagagtcaagttcctgagcttccccagtatgatttaccttatctaatacgatcttataaaactgctatgaatcaagccaaaaatgctataaaaaatggcaaaaaagacaagggatactttaattatggctatttactcatttcgcgagcgcctgccattactaaaagtacttctaatgttttgttaaaatcgcctctgctggtatttttacaaaaaagtgtgtaccagaaaaaacacaatatctctaacagccagcgactagaatttattatactgcaaaactacttgatgcagcattttcgagatcatttcattgctctatttccgcagtacatatcctattatacgaaataccaaaacatgttgaatatgattatccatagtattgcaactaaagataaagatcatccctttgcaggagccgtggtaaaaaaagtgttggaagatattgaaaacgccgaaaacattattgatcatacaaccattcaaaactatgcccatcaaagcaagtacgccatgctttacttgtcaattatttcccatttttaatctaatacggccaaagccgcgggttttttaataaactaacatttaaaaaaactgttttattaaaaattataatacttttattatatatggaacatccatctacaaactatactcccgaacagcaacacgaaaaattaaaacattatgttttaatccctaaacacctttggtcttatattaaatacggaacgcatgtccggtactacaccacacaaaatgttttccgagtcggtggctttgtgcttcaaaatccctacgaagccgttataaaaaatgaggtaaaaacagcaataagactgcaaaatagttttaacacaaaagcgaaagggcatgtaacgtgggccgtcccatatgataatattagcaagctatatgccaaaccagatgcaattatgcttaccatacaagaaaatgttgaaaaagctcttcatgctttaaaccaaaacgtactgacgctcgcatcaaaaatacgttaaatataatttttgtagaggataaaaagctattttagctaaaaaataattcatatacgtttatgcagaggaagaacggtggctttcaaattcagattgcatccacgtagaccgtagcgttttttttgcttctggtttatatcgtaaaccgtaataaacatcatcatttgtatccgttggatctttttcccactccggataaaaaatcggttttcttttttttggtcgttttttgcagtaagctgtaaattaagggaatatagcttatcgaaaagttgttcctgatccatataaatagcagcatatattaaaaaaaataaaaaaagacgcttcaacgagtcagtaccactgcttgccaacgatttacgttggttggtgcattatggtgatatagtaatgagtgcctgcacaagtgcttgcacaagtgcctgcacaagtgcttgcacaagtgcttgcacaagtgcttacacaagtgcttgcacaagtgcctgtacacattactgcatcgccaaagcacctgcaatgcctacttcctcaacagagtacgataactaaatgcttttaagcaccgcttgcgtcgatgtgtccttcggggcaatcgggttcaattggatccaatattattagtcataattacctaatacttattcaattttatcttttttaccttgtaagatttaaacagcgttttagcttgtttaaagcaacgtttaaaacaagctaaaatgctgtttaaaacaacgttttaaacaagttaaaacaaataagcttataaatataccatgacaaaattagcccaatggatgtttgagcagtatgtcaaagatttaaacctaaaaaatcgagggtccccctcgttccgcaaatggctcacattgcaaccctcactgctgcgctattcgggtgtgatgcgtgctaacgcctttgacatcctaaaatatggctatcctatgcagcagtcaggttatacggttgctacgcttgaaatccactttaaaaatattaggtcttcctttgccaacatttactggaaccgtgatagcgaggagcctgagtacgtctgctgttgtgccacctatcaatcgcacgatggcgaataccggtatcgatttgtttggtaccaacccttcatagaggcttataatgccatagaggcggccctggatcccctggaaaccattatcctgaacctcattgcggcacgagatctagacttcgttgttcacatatttccttataataagggccatgaagactatttggcctccacgcaacttattctcaaaatctttattgcgacgcttttaatggacattttaagaattaaagacaacacgttggacgttcacttaaattccgactatattattgtgatggagcggctttggcctcacataaaggatgccatagaacacttttttgaagcccataaggacttactagggtacttaattgcctttcgcaatggggggaactttgcaggaagtcttagaccctcctgtgggcaaaagattgttcccctaacgattcgagaggtcctacaaatgaatgatattaatttagccgtatggcgggaggtgtttattatgcaggaatgttccgacttagtcatcaatgggatagcgccctgtttccccatttttaacacgtggacgtatttgcaaggtattaaccagattttttttgaaaacacgtctttgcaggagaaatttaaaaaagattttattgcccgagagctttccaaagaaattatcaagggccaaaaaacgttgaatgacaaggagtttaaaaagttaagcctacatcaaatccagtacatggaatcctttctacttatgtcggatgttgccattatgattaccacagagtatgttggctatacccttcaatccctgccgggtattatttcgcgatccagctatttatcccccatcgtgaaaaacattttgatggacgaagactcttttatgtccctactatttgacctatgctatggcgcctacgtgttgcataaaaaagaaaatgtgattcacgcggatttgcacctgaataacatgacctactaccatttcaacccaaccagttttacagatcgcaacaaaccaggaaaatacaccttaaaggtcaagaatcctgtgattgcctttataaccgggcccaaagtcgaaaccgaaacgtacgtgttcaagcacatagatgggttcggctgcatcattgactttagcagagccattatggggccaaaccatgcaatcaagcttgagcggcagtacggcctcgcttttgtaaacaccttttaccgcaatcaaagtgagcatattttaaaggtattacggtactattttcctgaaatgctaaccaatcgcgaaaacgaaatacagggggtgattttatcaaactttaatttctttttcaatagcattactgccattgatttttacgccattgctagaaacctacgtagtatgctttctttggactatttacacacctctgaggtgaaacgaaacgtagaaatttcgcaaacatttttggatacatgtcaatttttggaggaaaaggccgtggaatttttgtttaaaaatcttcatactgtcttatctggcaagccggtcgaaaaaacggccggggatgtgcttttacccatcgtatttaaaaaatttttatacccaaatattcctaaaaatatattacggtcttttaccgtaatagatgtatacaattataataatataaagcgttattctgggaaagctatacaaacgtttccaccctgggctcaaaccaaagaaatcttgacgcacgccgagggtcgtacatttgaagatatttttcctagaggagaattagtttttaaaaaggcttacgcagaaaacaaccatttggacaaaattttacagcgtattcgtgagcagcttgctaatgaaaatttgtaaggcttgcagttcttgtatggtcagaacctatgtcgatggaaacattatttttcgctgcagctgcggcgaaagcgttcaaggggatagtcagaacttgctcgtctctagcaaggtgtaccacaccggggaaatggaagataagtacaagatttttattaaaaatgcaccctttgaccccacgaattgccaaataaaaaaggattgcccaaattgtcatttagactatttgacacaaatctgtattggaagccaaaaaatcattatattggtgtgccgctgtggctatatgagcaacagaggataaaccatatcatcccaccgaattatgacattcctttaaaaccgtccgcctaaatagttttcacacctttggtggcagactattttataaaaagtaatgttggttcatgaagataaagtgtgccaaagaaacttttataaacaaatgattaatgtaggtgctagtcgtgtgtacttaaacagggtattctatagccaagtattttctatagccaagtattttctatagccagtattagtcaagtatttagatgtcagggtatttttatagccagtatttttctatatgtacaaactattccagtaaacatatgtgtgttctttattgagcagcatcatggcattaacaagtttattaaactgctctaatgggcattaaatgacaactcggtgcttagcaaaagtgcctataccttttaacaattagggccgggaggcattcccagcttttttctataatcagccatacagtacccctgagcctcatacacgggaataaggtccttccattccttgttgggatcggcgggccagctctcaaatgaggtgtgaatgtaagggtcctgttctttttccttaatgaagcgtttaatctccatttgatgttgtttacttttttgtttgcggcggagcgtgttccgcaccaatacgtaaaaaataccaagaatcacacataaaagaattattaaaaaaaatatcatcatcgcggggtttaaaaaacgatcccatgcaacaggaatcgttcttaaaaccttgtctggcagggctgtaaacatgaagtctcctcctataatcggggtgggactgtagcctaacagttcaaggtcctgtcgttctagatacttattggcgaactgcccaccctttgcccccgtttttttattaatcaagcagcgctgcattttccaccattctaaatcttcaggagaaagctcaatgccatatatcaactttaacgttattgcatctttttcaatatccttatcaatttggctgagcttttgagctttaagcgggtctagtgtgtacttccatttaaacttagtgtcctgtagtttggctacatgaaatacggaacatttcggcggggcctttgtgacgcccttacactgcggaagtttatcattaggacaggcgcatagatgagactgcgccacagcatcgcgaactacatcgcagacggagtacattttcctcctatgttaaacaataaatttttttcatagctgaaatttgtgggcctatcttttcccttgcccggataataattataagggagtgttgaaacatctgggagagaattgcttaaaaaatgggtttttgggaggggtaactgcgactgttgtacgtcgttggccagggagattctatatgccgggctaaaggtgcaacgttcctgtgaacaacttagtacgcgcgttgttaatacaaatggactggtattagcaaacctcgtaaactcttccggacttgtttgtttttgtatgatgtttagcagggagtctgccttttcgagaatccaaagcgtcgcattgtagtaaaataaaaatagcgacttatcggcaggcgttgcaaaagcgccgtatagaaaataaagcagtaagtactggggagacaccacaataaggttatcttgaatgatagatatcgctagctctttaaacatagtgctaaaaaaatgtatgtcgttcgtcttgaatatagggggactatagtccatgtagggctcacatatctcagtcaggtgaaggcccatttcttttatgacttcttccgggttgtacgtcgctaacaccagcgcgggataggctttgggcatatccacggtaagtgttatgtttttatcattcttatggtaggagtaagatggttgtggaaattctgttttccactccgggactttgcaggtaattctcagctcatttagagtctggtacaggagggcgtatgccgcaaagccgtgtatggccacttgtttaaagggaattgaaaacgttttactttcgtatgtcgacttcacaggaacaacgggaatggggtaatatttttctatgaggttataccgctgcaaatcctttttaaacctgctaaaaacatcttcccttggtgggttatcaaaaggaaagcaaaatgctaggtgtagcccggcccgctggtaatcggggtgaatgattttaaggtttttatacgttaatgtgggtatggtgttaaagatattggggggcatatatgaaagatcagcaacccacacaaagtccgtgcgcacccgcatggtctgcacatggatggcgcgcaccgtgcccacctgcttgaagcccttttcatacaaaatgtcagcaagttcgtaggcgtcctcaacgtggttgggggaaaacatatcaaagtcgggtctttctccctcgggataaattgagctgcctttaagatgcagggcataatcaatggcaatccccccgtacaaaataagctttttctttatgataaattcgcggaccacctccaaagccgcctcaatctccacggcatttgcctcacgtttttgagcaatgagccggtacttagaaacattaaaatcagtctttagtaaagacgtcataaatagtgtttaatatatattaaaggtttgaataaaatactaaatagtaaaaatggatgccctattaaaggaaatagaaaagttatcgcagccatccttgcagaaagaaaacaatgatgtatgcgatctctgttttatgcaaatgaaaaaaatttctaactatcagcttttatgcgaagagtgcggtcagctgaaggactggtttgaacctgaatataatgaaaaattcacggtatattctcgtctaaagatcgtgggtgccaatagttcctatcaccagcgcgatttggacaaggccaactcaagtgactatagctccttgcaatttcatcacattttagaggagctcaaatccctaaatgttaagtatatggatgcggggcaaaagccctttcctattcaggtgttaaaagaaactgctcacagttataaccaagtacaacaacatcgggtcatacgcagcattacaaagcttcagatcttagccagtattctacgtagcatttgtttaaaattaaacattgcttgtacggtggcagacgccgcgaggtttactcaacttaataccaaagggatctcaaggggcatggatcttctgcgctccctatttgtagacaataaaattactttaaacgttgatttaaaccctatagacagctttattaatagtacctacagtgccttacaaattaaacaaatccaccaagaactgcaggaggaaaatgtttataatttaaaagaaattgttaagagctttatattatacgcggatgagaagaacatcggcgtcgatcttaacaggagaaccgttgtgattgctacgatgtataatgttttacgccgtgcctactaccccatagaaattgatacggtggtgtatcaatgtaaaatacgaaaaaatacaattacacgtgctcttaaaatgtatgaggattactactcccactttaagtctctttatgagcagtatcatttaaacgcggcaaaaaaattaatttaaactaaacgtttaaactaaatgtttaaactaaacgttaaaactaaacatttcgactaaagtttaaaacctagtctaacagcgggatgcccatttccctggggttccatatttcaacaattttttgaccttcgggtgttaccttgatgcagcgcatgacgagcagtggaattttcctattaaagagttcttgcttagctatatcaataggactgctatatttttttttaagcattgtagatccattaattgccaattgttgcgctctaacggcgaccaaccttgtggcctcaaaggtggttaaaacgttggaggtaatgcgctcgttatcgggtataatgaccaatgtttgcgacgaggcctgcacaaagccctcgcagatggacggagactccacgatctcgtccttgtcctcggactcctcctcactgtcgacgaggttctcctcttccgtttccacatattcctccacgaggtcatccatgataagatcctcgttgtcattatcagccatattacactgttatcaaatgtactgtttaatacgcaaatggatttactacgttttaattgtatgtcttcatgtgcaggctctagtggaaagtaattttctcacaatttttggcaccgttacacttgtgcccacaaaaacccgcgatttttttattttatattacttttggaagtacgagtttaaccagtcgctttcaaaccttatgcgtctatctcgccaaaaaacgctcacagcggtgttggatattacctttaaaaaaataacattaatttttaccacagagggcgtattgcgtatggattctacgaataagccaggcgtgccactcgatatagacccccagttcattgaccttgatagtattttaatggaactggatcattaggacctctcccgcccatttaaatttttagtttctacaataataaaatgcgcgaggaatcatgggaagaccacgataccattcagctcaccgctcagcgcaaatacctcgccgaggtgcaagctctagagacccttttgactcgagagctttcagtctttctcacagagccaggcagcaaaaaaacaaatattattaatagaatcacaggaaaaacctacgcacttcccagcacagagctactaagactctacgagcatctcgagcaatgtcgcaagcaaggcgccctcatgtattttttggaaagacaggggacctactcgggtctcatgttggactatgaccttaaactcaatacaaatgctgttcccccgctggaaccccccgcgctatcacggctttgccatcgaatatttgtgcatataaaaaacagcagtgtgctgcctgagggcagccataaaatccacttcttttttacattaaaacctgaagtggttcagggcaaatatgggttccatgtgctcattcctggtctcaagctggcggcttctaccaaaaaaagcattataggatccctacagcacgatgccaccgtacaaaaaattctacacgagcagggcgttacaaatcctgagtcctgtctggacccccactccgcctccgttccctcgctcctctacggctcctccaaactaaaccacaagccctaccaactgaaaaccggctttgagttagtctttgatagctctgatcccgactacattcccattcatcaaataaaaaatttagaatcttataatttagtttctgagttgagccttacgaatgaacagggaagccttgtaagacctgtctattgcgcggcagacattgccgctgagaaggaggaagagatcccgaccgaggatcactcgctctccatattaatgctacatgatcccgaagcccggtatttacataaaattttaaatctgcttcctccggagtattatgtagagtaccccctatggagcaacgtcgtattcgctttggccaatacatccgctaactatcggcccctcgccgaatggttttcgcaaaaatgccctgaaaaatggaatacgggaggaaaagagaaactagaaaaactttggaatgatgcctcgcaccacactgaaaagaaaatcaccaagcggtccattatgtactgggcccacaaacatgccccccagcaatacaaagaaattgtagaacaaggctacttttccattctcgctgaatatgtgtatagctataacggcatgcttgagcactacatgatcgccaaagtcatctatgctatgatgggcaacaagtttgtagtggacgtggattcaaacgggaagtacgtttggttcgaatttgtgctaccgggccagccaatgaatcagggagaaatatggaagtggcgcaaggaggtaaacccggatgagctgcacatctatatttccgaaaacttttcaagggtgatggaccgaatcacggagcacatcaaataccacctcagtcaaccccatgaaagcaatattttaaattattataaaaaactattaaaagcctttgaacgctctaaaagtaaaatctttaatgacagctttaaaaagggagttatcaggcaagctgagtttttatttcgccaaagaagctttattcaaactctggataccaatccccacctactgggggttggcaacggggttctctccattgagaccatcccggctaagctcattaatcattttcacgagcatcccattcatcagtacacacacatatgttatgtgccctttaatcccgaaaacccctggacaaaactattattgaatgcactccaagacatcatcccagaacttgatgctaggctgtggatcatgttctacctaagcacggccatatttcgcggcctgaaggaggctctgatgcttttgtggcttggaggcggctgcaatggaaaaacttttctaatgcgacttgtggccatggtattgggcgatcactatgcctccaagctcaacatcagccttcttacaagctgcagagaaaccgcggaaaaacccaacagtgcctttatgcggcttaaggggcggggatatgggtactttgaggaaaccaacaaaagcgaggttctaaatacgtcgcggctgaaggaaatggtaaatccgggcgatgtcaccgctcgagagcttaatcaaaaacaggaaagctttcagatgacggccaccatggtcgccgcgtccaactataacttcatcattgacacgacggaccacggcacatggagaagactgcggcattatcggtcaaaggtgaaattctgccataaccccgaccccagtaacccctacgagaaaaaggaagatcctcgctttattcacgagtacatcatggatccagactgccaaaacgcattcttcagcatactcgtctatttttgggagaagctacagaaggaatacaacgggcagattaaaaaagtgttttgtcccaccattgagagcgaaacggaggcgtacagaaagtcacaagatacgctacataggtttatcacagaaagagtcgtggagtcgccctccgcagaaactgtgtacaacctatccgaggtcgtgacggcctacgcggaatggtacaacaccaacattaacgtaaagcgccatattgccctcgagctatcccaggagttagaaaactctgtgctagaaaaataccttcagtggtctcccaacaaaacgcgaattctaaagggttgccgtattttgcataaatttgaaacgctgcagcccggcgaatcctacattggggtgtccacggccggcacactcctaaacacacccatatgcgagccaaaaaataaatggtgggaatggtcccctaatccctctgcccctcctgagaaagaagcgtctgcaccaactccttagggaatatccttagaagcatgtctttcggcagagccattaccggtagcaaaaaagcaacattgagtatattatatgccttagcctgctcataagcgtccttttttttcatggtattttatgtttttaaatatttttaattattttttaaatacgatgaacagttcgtgctccgaaggctgtttactaaaaatcggtgtgaatccgcattctttaaatatggtttcccattcggggatggtatggaaatccatgtctctacgaatagtatggtgcccaagtgcgtcctgcaggctgtgaagccagaaggcctcctgaccttgatgaaggtcgtacatgataagaaaaccatcaggtttcaacagatggtaaagcttgttaaaatcgtttatcgtaagatgatgcgccgccataggtaaccctatgagctccacagagttttcatgctggacatcgtccatatcggtataaaacgtttcacagtaaatgagacgcttaaacgagtatcgatgacaaacatttatttccaagtaggtttgcactacgtttttaggtatatcgggaatcatgttgattaaggttgtttcgggaaacttaatcatctgactaggcttcattttcaactctttaaaggatttcccggagaagtgaaaatgggtctttacgtatttatgtaaaaatacctgaatgggcagagggggctcctcctcttcgttctcgacgcctcccaaaatatttggaatttcctgacgtggcaaaagaaagtttatgtccacgtttacgaatccatcgaggacggacacaaagcttggctctaatctccattccatatactgtttagaaacgggagatagcataatcctaggcgtcacaatgcacgaagggtttttaatcaccgcatcgtggtaagaaaagtgtattccatttcttccagtataaagaagcctatgttcgtcgtagcagaaacaattaaggcggtatgcctcatacatacactgtttcaaagtacaaacacgttttaaaaaggtttctgcattggcggaggccaagcggttttgccattggtggaaggggttcaatcctacaatggccagctcgtttaaaatatcttcgcggcgcgctaaaatctgcaccatagaagaatactttagcatttttttttcgcaccattcgcgaagatgtttagctacattattaaccttattattgataaagtatacgatggcatgttggaagccttcaaaaataaagagcccctccaaaagatcatctgccaatagaagatggatgttggtgtaagcattgtcaatattttgtagaaacggcggaatgcctgccaaaaccgcttcagcaagcatagctccgttccgttgtttactgtccaatagattcgtaagttttttgtccgcaacagacacgacggctaggatggttgcaatgtcagaaatggcggcttgccagaaataacccgaaaagcacatgcgcgcttcttctatagataaaaacgaaaagcgagaggcaatgtctccgagctgcgtgagttgaagacctttttctcctctggttaaaaggcctgccacaatggcccgctcaatggctgatgccagcgcatccgtggggggaggatccagcatatcaatctcctctgccttaaacacgccttccttattttttttaatcgtttctacgacaatgctaagaaaaatggccccagggccttccgtaatgatttcaggatactgctgcactggtatttgctcaaagacgtgttttgtgtaaagcgggtaaaagtgcccaggaaatactctccctacacgcccctttctttgctcgatacggctttgagccgcggggcgcgtaataagccctcccgcccattcgggatagtaggtttcaatgcttctgttccacccgggatctatgacgtacttcagcgtttcaatggtaaggcccgtttccgcaacaaccgtggaaacaatgacccttcttaaaggtttttccactttagcggttaagggatttttcacccacagattcttaatttccgctttcaggccaaggtaggcctcattttcctgcgcaatcgcctcactatcgatcggcaaaatcaacattaacggcagcttttctttggcaaggtccatatttgcattattcagcaacatcgaaaggaagcgtatttcagccataccgggcatgaaaattaaaatatctgcttccgtgggacgatcatgaatgttttctttatgaatagtgagagccgtttcgcaggcggtcttaatgtagttgttggtgttatacagcggccagtgggtttccacaccgtactgtcgtccttccaccaaaataatgttttcttttccgataccaaaataggttgagtatttatgggtatcaatggtggcggaggttaaaattacaaagggaatacgcagcgcccctatgcttcctctttgcaacatgcgctgaagcatacttttaatatacatgagcataaggtcgatgcctagggctcgctcatgggcctcatctataatcataaaggcatagcgggaagctatctcatcatccgtcattgtatgtagctgcgccaacagaacccccgcggttgcataaataaggccccgattgggtttttccgtcagaggcttcgtttggtagcccactgtttggcctaatatcatgtcggggtagtgggttgaggcgccgatgtctttggcgagggtcaccgcggttaggactcttggctgggtacaaataaccgagcgtcccaagtatttttggaaagaatgcgtgttttcatttctcagaattctgaacacgtgtacgggtaaggccgtggattttccggaaccagtgcgtgactttataatgagcacccggtctgcgagggaggttggaatggcccctccaaactccgggagacgttgttttatccaagtgatgatgtaatgaataggaacatcattcttgtgctcagcgggcacgttatagagatgaccaggctccaataaagtcggttttcccatattctattgttttaaggattgattgttcataaatatttttatactctgaccaagaaattatttttttattaagccggttatttacgttgttatggaacgcgaaggtccagtactgccggagaaaagtcaaaaggggcaggcaattcatacaccaaaaagttttttttttctgctagcaagagcgtgtcaataattttaagctgatcgttaattaatttttggtttaactctttgttattatcaagatccttcgcataaaccgccatatttaataaaaacaataaattatttttataacattatatgttacgtcctgtagaaaccccaacccgtgaaatcaaaaaactcgacggcctgtgggcattcagtctggatcgcgaaaactgtggaattgatcagcgttggtgggaaagcgcgttacaagaaagccgggcaattgctgtgccaggcagttttaacgatcagttcgccgatgcagatattcgtaattatgcgggcaacgtctggtatcagcgcgaagtctttataccgaaaggttgggcaggccagcgtatcgtgctgcgtttcgatgcggtcactcattacggcaaagtgtgggtcaataatcaggaagtgatggagcatcagggcggctatacgccatttgaagccgatgtcacgccgtatgttattgccgggaaaagtgtacgtatcaccgtttgtgtgaacaacgaactgaactggcagactatcccgccgggaatggtgattaccgacgaaaacggcaagaaaaagcagtcttacttccatgatttctttaactatgccggaatccatcgcagcgtaatgctctacaccacgccgaacacctgggtggacgatatcaccgtggtgacgcatgtcgcgcaagactgtaaccacgcgtctgttgactggcaggtggtggccaatggtgatgtcagcgttgaactgcgtgatgcggatcaacaggtggttgcaactggacaaggcactagcgggactttgcaagtggtgaatccgcacctctggcaaccgggtgaaggttatctctatgaactgtgcgtcacagccaaaagccagacagagtgtgatatctacccgcttcgcgtcggcatccggtcagtggcagtgaagggcgaacagttcctgattaaccacaaaccgttctactttactggctttggtcgtcatgaagatgcggacttgcgtggcaaaggattcgataacgtgctgatggtgcacgaccacgcattaatggactggattggggccaactcctaccgtacctcgcattacccttacgctgaagagatgctcgactgggcagatgaacatggcatcgtggtgattgatgaaactgctgctgtcggctttaacctctctttaggcattggtttcgaagcgggcaacaagccgaaagaactgtacagcgaagaggcagtcaacggggaaactcagcaagcgcacttacaggcgattaaagagctgatagcgcgtgacaaaaaccacccaagcgtggtgatgtggagtattgccaacgaaccggatacccgtccgcaaggtgcacgggaatatttcgcgccactggcggaagcaacgcgtaaactcgacccgacgcgtccgatcacctgcgtcaatgtaatgttctgcgacgctcacaccgataccatcagcgatctctttgatgtgctgtgcctgaaccgttattacggatggtatgtccaaagcggcgatttggaaacggcagagaaggtactggaaaaagaacttctggcctggcaggagaaactgcatcagccgattatcatcaccgaatacggcgtggatacgttagccgggctgcactcaatgtacaccgacatgtggagtgaagagtatcagtgtgcatggctggatatgtatcaccgcgtctttgatcgcgtcagcgccgtcgtcggtgaacaggtatggaatttcgccgattttgcgacctcgcaaggcatattgcgcgttggcggtaacaagaaagggatcttcactcgcgaccgcaaaccgaagtcggcggcttttctgctgcaaaaacgctggactggcatgaacttcggtgaaaaaccgcagcagggaggcaaacaatgaatcaacaactctcctggcgcaccatcgtcggctacagcctcgggaattgctaccgagctcgaatttccccgatcgttcaaacatttggcaataaagtttcttaagattgaatcctgttgccggtcttgcgatgattatcatataatttctgttgaattacgttaagcatgtaataattaacatgtaatgcatgacgttatttatgagatgggtttttatgattagagtcccgcaattatacatttaatacgcgatagaaaacaaaatatagcgcgcaaactaggataaattatcgcgcgcggtgtcatctatgttactagatcatcgccagtatttaggtccccaatgcaacatttataaccttttgaaaaatctcattccatatagaggtaaatattttttttccatggagaatttttttgcactcttgaagggattgcgccacatcgtcaaatgttttttgttttccatgtattttggcgtaattccagccagtatctgtgtcatggtccttaatgtcatccgctaactgaaaggcatgtccaaaacaatgggcagccctttcaatcatcccaatgtcttcaacggatccagttcctaaaacccagcccataataaacgcgatcttaaaaaagggaatggttttttctggagtgtctactaactgaccggaacccgcgctgtttagagagtggcttacaaaggtacacagcagcgctcccagttggttgggatccggaaaccttggacagtgttccttaatccagtcgatttgccggcaaatattttgaaatccttgcatggttagcgccagagcgctcatctgcgccttggctacgccaaagcgggcccacactgtatctttatttcgccgcttcacatcgttgtcaaaggagggcatatcatcgataatcaaagaagctacgtgaaagtactccgctgctagggcggcctctgccggataaataggcgccccaaaggaatgttgcaactgacaggcccgaacaatttccatcaggataatgggacggatatacttcccacctcttagagcgtaagagcaaggctctgttagttgtcccttaaagtccccatcttcaatagcattatttaagatggtctcaaactcttcactaaaggttttataatttttaggattcagtggatgtattccatgaaaaagcgcgacactacgcggtgctgtgattctaaaatacttaggtttgcgcgtataggatattaaaataataataagaactacaatgatggagatatagatgagatgcaacatgctgagttgtctccccgcagggaatggtccttttccgcgcttgttaacggtaccgaggaggcgttgaaatctttaggaaaggtgctgtctagtttggaatctccaattcctcccgtatatttaggtatataattattgtgtctagaaattgtttgctttgaggtatcaaaatattcagcctgaccgctatttcttttagaataattcggtatagggcttgagtagttggcaatactcttaaaccggggcaccaaggtaacaatattttccatataatgggtttgatacgctttgtttaaaaatgggcttaccggctttatgcttgttagttgtgcattgagtaccggtatgtcttctaggatttgtggctttatagaatgattagcaaacacagaatgtagtatattagatacttgtagcatatgtctatttgcggaaaattcctggtattctctgccgtgttgcgaatctttgggcggaaggggaccaagcatcggcacgtccgtgtaggtactggtggattttatgagttcctgctctatgttcggtttgacatgtggatttcctaaaggaatacctctacctgcaatccctttttctaccgacgcaggtagattgtgcgctaaacacaaaatattgtacacgtctttgtgcggaatatatccgttatagtgctggcccggcatctgatcgccaaggtgctgctcatgcttaatggtaccctttgttctgagtttaggaagatcctcgtacgaaaaaaattttgtgtgctcgctgaacctcgtagaaggaaccgaactattttttgggttttttaaggaaggcaatgaggaaggctgggtcagacaatttttctgtgtgccctttaagctagccacctgcggaaatgtttttttttccgtacgaacaacattgcgcctaattaggttttccgtatgggttgaaaaagcaggacgatgatttttaaaatgattaaaaagtttattttttggaatggagctgtacggctccagatcttgcgcatcgccgtaaccaatgtttttgtgctgagggttcagcataaaagaaaagttacgtagatcactgagttgcaatcccttttcagccttttcaggactattagtgtattcattgtatacaggcgcggctccatttttgttgccgcagtaccgggaatttagtatattatcagaataccggttatgacgcggcaaatcgctttcccaaagaggtggatctgacctataatcggctaacagctttgaagcataatcatgatacattgtatataaaagttaattattatattgagaaggcataattacttcttgtaggggtacaagaggctttgaatcaggcaaactgacgggttttgaatcggccggctttggaccggcaggtatctttttaggttgatcttcttctagctcattagacacggatgggggagaaataggaggaataatttcatctccgcccttatatttgtcatggatagaagaaacaattacatccatgtttgatttattataaatgtcgtttaactggtgatttaaaacataataatgcaaaaataatagggctacaatgcatatatatacgtaaatagccgtcttcgtttttcgttttttatccaccggcggattacaaattgcaaaaaatacaactaataccaccgctgtaatgattaaggccacaatgaaaggattttgaaaggatgttttgaacggttcgcacgtataaattttttctcctaaattattgatacccgcaataaaatctacattcattttatatatttataaattatgaaaaatttagagttacatctccgccggaccaatcattgctaaaatttgaagattcttcaaaaaggcccgactggttgaatgtcttctgctcaggtttccaaaaattttccaagaatggattttgaacaataggctcatcttgattttcttcttcaaggatattttctttgatatcaagaacagcttctttaaactcaggtgtatcttgattaaactcaggtttatcctgatcaatcgcaaaaatattatcttcttcagatatatcctgtttaatcgcaagaatagtttcttcctcaggtttatcctgatcaatcgcaagaatattttcttcttcaggtttatcctgaccaaactcaacaatatctttctcgctaaatccgtttttagtgtgaagctcttggttttgaagagaattatcaaaatctattttagttgttgtcctagaccgtggcacgggatagttatctaatggtttacttactatagtcctcgaatgtggcacgggataattgtttggtgacttgctggttagctcttggcttgttaatagttcttgttttctcaataattccatctctactacttctttttgatccgctggtgtctctttttggtattcttcattagaaaaatgttcagagggtaatgtttcaataaactttgtgagtggatagctgctctttgatgtagaagagcgttgaatttgctgataaaggagttgaacaagtcgccggtattcactctgtcttttttcatattttttacgtagcgtggagagatctgctaagagcgacttgttttcagatgttaattcttcaatttgatgaagaaggctgcgattgtatgaactaagtcttgcatacgtttcttctaattctgtctccggctccacataggcctgttttcgcagaaatttattgtatagttccattctttttttgagcagaaaggtaagactataatcttgcatttctttcgtaactttatggtagttttctttccggtttttgataataaagggcagcattttttctgttgtgataaaggtgcccagattgctaatgtagtcgcacagtagcaattccaagatagattctttcttttcaaggcttatagattggctgtattctttaggtatgaaagaatcaacaatcgttgttacgaagtttgaaaagtttaatgttttgctgttaatttgggtaatgttacaaaaatatttgtaaaaactatctagcattttttcataaagttttttattttgtttaacccctaaaatatagccctttacttgatactgatattccgtaacaatggaatgttttttgtatagtgcatttttgtataaaaagttataaaaaatgttgataaaatacgcaccaagggtttcaaaaatacttataacgtgggattcttcctgatccattatatcatatgtaatattattttaataaaaaattactgacgaataacatgcaaaaaaaatatgtttaaacttattttaagctagcacttatttaaaagtgttttaaacacgttttaaattgtatgttaatacacttaaaaattaagccgaaatttgctccaataaggattacttttatcaatgaccacctctttactataaacggctttacataattttaataatgctttagagccaaagctgaaggcagtgggaagcggcactgtactatggtaaaaatgttgccgatgttcatcctcgcggatgtacacaagtttcctatatcctttaaacacaatatggctaatttcttccacatactccttatcctgtttggaatagcggttgctttgacgggaaaaattcgacatacaaatagaggcatttgtaaaaatggaaacaaatgcgtttttacgaagattggcgggtaaatcggtatcatcttggcagcaaataatcatcgaaataaaacagtgacgattttggtaaaaaaactttttaaaaatttcttttgtaaataatgggtgcagttcggccgcgcagtcgtctaatattaaaagtaaacgaggattaagattgatatagtttaacgtaaacttttcatcctctgtaaggcataagtttttatacatatgaatgttctgtataataattttttttaaaagttgctgataaagcgatgtaatcttttcttcttttttttggtccgtttgttcagcctttaagcactccacttttgcaatatttttgttttccttttgctgtatatcgatcggaagtttatgatacaatgtttttagcatatcgatgttgtttactcgactgtagatggaggacatcatagtttgccgctgccagatggcctccaaaaagcgttcagcgcccttgttgtcattttttttttgcttatcggcgagccacaagcggtagtgtattagagttggatgtacaaaaccctcatatgaacgatttgagggttccgagggggcaaccactaaaatttgttcaatatggggttgcaggattttcataatatgtttaacgtacacggttttgcctgtttttgaggggccatatagcacagttgttttatctataaaatgatgtgctttgaactgtagttcaggaattagcttccctgaatgggtcgttagggccatctctatattattacaattctgcttttgtatataaaatttctttttcgagtttattattattgttgacccacatatctacccgtatcgtatcatcaggcacattgagcatttcaagcgcattatctaactgtttttttgtttttatcagctcgctttcttcatcgggggttaaattttctttactaagcagttgcttaattttttcttcgcagtcgtctataaaatcatactctcgagcttttttgatatttccagatgctttttctaggttttttagctccttaaaggaaagcagtcccttaatcccgctatccgtgtgaaaggttgaattatagatggagagccccggagcatccgggccagtttcttgtatattttttgcttttttgtggtaaatagtatttcgtaaaatctcttttcctatctttaggtcttcctcatgacggtccaaaatccgttttattatttcattattttgattaaaataattgtagcgctctctgttggccttaaagcttcccaggagtgtccagttgcctaattgaatggatgaaacctctgagaaaatctggtctttatatttataataaaattcatcaaccttttgttggttgctgctatccaccacatcataaataatgaaggcaaactctaggtcgggtttttctgggtagatgctttccgtagcggcccgcaactcttcgtaattatcctcaatgtaataattccacttataaaaagtatcctgaggtggaatatgctgcgaaagatatctagtaatttttgtgttaaagagaatgggtttaaacgccctcggattttcaagcatatgtttaatgctttggtgaagttctatattttgtaatatgtgggctgctgccctatagccctgtggggtttgggtgattgcatcaatatcggcctgaagctcattaggcacatttaatgttttttgcatgatgtgtaaagggatgcgctcaggatctgctaaatcggtgtattctgtgcttgtacaagtgcttgcacaggtatctacattggtatctgcacacatgcttgcacaggtgtctacattggtatctgcacacatgcttgcacaagtgtctacattggtatctgcacaagtatacgcactttgagcatgaagattaggatcaaacacaaaatgttctcgtaaaaagctatcgatcgttgttttagcttccttgcttttctgcgtctgggttttgcagctatctgctatagataaaattgtatttactaccgattcagagggaacatcattagtttcctgtttcaaagtatcaactaacgttattagctcactgagaagagttttggtcgtgtgggtaggttttgaataggaaggcatccattcctgcagagctttgaagacatatccaataaagctagtcattataagacgtcgaatatactgctcccgcaaatttgtaaaagagcaaaaggccaccctgctatcatttttgaactgtttgtaagggttcgtcctttggtaaagctgtttaagcgtttcttcggatatttcagtagagggatcctccaatacgtttttgagaagctcatcaatattaaattctgccatatcttagagtttattatatacatattaaagctttaatataaggggggtataacaatggacgaaatcatcaataaataccaagctgttgaaaaactttttaaggaaattcagcaaggattggccgcgtatgatcaatacaagaccttaattagtgaaatgatgcactataataatcatatcaagcaggagtattttaactttttaatgattatttcaccttatcttattagggcgcatagcggagaaacgctgcgaaacaaagtaaataatgaaattaaacgtcttattttggttgaaaatatcaataccaaaatatctaaaacgctggtaagtgttaattttttactacagaaaaaactttcaacggacggggtgaaaacgaaaaacatgtggtgcaccaataatcccatgctgcaggtaaaaacagcccacaacctttttaagcaactatgcgacacacagtccaaaactcaatgggtacaaactttaaaatataaggaatgcaagtattgtcataccgacatggtgtttaacaccacgcagtttgggctgcaatgtcctaactgcggttgtattcaagaattgatgggaaccatttttgatgaaacacatttttacaaccatgatgggcagaaagcaaagtcaggtatctttaaccctaaccgtcactatcggttttggatagaacatattcttggtagaaatccagaacaagagttggggaccaaacaagatccctgcggaaccaaggtgttgcaacaactaaaaaaaattattaagcgcgataataaatgcatcgcgcttttgacggtcgaaaatattcgaaaaatgttaaaagagataaaccgcacagacttaaataattgtgtttctcttatattgcgtaaacttaccggagtagggccgcctcaaatatcagagtcgattttactacgaggcgaatacatatttacagaggcaattaagatacgggaaaaagtgtgtaaaaaagggcgtattaataggaattattatccgtattatatatataaaatttttgacgccattttgcctccaaatgataccacgaatcgacgcattttacaatatattcatttgcaaggaaatgatacgctagctaataatgatagtgagtgggaatctatctgtatggagctccctgaaataaaatggaagcccacagatcgaacccattgtgttcattttttttaaagatgaagattttttagatgattttttttagttttttaaaagacgaaaaaattttttaaaagatgaatattcttaaaccccgcaaattacttttttttaggtactgtaacgcagcacagctgaaccgttctgaagaagaagaaagttaatagcagatgccgataccacaagatcagccgtagtgatagaccccacgtaatccgtgtcccaactaatataaaattctcttgctctggatacgttaatatgaccactgggttggtattcctcccgtggcttcaaagcaaaggtaatcatcatcgcacccggatcatcgggggttttaatcgcattgcctccgtagtggaagggtatgtaagagctgcagaactttgatggaaatttatcgataagattgataccatgagcagttacggaaatgtttttaataataggtaatgtgatcggatacgtaacggggctaatatcagatatagatgaacatgcgtctggaagagctgtatctctatcctgaaagcttatctctgcgtggtgagtgggctgcataatggcgttaacaacatgtccgaacttgtgccaatctcggtgttgatgaggattttgatcggagatgttccaggtaggttttaatcctataaacatatattcaatgggccatttaagagcagacattagtttttcatcgtggtggttattgttggtgtgggtcacctgcgttttatggacacgtatcagcgaaaagcgaacgcgttttacaaaaaggttgtgtatttcaggggttacaaacaggttattgatgtaaagttcattattcgtgagcgagatttcattaatgactcctgggataaaccatggtttaaagcgtatattgcgtctactggggcgtccagctataaaacgtgactggcgtacaaaaagtccaggaaattcattcaccaaatccttttgcgatgcaagctttatggtgataaagcgctcgccgaagggaatggatactgagggaatagcaaggttcacgttctcattaaaccaaaagcgcaacttaatccagagcgcaagagggggctgatagtatttaggggtttgaggtccattacagctgtaatgaacattacgtcttatgtccagatacgttgcgtccgtgataggagtaatatcttgtttacctgctgtttggatattgtgagagttctcgggaaaatgctgtgaaagaaatttcgggttggtatggctacacgttcgctgcgtatcattttcatcggtaagaataggtttgctttggtgcggcttgtgcaaatcatgaatgttgcataggagagggccactggttccctccaccgatacctcctggccaaccaagtgcttatatccagtcattttatcccctgggatgcaaaatttgcgcacaagcgttgtgacatccgaactatattcgtctagggaatttccatttacatcgaatcttacgttttcataaagtcgttctccggggtattcgcagtagtaaaccaagtttcggtacgcattctttgtgccgggtacaatgggtcttccaaaaggatctacaagcgtgtaaacggcgccctctaagggtgtttggttgtcccagtcatatccgttgcgaggaaacgtttgaagctgcccatgggcccccatctgggacgtgccctgaatcggagcatcctgccaggatgaatgacatgcacccaatatatgatggcccaccatatcatggaaaaagtctccgtactggggaataccaaaggtaagcttgtttcccaaggtgggggtacccgtatgcgggcgtactttattgtattcaaaccctactggaacataaggcttaaaatgcgcattaaaatgcaccaaatgtgtttcttcgatttgactcaaagtgggttcgggatcgggtttcccataacttttgttcacatttttaatgttagagatcctgctattcagcaagtcttgggccaatataatcttgtcggccttcccatcgttagcaataagacaaaaagctcctcctgatgccatatataatgttataaaaataatttattgtttttattaaatatggcggtttatgcgaaggatcttgataataacaaagagttaaaccaaaaattaattaacgatcagcttaaaattattgacacgctcttgctggcagaaaaaaaaaactttttggtgtatgaactacctgccccttttgacttttcctccggcgaccctttggccagtcagcgcgacatatactatgccatcataaaaagcctcgaggagcgcgggtttactgtcaaaatatgtatgaaaggggatcgtgccctccttttcatcacctggaaaaaaatacaatccattgagataaacaaaaaagaagaatatctgcgcatgcacttcatacaagacgaagagaaagcattttattgtaaatttttagagtctagatgagcttttacgcaatgttgtacagtgttgtatatatgtcttgtaagcatttgttgtagagtaataagtaaaagataaataaaaatgactattaaaataaagcccaaaccattaaaaatatttttatctgttagatttaatttaataaatggctcatggaatgtgtggtgcgccgctgcatgaggtgtggccgcatgggatgtggtcgcataagatgtagctacatgggatgtggcatttgcttgcatgtaaggatcatgatgtgttgggtcttcatcccagcaataatcgccatctttatctagctgaattgtataccccattatatatcacttattatttttttttaatgtttcatgaatttcattataggcggtgaaagggtcctcaggccccttctgtaaaagattatagagatcttcggacgctttatgtttcgtgcgaattaaggcgggatataacaaaagagagggccccagttccaaacaaattttacttagcgggctcatattttgcaccaagtttcccactacttgcgatgtttcataacgcattttaaagagctttatcataaaagtgttatgcaggccggtgtagtctggcctatagttaaggaaggggatttctctggtaccgtcaaacacgatctcaagtcctctagcaagcccgatcaaaatttcttcagcaatggatgagtatctaattcctacattacgaagcgtaagcatttctataacatcatctatttcctgcatagaggaatctattgtaggaattttaatatcatctgtgctgatttgttcattcccaagataggtaagcagcatattaattttttctagctttactagcttagtcttacgctcataatcatgatcttttttataaaaagagttgggatcaccgttggaccgtagatgattaataaggcggtctacttgctttgtactaggtttaatacttttttcactatactcgctttcagcatagtggtttttacgatctcttttagaaatagctgttttttgagatgcctcagactctgcatatttttttctatgcgtagaaagagaataaccgcggtcattacgtgaactactgttgcatgcaaggcctcggcgcgtcttaccgctgcgcacactgccattgcgtatactgccatcgcgcacactgccgctgcgtatactgccattgcgtatactgccgctgcgtatgctgccgctgcgtatgctgccgctacatacactatcactacatatgctgtcagtacatacgctatcgcggcgtatgccgccgtgtaccttatcgccgcccctacccgagggttttttagatataatactgtgtggggagtcaagcgaaaattcagggtcattaaagttaatgcccaatgactttgccaatccattaagctcttcatcaaaatgatcggtaggaaaactttgttgcttgcccatgacctgtttttcaagttcctccaaattggcttgctcatttatatggagattattcataagcgtcgtaattccagcaagatttgctccttctaaaaatgtggtgtcctccatcggatatactatactatttaaaagcttttaaataaaaatgtgtttggaagaaatgctctcttcaagcgtgtgtagctcagatataaatgcctcctcagaaagctttccaccatactcctttctcatcgtataggagggcgccggtttaatgtaggaaatccactgggaggtaaaaaaccggtacaacatatttagcagctcgcgggcctcccaccttttgggctccgtatagtgcacatcaacataagaggcggcgcatgaaaagctgcaaaagttgccgagaacgcccatctcaatctctcctcgctcattttcacgcatataggtgggcacgaattttgggacagtcttgaaatagagatgacatgtccagcatttaaagctagaatgggtaacccatttggaaacagtggtgaatacggagggtagctttttttcgacctcggcttcatcgtcattcgtatttaacgtatcggtggcagtttttttggattgcaagcattcttcaatggtaatcccggataagtataaaatattaggacaattagtttccataattttgatagttatttttatacaacatggatttaattaaagataaatggaggacgaaacggaactgtgttttcggtcaaacaaggtgacgaggcttgaaatgtttgtctgcacatacgggggaaaaattaccagccttgcatgttcgcatatggagttaattaaaatgttgcaaattgctgagccggtgaaggcattgaactgcaactttggccaccagtgcctaccgggctacgaatctttaataaagactccgaaaaaaactaaaaacatgttgcgccgtccgcgcaaaacagaaggcgatgggacttgcttcaatagtgccattgaagcctccattttgtttaaggacaagatgtataaattaaaatgttttcctagtaccggggaaattcaggtcccgggcgtcatttttccggattttgaagacggaaaaaacattatacagcagtgggtagacttcttgcaacatcaacccattgaaaaaaaaatccagattattgaatttaaaacgattatgattaattttaagtttcaaataaacccagtgtctccccgcgtcatcattcatttaaaaaaatttgcagctttgttggaacacatccctactccatatcccatacgtgaaataaagcctccattagaagactcaaaagtatccgcaaaatttatggtcagtccgggaaaaaaagtacgcattaatgtttttcttaaaggtaagataaatattttaggctgcaacacaaaggaatccgcggagaccatttatacgtttttgaaagatcttatcagcgtacattggcaagaaattttgtgcgtgttaccggtacccgattaaagaatgttttcattaataaggtaatcgactatgctaaaaagaataacaagaaaaataccttgaagaactataccaaagtaggtaggttttctgcatgtcacggcatggttaaaattgctaataatgtagtccacaaaagcattgctcaatacgactaaaaatagtaaaaaaaggataagtgctctttttatatccatatactttaaaacttattttttacactaataatttcctgcggccgcaatataaactgtaggtcatctataacgcccagacctgttaaaagtagagtactatgttttaagggatttaaaatatccgccgcaagaatgtgaatataattttcaaagtggtttacaggaatgcgtaagcgtttttttttgcactgcggttggtttagggtcgaatactggcaggaggtatatatattaataagaccgcggtcgatggtttcaatatcttcatagaattcaatgcgcggcgtcaaaagttttttaagatgttgacataactcatcatacgtgtaggactggaggggggaaagaagggtgtagtcaaagttaaaaatgtttttttgaagaacctttaaagcatgttccgcgtccgtggtttccaaaatatgttttatggtatgaatgtcatttaaatctacaaagtctgacagctttgtgtagaactcggtgacggaggttattttctggaaatcggttttttgaaaaagattttcaatgtgtttgcgggttgagttgctttgcagtccatacaagacatcaaaaaattcaatcagcaaaaacttatacaaatggttaatataaaaagctttgttggccttattctgctgaggatatggttcctctaggggatatagaatggcttggtctatatccctaggatcaatagtcaatgttgcgatgggaagcttttccagcgtagcgggaagagtttgggttggagcgtagtaaaagtatagcccggtttttccctctgaaagaaagcccacaaattctttttttatattttgcagcaccgctgagggtacgatttcgtactgtttatactgtttgttgaaaagggtaataaatttccaggtttcttcaaagcttgcaatctgggtgggccgcagatcaaagtcgatgggaatgtcgtcatgaatgtaggatgatagtcttataggaaaataaatagggcgatcggtgtctgaatcgataagtaaagcataacaaaagttatgcctgttgataagttttttaccaaccgtgtagccgggaatgtttttcacgtcatggatatcccaccagttatccttgcacataaactcgctcatagactggatgacctccatcacagggtcatcttcggtaaaaatatactgggcctcactgtttttcagaaatcttttttgctgggtgatggccattgggtagatcccttcgtccgtgtcaaagataatggctatcttcttcgatgggctaagaattttttgtattgtgctgggggacacctcaaacccgatgtcgccctgtttatctttaaaaaagacacagtgaaggtcgtagcatatggcaacaaggtccagaaagatgtcctgccatgtggtgtcccattgaagcagttggtttttttgttcaacaaaggtttgtaagataaggtttgccagctccgcgccgctggaaaacatgttgccggccccattccccaaaatatagtactgcggtgtgttggccgcctttgcaatttcaatggcaagggccttgggggcaagatccaaaattcgagcaagggaataaaaaagcccggcattgctaattccaagcatggtttgctccacccccacaatgcaaaaaatgtcgggctcttttatcgtatttaaaaacagttcatctgctatctggtggggtagaaaggcaatccggttcaccggtattttttttccataggacaaggtatgacgcgatgtttgtgtattaagatcctccaggtcttgttctacaaacgtgtgcttggtgaggcaggtattgttaatatagaaccgctttgtgcccagcagggccttcgtcttttggcagcacggcagacagtaatttagggggtggcggccttctagtaggcttagatgagggtagtcaggatgcgggcagctatagtaggcaggtaccccctccgtgaaattccaatactttactagctccttgcgcttggctggcggcatggacttcacctcggcctctgagtaaatgacgggtggccgtgggtgctggcataggacggagtaaaccgttgcctgcgtgtcgtacttgcgcaggtcatacaggtcggggtcctgttcttgaagcgcacgtagctgagaggctccctttccttgttgtttatcgtgcagttgagagagtttattaaccaaaattttgtcaggcccggtgatcaagttatctaaaaacacaaataggtaaacccaaagatagttaaactcttcctgggtaatgttaaacatttctattttgatatctgtaaccctatggtagatgcgaatgttgcggccgccgtagattgtttcccaccgggccgcaacatttgtgtcaaagaggtacgcatacgtgttttggagcaacgcaacattgatgtccattttgcgccccggaccggaggaaataatgatcatccgttcgatttcgtggggatcatacgaataaatcccctttttaaataaaaaattgtagaccccggtttgctggaggccccgcacggaaataatccctgcttgctcgtattcccgccaacgacttttgagctcggtaaatcccttgctagaaagcgtatagggccaaaaggtggacaccgacatggagctgatagaaatttggatgtcctcgttggagggaaggggcagactccctccacgaggaaacgcggcaggccccatatcattaattgtatgaataataggatttatgaaattatttagggtggacaccacggagttaaagtcgtggcgctcgttttctgaccaattgctttcgataaagtagtgcccattattttgtatggtaagaataaaggcctttttattgataaagcgtattaaaataatagtgggtacacggaatgttttattgctgaatttttcaggctccgtggaagttatgtggtgtttggaaaccacggtgggacctgttttactataaaagaacaccaccagctgaggaatatcgggagtagctggaaataggtcgaaaacattgcgcacattaatttgaatatttacgaggggtgaaattttaatcattgccgaggtgacggccaacgtgccgcgtgttagtctattcccctcgtacttggcaatgacttgttgtgctctggcatacgtaaagtttattagtttttgctctaggagaagcctctttttaagactggtcaaggatggagaaagagcaggatactgtttttccatttgtaagggagattgtaccaatagtttaaaggcatcgggggaaagaagaggccaatacttcataataaggccgtaatagagtaagtcaaattggtaattatcctctatggcaatggagatttggcgccgcatgggggccactagcgtgttgaggtctgctacaaagatgtgatgaatgttttttatgagctggaagctgtcgagcgcttccacatagagctcatctttttgactttccatagatgcgtcgatgttcaccccacccacctgttgaaactcctttttgtagtcgcgaatgtctaacgccaccccgctaccgcttaacaataggcgatacgttacctgaagcgcattgttttgaaaaaagaaaatgtgttgtctataaggggggatccctgtggcaacgtaaattttttctcgaatgtctttaaaagtgtcttcagggaaaatactatactcgctatacatcgtctcaatttctggcatcatcacgtttgtctcctcgccacgatcctccacaaaaagtttttcaaactcatctaaatcatcgctatctccacccaccacgtattgggaaagctttttctcccaatcctcgccgtaaaaattttgtaaaatttctttgtccttaggggttcgctgcaggtctttgcggcaggcctgtaacacgtttgcaggaacggatcccaaaaaaataaacgtcttcgtgtactcattttccacaggattataaagagtaactcgtagaggatttgttaaaaagtcattttggaaatccattatacccggtatagaaaataaaatttaaaataaaaacggatgatatctatcatggaccgttctgagattgttgcacgggagaacccggtgattacccaacgagttacaaatctcctacaaaccaatgctcctctactattcatgcccattgatatccatgaagtacgatatggagcctacacacttttcatgtatggttccctcgaaaacggttacaaagcagaagtaaggattgaaaacatcccagttttctttgacgtacagattgagttcaatgatacaaaccagctttttttaaagtcgctactgacggctgaaaatattgtgtatgaacggctggagacgctcacccagcgtcctgtaatggggtaccgcgagaaggaaaaagagtttgcaccatacattcgaatattttttaaaagcctgtatgagcgacgaaaagccattacttacttaaataatatgggctacaacacggccgcggacgacacaacctgttattaccgaatggtttcccgagaattaaaactacctcttacaagttggatacagcttcagcactattcctacgagcctcgcggcttggtacacaggttttccgtaacccccgaggatcttgtttcctatcagaatgatggccccacagaccacagcatcgttatggcctacgatatagagacctatagccctgttaagggaaccgttccggacccaaatcaggcaaacgacgtggtgttcatgatatgcatgcgcattttttggattcactccacagagcctctagcgagcacgtgcatcaccatggcaccctgcaaaaagtcctcagagtggaccaccattctatgctcctctgaaaaaaatttgttgttaagctttgctgaacagtttagccgctgggctcctgatatatgcacagggttcaatgattctcggtacgactggccctttatcgttgaaaaatctatgcagcacggtattctagaagaaatctttaacaaaatgagccttttctggcaccaaaagctggataccattctaaaatgctattacgtaaaggaaaagagagtcaaaatctcggccgaaaaatcgatcatttcctcctttttgcatacccctggatgcctacccattgatgtccgcaacatgtgtatgcagctttaccctaaagccgaaaaaacaagcttgaaagcgtttttagaaaattgtgggttagattcgaaggtagacctgccgtaccatctcatgtggaagtattatgaaacacgagacagcgaaaaaatagccgacgtggcctattactgcattatagatgcccagcgctgtcaggaccttctggtgcgccacaatgttatccccgatcgcagagaggtaggaattctgtcatacacctcgctgtatgactgtatctactacgcgggaggacacaaggtatgcaatatgctcattgcctatgccatccatgatgaatacggccgtattgcttgcagtaccattgcccgaggtaagcgggaacacggaaaatatcccggcgcctttgtgatagaccccgttaaagggcttgaacaggataaacccaccacaggtctcgactttgcgtcgctgtacccctcactcatcatggcctacaacttttcgccagaaaaatttgtagcctctcgggatgaggcaaatagcctcatggccaagggtgaatctcttcactacgtctcctttcactttaacaatcgtctcgtggaaggatggtttgtgcggcataataacgttcctgataaaatgggattgtacccaaaagtactcatcgatctacttaacaaacggaccgcccttaaacaagagcttaaaaaactaggtgagaaaaaagaatgtatccatgaatcccatcctgggtttaaggaactacagtttcgccatgccatggtagacgcgaagcaaaaggcgttgaaaattttcatgaacacgttttacggcgaggcaggtaacaatttgtcgcccttctttctgcttcctctagccggaggagtcaccagttcgggtcaatataatcttaaacttgtctataactttgttatcaataaaggttacggcatcaagtacggtgacaccgactcattatacattacatgcccagatagtctttatacagaggtaacagacgcatatttaaacagccaaaaaacgataaaacattatgagcaactctgccacgaaaaagtgcttctgtctatgaaagccatgtctacactatgcgccgaggtgaatgaatacctgcgacaagataatggcaccagttacctacgtatggcctacgaggaagtactctttcctgtgtgctttacaggcaagaaaaagtattatggtattgctcatgtaaacacacccaattttaatacaaaagaattattcatccgcggaatagatatcattaagcagggtcaaacaaaactcaccaaaacgataggaacgcgaattatggaagaatccatgaaactacgccgccctgaggaccatcgcccccctcttattgaaatcgttaaaacggttttgaaggatgctgtggttaacatgaagcagtggaattttgaagacttcatccaaacagatgcgtggagaccggacaaagacaacaaagcagtccaaatctttatgtctcgcatgcacgctcggcgtgagcaactaaaaaaacacggcgctgcagcatcgcaatttgctgagcccgagccgggagaacgcttctcctacgttatcgtggaaaaacaggtacagtttgatatccagggccaccgcacagattcctccagaaagggggacaagatggaatacgtctctgaagcaaaggctaaaaatcttcctattgatatattgttttatatcaacaactatgttctaggcttgtgcgcgagattcattaatgaaaatgaagaatttcaaccccctgacaacgtcagcaataaggatgaatacgctcagcgccgagctaaatcctacctacaaaaattcgtgcaatccattcaccctaaagacaagtctgtcattaagcaaggcaatgttcatcgacagtgctacaaatacattcaccaagaaattaaaaaaaaaataggcatctttgccgacctttataaggaattttttaacaacaccacaaaccccatcgaaagctttattcaaagcactcagtttatgatacaatactttgatggagaacaaaaagtaaaccattctatgaaaaaaatggttgaacagcatgctacggctagtaatcgagctggtaagcccgctggtaatccagccggcaatgcgctgatgcgggctatatttacgcagctgattacggaagaaaaaaaaattgtacaagccttatacaataagggggatgcaatacacgatcttctcacctatatcattaacaatataaattacaaaattgccacgtttcagacgaaacagatgttgacgttcgagttttccagtactcatgtagaactgctattaaagctgaataaaacgtggcttattttggctggaattcatgtggcaaaaaaacatctgcaagcttttttggattcatataacaatgaatcgccgtctagaacattcattcagcaggctatagaggaagaatgtggcagtattaaaccatcttgctacgactttatttcctaatacttcttaagaaactctttaaacaaggacttcgcatggtcaaaggttctaaacccatggcccttatgattcgccaaaaaagcggtttcatcaagattttctaaccctttcacggatgaagaaataaggtgttcggcctcgtttgcccattttctatgattttttttcacctcgggttctagatctgttttctccatatactcattgtggtcatatttttttttgggaggaggcgtgggtggaggaatgggtggaggaagtacacccgactttcccgcttcaaccgttttataaaaaaatagaagcataatacaaagaataaggactatcgcaaatatgataaccagtgtcccagtcgagggcattttgttatataagtaacgttttttttattttttataattcgaatgaagaaccatgttgaatagtcttctactcaaagacattttgttatacggtaaatgagaatttataaaatccgaatatcactatcatactgtttatctgagaaggtctcactgggtcctgtgatggagaacccatactctgtaatgctggggtttataatgtggtcaggactgacaagcacatttctgaactgcgagagttctaggtttagacgcagtcgtaatagtcgctgtatatttgtaataaatattagattgcgtatgaggcgagtgtcaaagcgatcctttccaatttgtactaaggtgggcttttgtattccaactcccacttgtttaacgatggaccagggtccttcttcccgattttgttccgtgatataggtcagcacactattttctgtatatgaggtatgatgtcgcatattaatacctggtgccattccaactggcggttgtgcaattcgggctgtaccgggacccaaccatcgtggagttttataaacatatcgttctagcgtatttaaaaattccttaaggttatttacgagtagcatgaagggtgctattaaaacaggtggatggtttataaccattgtcataaaccattgcattgcttcaatatcattttgtaatgcttgacggggaggcggggcaggtaatccacgtatgttgaataaagcggttaattgtgcaccggctgtttggggcgtaatattttgtattaaatttatcatcgaattggcttgcccggcatttcctataagatcgattaaattggttatttgacctcgatattgttgtacccagttttgaatggcagcgatgatctcaggggttggattgttttgaatttcaggtgtttgtattagattattcacttctcttcgtgtatcttcaagctgagtcctaaatgcatttaactcgcctataatttggtttctatcaataacatttcttaaacctcgaactgtttcagccaatcgtatagtacgcacaatttcatgtaaggcctggtttatgtatattgacatgggatggccccaccgctcacgtccacgttgaatacctgcggccaaactaggacctgcctcgtcataatcaaattgtgtaggataaaggcttccaaatagcactttattgaaaatttggtcagaaagaaatttagggcggcccatatttagcgcgttgtcccctctaaagatgcgtgacatgtatccggcgttgcctttggatagtaactcattcccatattgagtaatagagaccgagacataggggtttataagaagttttagcataaattctcgagtatttatggggggacgattcggaatgtttaatacctctgcaacatctggttgaggagccgtggtgtccagagatcgtactttttcagccgaaatgccgtacataagacaagcaatttcttcaaaactatagtcatagttgtaaatattggcaagtggtatagatcgcatcagcgcatttacattgataggtataatattcatatcaaacaagttaaatatgcgctcgcgctctctattagagccaagagtgcgtgtttgacctttcggcgacactattttgtgaatatgattgatttgctcctcttggtaagagctttccacgaaggaaattacgtcttgcaatgttttacgaagcgaatacactgcattcatccctattcccgctgttataatgggtttatcgtctctgttctcgctaataagattaactccaccaaaagtattttcattgtacatcatcactgttttaaaactacggatatttatgataaatcggagagcctgaatggcgtgggtataaaagtgttcaaatcgcgtgggagtaatttgttcgcgagcaactaccgtttcattatagtttttcatgataagctgtactccgggcatatctgagagctgtaccggatcatttcccagtaattttcttgtgccgtatagtagtttaaactcgggggagccgctttcaaggttcgggtaaagaagaggatcatatacctcattattttctattcttaggtcatgtaaataatagagcgaaagtgaaaatggcataagaggctccttattgtaccgggacatatagttttgaatgaagtgttcttctgtttcaagatagatgggatgatcggtaagctcgtgcaggacctccatggcagaatctgccagagtgtgagagcctctaatgatcccgtcgatcactgcgaccagtcgctttcgcacaacatcgctcgtattattttgtgcgtctcctaggggcataagcgtaacattgggacgaaatacgccgccaattccccgcagggccgcctgaccgacggatagtcctgtcgcaggaacattgttattattataataaataacggaatcattattggctcccaagagtgccgtcagattagggcgagctagttggacatttgtgtattgtataaattgttttagaagctctccctggctaataagaatattaaacattttgttaaatagtggaagattggctctataattttctttaaggtaaatgggaatttctgttaaagtagaaataagatgctgactcaggccctggcgattggtatccttaataagccgctgaagtataagtcccaaagacagaagaagcaccgactgctctgtggggtcgcctctatgaccaaagacgttgttattgcgtgctaagtcagggtgagcatatcccatctccatcactgcttggctaaagttcccattagcgaatgcattaataagatttagatatatttttccgctgggagcatcataaaatcgggtaatatatgaagctatgagctggttaaacaccatcatcatactacgattattttgaataccatagtctgatccgtataggcgataacgtcgaaggttgtttgcggcatcattgacattggcataggttctgagcgctatgttgtcccagtagctaagagtattttcctcctgggcgttgttggtacgaataagattggagagtctaaagtctcctagtgccacctgctctacacgaagtccagagttattctccaaagcatcgtaaaatacgagtctactgaatactcttccgtattgttcaaagcgttcagaggattggggattgttatttatttgaatattagccgcgtcccttctttgcgccccacctcgaagttgcagtacattataaggctttgtaagcaaggtgtaggttttattaatgatttggttaaccccctccaggcccaattcaccgccaggaagcggccttcctccggcatcggtaggtggtttaataagtttgtcaattaaatgttcttccaaccagtaaaatgagccaggattagatctattttcatagtattgaataatgtttttatcaatatgcgggcgtagaagatcaagaaaatacttcgtgtcggccatcaaagaatcaattaaggaaataagacctgtaaaatctaaatgcacttgagcggtgctggtttcagggaagcgaacttgaaccattttgttaaaactggaggtcatttcgaagatattggtcaacaggagctgcatgattcgctgattatctactaaataccttgcggccaactcttgctccggacgaactcctccaccagcaggaatacccacatatggtacaatccaagcaaaaagagtttctgtggttaaatttcggtcttgggctgctgcagccgcttcggtagtgggatcagggtacaccatagaaagccgcatattgatttctttaatgactaatcctggatttctaatctcagagatggccccgtgttttcttccgagccagtcaataagattggcgcggttcacgttggcagcttgtgtctctcgtaaccattcgataatgcttttttgaatcgtatctaggtctaaacctttaatgttattacgaaagttattaagaagtacgtaaatagcactcaataagttaagacctgtaataacggtttcatgaaacagaaatattttgttaacatctgtatctgccagtgactcagagccttgaataagttttgaaacgatttgaattttatcggtatgctcctttttgagttcattgatagcctggcgaatgagttcttggtaggaaattttgcccaattcttgttgcagactgggatcttcaaacatctcactaagctgtttcctaaatttttgtaccaaatcccactgggagttgggctgcagcattcctgtttggacatccacagagtctatattgtatagtgccgggcgccacttgggggtaggctgggttgaaggactaataaacctatcggagggaagtaattgtgaggattgtgtatagccatcctcatcaggaagaatggagtagttggtttgattcatcattccaaaatcattcatagttcgcgcttcctgaacaatgcgttgaaatttttcccattcggtgcgtgtaatgacaccgaatctgcggtttatttcatttacaaaatggataagcgcttttttggttgcttcttgttcaccatactctaagttaaagtgttggtaaatgacgtttatttctttgataagctgacgaatttcggtttctgagtagtcaccaatgttaataagctcaataggacgcataaagataatgcgaataagtcctgagaagattccttccagctcaggaagcatcgagatctgtacattttcatctctaaaggaaaacaacttttgataaaattcggcgaggcggggaaggcggaagtaaagctctgctgcctcgggaattacctcgggctctagctcatcggcaccccccaatatcatacgcgtgggtataagtttgtacacgggctcaggccgttcaaacatgtcgtaaatccctaatacaataaaaatcttggcggccatacttttcagcatgaaggtgaagaagacgtcctcggtttcccagcgggttgatagggcgtcgttaactctcacagtagagaggtagacccgctgagccgcttcctcggcagtctgtgcaagcgccatcctttgtcctccaatttctgattgatttagatttttaagtcccacggaaagcgcagaatgttgaagatattcaagcaaggttttatagatttgcaggggcgacatgggcaccatttgccgcagctcctctcccccaagcatgtccccaatccgggcaaaggcattgatgatatttttaagcgcctgaaagttagaaagagagcgcccgataaggtcgcgaatgtttttagcctggcttgctctgacgggacggagggtaccaacgcttcggccttgttggatttcagccgcaactttttcgtagtagtggcccgcaggagcattatccgtaaagacgttggagtcgttgcctgtggaggtgggaaaactttcaaagacttgtgcaagcgtgtcccctgttgtctcggtgaaccatcgtcctataatgcgcacgccatccagcatctgttggactgtttgaatagaatctatgttgtttacaaacgttttggtaatgtttttaagataaagatctagcccttccagagctcgatagaatcggcgttttacatcatactccagctcgatggcgcttacggttgccttccagtctacttcctgggcacctccaggatttgggcccacgtgtcctctggcaagatctacagccggagaattaatgcgcgcatttttttccgtatccaactgcatgaggcgtcccgcaatagcatctccgagaatagtggcatagttttcctcgtaggattgaaactcctgtttgttatgcgttaaattggagtaaatctgggccacataatagtaatacataaaggtgttaattgcctggttgaggtcaacctgcgatcgcgcggccttgctgagcccaagctcttcaactgttagggcagcaccgcctacccttgtacactcgcagtcctcctcgcctccatactttttttgcacaatatcggtataaaaatcaataatctgtagcaagcgagagcaggagtcataaagatttttaaaattagggtcggttttagatatctcctccaaaacatttttaacaagcgtaagctgtgttaagaaggtttcgcgttcttctcgtgcggccgcattggtgtaaaagccgataagacttagatcaagtgcgatggtgcccatatcattaatgcgcgaaagagcatctcgaagcctcgttatgttcggcgtcaaggcaatttctttaacaagtttgatgcctatttttttcacattttccaaaaagtcgttataggcttgtgtgcttttattcaaaaattccatgaggatgtgctttctatccagtctttgcgcttcaatcctcctatctagtggcgttttctcctcatcgcccccctttttggcacaactgttctcaaggattttgtggcgttcattaaaggtctgtcgcaacaggttcacggctttttcaaactcagcaatgttttctgcggagacaagaccactaaaccttttgaggtcaagctccttgtcaaactccgcccagtttttgctttgaaggtactgttcaaccttgagtcctactttctggagagccttattaattttattcgcaacagacgcagcaatacctagattacaaagtgtgtacgaaagtacttttccaaaatttttggttcccaagacactatttgtatcatttaaaagtttaataatatccacctcatccgtctgcagtttatcaagttccttttgggtgggagttaaaatattgtcaataaaattcgttaaaatgttgatttgcaggttttgttcatttaaaagtcgacgatatactgcttcaatcatggtgactgcattaatgacttcctcattgggggctgctttggttacctccgtcaccatgcgctcgtgaagttgcttaatggcgtcgtttaacagcttgatattttcaagtgtattttctatactgccgtgtacatcaagatactctgcgcgcagtccatgagttagggagttaatgtacagaactatttgtcgacatatactggcggccccttcggtggtatctataagcttatcctgacctaaatcaataaattcctggttaatggcgtctgcaatcattttacagacggtctcctgtttttccgcattttttacaaaggtggaaccggctcgaggatcgggcagttgttttttgatatctttaagaatatcttcgatgggctgctttgtgtctactttgaaccctattttggcaatcgccctgataattccttctataatccgcagctttgctttactcgatacggagtctatgtgataatctttaatgtgttgtacaggatttttgtcccccccgccattaaaatatcctccccctgaaaaaggacgagtttgtctttgtatatgatcctgtaacttcgcatatatatttgcttctgatgaaggcagtggtctactagaggttgaagatccacggttacccattataataaaaaaaataaagatttaaaactacaaatattttgctgtttataaacccaatcatataagactaactaaaacattaaatgtaggtgagataaaagcttattttttttaaaagtttaataaccatgagtcttaccacctctttttcttcttcctttagaggggttccataaatggtttgaataaaattatgtgctctaataaccttgttaaaatcaggtgcctttccatattgttcaatatgttgcacagtcttttgtgcaagcatatacagcttggagtctttaggtacctccgatgagggctcttgctcaaacaacgtttcaaaggaggatgtgcattcattggtttcattatcatttttttcatgaatgttctccgaagatgctgaggattccgtctcctcttcaaacagcacatgcagaatcatattccattcttcttgagcctgatgttcagtatacccttgccctgcatatatacgagcagatttcacaatatcatacttaacagtactaagcaatgtttttatagcggtcgtaacaattctaccgctattgataatctcaacagaaaaccaattatacaggctacccgcatgaaacacaacttgtgaagatgatcttaaatccgttttgaagatgacctccattttcatggatatatttaaaataaaatccattcaattttaaaattataaaataataagaagatgccctctaatatgaaacagttttgcaagatttctgtatggctacagcagcacgatccagatttattagaaattatcaacaacttatgtatgcttggcaatttatccgcggcaaagtacaaacacggagttaccttcatttaccccaaacaggcaaagatccgcgatgaaataaaaaaacatgcctactccaatgacccttcacaagccataaagaccttagaatcactcatccttccattttacattcccactccagcggagttcaccggggaaatcggctcctacaccggagtgaaattagaggttgaaaaaacggaggcgaataaagttattttaaaaaatggagaagcggtcctagtaccggcggccgattttaagccctttcctgatcgccgactagcggtctggatcatggagtcaggctctatgcccctggagggtcccccctataagcggaaaaaggagggtggggggaatgacccgccggttcctaagcatatctcgccgtatactccgcgcacgcgtattgccattgaggtggaaaaggcctttgatgactgtatgcgtcaaaactggtgtagtgtcaataatccctatcttgccaagtcggtctccttgctgtctttcttgtcgctcaaccatcccaccgagtttattaaggtactgccgcttatagactttgaccccttggtgaccttttatctacttcttgagccctataaaacgcatggggatgactttttaattccggaaaccattttattcggccctaccggatggaatggtacagatctgtatcaaagtgccatgctggagtttaaaaagttttttacccagattactcgccaaacctttatggacatagccgattcggctactaaggaggtagatgttcccatatgttactcggatcccgaaaccgtacattcctatgccaatcacgtgcgtactgaaattttgcatcacaatgccgtcaataaggttacaacacctaacctcgtcgtgcaggcctataatgagctcgagcaaaccaataccatacgacattacggccctattttcccggaaagtaccatcaacgcactgcgtttttggaaaaagctgtggcaggatgaacagcgatttgttatccacggcctgcaccgcacgttgatggatcaacccacctatgaaacctctgagtttgcagagatcgttagaaatttacggttttcgcgtcccggcaataactatataaacgagcttaatattacaagtcccgctatgtacggcgacaagcataccaccggagatattgcgcccaatgatagatttgccatgttggtggcctttatcaacagtactgactttttatacaccgcgattcccgaggaaaaggtaggggggaatgaaacccaaaccagtagccttacagacctagttccaacacggctacactcttttttaaatcataatctaagcaaacttaaaatcttaaaccgcgcgcagcaaacggttagaaatattctttcaaatgattgtcttaatcaactgaaacattatgttaaacacacgggaaaaaatgaaatactaaagttacttcaagaataagtatgttgatacctgtggtgtgttttacctgtgggtttcctattggaacctacgcggcaatttttgacaaggctcgtaccgagtatattaaaaccaaaatgggcggaacattgccgcaaaatatcccattagatgcttctctccagattgagttaaaagacctcattacagctctgggaatcccaatgcgggtgtgttgtcgcactcatttaattactacgttggattatcgtaaatattattaatatctaaaattgaaaaaatatttttaatgttactagtaaaaatgactacacacatctttcacgcagatgatctcctacaagcattgcaacaagcaaaagcagaaaaaaatttttcatctgtattttctttagattgggataaattacgcacagcgaagcgtaatacaacggttaaatatgttacggtcaatgtcatagtaaaaggcaaaaaagctccgctaatgtttaactttcaaaatgaaaaacatgtaggaaccattcctcccagtaccgatgaagaggttatacggatgaatgctgaaaatccaaagtttttggtgaaaaaacgtgacagggatccctgtttgcagttcaacaaatacaaaatctcgccgccattggaagatgatggtctcactgttaaaaagaatgagcagggtgaagaaatataccccggcgacgaagaaaaatctaagttgtttcaaattattgaactgttagaagaagcctttgaagacgctgtgcaaaaaggtcctgaagccatgaaaacgaaacatgttataaaattaattcaaagaaaaatttctaatagcgcggttaaaaacgcagacaaacctttgccgaatcctatcgcacgcattcgtattaaaatcaatcccgctacaagtatactaacaccaatattgcttgataaaaataagcccattactttacagaatggtaaaacaagctttgaagagttaaaagatgaagacggcgttaaggccaatccggataatattcataagcttatagaatcgcattctatacatgatggcatcattaatgctagatctatttgcatcagcaatatgggcatttcatttccgctttgcttggaaatgggagttgtaaaagtttttgaaaaaaataatgggattgatgtgaactccatttatggctcagacgatatttcaactcttgttaatcagattgctattgcttaaacaatttgctcaaaacaagcttataaacgtttcttaggtatgcgatacgtaaatcctaattctttaataagttctttttcagtagtgatttttagaggtactaaagtttgatttttaaataatccatactgatttagcttataattctttttttttaacgcagctcgaattcttattaaataagaaacgggacccgtaaaatgaagtactgcgtatggcttttcctcggctaaggccgtaaaaagatcaagttgatatgtgttttttttccattcaataaaaagtacacactttcgttctccgcagacttttacagaaaaagaaagatcctttatgcgaatgttgggcaggacgtgttttaaaagttttttttctggaacaataataagaagatccacgtcattaagcattttctcttcgcgtcttaagctaccaacagcaacgatgttttttgataaaatttttataagttgtccattatattcaaacgcaagtcgggagcgtaagtcatttacaattttttttccttgaataagcgttaacattttatatttaatattaaaatcttttcattttatatattatatacgcaaaatggcacttgatggttcaagtggtggaggctctaatgtagaaacattacttatagtagcaatcattgtggttattatggcaatcatgctttactatttttggtggatgccccgccagcaaaaaaaatgtagcaaggctgaagaatgcacatgtaataacggaagctgttccctaaaaacaagttaaaacatgcaattatatgcatgcatataaacgcatgcatataaacgcatacatataaaatgcgtaaatactatataaaaaactataacatatcaatcaaggaatcaacacttttataattttccgtaatatatttttcatccataatgatgtcagagtacatggtccctatgcgaggaacagagcccataagggtaggcgcggcaataccgtaaatgggattcacggcggagtcaaccgcagcatctgtcaagacctggactggagacgacaaggccattcgcaacaacacgttggaaggctctcttgcattaagccctgccttttctagagaggtaacctgtcccgttcttgtcatgagatctgcgtacatgagtaaatgacgatggttgggacccttgtcccccataaccgttctaatttcactaataattttttgccgtgccgcttctatgccgtaaagctccatggtgtctcctatagaggacgatacgatggtgtatgggtcgatgttatcatcaagcattgcgccaaaaatattagtcccgtttgttttgatggcgtagatattgtctagtcttaccagtttcccctgggcatccacacggtggcgcataagcttaacaacattcgcatttttgatgcctggtattcctctaatcgtgctatttaatagtttatccaccacatttacggcaattttttcatccgtagccattcgggtattggtactgcgtctaaaggcgctttcccgtaggtatatgcgaataatgatgggaatccctgaggccgtgttttccacagaatgcatgatgtaggtgttggggtgtttagctcttagactattaataatactttctagactaatgctttttaatatcatggttgttttgtttaattccaagcggatacaccagtttgcaatatcctctgggggctgtagtagaggatggttttccagaaaatccgtcatccattccacatcacttgcaaaatcggggtacatcacatttttttttgtgcttgaatacgtttcgtacaataggtgccactgcaatatcaaccgttcgaacgttataagctctatgctgttagcaatttcttgcgcatatgttttatttgtttccacttccgggttctttagacgtaaaagcatttcagaggattgttcagcctctacgggcttcgcgctaaagatctcctggggccgcacaattcccgacttgttggttcccccggccacggaccggtggtgggagtccagcatatattgtgtcaagggctctgatacggactgcgccgccaggattcccactgcctcaccgtagttaataagactttgagtatattgtagccttatgaggtccaggatggcactcatctgctcgcaggtaatgtttaatgttttaacggttgccagttcgatgcgaataagcatgcgcatcagagaggcagcccgtttaagataaacgggtatgggcgtttgtagtcgttcctgaatgttgttaataaacacgtatggaagatttttgcaaaacgttttgaccatcgcgtatttttgtagaatacttttttcgtcgaagggaagcacgccactggtggagctcagtagaatgttttttacgatgctggccacgtttaccggcacctgtctaacatctgtaagcagctgactgaaattaaaattttcgacgtttaggaagatctgtcgatatttatctctatcctttttaaggcgtgaaaattcttcttcaaacaagggcgattgtatcccggtgtacttgaatttgtcttcaagttcctggtccgacagcatgatggtttcaaaccgtacggtttcaagctggcgcgcatcaaggccgtcctctccgtacaactgctgcacaagacgcgtatcgatggaaacccgtcggtaataatccacaatacaggattgaaggccaaagatggctttacggttggcatagcctgtggatgatgtcgataatgctttgttgatcaagtcgaatcttccattcatttccccaaagataaattcaggggaggtaaggcccgcaatatagctgttgcagatgaacccgtaggcctgcgcctccagggcaaacctggggtagtacaccagggtcctaccgaaggaaaactggggttgaatgcgttgtgtattaatttcaatttggccgatgcccgccatgatgtgaatcatattggggtttgagcccttggcgccagtggccaccatctgaaaaagcccattggtttccggattaatggaattcataatcggctttaaaattctatcgggaaatttaagcgcattcagctgcaatttttcgtagaagtcatgcgttgtcaggcctataggcggcatgatgtctccatgaagcagccggttgtttatttcctccgactcaagcagcagttcattgataatttcttggacctcctgatgtgcctccggggttaggagcatgtcggccgtggacactgtgaatccggcgttgcgcacgtagtttagggcgagctgctgggtcgcaaatatcattttcaaggcctgctgcggcccatacctacgcgaaataaggtgatagattccaccggaggaacccgctccgacggcctttttgtcaaggacgccttcaatgagttcgccgttgcgtatttgtgtagagatgtcctgcttgttataatgcatgtagggtgcatacacttctgagtaccatgtgggggctcgttgataattgatgggggtctgcctcagtagcatagatacaaccgatttgccatccagcaggtcagttggggagtagttggcaaaacaaggtgggtcggtttgggttgtttgaaacaaccccatggcgtgcagcttgttcatcacatttttccccatgggggtgttcgtgcgtgtaagcaaaaagcttcccaccgtggagtcctgcacctgcccattaacgggacccgagctctttgtggaaatgaaccagtttcgcacagaacaaagtagttcggcctcaacgcggctcatgacgctccagggaacccagagattcatctgatccccgtcaaagtccgcattataccaggcacatgcgctgacattcatttgaaacgtagaaatttttgggttttcaagaacgacaatccggtgaacccctatgctgcttcgttcgagagaaggctggcgattaaaaaacgcgacgtcgccagtgacgacgtcacggtaaaggatgtctcctacctccagcctaaagtcttgtttgagaccctcaatgtcgtgaacggattgtgttatttgcttatacactcttgaacaaccagggtactggcgctttccatttaaaaaatagggcattaatctattaatattataatgttgcactgtttccgcaacttgcagcgttcgtgcaaaggaaatgggatagccaacctcgtccaggtgaaggtctgagttcccgcagatggtggaccggctgatcgaccatacctggctgcccagtagggatttacgaattcttccctccttgcgaggaagtcttcgcatgatggagggagcagggcgtgcccccatgacgatcccacgctttcccgtgcctccctgggttgcggtggtggaaacggaatccaacaaaaagttatagtaaagttgctgtatggtttgcaaattgcggtcaatatttaaaggtattttttggccgcgcacgatttgtaggtccttcgggatcagcagattctttcgaaccagatactgaatcacgttgttaatgtcgtgaaagctttgggggcctgacccgattcccaatctgatgccaggtcgtatgctgatgggggggatctgaatggccttaagcacaagtttttcgggatgggagtttttacttcgccccagttttacaacggtgtcgtaggttacgcgcgaaaaaatctctctgatgatctgcgggtacagtttgtcaatcttgccctgctgatccgcccaaaaggtaaaataatcttccgagtccttaacaattttggggtgtactgccttacagacgtagcactgctttccttcggtttggcttgaagccgcttcaataagacgcttaggcctaataaggtgctcgtacctctttaggtcaacgatgggagccccgcagttgagacatataacccttaaccatcgtcgtatttcggcgatgaagagcggctgaagcaccggagcatgcatctgcagtatcccagggtgtcccatacattgcttgcgctggtgtgagcaagtgatgcatttataatggtgatcggtggttcccattcgcgcatcatagatacccccttcggcgggaagggtgccctcaaataaattagaaatggtaacctccataacgccttgcctcttatgatcattgtcaccggcaatattgaactgaacggcggctatttcggcatatccagcctccatatttttgctaaatacataataaaacttcaaatgttaaaaaaaataacatcggttggcatatttttttgttaaaaccaagtgttaaatgatttctaaaacatttatcggttcacgaaaacctaccgcacgggcctgaagaggaatgccagttttgggggaaagctcggcatattccacggtaagctcttttccataaagatgttttttaaataaggcgggcgtgagtttttgaaaaagagcataacgatccgcgtacgtcaaatgcttaggagtgactacaaaccgctttttgtttggcaattcgcaaacccataaaatggcgcctaagtcctttcccttttttccctgagtatagtccactaaaataaattcagcgtctagcagcggtttcagcttggcaagatgcgctgagtggtagttgttgtatcccggctcatagggcccattggcattgcgtacgatggctccctcgtagccctccttaataaactgcgccttaagcctaagggcctcatccacattcttcacgctaaaattttcaacttggtggataaaggtaagatcttccttctgtttaaaaatatttgttaatagctgttgtctcttgttggaaggcatttgaagctgatcactccaaaaacagtcaaacacgtaaaagtgcagctcggaggaatctgtcttcgcattcgcctgccccgcgatccattgcagaggtttgcggtgtaaataaagctcaccatccaaatatactctcacgtctataaataaataaagctgtttgagctcttttttaatattgtcaagacctaaaaattcctttttcgtgcgcgaatacaagagaatgctaccatcgccctgctggcaggccacagctcgaacgccattacgcttgcgctgcacgatgggatctgtttcttcttcaaaaaatgtcttaggaattatattaaaatattttaccagcataggggggataattcctctatttgtgtgggctccccgcttttgtctggcatggcgattatatttactaagggcgtccttgaatgcctgatggactaccgttgtggcattttttttacccaagttttttccctcggtaacacgtgtcatttttgatatccgcaccgccccttcttccacaaaaaattttgtgaaaatttcagcaacggcgtcttttacatctgtggaaaacatctcatctgtgatgggaatgatcgtgttgtgctgcaccacttgcacacaaataatccatgaggccttttttccgcttttcgtttcagactcaatcggaggaaaacaaaaaatgttgtttgaatattgcccaggaaattgatttagcatggttttaacaataaaataagcctatcaatttttttataatttgaatagttattccaaattcaatatggcttctttagataatttagtggcacgatatcagaggtgctttaatgaccagtctcttaaaaatagtactattgaacttgaaatacgttttcaacagataaattttttattattcaaaaccgtatatgaggcacttgtggcacaagagatccctagcaccatctcccacagcatccgctgcatcaaaaaagttcaccatgaaaaccactgccgggaaaaaattttgccgtcggaaaatctttacttcaaaaaacagcctctcatgttttttaagttttcagagcctgcatctctgggctgtaaggtctcgctggccatcgagcagcccattcgtaaatttatcttggactcctccattctcgttcggctcaaaaatcgtacgacctttcgggtatctgaactttggaaaatagagcttaccattgtaaagcagctgatgggaagcgaggtctctgcaaaacttgccgctttcaaaacgcttctgtttgacaccccagagcaacaaacgacaaaaaatatgatgacgttaataaacccagatgacgaatatctttacgaaatagaaatagagtatacaggaaagcccgaatccctaacggcggcagatgttataaaaattaaaaacacggtgttgacacttatttctccaaaccatttaatgctaacagcctaccaccaggccattgaattcattgcctcccatatactgtcctcagaaatccttcttgctcgtattaagagcgggaagtgggggcttaaacgcctcctcccccaggtgaaatccatgaccaaagcggattacatgaaattttatccgcccgttggctactatgtaacggacaaagcagatggaattagaggcatcgccgtcattcaggacacgcaaatttatgtggttgcagaccagttatacagcctaggtaccaccggcattgaaccccttaaaccaaccattttggacggtgaatttatgcctgaaaaaaaagaattttatgggtttgacgtcatcatgtatgagggcaatctattgacgcaacaggggtttgaaacaagaattgagtctttaagcaagggcattaaagtcttacaagcgtttaacataaaagcagaaatgaagccctttatttcgctaacaagtgcagatcccaacgtgctcctcaaaaactttgaaagcatttttaagaaaaaaactcgcccatattctattgatggcatcattttagtagaacctggcaattcttatctaaatacaaacacctttaagtggaagcccacctgggataacacattagactttttggtgcgaaaatgtccggagagtttaaacgtaccagagtacgcgcccaaaaaagggttttccctgcatctactatttgtaggcatctccggagagctttttaaaaaattagcgctaaattggtgtccaggatatacgaaactattccccgttacacagcgcaaccaaaactactttccagtacagttccagccatcggattttccattggcatttctttattaccacccagatacctcgtcattttctaatatagatggaaaggtccttgaaatgcgttgtcttaagagagaaatcaatcacgtcagctgggaaattgtaaaaatccgggaggataggcagcaggatcttaaaaccggcgggtattttggcaatgatttcaaaacagccgaactcacatggcttaactatatggatcccttttcctttgaggagctggcaaagggcccttctggaatgtacttcgccggtgccaaaaccggcatataccgcgctcaaacagcacttatttcctttattaaacaagaaatcatccaaaaaataagtcaccaatcctgggttatcgatcttggaataggaaaagggcaggacctaggacgttacctggacgcagggataaggcatcttgttgggatcgataaggatcaaaccgcgcttgcggagcttgtttatcgaaaattttcgcatgctacgacccgacagcacaagcacgctaccaacatttacgtgttgcatcaagacctcgcagagcctgcgaaagaaatcagcgaaaaggtacaccaaatttacgggtttcccaaggagggagcttcttccattgttagcaacctgtttattcactatcttatgaaaaacacgcagcaggtggaaaacctggccgttctgtgccataagcttcttcagccggggggaatggtgtggtttaccaccatgttgggagaacaggtcttagaattacttcatgaaaatagaatagagctcaatgaagtatgggaggctcgtgaaaacgaagtggtcaaatttgctattaaacgtctctttaaagaggatatattacaggaaactgggcaagaaattggagtcctgttacccttcagcaatggcgacttctacaatgaatatcttgtgaacacagcgtttttaattaaaatatttaaacatcacggcttttccctagttcaaaagcagtcctttaaggactggattccagaatttcaaaactttagtaaaagtttgtataaaattcttacagaagccgataaaacttggacaagcctttttgggtttatttgtctgcgcaaaaattaaatattttttcataagaagtactacccaggttttaaagaaatagctaaaaatatcatatggatactgccatgcagcttaaaacgtctattggtttaattacatgtcgtatgaacacccaaaataaccaaatagaaactattctggttcaaaaacgttacagccttgctttttcagaatttattcattgtcattactctataaatgctaatcaaggtcatctgattaaaatgtttaataacatgacaattaatgaacgactgcttgtcaaaacactggattttgaccgcatgtggtatcatatttggattgaaactccagtctacgaactataccacaaaaaataccaaaaatttaggaaaaattggcttctcccggataatgggaaaaagcttatttcattaatcaaccaagcaaagggctcaggaacacttctatgggaaatccctaagggtaagccgaaggaagacgagtcggaccttacctgtgccatacgggagtttgaagaagaaaccgggattacccgcgaatattaccagattctcccagagtttaaaaaatctatgtcatactttgacggtaaaacagaatataagcatatctacttccttgcaatgttatgtaagtcgttggaggaacccaatatgaatctttctttacaatacgaaaaccgaattgccgaaatttctaaaatttcttggcaaaatatggaggctgtacgttttattagcaaacgccagtcattaaacctggagcctatcatcgggcctgcatttaattttattaaaaactatttacgatacaagcactaggatgccgcattaaaatgccacataaggtaatacactaggaatgtcgcacacgcacaagaatacaacgtcgccggagatttattatctagtacacgttttatgtatgtacaatccgccttcatttaatatattgagcggatgtactatgtatttattttaacaaaaaacattattttttttaatcttcatcatctgtttttataaactcagtaatatcaaaagtagcttgtggggtttcagagggttcaccttggttatcctccgtgaggataacatgttcttcaggttcgtcgtcactggagaacccatcatttaattcctcttcactcaacatctgtaaaaaatcttccaagctttcgctatcgttaaaatcctcatcatccataagaataatggtaccttcctcatcgtttcctccttgtttcgtgtctaaataggcctgcatggcatttgcaaaagtatcaaaataggctgagtcagattgctgttccaaaatatggccttgcgtattaaatgtggttgcatcgttgttaaatgcttgcaaatacagtaagggatttatatccattattattaagcaaaaaaaatttaaattatttttcgaccgatgttaggtaaaattaaacaattgctataggtgttaagcaatgtttattgattttaagtactcaacaaccatgatgtaaatactatacagcacttttggatttttaatcaaatccagattaatactaacttcttttgtgatacagttcgtaataatagtatcctgctcatcgttttgtaagatttcttttaatatatttttttttaccgggatactaagcaattgattattttcttttaaaaactccttttgatattcaatcgtcttattcattgaatatttgtatataactataattacaaatgttcaatgaattgttattcatgtcgggagatggctatttaaaaatcatgtcctatttttctttgctcaataagcatccaaatattttcatggcgttttattaattgttcattattgaacgtatcacaaagatcatttataaattgcagatagtttattatttctttcaagagagtaacaaacattacttcagcagaacatataataggtaattcagtggcgttaaaagaattttgatcttgttgatacgccaatggcgaggacttaaggagatttgggggtcttgcccaaaaccctaggctgctgttcttgttttttagggcgtcataaagaaatgaaagcacattgcaaggcttaagccgcgacatctccttccccttgggccctttccatatttttagatctaagatctcatccgagcttatagagtaggtatagtaaagtttttcaaaaaagcatatctgcttgaagtcttttttagaacgactttcaagaagcatttctataatgttaacaagttttgttaggtttaaggcctgttcctgtgtaagctcctcttgcacgtgatagactgaaaaagtgtgcttaggaatgaaaatactccccgtggcactggcctgttgtctgccaggtatatagtacacgctgctgttagcaagctgtaccggcacaatttgccccacttctgcaacattattttgcgattcggacgagggtatgacaatagttacgggttcagtcaataggctttcgccgagaataatattactgtcatttttaataattttaacggccgctattaaatcaaaggcatttaagtaagaaacaacagcagaaaatcttacatgcatatatcctcttccgctattattcgtacgcataataaaacaaggggagcgttgtataacgccagtaatattaagaataaaactgtttttgaaacacttacccacataaatgttttcaagctccttcaaaagatgagcctccacatttgtacaaaaattggtaggatcatcaatattcaacgttgtctcaaaaattttttggtcgatcatatctataatatattctgtctatttcaatttaaataatatacgaataaataacgagattattttattaaataagcaatggtgtatacactttgtatttactttgagatatactttgtgtatcacaacgtgccctaagatgtgtgcacaagtgacggcattttgtcgttaaaaaggtaaaaccagcggattccatcctgcattccatttggttgattacgagcctccatttctttttgcaaaaggttattgcgaatgagtaagcagagcttgatggcactaatctttgtaaggtttaaacttatgcccaattggtcagcaattttttgttgctcctcccgtccgcgtgtttcgcatacggctccccggtttagcatgcgaatatcagtaatctcattcttttttaaaacctggataggtgggcggattttaaatttaagggcctttcccttgctttccatatagcctatgacgatgtcgttttcttttcgtttaacattaatattaagcatataaagcggaatttcatgccaggttttatcttctcgcgaggtaataagtcgcacggagtcctccgtggcatagcccactagagtgttgtcatccccaggcacgtggcttataattttaaaaatgtccggaaatggctgaatatctttttttgaaaaagcgatgaaaaactttttataaacctcgacaagggcccccatacctgcaagattatctataataagtgcttctagcatcgtatagtgaaatgaagcggggtagtggatgagtacctgctccattggctcatcctgaaaatccttctgaaacttttcatacaatacttgaaagggttctttggtctgcgagtgttcgaggtatttggtaatacggatgctgtgcatcgcgggaggctgaaaatcccgaatatatgtttcaatatctaataccggttcctttttatggttaagcaccgcagcgacgtacaaatgctcaggctttgccggcacatgcataatggtgcaaagacgattctgtatccataattccttgcactggttttttgagtagcatagagaaatgagcgccagcgcgaagttgtcctctgagaagagtttattatcgatggtaattccctgtatgagcttgggagtggaaacagccttccatagctcggagtacgtccacacggggcgtgccataaacaaagatataataatattagaaattgtttttacctcttgctccccgtatccataggcctcaaaggtattgaggacggtggctccgacgtttgccggcgtgatggatggactaaggggcagactttccaacataggcttatcaatcttaatctggttggtgaacccatcaatggcgtgctttcgcagcgccttatccccctcctgtattaaaatgtattcttttaatttttgtgcgtacttagcgagctctggccctccatcgggtgttgtcgatacgtacaaataaattgtcacgttgcgctcactgggggggagctccatgtgtgaattttttcgcaccaccctcccaaatacctgaataagccggggaatatcaaggggcaatgacataatcatctcgtaccgcacggcctgaaagttcaaaccctccacaatcaccttggacccgatgagaatacgcagctggtggccttccaggttggacgaggcgttaaaaagagccaggcttcgttcgcgtacagcgggctctatttcgctgtgcagaatggtgaaccgtactggaataaactgatggtcgctatgtgtgtgctcatcgcgaatcgcggcgcagatggagcagcgggtcgttcccacaggggacgaaacttcatttaaaatgccattactttgtaaaatttcttgcaagataagaacccccgacatgcggacccgattgtggtaaattaaaattttcccccggccttgccgaataatggaaagaatgtctttcatcatttgagtgtattttccgctataaaaggccaatcccgagatgtgcgttggtggctgcagcgacaaaaagctgccactcacattaaagggggctctacgcgaaggctcaataatctgtaccccgttttccagaagccagtctgtgcttgccatagaaagggcggtgggggtttccgtcgagttaaacaggccgtaagccttgggttccgtttgttttgaaaattttgggttgggaaacaccatgtcataaatgctgtacgcattactcgagattttagggtcagggcccagctgtttaagcgtttcaagctgatactcagacatggggcattcgatgaaatgtaagtacggcaatgtttcgtctttataggacaacatctttccggcaaatattctttcggggtaaaaattggtgttggtatccaacaaaaaagatacccttccggtgctcagtctttccacaagagctagggcgtcctttttccatttaacggaatgcccactgctgtcaaacagttgctggcgctggaggggctggccgttgggcagctcatgccgcggaaccaaaaggtttaacaggtcgacgtattccatgacactcccggttacgggcgttgccgacatgaagacggccctgggggcctggtgaggtggaaaggcatccaggacatactgtaaagcgatgccataattatttcgttcctggatattgtacacgttgtgtatttcatccgcaatgagcagtcctcccctaagttgctccatgattttttgattcacccggatgaggccgtttgtctcggcctcgctaattttttgcacgaactgagatatatcgttctcattcaatgtatcttctgcttcgtcagaacgatgaaacagagaaagcacatcaaagtttttctcttcacccttactcgtaatattgaaaagcttggatgcaaattccttatagccgtaaaactgaaaaaagcctccgcggtttctatcggttaaacggcgctttaacgtactaacgaacccatttagatgccgtgattcgaccgacgtggtgctgccagactgctttgcaatgtgaagaagccggtgtagctcagcgacctccttgtaagaaacaaatcccagctcaggacgtcttagcatttctgtttgaatgatggcgcgtgtaaagcctaccacaaaaatccagggcgcattttcaataaaattcatgtagtggttcataaattgacgcgcgatggcaatcgcggcaatgctttttcccgtcccggtctgccagtttaataaaagacgcgagtagggcgtgttgggattttgaaagttttggacgaaaagctgggcattatgcaattggagacccttgatggaaggaaagggcgacgcgtaggggtcacacggaaaaaacgctcgcccccccttctcgcagccaggcccaccgatctggacaaaatgagcccgcagatcacgaatgagctctttttggtcgacaggaggggaaatcaacgatttaaactcctttcttcgcgccaactgctgcaaaaagtctgcggcatccaattcgggatacgccatattatcataaaaaaataaacctttttatgaaaacttttatgtgattctgtattgcaattgttttttatgaatactgtaaataagcgtatcaacttgtttttctaacgaagaggcgttattctttttttctggatataaaataataataagtataataattaagactaaacagcaggcaatcactatcaaactcatattatacttacttttttataaaaagtattatatcttatgaatgcgcaagttcagctaattgttcgtcgcttggaatgtgggactgcagggaggtggagtttttcctttttctaaagaataccgggaaatggtggtgaggctcaggttgttgtacatagtagctaggaggaggtttaggtatgctcgacttgcagtcaatagtccggttatagtaaacgatggcaacgatgataagaataataatgagcaaaatcaaaatgcccaggagaatcgcagttgttccgggatatttggcgattgtatgggctaaaaggccttgggtgctttgtttaattccctcgcgggttgacaggttatgagaaagcagtggagacgtttcagtgtccatttattacaattgaacagttatattaatctcaaataaaatataacacaaaattaattatggccatgcaaaagttatttacgtatatttacgagtttattgaatatcgtaagatggtgctgttggaagaaaaggtaccatatgataagtttgttcaaatggtacttaatacaggattttttcgtattaacgcggagacgctgaatcacggaatcgtatccgtgtttatctttggagcaaatggcaagtacgttcaccacggaggcgacatgagaacgcttttaacgaatacgcttaatgaaaaaaaacattatgaagaattaattttaatcgttgataagcccgttttaagcaaaaaaaatattttagatataatcgtcgagcagcgcgctgcaaatcccacgattgtaataaacatatatccctaccacctgttctgcattaacattcccaaggtgagtgccattcctaaacataaactaattactcaggaggaggcgcaggagtttttaggtcgcgaatatctgcaaccgcaggacctcatgcaaattagcgcgtcagaccccccggtggtctggctgggaggaagaccgggagactttgtgcaaattgagcggccctcagagacagctatgcacgctgttgttatccgctttatcaccaagtccaaaatttgagtcccgtgtttaaagatgacagacagctaagtaagcatatctgtaaaattgtcgatgtcctctgtggatagagcgctttcctctgagcagcaaattttttcatacatctccatgggggatggcgaggctttaatagtatgtaggtcacgtaagaactgttgtatgatgggatatttgtcttttaaaaactggggatgtttcataactggaattatttgaaagataaagaccttccatccaaagtagccaaccacatttggcatttcgggacacgcggtttcataaggcatagaatagtgaatagtgtactgatctttttgatacagcgtttcaagtagttggcgaaatgtttccgcgtcgagcgtgccaaaatcttgaggagcctcggtgtgctcctgtgtagagcagatcgtgatgattccccaggcaagcgggagcatggactctggagggtggatatccgtattggtctcattattcgatcccagctgatgaatgccgcacacgcgaaacatggcctcgacgtagatgcccatagagataggcggcgaaagggcaagaccggattgtatttgcggcatatagtaggagggcaccgagttttttatttttcggttgaatggggactttatttctaccagcacggggatgcgtttcgtggcctcatagcgtacgttgttaaaaattgttttgatttcccaggactgttgagtgtatcccagcgttaggtgacaaaacccatcggggctattactatgtccggggtatcccaaataggtcccatcaatatgaatattgtcacctatgacggtggtttggcagaacaactcaagcagatctttactaacacgctcaaaaagggttccccagctacaagcagcgcggttcaaattcttcttaaaaagatttgctttttccgccaaggttatataatagcttttgtaagggtttaaacctaaaacgctggcaaggtcagagccacccacctgagtgcgacgaatagcatgccaggcatcggagcgctgctgaggagagtctttaaacaggcgtacaaaggtttccattatacttgttttaacaggaattcaatataaaaagtcaacacagtttgcaatttttccaatctcaagatatagccatacatttttttttccaattggcgaatatgtttaagctcatgtgtttcaatattagcatccggaaatttaaatgcataaagatgttcaaaggcctgatttatacacgtatcaaaggatctgtggtatgttattagcttcagcatgtgtgccagatcttcaagatggtctaaatttatacggttttccacgtggtggatcatgtctgccacatcttgagcccccatccaggggatcacaaggtactcccccttaaagatgattcgtcgtttttttaaaaaatcatgaaaacgttttaaagcttcaagaaaggggcagttgggctttgaccccaaaatgctgacgacgatatcctcgggcatgatgtattcgcagtgaggatagtagtttacggactctaattcagcggcccgccgttttatttcgtatcttgcccagttattcagagagtactccacgcctccgaccacaacagacatcctatctattaaaaaataacaataaaaaccttatgaaatctatgtatagtggccgctaaaatgtctatattagaaaaaattacgtcaagtccctctgaatgcgcagagcatcttacaaacaaagatagctgtttaagtaaaaaaatacaaaaagagctcacctcttttttggaaaaaaaagagacactcggttgcgattcggagtcctgcgtaattacccaccccgccgtgaaggcctatgcgcaacaaaagggactggacctctccaaagaactggagactcggtttaaagcgccaggacccagaaacaacacgggtcttcttacaaacttcaatattgatgaaacgctgcagaggtgggccataaaatacaccaagtttttcaactgtcctttttccatgatggactttgagagggtccattataaatttaatcaagtggatatggtaaaggtatataagggagaagagctacaatatgtagaaggcaaagtggtcaagcgtccttgtaacaccttcggatgcgttttaaacacggacttttcaacgggcactggaaaacactgggtagccatctttgtggatatgcggggcgactgctggagcatcgaatattttaattcgacgggaaattctcctccaggtcccgttattcgttggatggaacgggtcaaacagcagctattaaaaatacaccacaccgtgaaaacgcttgcagttaccaacattcgtcaccaacggtcgcagaccgagtgcggcccctacagcctgttttacatcagggcacgcctcgacaacgtgtcatacgcccattttatatccgctaggattaccgacgaagacatgtataagtttagaacccatctgtttcgcatcgcataaactaataaagtttgaattctttataggaataaaaatggaagcgtttgaaatcagcgatttcaaagagcatgcgaagaaaaaaagcatgtgggctggcgccctcaacaaagtcactatttcgggtcttatgggggtctttaccgaagatgaggaccttatggcgttacccattcacagagaccactgccccgctttgttaaaaatttttgacgagatcatcgtaaatgccacggatcatgaaagagcttgccataacaaaacaaaaaaggtaacttacattaaaatttcgtttgataaaggtgtgttttcttgcgaaaacgatggcccgggaatccccattgcaaagcatgagcaagccagtcttatcgccaagcgcgatgtgtatgttcccgaggtggcttcatgtcactttttagccggaacgaacatcaataaggccaaggactgtatcaaggggggaaccaacggcgtcgggctgaagctcgccatggtgcattcgcagtgggccattcttaccaccgccgacggcgcgcaaaagtatgttcaacatatcaaccaacgcctagatatcattgagcctcctaccattacaccctccagggaaatgtttacacgtatcgagctcatgcccgtataccaggaactagggtacgcggagcctctgtctgaaacagagcaggcggatctttccgcctggatttaccttcgcgcctgccaatgcgcggcctacgtgggaaaaggcaccaccatttattacaatgataagccttgccgcacgggctctgtgatggcgctagccaaaatgtacaccctgttgagcgcgcctaatagcacgatacatacggcgaccattaaggccgacgcaaagccctatagcctgcaccccctgcaggttgcggcggtcgtgtcccccaagtttaaaaaatttgaacacgtgtccgttatcaacggggtaaattgcgtaaaaggagaacatgtcacctttttgaaaaagactattaatgaaatggtcgttaaaaaatttcaacaaacgattaaagataaaaaccgcaaaacaacattacgagacagctgttcaaacatctttatcgttatagtgggttccattccaggaatagaatggaccggccagcggaaggatgaacttagcatcgcggaaaatgtttttaaaacgcattactccattccttctagttttttaacaagtatgacaaagtctatcgtggatattcttctgcaatccatttctaaaaaagataaccataaacaggtcgacgtagacaaatatacgcgtgcccgcaatgcgggaggaaaaagggcgcaggactgcatgctactcgcggcggaaggggatagcgcactttccctgctgcgcacgggactaaccctgggaaagtccaacccaagcgggccctcctttgacttctgcggcatgatctccctgggaggagtcatcatgaatgcctgcaaaaaggtgacaaacattacaacggactctggagaaaccattatggtgcgcaacgaacagcttaccaataataaagtgttgcagggaatcgtgcaggtattgggtctagacttcaactgccattacaaaacacaggaagagcgagcaaagctgagatacggctgcattgttgcgtgcgttgatcaagatctggatgggtgtggaaaaatccttggactgctgctggcctactttcacctgttttggcctcagcttattatccatggtttcgtaaaacgactgcttaccccgctgatacgtgtgtatgaaaagggtaagaccatgcccgtggaattttactatgaacaagagtttgatgcctgggcaaaaaagcagaccagcttagccaaccataccgtaaaatattacaagggattggcggcgcatgacacccatgaagtaaaaagcatgttcaaacattttgacaacatggtgtacacgtttaccctggatgactcagcaaaggagttgtttcatatttattttggcggggagtcggagttgcgaaaaagagagctttgcaccggcgtggtgccgctcaccgaaacccagacgcagtccattcatagtgtccgacgaattccttgcagcctgcatctgcaagtagataccaaggcttacaagctggatgccatcgagcggcagattcccaacttcttagacgggatgacgcgggcgcggcgcaaaattttagccgggggggtgaaatgcttcgcctccaacaaccgtgaacgaaaggtttttcagttcgggggctacgttgcagatcacatgttttatcaccatggcgacatgtcgttaaacacaagtattataaaagccgcccagtattacccaggctcctcccacctctatccggtattcataggcataggaagttttggctccaggcacctgggaggaaaggatgcaggatccccaagatacatcagtgtgcagcttgcgtctgaatttattaaaacaatgttccccgcggaggactcatggcttctcccctacgtctttgaggacggccagcgggcggaaccagagtactacgtgcctgtgttgccgcttgctattatggagtacggcgccaacccatcggagggctggaagtacaccacttgggcccggcaactggaagacattttggccttggtgagggcctacgtcgacaaagacaacccaaaacacgagctactgcactatgcaataaaacataagattactatactcccgctgcggccctccaattacaatttcaagggccatttgaagcggtttggccaatactactacagctacggcacgtacgtcatctcagagcagcgaaatataattactattacggagcttcctctgcgtgttcctacggttgcatacatcgaaagtataaaaaaatcgagtaaccgcatgacatttattgaagaaatcatcgactacagtagttcagaaactattgaaattctggtgaaattaaagccaaatagtcttaaccgtatcgtggaagaatttaaggagactgaagagcaagattccatagaaaattttctgcgcctgcgcaattgtttacattcacatctaaactttgtaaaacctaaaggtggcattatcgagtttaacacgtattatgaaattttgtatgcgtggctaccttacaggcgtgagctttaccaaaagcgtcttatgcgtgagcacgcggtgcttaagctgcgcattatcatggaaactgctattgtacgctacatcaatgagtctgcagagctaaatctttcccattatgaggatgaaaaggaggcaagccgcattctaagcgagcatggatttcccccgctgaaccacacgctgatcatttcccctgagtttgcctctatagaggaactcaatcaaaaagcactgcagggctgttatacctatatactatctttgcaggctcgagaattgcttatcgcagccaaaactcgtcgggtggaaaaaataaaaaaaatgcaagctcgtcttgataaggttgagcagcttttgcaagagtctccctttcccggcgccagcgtatggctggaggaaattgatgcggtggaaaaggctattataaaaggaagaaatactcagtggaaatttcattaaacgctaccggttttatgatgtccaataggtgttaagcaatcagttcatcaacatttttttcaagaatttgaaaagtttggataatgttctgaatacttttttctaaaagagttatcaaatcttcttgtgaggccttatgaataattgttaataccatttcttgcttatggggaacacactgataccccacaaagctaatatcaggaatcatttcataaatatatgtttttagcagatttccgatggtatgggtttcatcttttatcgtgataatggcctttgttttttcctcatccatggaaaacagcacaagttccggctgcggctcttcaaagttttcataaattttttgaatgctttggattcggccaataatgatccggcaggcgttttttaaatacgtgcgaacggcctggttgatatgtggcagcggcaccgctggaaagcaaagccccaggcggtggtgacgcgggtctgaggtcatagagctttgcttgtaaccgctaagcgccatatattcttttttatccgttgggtactgttcaatgtcaaggtgggaaaaatgtgttttaacggcaagattaaaggcggcatgctttcgtcctatgccctttttaatatagatatcctctataatcaacgattttccgggttgtaggaagccaatctcaaaggtaggattaaaaatcgggtatttaagcttagggcctgccacctggatgagatcgcggctatagatggttttaacctcacagctattgtttaaactccgcagagcaaataccagtgtctcgtttttcgcataaatcggaatgaaattaatgcggtttctaataaattgttccgtcataaacaggtccgtggaatcctcgatcttatacccaccgggcttaatatctagcatataattgggaatttcatcttgcaagacccgcgacaggccgtggaccgcggctctgctaatgcccttaaagtccataacaacattgaccgggacgaggggcaactgctcctcgagctgaaatagttttttggccgcatttttaataaagaggttggaaaagtctatcaaaaacggtttgatttccacgttttggaaaattttttccatttgtattataaatatatctatatatattcaaattatggtagtttatgacttgctcgtttctttaagtaaggaatccatagatgtgctacggtttgtagaggcaaaccttgcggcgtttaaccagcagtatatttttttcaatatccaaagaaaaaactcgatcacgacaccccttctcattacgccgcagcaggaaaaaatttcgcaaattgttgagtttttaatggatgaatataataagaacaatagaaggccctccgggccgccgcgtgagcagcccatgcacccattattgccgtatcaacaatcctcggacgaacagcccatgatgccgtatcaacagcccccggggaatgatgatcagccatatgagcaaatataccataaaaaacacgcgtcgcagcaagtaaatactgaactgaacgattattatcaacatattcttgcattaggcgatgaagacaaaggtatggacagcatgttaaaacttccagaaaaggcaaaaagggatagcgatgatgaggacgacatgttttctataaaaaactaacgacgtaacaattaaacaaaaataaaaatcattataaaatgaatcttgaatacgtccaagttgttcaaaaatttaatcaagtactcctagaacttaccaaaaaagtatgtaccgttgtgggcgggagcaaacccacctattggtatcaccacattagaagggtttgctcagaatgtccatccatgccgatgagtatgataggtccgtatctgaatgtctataaagcccaaattctaacaagggacaagaatttttttatgaatttcgatcccgcgcataatgagtacacctttatcattcaaaaactaaaagaagcagcccgaaatatgccggaagacgaattagaacagtactgggtaaaacttttatttttacttaaaagctacataaaatgtaagccctttattaattaaagaattgatgcataactaataaatggccggtcgtgttaaaataaaacagaaagagctcatagactctactgtaaaaaacaaaaatgtgatgaatctgttccatgaaattataggctcaaaaggcaatattaattttagcgttgtctggcccaagtttaaaaaaatcaaacagagcgtttatgactacatttccactctttctgtgctggaaaaagcaaacgttatgcaaaactttgaagctgataagaaactgttggaactttttgtacaaaagctgtgggctgcctatgaaggctatttcaaatatcccgagattgaaaaatatgaggtggaaggccaggtaaatttcaatctcgtacctcagtgcgtcctcgaaaagtttagccagttgtataggataagaatcaattcagagcttgtcacactcatcctaaacagctgtgcctttatgagtaaatataacgattatattctcaaaaaagatccctacatactaaccataacccccggcctatgcttttcccccattcccaacttcgaggacctaaattttaaacatctttacaacagtgataaaaattctcagcatgacaaagagtttatcatgtttatattatataagctttatacggctgccctaggagtgtacaatgccatctcgattccagacatcgacgtagaagaccttgaaaatatcatcctatcctcggtgagccagattaaaaaacaaattccgcgctgcaaagacgccttcaacaaaattgaatcttcggtacacctgttgcgcaaaaattttaacacatattacagtgactatgtgggctcaggctacaacccaaccatcattatggaacagtacattaaagacatatcacaggattccaagaacatatcaccacgcatttcctaccagtttagaaccatcatcaagtattaccgcgacatgattgccaccaggcatcaaacgatggacccccaggtattaaacctcgtaaagcacgtcgaaaagaaattagatatgcttgatagagaaaaaaattagtatatatagttatggtgaatctttttcctgtttttaccttaattgtgattattacaattttaattacgactcgagaactatccaccacgatgcttattgtttctcttgtaacagattatattattattaatacacagtatacggaacagcagcatgaaaacaatacatttttcatgccgcaaaaaaattcttttaacgaatcttataataaagacaaaaaatctaatatacatattccctaccagtggctggcgcctgaactgaaggaagctgagagcaagtactggtggggcaattatgatcctcatagcgagcccgttctcgctggcgcatcttgaatatcttcatacgtggcacgtcaccatcaaaaacattgcccaacagcacgggcttgatataaaggtggccattgtggtctcaacatcgcatttaaataattttttgccaatttccggggcgcttaacatcgaatgtataaccttccccagttgcggcatcaaggagatagacctcctatgggcgcgcattaaactatttcaacattactgcgccatcggtgcccgtcttttatggctggtaagtgctgacatcaggccccctgtttcagcgtggccagccatcgccgacagtctaaaaaagggagcagatgcggtcgttattccctacccctcccgatggaacaatcttatacctaccgtcatcaaagaaatagttgtccaccaaaaaaaatgccttgtggcggtggatgcacgccaccttgatacagatacccagattgtaggggccgggatgggctgcatcgtcctaaccctaaaggcccttatggtgcgcctaagtattggcaaacagcccgttaagatactgtggcccgaccttcacggcactgccgagggcattcctctggagggggtggaggttggctggtttttaaacgcttatgcgcataaattaaatatacgctgcctaggggctgatcatattgcgcagcacttaacttaattctttatttaaaaagtccacgcatccagtggcggcctacattaagggcctacgcacataaatatacactggctagaagtacgccttcatttaaaccattgaattatttatataatggctgcaaacattattgcaacaagagccgtgccaaagatggccagcaaaaaagagcatcaatactgtctgctagactcccaggaaaagcgtcatgggcattatcccttttcatttgaattaaagccttatgggcaaacaggcgcaaatatcataggagtacagggctcacttacccatgttatcaaaatgacagtatttccatttatgattccttttcctttacaaaaaactcatatagatgattttattggtggacgcatttatttattttttaaggaactggacatgcaagcagtttctgatgtaaatggaatgcaataccacttcgagttcaaggttgttcctgtaagccccaaccaagtagagcttcttcctgtgaataataaatataaatttacatatgctataccggtagtgcaataccttaccccaatcttttatgatctttcgggaccgctagatttcccattagatactctttcggtccatgtggatatcctctccaatcatatacagcttcctatccaaaaccataacctaacaacgggtgatcgtgtttttatttctggatataaacacctgcaaacgattgaattatgtaaaaataacaagatttttatcaaaaatataccgccgctttcatccgaaaaaataaaactatatatactaaaaaatcgaatcagaattccgctatactttaaatctttaaaaacgtctaagtaataacatttttatagtctactcctagttccgaaataggctgaatttcttttttaagtcctttaaaccaaggatgtgatacaagactcttaaaggaaagccgcttattttcattaattgttaaacattccgtgataaactgttttcccgtctctgaaatgttctcgggaatataattttcccgtttcaggatatcatttaaataaaaattttctgcacgaaatctaaaaagattaaccgcgaccatacctatcgtccacacggttaaaggaagctggtagtaataaccataataataaaattctggacacacgtattcccatgttccaaacatattatattggggacgggtttcgtctaatctaacagcgcttccaaagtcaatgaccttaatgatcttttgatttatgtctataataaggttctcatccttaatatccccatggataaagcccttctcataaatgttttgtataataagaataagctggaatattatttttttggcttcggtttcctcaagttttttaaagtaatgataatgaagtagatcaacactatttggaatatattctatgattagtatatgatacatagcattttcggtatattcgataagcttaataacaccgggagtatcttgcagggctttcaacacgatgacttcatttcctggaatttcttttttagaaacgtacttaaatataatgggttgccctacttgatgacccaaaaagacgttatttctgccaccctcaaacatgggtctcgtcgcaatgaaatacatgtgctgcgttgtggagatcctttccacctttgctgtaggataaaacgcatattgtgcctggggattttttaacatttttttaagctgttgttccggcctggacatgttttattagctttatatataaagggttagaaggtttaatttcaatatatgccttaatgatgggattatattcgtaaaaggtatagcctaatcctacgtctttgtttttttggtaaaaaaactgtttgccctcgtaggatatgctataggcttttacttcggcttttacaagcggttggcagggattgggcaaacgtaaatcgcgttcaaagttttcatgaaaaagcaaagcatttgtgggctgacacatcagacagccgctttcgccattgaaggcacattcaatggccgccctttttagtaaatcgcggaaagcagaattaagatggctcttttcaagccccctttcgtgaaaacgctcatcaatcgttttttgttcctgactgccttcgggaatactataaaacattttttgattagccaccgcgatgtacaaaaaaggctgtacggttttctcctcgggcggtagcgcatcgtggctaccaatgcgtataatgcgcgccttcacttgatcctctcgggccttatcccagtacggctctaggatatgaacctgccgcccgtatttgagatccaatccctcagctcctgttttagagacgagtaaaattttaataacctctccgtgtatattcagcggcgaattccaaagctgctggatcatgtcgcgctctttagataaaattttccctgtaataagcgtaaatcgtgttattttggaggacaggactaacgtatgggtcggcccatcttccgcaaagtttttcaccataagatctttcccatccttatgaaggaggatggtgttgtgcccttcttccaatacttttaggggctgaaggcactggtagccctctatttctaaaaagcgggccacgacgtgaaggcccaattccacaaactgtgagtaaatgagcacagggcccggagacgttttaatattttttagcatgcgtactattttgggactagaattttctgtgaaggcctctttgggcagctgctgaacagcctctgataatttttcatcctcctttactgttagcatttcggacgcgaagatgctgatcatacgggaacgcacatagtaggaggagcctgactcttgctccgatcctggcaggcagagggcggcggcatttattttttcatacattcctgagctggcgtgcttttccgcgttttcaacgtctcgggccagcagatattgcctatactgctcgggtgacatttcaaccttttctataataagaggaagctctgtggggaatagcttgttgagctcattctggtttccagcgtagcttatcatacccactaggcggtttagtagtttgtccgcgtttaaagggctattcgttgttttattgacataagcggtgtagaatctttcatagtgaagaggtaataagattcgcccgcttagcatattaaaacagggcaccatttcaaaggggtccttcgaacacggggtgcctgttaaaaacagaatacgaatatttttagcttgcataatattattgtacagctggcgggcatttgttttatcattggcgctattgataattcctctaaagaggttgtgtgcctcgtcaacgatgagcaggcatccatttagggaccctcccgcctttatgatctgctgccccatgttgtaagcgtctagggacacaaacctgaagcgccgcgagattttttgtagctctttggagtgatccgtcgtttccggatataaaagtttaataagctttaacaaagactgttggaagtttgagtgcaacgacttgggtgcgatcagaatcgggttgtaaatatgtgaaagtgagatggcaagcgacaggctcaaaatggttttccccatgcccatctggtgatagatgaggaggccccgtgtgttttccccctggcctatcccaaatttaggatccgaaaaggcggtgtaaattaaaaactggtagtatttcagggctcgtgcaaagcgggcagtgagtgaggtgtctttgctttcctgaagctctttatatttttcatatacctcttttaggtatgcttctatttggacggggaaggaggtgttgttgtgcacgcaagacatgactcgttataaggatcccatattaaaacttcattagaagaatagggctgctgatagctagcgctgcacttaaaaatggggtagccctttttcttgtaaatccggtgcctgtcgtagacctggctagaaagcgggcttagtgtatctttaatgtccacaacgatgcgtacctttttttcatccgatccctgccgggtaatacgtcccaagatttgctccatgttgtttctgcggggcgttgccatgatgatcgatgtcatatgcttgaaggaaatgcctctacgcccgtagccataggtcagcaagataatggaagcgctgtgtgcctgagaaagagcggtatttgaaaccccgccgcataggagcgccacctccggaacgataatttgaacatctttgaattctttggaaagcgcctgataaaaaatttctaaaagtttgcgaaattccacgaaaatgatgatgccatacggctcatcggtcccccatttgtgaggctcagcggtatgcagggagtaaagccgctttgcctcatttacgacaagttgtatacgcgaaggatcttgaagtagtttatcaatggtggcaatggccgataccttttcattaatatacacagggctaacgaagtcaggatgtccctgatattcgatttccctcacgtacccggaaaaggttgtggtgggacttacagtcctctggggctgtcctagatggtgaataataatcttgtccataccatcgggccggtccaggggtgtagcggacagtcctaatatccgactaagttgtattttccaaaaaattttgtaattctccggcgagtgtaattcatgtgcctcatctaacacgactagaccaaagggctcaaagaactgctcaggcttcttgcgcagggtattaatgattcccacgatgacgtcgtactctttgctcgtcatgtcctttttcttgcacgctgcattattgtaagcagctacacgtaggtggggcaggagcaatgttagctcgtcgatccactgtatttgaatcgccttggtgggcacgatgaccagggtagggtacaaaagtttttgaataatgctgatcgcaatacgcgttttccccaaaccggtatttagatgtaggtaaaagcgcccatagggggacaggagctttttatgaatcttatcgaccatttcttgctggtagttaaatagtggaaattctgtttcaacgcatgggagggcccgcagcgacacggggcgcgtcgtgtaaaccatgttaaacatttcaaactgcttttgcagcaatatgggaaaataaatgtattccccctgcagcgtgaaggcagtttcctgtcttatggctatgtgctttggctgcccgggtaatgcccgcgccgtaacggtgagcgccttaagaacgcgcccgaaatcatgttgtaatttactttgtagcttcttataatttattcctattccagcaaaggatataatggcctccattctcacgctggacgggttatatgcagaggttccaaaattcttaccagaggcgttacgagagggctgtgctggcaagaatcctctaagcttttatattcaacaaattttaaatttaatgggatgtgacggtaacgagtaccatgttctttttaccagcagctccgaggaagcaaatactcatatgatcatggccgccgtgcgtcgccatttgctgcggacgcagcaaaggcctcatgtcattatcggagcagccgagccccctagcgtcaccgaatgtgtgaaggcattggcgcaggaaaaacgctgcgtatacaccatcatccccctaaaaaattttgaaatagatcctgttgcggtatacgatgccatacaaagcaatacctgcttagcgtgcatttcaggcactaatgctgttgtcaaaacgttcaacaaactccaggacatcagcaacgtgttaaaaggtattcccctgcactcagaagtgagtgatcttgtttatcaaggatgtattcaacaaaatccgcccgctgatagtttttcaataaatagtctctacggcttcctgggagtcggtgttttgggaatgaagaaaaaggtcatgcaaggattggggccgctcatttttggaggagggctgagaggcggaagccctaatatacccggaattcatgccatgtataaaacgctaacccagcaaaggccttctatgaaaaaaaataaatacaatacatacgctgttcatgaaaactttaaaaaacatcagcatgtatatctacccatagggggcgtgtctgcagaggacacgtctgcagaaaacatatctacaaaagacatgcctgttgaaggcccgaagggactcccgggctatattttatttagcgttggccgtcgcgccgaggagctacaaaaaaaaattttcactaaatttaatataaaggttggccgtgttgttgacttacaagagatactgtttcgtatcaaaataccccaaaaatactgggagacattattgttcatccaattaagagataatttgaccaaagaggacataaaaagagttatggttgttttgatgcatttagataccatcactcctcgtggctctcttcctcctccgagccactcttcttctttttcttaatcgtttttgtttgttctataataagggaaaagaactccgtgggatcttgttccccgtacaggttatctgcgaccataaggatgcttagaatggtaaacaggtgagaatacataagggtttgcgttttaagaaaaccctgacgttgaatcataattgaaaacaccttgcaaagccgactcatcagttgttctgtaatggcgttaagcattttctggaatttttcttggttttcgggtgtgattttatattcatgtagaaagtgtttcacacctgaggagaagaatctttcctccttcgagagcccatctttgatgatgggaagttccttgatcagggcaaaccattcctcctcttgggcttgcggattctgaagatactgatggcagatatggtttagaatggtgcacacgtagctaataagctctgagctgattctttggttggttttcaaatgttggcgaaagtagtttttcaccgaagtgcatgtaataaacgtcttcattttcttataatatacaacagtatgttgagtctttaatttaaaattacaaggagttttctaggtctttatgcgtataggtgtttctttgtcgtaaattttcaatagccgacattgtttgtgaagcagtgttctgagtagtgactgtcgtgtaaggctcagccggatgagcaggagcactcgcggccgcaggtgcggccgccggcccgccagttgccatgactagtctgtccgtaactgggttgtccgtaactggtttgtttgttgctggtctgtttgttgccggtctgcccgtgactggcttgcctacacttgctgtagtcgctccagctggtttagaggtacctggttgtggagtgacttctacccactgctgatcttgataaggatttataaactgtatatcttcctcctcaatagcagcagcttttttctttcttgaagagaatagatagattagaacgatgataatgatgactaagaccacgatagcaatgagaatagtatacatatgtgtggagaagaagcttggtgtagtgactggtgacaaacactcaccataatgccgcggataaaccggttgaaaaaattcagaatccatttaagatactattataaataatatataaaaatgttgtggcgcaatgaaattacagaatttatggaccaactttccaagtattctcaagaaatcttaaaaacgtttaagcaattgcgtcctagtgaatataaacaatacaatgaatttttaacacaagttacaccgttgctgcaaaaaacccctgaaaaaattccagagttggttgaccatatattcaattacctagacaacgttgaaaaaatttgtgagctcctcgtgaatgctagctcaattattattagttcaaaaatacgagaacaagtaaaacacggaatgagcttcagctataaagccgacctcgactccttggcggacattctctctcaaaaacagtacgtgcttatgcatctttcaaaaaatattgcggccgagtattttaatacgtgtttaaaccaagggaaatccaagttagatctcaaagctgcctctgtattttatagtagtcgttcccgaacggcaagctcagcagaactctatagaaaaatgctatacgcctatggttcaccgcaggaaattaattattatactgaaaaagcccgaaataagacgttggatgtggaggagagcgacagcatggccatcatcgaacgaacggcccgacacaacctttcccttatgcacccgctagaagccatggggcttacctttggggcaaccaacacggacgccgacccggaggatctgaaggacaaaacggtgataaatttaacgctcccgcaggcaacagaaagcatcacctaccatcttaaatccctaatgcagctaaaaaaagtaagtacggcttcaggactaaatacaaacattttgaaagcatttgataatattatttccacccctgtgaaaaaaaataaaatggcctccaagttggcgcccgggatggatgtcgtgttcactagcgataacggaaaaacattttttactaaaaacattttaagcaaaaacatgctagcggggcccaaagagcgggtgtttgcatataataatctcattagtaatttaaataactcctgtttcatacaaaatcacaacgattttttaagacagcaggactcttggcccttctatgacgcgcacaattttaccaacaagtttttaatgcagcctattttttcggggcagacccgtcctcggcttcagggagccatggaggcggcgcatgtggaaacgcatctcacggcatttttacaaagtattcagccctctaggccacaagatccctctgttttggcttcccccaagttatctgctctaatcttgaactaaaaacagcctttcttggacttaaatgatggtctaccagtttttgaaataacttagagaactatgaagattttcatgaaatttaaattagagatttgcaaaggttacttgcggtcattttctgttgaattaaataattattcgaatagtataatgtctgaagatattcgtcgtggtcctggcagaccgccaaagaaaagggttgttcccaactttgagcgcaagggcattctggaaaaaccagttcggccacaaagccgtctcgagttttcctatgataacccgctgatatttaaaaatctttttatttactttaaaaaccttaaaagtaaaaatattttggtgcgatgtacccccaccgagattacctttttttcacgtgaccagtcgcaggcaagctttgttattgccaccatcgacggaaaaaacgtgaaccattattacgccagtgatgtcttttggctaggcatcaacagagagctcgttgaaaaaatgtttaacagcattgatcgctcttttttaaaaattaccatcgttcaccgctatgacaagcctgaaaccctgttttttatctttacggattttgacattgacaaggagtgcacgtatcagattacggtctcggagcccgagctcgatatggaccttatcgaaatggaaaaaagcatcagtgaagaaagactcaagaactatcctctgcgctgggagtttacctccaagcagctcaagaaaacatttagcgacttatcaaactacaccgagctcgtgaccattgaaaaactcggcggcgatacgccgctgcacctgtatttccaaaagtttaactccatctcataccacgagatgtataaatcttccaacaagatcaacctgacctcgaccattcctaagtcgcaggtgttccagataaatgttaaaattgctcacatcaagtcgctggcctcggctatggtcaccgacaagatccgcattctgtgcgaagaaaatgggaacctaatctttcaatcggaaatggatgcccttatgttaaatacgattaccttgaacaccacgatatagttcggtaacattagatgttctaatatttagcatctaaataatacgctgtagtccggtcagggttgcgtcacagttttcccatttttttgcctcgtcggcggtggccaccgttgccctatcatttacgcccggtaagacaaagctaaaggcgttcagcggggcttggcaatgcccgcccagcgtgaaggagctcggaggattttgcgcatcccgaaatcccttagccatgttgtttaacacttcggttacgtcaatcgagtgaagggatcccttgggatccgtgaatgtaaagacgcagtttctaaagcgcatgtatgcgatggacgattcatcgggggttttgaaggtaacagtgttccccttgctgtacttaaagggggaccatccggtaaaattataccaaatgaaagcaataataattaaaataaccaacacaatagttatagacaacacaaagtctgtagtgccgcccattattaaataaaaatattttagaccgccggcttaaaatttacttattgctcatagcttaagtctattttattcatagcttaagtttattgctcatggcttaagtctattgcttatagcttaagtctattttattcatagcttaagtctattgttcatggcttaagtttgttgctcatagcttaactccattactgatagcttactgatcatgacttaaataaaaatattttgcccgcttaaaaattgtttaggtttgaaaaaataagagatggagggggcaacttatcgtcattgtgtttacccccactggaagacatcaaacggtaaataattataagaatcaaaatgattaatataagggttaaaaaaggatgattcatcacattaattaaaaacgtatttataacgctgttgcagttgaaattttggtataggtcggaaatattgcccgagcctccgtattctgcaatgttctgacatatggtgagtccggaggggcactgcttgttggtcaaaatatttctttgctccgttgttttataggcatttttatttccattacacggagcaaacgcacattcaggccatagggtgccggagttcacacaggcacaatactggctatacgcatactcatcctttgagcacaatccctgtttatcgcatatgctcccaataatattgtcatcctccgccgtttgttgatttgtatgcgagcgtaaaatagcggcccaggccttgggctcctttttttgcagctcggaaatcgaagggcctgtacagctaaagtcgacccaaatatcattgcatttcgtggaaactggcatgcaagacataattgaaataattaataagtatatatcatggcaacaaatttttttattcaacctatcaccgaagaagctgaagcatactacccaccttccgtgataacgaataaacggaaggacctgggggtagacgtatactgttgctccgacctagtgcttcaacctggactaaatattgttcgcctgcatattaaagtagcatgcgaacacatgggcaaaaaatgcggttttaaaatcatggcgagaagcagtatgtgcacccatgaacggctgctcatccttgcaaacggaattggtttaatagacccgggttatgtgggcgagctcatgctcaagatcattaatcttggcgacaccccggtccaaatatgggccaaagaatgtttggtgcagttggtggcccaaggtgaccatgtgcctgaccatatcaacatcctaaaaagaaaccaaatatttccgctgtttgcgcctaccccaagaggcgagggtagatttgggagcacgggcgaggccgggattatgagaacttaattttattttttttcttaacataatgggaggctctacaagcaaaaattcctttaaaaatacgaccaacattatcagcaattccattttcaatcagatgcaaagttgtatttccatgttggatggcaaaaattacataggcgtattcggtgatggaaatattttaaaccacgttttccaggatttaaacttatcattaaacacaagttgcgtgcaaaagcacgtaaacgaggaaaatttcattacaaatctttcgaaccaaattactcaaaatttaaaagaccaagaagttgcgttaacccaatggatggacgcaggaactcacgatcagaaaacggatatagaagaaaatataaaggtaaacttaacaaccacacttattcaaaactgcgtttcatccctgtcgggtatgaacgtgctggtggtgaaggggaatggcaacattgttgaaaacgcaactcagaagcagtcgcagcaaatcatctctaactgcttgcaggggagcaagcaggccatagacaccacaaccggcatcactaacacggtaaatcagtactcacactacacctcaaaaaacttttttgacttcattgcagacgcaatttcggctgtttttaaaaacatcatggtcgcggctgtagttatcgttctaatcatcgtagggtttatagccgtcttttactttttgcattcacggcaccgccatgaggaggaagaagaagctgaaccactcataagcaacaaggtattaaaaaatgctgccgtttcgtaataatttaattaaaagtaaaaaaaaaggtattgttatagtgatggcagattttaattctccaatccagtatttgaaagaagattcgagggaccggacctctataggttctctagaatacgatgaaaatgccgacacgatgataccgagcttcgcagcaggcttggaagagtttgaacccattcccgactatgaccctaccacatcaacttccctgtattcacaattgacccacaacatggaaaaaatcgcagaggaagaggatagtaattttctacacgatactagggagtttacttcactggtccccgatgaggcagacaataaaccggaagatgacgaagaaagcggtgcaaaacctaaaaagaaaaaacatttgtttccaaaattaagctcgcataaatcgaagtaaaaattgaagcgaaaaaaagtagaaaaaaaatgtttggagcttttgtaagccaccgtttgtggtcagatagtggttgtacgaccacctgcatcacaaacagcattgctaattatgtagccttcggcgaacaaattggatttccctttaaatcagctcaggtatttattgccggccctagaaaggctgtgataaatattcaggaagatgataaagttgagcttttaaagatgattgttaagcacaatctttgggttgttgctcatggaacctacttagatgtgccctggtcccgtaagagtgcgtttgttacacattttatacaacaagaactacttatatgcaaggaagtcggtattaaagggttagttttacacctaggcgctgtggagcctgaacttattatggaaggactaaaaaaaattaagccggttgagggggttgtcatttacctggaaaccccgcataacaaacatcatacatataaatacagtacaattgagcagatcaaagaattgtttttacggatacgaaataccaggttgaaacagattggtttatgcattgatacggctcacatctggtcttccggtgtcaacatctccagctataatgacgcggggcaatggctgcgctcgctggaaaacattcattccgtgatcccaccaagccacattatgttccacctaaatgatgccgccacagaatgcggaagcggtatagaccgacatgcaagtctttttgaaggaatgatttggaaatcatatagccataaaataaagcaaagcggtttatattgttttgttgaatacgttacgcgacaccagtgtccggctatattggagagaaacctcgggtcttccatgcaattacaaaccgctttaaccgcagaatttactacattaaaatcgttattaaaataaggatgagttttagcgaatgtcccttagttattagtgcatgcaaaaaatttctacaaaagcgtattacaatagagaatgaagcacttataaatgccttaataaccgctttagcgcagaccagcacgttgaatgatctttgtttattacctattcaaacctatttgcttagttataaaaatgcttttgagtggatacacttcgtatgtattgcaatcaccactattttggataataagtataactggaaggactgtacggtagatattaattatatttttctccatgtaacctatatttacaatattaaaaccaaggaatacctagactactgttcttaaactttattttttctatatttacgccaaagagaatatttaaagtttttttgaaaaaaataatatatgtagataaaattcagttacatgatatatgtgtaaacatgtgtggtaaacaacatatggttatgctttataagataaatgcgcataatatatgtaaacaaaatatggttatgtgttaaatgcatataaatgtattttaacgtatatcttgtgataatggatatatgcatttattaaaagaggctgtatttattataaatcttgctaaggatgccattgtcaacatatatcccatgttggacaaattgcgttgcgatccagttctttttttttgattttgtttaatgctatcctttttgaagggatggttgtccaccatatttattcgatgttcaatgaataggtctgctttttcgtaaggcagtgaaggtcgttccaagactccttgaacgatggacgtgttttcttggatccacttaaaaagcacgtggcattcaaaaacaggacagtgattggatccttggatatgctttggacagccaatgcttgaagagatgtagtcccttttctttaggacaagcttctccacgctggggcaacagagatcgttcaagttctggacggtcgcatttggaatgttgaaacttcgtatccattcaccctcgggtcctcccttatgaagaaggagtatttgctcatggtccttagtaatcttaaccaaatgttggaagatcatttttttacctgctttaaaggcctgaagggtgtcagttggcaaagctattgaattcgggagtgggctttcatcaagcgtgaaatggtgaatgtgacgcgactggaaagaaaacgaccgttgatttattttttcaaagattgggtcgattccgccatgaaagaacagctgcaagattttagaaggcgtatttttttcccaataaaaaatgaccacttctcgtgggattaaaatcgtctgtgtcccattttcattatataattggcccataaagccatcaacgtcaatcaacaccaaaagcatggtatagagagcttttagaaccggagttcgttaaaaaaatacaaagttcgtttaaaacgtgtaatgttactaaaaaaatgtaatgtttaaatgataatgataccacatgcattaatgaaaaaaacttttaaatttttgttttaatatttgcatgaaaatggaaacatttttagtctgtttatttcacaatgcagatggtttacatcaacagattcaggaaattttgtatttattgcggatgcatatttacgaaacaaatctttacttaaagcaggaactatcacggcttatatatccaaataggcaactttcttttgtgttacttatgcccctttcccttctaagaaactgggatgacattgaatatttaacggacgttgtagatgataagcagactctacattacgcggcaaatttgctgacaaactacgttctacatctatccatgtttcaaaagctgacaaaaccatacttccttttagcggtcaagcgggtcagcgaaaaactcaacaaaaagcagcgacattcattttacgaggtattggtaacctccgaaaccttgaataattatgaaaacctatctaaaaacattttaaatacgttgatgtttgccgtgcgctacgtatttaaacctacgccgaactattcagaaattctcgcagagttggaaaaaaaaaataaaattcaccatattatttttaatatggtaattacggattttgcgcaaatccgtgaacaacaaatggataaacatctgtgtgaaacaaataatgagcttcgtcaggaatgtaaagaaactatttttgatttaaaggtggtaggaaatgtttagccaataaactcatgcccgcattttttacaggtacaaaatatcgtggatggctcatcgagggcgcgtgtttgtacttctctgtaggtacacatacgctgcttgcagttgggacacttataaagttgtgacgtcttttcggcgaccttttgctgcgaacgtagagtaatttctgtcttctcctttaaggcggcagaggggcaaagctcggcgaacgtcatgctaccaattgcctccggttttagctcgccagaaattagcttattaagggcatcgttatcctgttgttggtgactttttttttcgcagttaataatatgattgatcgtcccacaacgggttgaatattcttctaaaaaggttttttcttgttgctggtacgtataatgataacacgaggcctcgattttttgcgcgtattcggtgcataaatcagtatgttccttaaaaaacatatgtttttgaagcgttctaaaaaacatcatttggatgatatcacgcatttccaaaataatatagggttctagtcttttggaatctttcataactagatcggtggtaatattcttagtcatacaatttattaaaaatggtttaatatattgtaaatattttttaggcgtgtcagcctgtaaaaaacattcttgttcaatcttatttgtaaggatagtattttgcaaatacttatttagcaaaaatacgatagaatcgcgggctatatgcattttcatataatttttttttaaaatttaatacaaaaaaaagaagtatagactcttcttctagtccggttagttcgttggttgcctcaacatggagactcagaagttgatttccatggttaaggaagccttagaaaaatatcaataccctcttactgctaaaaatattaaagtagtgatacaaaaagagcacaatgtcgtcttacctacaggatctataaatagcatactgtacagtaactcagaactttttgagaagattgataagacaaataccatttatcccccgctttggatacggaaaaactaattgtaaccagtagtacatttaaggatagtttaagcagtaaatgtagaataacacagttaagcaataaataacaagtatataggaatatataggaatatatagaaatatatagaaatagctaagcttaatactaattcagctttttttttaactaaaacctgaatagatgcgaagtagcggacatatacatactaaaataagccatacatttactttcttcttgaacatgaaacctttttttcttctgttgttggtatataaacaataggactgtttgctgaggttgtatgatcttctacaactgctgtctcaggatgacgatgtttttttaaactaaaagtgtaggatggaatgagtggaatatagttatggctcgacttatcctgtttcgtacaggaatattttttacaaatagaacgcaacaagcatatgaataaaaacagaaatgatatacaggagcataaaatagatatgaacactaaggggtagcagcttttataacgttccgtatttttcttagctatcaattgatttaccgtaatatttatctcgggaaactttgttctacaatattttgtttggtattccagaaactcatgtcctggcttattcccgcagcttaaaaaatgatacaaaaatgtgttattgttactaaaattaattcttcttaagaaaaactgcggaagacgctttaggtacgtctgttcctgttttagtaggaagtagtataagggacaatttctttttccacacattagattattgtaatataggtaggttggggtgttggagcgaataagttttctgagtatgttataatctatgacttgtaaatcgttataccttaggtccaaaaacttgagttctttaccaaagccacctgcaatttcagaaatatttttcatcccgcagcggataatacggatgtcctgaaacgtctttaaaatacttgtattgtagtgaatacttatgttatttttttgtaaataatctatgtcatgacaagtgcatgaaatgccagcagcattgcttggtatagtattatatgcaggaagaactatactactattgagaatagtcacattgtacttataccatgtattattttctgatataaagtatttgcaggtgacctgtggtttaatcctacctgttaagccacttcctaaaaaaacaaaaaatatgaaaacccttagcatcctgtatatactattaaaaatttataaaattttctgtttaaatttcatttagacaaaaaaataatatatatacatcagcaagaaattatatacagattatataattttctgatttttttttgccacaataagcatcattatatgcattaaaatctcaatactaaacactaaaatctaaattctaagcattaaattctaagcattaaattctatgcactaaactgtaagcactaaaatctaagtaactaaaatcaacactaaatgtatgcaacctaaaatgtaaagcattactcatcatcctcctcttcttcatcctcatcatcataggttaagatatatgtgtcatcctccatttcttcacattcatcttcataagcatcactgggtattggtggaacattggatgcagcatttttaaaatattctatgtcttctggtgaacactcatctaatgattttttgacagtccttttaacttccatgggatatgattccaaatcctctttatataagagtttacggtagcttttagctgcatccacatttgctggagaatctggatttggctcattgagcagtgaaattacactaagaagaatggtatcaatcttttgagccggagaccaagtcattccctgttcttcagcattgtctccgtgtaagatagagatacatagttttccatcagagtaaatattaggatgccacatttcagaggtgaatgttaatctgggtggtgcatatgggtattctggaggaaaggcgatttttgccttgaataagcctccctcataaaaagtgtcaggtgggccccttaagatcacatcccattcagtcatatccttctcattcaccgaaattttgaaattctcagagggattctctatcaggtgtctgtactctgctattaaaaacctggaaaccatggttatttaatattaattaaattccctggtttattcctccttaaaagtagatgaacctcttttgttttttattgggttcatttttactaaatttatgaactggaaaaaactttaacggcataattatcaaatgcgaagggggatccgtataaaatcctagcttgccggtaatggctattaagttaaatttggtaccagtaacactaatatttaaaaagccctgatcattaactttccacattaaaagattattatattcgaatgtttgtccaatatggacaactttgtcaccagatgttacatttgatttggttgttagtggctgaagcttggcacaatcaaaaataagcccattaacactaagatatagaggagtgggttgatctattttctcatagtttaatattccatctttccacgtaatagcttgataattatccgcagcaatgagttgaaattttataaatagtacaggggttttagttgtcgttatacatttaaagggtgttttataaaaataaaaataataattgttaaaagtatgataataatcgccaaaataatttcatacattttttataagaattatacatagtatggtatttaaaatattagctaaatttaaaaaaacttcatgatttttaaaacagggaaaaaggggattaggttgaataaaaaaggtaagcacttgtctatatattttttttacaatgttgccttgagtcgcatttttaactggctggggagtatcagagtggaatatcactgtagtaggtctataaggtcttgttaaaatatgatcggtcattgttttcgtactagtgtcatttagggtcgacctgatagctcgatataaagttataggggataacctatcaaatacagtcttatctgtgctgaaatgtatatcgtcttctttatcactaataatattaggaatggctgtcattaaataattactacttgttgttgtgggtgaaatagttgtactggtattattggaaatggctgtcattaaataattactacttgttgttgtgggtgaaatagttgtactagtattattagaaatggctgtcgttaaataattactacctattacaagtaaactaatgctaactacatttttaacctcaataaacctaaaaagccatactaaatacctaaacaacatcctgttataatatgagcagaaaaaaaaataagtataattagggaattattcttattcgcttactattaagaataattcagaatcttatttagttagaaactatcataaagtgaataggactcatcgtcggatgaagattccgtttcagagatagtttctttttcttcctcagaataatctgttcctacaatagaatcggtgtcatcctcagaaagagaagtatttaaatatggactatctatagcaatatcctcttctatctcgcaatcctcctcctccatttccatagtgtgtaggagaatatttttatcatcatgctcacttctttttttgttgaaagatgaaccgtcctcaatacggttcatgttaagttccttcatcttatgtataatttccgtaatccgtgatgtttttgacatgtaagatggttttaaggttatatccacaataacaggagaatctctatcattttcatttgataaactttgatctttgatttcttcgtctaaaattcttgtctttttttgggtactagatgaaatagaggaattcatattctgaaacgatatatcaaggggagctggacgcttttttccaattaaaccgtttttcgagatactatgattagatgaatgatctttagccaagctgtccttggatatactatagttagatattttacctttaaataatattcttctatacaagttattcttaggtaaagaattagtatggattcctatatttttatctgaaggagtgtccatatcggagaacgtcctcttacgaatattttgaccacgagccatttcatccactataggcagtattttggctggctatggttctttgttgtgacaattctatgagatttgattgcaaatcaatttttagttttaaatatattggtacctaggacaaagaaagtatatatagccaataattattccactaaattgatttccagactgatgggtatggagccatgttgtctctgcagacgatcgcaaaaatggccgtagcaacaaacacctactccaagtatcactatccaatactgaaggtctttgggctgtggtggaaaaacaatacgctaaatggccctattaaaatatgtaaccattgcaacaacataatggtaggagaatatcctatgtgttacaatcatggaatgagtctggatatagctttgattcgggcagtaaaggagcgtaatatatccttagtccagcttttcaccgaatgggggggaaatattgactatggggcactttgtgctaacactccatctatgcaaagattatgtaaaagtttgggagccaaaccaccaaagggccgaatgtatatggatgctcttatacatctttcagataccttgaatgataatgatctgattagggggtatgagatttttgatgataatagcgtgttggattgtgtcaatctcatacgactcaaaataatgcttaccttgaaggcccgtatacctctcatggaacaactagaccaaattgccttaaaacaacttctgcagcgatactggtatgccatggctgtacaacacaacttaacaatcgctatccactattttgataatcatattcctaatataaagccatttagtctgcgctgtgctttgtattttaatgatccctttaaaatccatgatgcttgcagaactgtaaatatggatcctaatgagatgatgaacattgcttgtcaacaggatttaaactttcaaagcatttactattgttatcttttaggggctgatattaatcaggctatgctaatgtctttaaagtatggtcatctttctaatatgtggttttgcatagatttgggggcggatgcctttaaagaggcaggggcgcttgctgagaaaaaaataaaagagtgttacaacacatattaggtcttaatatctttaagcgagagttgattcccccctgtaaagatcctgatccttatcaaatccaaattctgttaaaaaactacattctaaaaaatgtctcaactgtttttacatattattgccagtagccattgtttatatcagaaaataacccatttgtttatctttttttgtggggcaaccattaagacccgacgcaaaaaaagattaatcttttatcagatacctaaaacgttctataagggagtctatgagatggatcatattttgatggtcatagtaagaagcaagctttttggcgaaaacaacggagttaaagaatttaacccgctcatgtttggataggacttttaacagcgagccaaaacagtatttaaaaatttggcaatagtttttttgggatgcaataaacaaacacttgatcagtgcccgcttcactttctgatcagacatgtttgccgcataacaggcctttttaaacttagtaatataattatgttccgcaagcaccattaacaagggaacgatgggaagctgcttttcttggtgaaatttacgtaaatattcgatggccaccgcttggacgactgtgtaatttactaagttagaaatgatagctttcatggttgtaaaaatatacataggattttctttttctgtatacagtttgaaaagcttatgattacgtgaaatgatggccatttttaatacaagatggtatagtgtatctttaggtaaaaatgccttgcaagccgcgatgatgtcgatgttgtctccatgaacagcgatagaaactaatgtttccaatctaaatgtttttatctgcattaatagaagaatgcagtcaatgttattatacttaataatactgtaatacaccgaatcaatgaccgtcatctgagaatcaagctgacttattagtaaatttaacgtttttttggaggcatgacctttgatcgcggcactaagtgcacacagtatagcaaaattgttaaatacattttgatttaggagaaggagtaatattttccttcggttatagtacgcagcatctgtgatgattattggccgataaatgttaaaatgtgttaacagctttttaaaaaaacggaagtaatttttttggatcgctgtttgcatcatcgaaataatgagataatcagggtatataatgggtaggtcacatgctacctctaacaaagaatagtcgcccaatctaaaggctgtgttgaaaagcgtactatcatcatacgtatcgagtacccctgctgttacaaaccaagcgataagatgaatgtgccgttccttgcaagctatcgcaaatagggagtttcctatggaatgtcgaataatgtactccctatttttttccaaaatgtttggaaaattgtatagcgttgcggcatacagtagacactccattctggcgttataatttttacttttacatatgaataggtggaagaactcgaataattcttgagaacttgttaaatgcataatatggtgatattttggtgtcgttaaatggtatgagaaaatgcattctaatacatcttttcggttatgctttagcgcctgagctaaggcatattcaggctcgacccataggactagtgtttctataattgagatattcgcctgctttgccagggcatactttaagacgctccggttagaaaaaatgttgttatgaagatggataaccgtatccatttttacgatgggaccattccagtatagtcctaaatgctgtagcagatcttttgttagttgtgaagcgttctcgggtgtcatataaatatgttgcagggcttttttctgtaaggagaacatttcgtcgtaatcgtacaaaaaaaattaaaatttgggcatggatgattcaaacataacaaaatcaagattttataacagtttgcattaacctatacatatatgcaagtaaatgagatattatctatcataacgaatcaagggatatttgtatatatcaggagtttctgaaataaagatatgaagattatcatagtagtatccatcaatcacaatgcaacttcctttaaggcataatttagtaaactcagcactcccatcttctggatgctttacaactaacattaaaaactcctcagtcatattatctgtaataaaataagatcctcctggagccatttgtagcatgtctcttattcctacaaaatcttttttgggatggtaaaaactcagcagtttcaaactcttttttagttttttttcctggtatttaagccatttgttataaaacagttttcttatgaaaatgcatttgaaaatattgggaatgtttaaccatgcttcttccgagcacatctccagatacttactttctttgtttcccatgtctaatttattgctcactaagttagtaatgaatctattttaataatctactttactaatctatcttaataacctatcttataatctatcttaataacctaattataacctatttataattggctaatgctgccggcatttcatgcctatctaaacaactcctactaagcaatctactattacatatatagattcactttttatatttgtaaatcatgagaattataaaatcattactcatttttattgtaaattagtgggtatttgtaaaaatcttcaaacgttttaagatagttttctagagagaagtaatctttgccatcaatatataatgcttttcctttaaactccagttttgctatgtttagtgagccgtttctagatctttttgggcaataaatagattttcattggttgcatcgtccgtaagcagaaaggtaccactaggcacgttaaaaaacatacgttctatttcatggtcggatttttgagaatagaaaaaatctaattttttaatccgcgttaactcttttttatcaatctttccagactgttttatatatactttattgcaaatcttacaatcctctatggcttcattatacttattttgcttatcctctattgacatgtccgtatttgataggtaacttccgttaaggcggttccccatggttttagatagatttttaattcagttgtatacttttattatgaggctaaaatatagaagtttgatcctaaaaaaataaaaagattttgtacatttatttatggtttatagcggtatagaggccgataaaaggtatccgggtagtctcctatgatatcgtcaattttggtataataacagttgttatggtagtattgtccaaaccgagtatgtatgcgccggtgaagcgtccgcccgctaatggtacagttccaggttaagacaatcatatcacacccaaaaagagaggaaacagcataggtgcccaaaggttcattatataacatacgccgcatatattttagttttttttctccatggtaataatcacaggttttcatgtcctgcttaataggatgattccccatgtatgataatatataataaatttagtttttagctttttcaaaaaattgggcgctcgaaactaaattttccttatcacagcgtttggagaaagcgtatttaaagatatatcttcttctaacaagactgcaaaaaaaatcttaccccttatttttataatgttcatcatagcgtttgaagatatcagaaggtgccaggttttataaaaatatcctttaggatttataacgatacaagggtctataaaatatatgcgggtataatcttataaaatcatcgattttttcataatattctccgtttatacaataaagatcataacagatattgatgcgtagatgcattattcgcgtgttcgttgggcagctaaaggatatcacaacgtagttttttttaagaaaagacgaaactacataagtccctaagggttcattgaatagtaaacgccatatttgttttaaattttgttgttcaccatagtagtattcgcactttttcaagtcttttttaataagcctattccccatgtatgcttataaataaaaatttagaaatgtgctatattatttgttgatgaatcatgaacacgtcttatatgttgatatgttactttaaaaacatttgtattttcaacagacgcgttctattcttattaagaatgatgccgtctttattttaaaccttggtttaaaatttaaagaagtatttataaactataatcatgggaactttttcagtaactgcctctgcaaaaagtgacgatgctgtttgtaagtatttagaagaaccaatagatgaaaattacagaaacatattaagaaatgagcatgttaaaaaaaatttaaatgaggctctgaatcgacatattactacctataatccagtagttgattggtgtaataactattcaacattttcatctcaggatttcgatgaatataaaatttatatacatagcgatcttatggatggacgacctcgtccaaaaaaaacatggtgtgtcatcatgtaatgtttgttagttttatataaacgcaaaaatattcttctaggagatgttgatatactacctattgaattcaatatattaaagtacatttctggctattcccattacggtattattattactatttttaagagctagatgtggatttaagtaataataacattctcccgttcctcctagagacacctcatcaaattcccatcctatgcaacctttatgttgtaaacataatgattgacagcattcatcttcttttgaccaagtcgtccaaatcctaccaagatctatacgtgtttttccaaatggagattgaagatcagcagtagtggcattaaacctataaaaaccaggtgcataatcacatgaacggatcgtaggatctaatttaatatcttttatatcttgttttactgcttctagacaacttttatcagtacatgttccacgtacacagtggtgtcctttatccttacaatccgtatctgtcttacatttttttttcggcggtttatgtttcagatggtaaaaacccagtattaaaataatcacaagaataattcctataagtacttgaacaacaggataaaacattttaatattaaatatattttttaattaaatgaatagatttaatccaagtagtattaaaattttttagaaatagtgttctacaaataatgaaatgaatggtccaaaaaaaataaggtgtacaataatgtaatatattgttaggctaagtaaatttaatattttaaagtatttggaaaaatattttttaacatatgatgtctaggaatattttttagacatttaaaaccatatagttactttatttattacactgaacttgaaaagacttattacctaaaatattaatagatgaagtaatattgtgtaattgagtccataacatgggtgggaaacaaaaatctcgtaatatgaaaaataaacatcctaaaaagagtgcaattgttataagtttatgtaactttattttaaagtaagaatataaaaatatgagtacaagaggaataggggccattactaacattggctccaacatcctgttgtctacaaaaaaaaatattttttttagcaaaaaaaaatccatggaaggatattaatacacataattatttgacatcacattagtgtacttaccaaatagtaatatacaaccatcctaatattcacctttatgaaatgatcccaacctatacggtaaaatagtataggttttaataaagaaaaaagatattctgtggtttttatttttgtatagtgtgtgaatacaaaataaaatcccaaattttaaccttttcttttttttctatacaggatgttagaaatagtattggcaacgctgctaggcgacctgcagcggctccgggttcttacccctcagcagcgggcagttgccttctttcgagccaatactaaggagctagaggacttcttatgctcagatgggcagtctgaggaggtactgtctggcccccttcttaaccgtctactagaaccctcaggccctcttgatattttaaccggatatcacctatttcgtcagaatcccaaggcaggtcagttgcgcggccttgaggtcaagatgcttgaacggttatacgatgctaatatttacaatatactgtctcggctgcggcctgaaaaagttcgcaacaaggctattgagctatactgggttttccgagctatccatatttgtcatgctcctttagttttagatattgtacgatatgaggaaccggactttgctgaactggcctttatttgtgctgcttactttggtgaacctcaggtaatgtatttgctctacaaatatatgcctctgacccgcgcagttcttacggatgccatccggataagtcttgagagcaacaaccaggtagggatttgctatgcttacttgatgggaggcagcctcaagggactagtctccgccccactgcgtaaacgtctgcgcgccaaactacgctcgcagcgcaaaaagaaggacgttctttcaccccacgacttcttactgctgctccagtagctttttttgccgcaggagcaccgcggataggagctcctccacgctcgcgatccggcgctggaagcggaaccgatcgaccgccacctgctcccagggacccttgcgctcgatgtcgtcggcttcccacacctcgacggctgtggcaaaatggacatgcttcgcgtcgttcgtccgttttttgcgccgcctccccattattcttcctgtaagattagtgtttaatacctataataacataattttaagatttaatataccaaaacttaaactatttttgtatagtaactattagcataacttcgtatagcatacattatacgaagttatgccggagaaaagtcaaaaggggcaggcaattcatacaccaaaaagttttttttttctgctagcaagagcgtgtcaataattttaagctgatcgttaattaatttttggtttaactctttgttattatcaagatccttcgcataaaccgccatatttaataaaaacaataaattatttttataacattatatggtgagcaagggcgaggaggataacatggccatcatcaaggagttcatgcgcttcaaggtgcacatggagggctccgtgaacggccacgagttcgagatcgagggcgagggcgagggccgcccctacgagggcacccagaccgccaagctgaaggtgaccaagggtggccccctgcccttcgcctgggacatcctgtcccctcagttcatgtacggctccaaggcctacgtgaagcaccccgccgacatccccgactacttgaagctgtccttccccgagggcttcaagtgggagcgcgtgatgaacttcgaggacggcggcgtggtgaccgtgacccaggactcctccctccaggacggcgagttcatctacaaggtgaagctgcgcggcaccaacttcccctccgacggccccgtaatgcagaagaagaccatgggctgggaggcctcctccgagcggatgtaccccgaggacggcgccctgaagggcgagatcaagcagaggctgaagctgaaggacggcggccactacgacgctgaggtcaagaccacctacaaggccaagaagcccgtgcagctgcccggcgcctacaacgtcaacatcaagttggacatcacctcccacaacgaggactacaccatcgtggaacagtacgaacgcgccgagggccgccactccaccggcggcatggacgagctgtacaagtagtaaatcaacaactctcctggcgcaccatcgtcggctacagcctcgggaattgctaccgagctcgaatttccccgatcgttcaaacatttggcaataaagtttcttaagattgaatcctgttgccggtcttgcgatgattatcatataatttctgttgaattacgttaagcatgtaataattaacatgtaatgcatgacgttatttatgagatgggtttttatgattagagtcccgcaattatacatttaatacgcgatagaaaacaaaatatagcgcgcaaactaggataaattatcgcgcgcggtgtcatctatgttactagatcataacttcgtatagcatacattatacgaagttatggatccctaatgcgctccatccagaagaataattaaaaaaaatattttttttagcaagtttttaaactatttaaataaatgtggtaaaaaaattcacataataattaaagtgaacgtgttagaattaatatttttttataatcggatataatatccattaaatcaataaatgatagtgttgctaccacactaaacaataacaaacagaaacgcacgatacctttcctcatgatttataatagcgtgttatctaaagatttttttgaaaaaaatattaaattttagttgattatttttttcagttacaacattgctttagaaaaaatacctaattactacatagcaaataaagcgagcgcattgttacaaacaacattttttttgcgcctggatactcctatatatgagaactataatacggtatattaatcctattaccaacattgtcaataatagtatgtaggcaatgacatactttaaataccaaatatccatggttatttctaaaaatcttgaaaaaacgttaaattttagatcggtcacctacgacagtaatactaattttaataattgatgactgaaatcataatataatgccgtgcgaaaaataattatttttcggttaaagataccattacataaaaaatatgccatctactctacaagtgcttgctaaaaaggtattggccttaggggagcataaagaaaatgaacatatatctagagaatattattatcatatattaaagtgttgcggtttatggtggcatgaagctccgattatactttgttatgatgggagtgagcaaatgatgataaagactccaatctttgaagaaggcatattacttaatactgcattaatgaaagctgtacaggagaataattatgaattaataaagttgtttactgaatggggagcaaacatcaattatggattaatttccattaataccgagcatgcccgggatctatgtcgaaaattaggagctaaagaaatgcttgaaggaaatgaatttatacaaattatattcaaaacattagatgataccaccagtagtaatataattttatgtcatgaattattcaccaacaatcctcttttagagaatgtaaatatgggggaaatgaggatgataatttattggaggatgaaaaatttaacgaacctattattaaataatgactctattagtgaaatattaactaaattctggtatggtatagcagtaaaatataatcttaaggatgcgatccaatatttttaccagagattcatggacttcaacgagtggcgagtaacatgtgctctttcttttaataatgtgaatgatcttcataagatgtatataacagagaaggttcatatgaataatgacgaaatgatgaatctagcctgcagcattcaagacagaaatttatcaaccatttactattgttttctattggggggctaacatcaatcaagcaatgttaacctcagtattaaattataatatttttaacttattcttttgtatagacttaggggctgatgcctttgaagagggtaagaccctggcgaaacaaaaggggtataatgaaatagtggaaatcttatcattagatatcatttatagtccaaatactgacttctcatcaaaaatagaacctgaacatattagttctttgttaaaaaacttttatccaaaaaatctgttcgcttttgatcgttgcaaccccggtttatattattcttagaggaccgctacaaaaattattttttttcttgatcaaagctccaaaataattattagattaaagtcgcctatagcagcagcccactccaaaaaaagtattttatagtacaaaaaacacgaaaaatagtttgcggccggcggcaaactatttgttgttgtctaaaacttaatgtttttttaatatttttaaatgcaaccatggattgttggactatcagggagaagaactatagctacatcatattgtcaatactggtaatactattaatatggtatcttatacttaactattgtcgatcgaaaaaaaatgcagttacaaacaacatgccgccaccatacacggtgtcaagtagctgttctcaataatagggttgattgacgctcttcgtaataatatgttgattgacgcatcataaaatgctgtggttgattaatatgttgattgtcgcctactttattatataagtaatgatttttgtataaaatacgggtttgtgagggctttattttttcttattagaacaaagcatgcaatttaaggcctacagcaagagtaatttaacacctacaacagtaattttaaggtcagtaataatgtttaattaaggcctgaccactaaaacttaaacgattttgtaaaaaaaaatgtctactccactttctctacagactcttgttaaaaaagtgctggccacacagcacatatctaaagaacactactttattttgaaatattgtggtttatggtggcatgaagcgccgattacgatttgcattgatgaggatagccaaatattgataaaatcggcaagcttcaaagaaggcttatctttagatatcgcattaatgaaagtcgtgcaagaaaataaccatgatttaatagagttgtttaccaagtggggtgcagatatcaactctagcttagttactgttaatacggagtatacccggaacctttgtcagaaattaggcgcaaaggaagctttgaatgaaagggatattttacaaatattttataaaacacgtcatcttaaaactagcagtaatattattttatataatgaattgttttctaataatctccttttccaaaatatagagagattgagtttaatagtttataggggcttgaaaaacttatcaatcaactttatattggatgatatttcatttagcgaaatgttaactagatactggtatagtatggcgatattatataaccttactgaagccatccaatatttttatcaacgatataggcattttaaagattggcggcttatatgtgggctttcttttaacaatttgtctgaccttcatgaagtatataacttagagaagacggatatagacattgatgaaatgatgaagttgacctgtagtacgtatgatggtaattattcgactatttattattgttttatgttgggggctgacatcaatcgggcaatgttaacctcggtaataaactttcatattggtaacttgttcctttgtatagatttaggagctgatgctttcgaagacagcatggaactagcaaaacaaaagaataataatatattagtagaaatattatcatttaaaaattattatagttcaaatacctctcttttatcaataaaaacgacagatccggaaaaaattaatgccttattagatgaagaaaagtatgagtcaaaaaatatgttaatgtatgaagaattatctcattgatacaaaattattttttataacagaactctctgatggtgacaaatctccgataggaatatatgacgtaacataattatttttttcgcccagaaaaaaattataaatgttattattgccagcacttttatcaactatacgtacaaaaaggtgttgaccaaaaaaataattttttttcttgatcaaagtatgtaaacgcccgcttacagcaaggatcttaagtgagagccattaaattttattgatagctgcttgccaccagtagaatacggccaaaccacctaacaggaaatacaaggcggcccttcggccaataaggtggataaaaatcacgcataagacggttgtaacatagcactttagtgcgaatatcaggaatgccaatagcatgtagataaggcaccaaacatcgcagctatacatggctaaagatcaaccagaaaaggtttaaattttaacgccggcccaaaacttaaactttttttgatatttttaagtgcagccatggattggtccggccataggatgacctatgcctacgtggcattctcattgatggcaatagcaataatatggtatattctacttatctattgccgatcgaaaaaaaatgttgttacaagcggtaatacgctcgctttagcgccaatatcgcatatgtgaaaaatgttcgccgaaaaaaacattaaaatttagaaccgccgcggcatctcaggggcggcaacatttttttttatatggatattgtcacacaccacctcatctatgacgcaatatattactgctaatatcaggttccccaatagtatgtagagaaaccacacaagatagatattcatggcgatttttgacgaaaaaacattaagttttagcttctttgacgcctgtgtactaataatgtttaacgcctgtagtataataattgatacctacagcagtaattgatacctacggcgataatgtctctctggccgccccaaaaaaaagtatttacggtagggtttattaccggcggcgtaacaccagttatggtcaattttgtctggcccgccgcccagccgcaaaaaaaaatcaattacaaccgcaaaaaaaaatatttccggccgcggcgtttcaaaaaataatctttgcgaaataattccgcatcttgtgaaatgaacgcctacagtaataattttaatctttgacacctacagcagtagtaataattttaatctttaacgcctgcagcagtactaatattttaatctttaacgcctacagcagtagtaataattttaatgtttaacgcctacagcagtagtaat

SEQ ID NO: 4 - protein, 61 aa, African swine fever virus
MLHWGPKYWRQYWTFAFHNNVNNRLNKKIISWSEYKNIYEQSILKTIEYGKTDFIGAWSSL

SEQ ID NO: 5 - DNA, 20 bp, Artificial Sequence
  Chemically Synthesized
tagagatgaccaggctccaa

SEQ ID NO: 6 - DNA, 23 bp, Artificial Sequence
  Chemically Synthesized
gttgcattggggacctaaatact

SEQ ID NO: 7 - DNA, 17 bp, Artificial Sequence
  Chemically Synthesized
gacggcctgtgggcatt

SEQ ID NO: 8 - DNA, 17 bp, Artificial Sequence
  Chemically Synthesized
gcgatggattccggcat

SEQ ID NO: 9 - DNA, 23 bp, Artificial Sequence
  Chemically Synthesized
gtcttattgctaacgatgggaag

SEQ ID NO: 10 - DNA, 23 bp, Artificial Sequence
  Chemically Synthesized
ccaaaggtaagcttgtttcccaa

SEQ ID NO: 11 - DNA, 20 bp, Artificial Sequence
  Chemically Synthesized
gtaagatacgaaaaggcgtg

SEQ ID NO: 12 - DNA, 17 bp, Artificial Sequence
  Chemically Synthesized
gacgctcctagctggaa

SEQ ID NO: 13 - DNA, 19 bp, Artificial Sequence
  Chemically Synthesized
gttgttatggaacgcgaag

SEQ ID NO: 14 - DNA, 21 bp, Artificial Sequence
  Chemically Synthesized
gggtttctacaggacgtaaca

SEQ ID NO: 15 - DNA, 22 bp, Artificial Sequence
  Chemically Synthesized
ctgttgaattacgttaagcatg

SEQ ID NO: 16 - DNA, 20 bp, Artificial Sequence
  Chemically Synthesized
cattggggacctaaatactg

SEQ ID NO: 17 - protein, 119 aa, African swine fever virus
MLHWGPKFWRTLHLYAIFFSDTPGWKEKYEAIQWILNFIESLPCTMCRHHAFSYLTKNPLTLNNSEDFQYWTFAFHNNVNKRLNKKIISWSEYKNIYEQSILNTIEYGKTDFIGAWSSL

SEQ ID NO: 18 - protein, 119 aa, African swine fever virus
MLHWGPKYWRALHLYAIFFSDAPGWKEKYEAIQWILNFIESLPCTRCRHHAFSYLTKNPLTLNNSEDFQYWTFAFHNNVNNRLNKKIISWSEYKNIYEQSILKTIEYGKTDFIGAWSSL

SEQ ID NO: 19 - protein, 119 aa, African swine fever virus
MLHWGPKFWRALHLYAIFFSDAPNWKEKYEAIQWILNFIESLPCTMCRHHAFSYLTKNPLTLNNSEDFQYWTFAFHNNVNKRLNKKIISWSEYKNIYEQSILKTIEYGKTDFIGAWSSL

SEQ ID NO: 20 - protein, 119 aa, African swine fever virus
MLHWGPKYWRALHLYAIFFSDTPGWKEKYEAIQWILNFIESLPCTRCQHHAFSYLTKNPLTLNNSEDFQYWTFAFHNNVNNRLNKKIISWSEYKNIYEQSILKTIEYGKTDFIGAWSSL

SEQ ID NO: 21 - protein, 119 aa, African swine fever virus
MLHWGPKYWRALHLYAIFFSDAPGWKEKYEAIQWILNFIESLPCTRCQHHAFSYLTKNPLTLNNSEDFQYWTFAFHNNVNNRLNKKIISWSEYKNIYEQSILKTIEYGKTDFIGAWSSL

SEQ ID NO: 22 - protein, 119 aa, African swine fever virus
MLHWGPKYWRSLHLYAIFFSDAPSWKEKYEAIQWILNFIESLPCTRCQRHAFSYLTKNPLTLNNSEDFQYWTFAFHNNVNNRLNKKIISWSEYKNIYEQSILKTIEYGKTDFIGAWSSL

SEQ ID NO: 23 - protein, 119 aa, African swine fever virus
MLHWGPKYWRSLHLYAIFFSDAPSWKEKYEAIQWILSFIESLPCTRCQHHAFSYLTKNPLTLNNSEDFQYWTFAFHNNVNNRLNKKIISWSEYKNIYEQSILKTIEYGKTDFIGAWSSL

SEQ ID NO: 24 - protein, 58 aa, African swine fever virus
SLHLYAIFFSDAPSWKEKYEAIQWILNFIESLPCTRCQHHAFSYLTKNPLTLNNSEDF

SEQ ID NO: 25 - protein, 96 aa, African swine fever virus
MSTHDCSLKEKPVDMNDISEKSVVVDNAPEKPAGANHIPEKSAREMTSSEWIAEYWKGIKRGNDVPCCCPRKMTSADKKFSVFGKGSLMRSIQKNN

SEQ ID NO: 26 - protein, 96 aa, African swine fever virus
MSTHDCSPKEKPVDMNDISEKSAVVDNAPEKPAGANHIPEKSAREMTSSEWIAEYWKGIKRGNDVPCCCPRKMTSADKKFSVFGKGSLMRSIQKNN

SEQ ID NO: 27 - protein, 96 aa, African swine fever virus
MSTHDCFSKEKPVDMNDISEKSSVVDNAPEKPAGANHIPEKSAREMTSSEWIAEYWKGIKRGNDVPCCCPRKMTSADKKFSVFGKGSLIRSIQKNN

SEQ ID NO: 28 - protein, 96 aa, African swine fever virus
MSTHDCSPKEKPVDMNDISEKSAVVDNAPEKPAEANHIPEKSRREMTSSEWIAEYWKGIKRGNDVPCCCPRKMTSADEKFSVFGKGSLIRSIQKNN

SEQ ID NO: 29 - protein, 96 aa, African swine fever virus
MSTHDNSPKEKPVDMNNISEKLSVVDNAPEKPAGANHIPEKSAREMTSSEWIAEYWKGIKRGNDVPCCCPRKMTSADKKFSVFGKGSLIRSIQKNN

SEQ ID NO: 30 - protein, 95 aa, African swine fever virus
  misc_feature (31)..(32): Xaa can be any naturally occurring amino acid
  misc_feature (42)..(43): Xaa can be any naturally occurring amino acid
  misc_feature (67)..(68): Xaa can be any naturally occurring amino acid
MSTHNNSPKEKPVDVNNVSEESAVVNNAPEXXGGNHIPEKTXXKMTSSEWIAEYWKGINRGNDVPCXXPRKMTSADKKFSEFGKGSIMRSIQKNN

SEQ ID NO: 31 - protein, 96 aa, African swine fever virus
  misc_feature (43)..(44): Xaa can be any naturally occurring amino acid
MSTHDCSPKEKPVDMNDISEKSAVMNNAPEKPAGANHIPEKSXXEMTSSEWIAEYWKGIKRGNDVPCCCPRKMTSADKKFSVFGKGSLMRSIQKNN

SEQ ID NO: 32 - protein, 96 aa, African swine fever virus
  misc_feature (43)..(44): Xaa can be any naturally occurring amino acid
MSTHDCSPKEKPVDMNDISEKSAVVNNAPEKPAGANHIPEKSXXEMTSSEWIAEYWKGIKRGNDVPCCCPRKMTSADKKFSVFGKGSLMRSIQKNN

SEQ ID NO: 33 - protein, 96 aa, African swine fever virus
MSTHDCSPKEKPVDMNDISEKSAVVDNAPEKPAGANHIPEKSAHEMTSSEWIAEYWKGIKRGNDVPCCCPRKMTSADKKFSVFGKGSLMRSIQKNN

SEQ ID NO: 34 - protein, 95 aa, African swine fever virus
MSTHDCSPKEKPVDMNDISEKSAVVNNAPEKPAGANHIPEKSAEMTSSEWIAEYWKGIKRGNDVPCCCPRKMTSADKKFSVFGKGSLMRSIQKNN

SEQ ID NO: 35 - protein, 96 aa, African swine fever virus; identical to SEQ ID NO: 27

SEQ ID NO: 36 - protein, 95 aa, African swine fever virus
MSTHNNSPKEKPVDMNNISEKLDVVNNAPEKPAGANHIPEKSAEMTSSEWIAEYWKGINRGNDVPCCCPRKMTSVDKKFSVFGKGYLMRSMQKDD

SEQ ID NO: 37 - protein, 95 aa, African swine fever virus
MSTHNNSPKEKPVDMNNISEKLDVVNNAPEKPAGANHIPEKLAEMTSSEWIAEYWKGINRGNDVPCCCPRKMTSADKKFSVFGKGYLMRSMQKDD

SEQ ID NO: 38 - protein, 96 aa, African swine fever virus
  misc_feature (43)..(44): Xaa can be any naturally occurring amino acid
MSTHNNSPKEKPVDMNNISEKLDVVNNAPEKPAGANHIPEKLXXEMTSSEWIAEYWKGINRGNDVPCCCPRKITSADKKFSVFGKGYLMRSMQKDD

SEQ ID NO: 39 - protein, 96 aa, African swine fever virus
  misc_feature (43)..(44): Xaa can be any naturally occurring amino acid
MSTHNNSPKEKPVDMNNISEKLDVVNNAPEKPAGANHILEKLXXEMTSSEWIAEYWKGINRGNDVPCCCPRKMTSADKKFSVFGKGYLMRSMQKDD

SEQ ID NO: 40 - protein, 96 aa, African swine fever virus
  misc_feature (43)..(44): Xaa can be any naturally occurring amino acid
MSTHNNSPKEKPVDMNNISEKLDVVNNAPEKPAGANHIPEKLXXEMTSSEWIAEYWKGINRGNDVPCCCPRKMTSADKKFSVFGKGYLMRSMQKDD

SEQ ID NO: 41 - protein, 96 aa, African swine fever virus
  misc_feature (43)..(44): Xaa can be any naturally occurring amino acid
MSTHNNSPKEKPVDMNNISEKLDVVNNAPEKPVGANHIPEKLXXEMTSSEWIAEYWKGINRGNDVPCCCPRKMTSADKKFSVFGKGYLMRSMQKDD

SEQ ID NO: 42 - protein, 84 aa, African swine fever virus
  misc_feature (84)..(84): Xaa can be any naturally occurring amino acid
MSTHNNSPKEKPVDVNNVSEESAVVNNAPETGGNHIPEKTAKMTSSEWIAEYWKGINRGNDVPCCPRKMTSADKKFSEFGKDTX